European Patent Specification EP 3 828 281 B1, published November 27, 2024. Title: METHODS FOR DETECTING CpG METHYLATION OF TUMOUR-DERIVED DNA IN BLOOD SAMPLES. Applicant: Epigenomics AG. The sequence listing filed with the application follows.

SEQUENCE LISTING (63 sequences)

SEQ ID NO: 1 - DNA, 34993 bp, Homo sapiens
ggataagaatctctcccaactagaaggcaattctcaggcctttcccctctaaggacttccaccaaagttcccaggaaaattgaggagactctgagtcaggggcccagcctgagctctgcccacagcaagtgacccccactgaggcatgaaaacaggaagtaaaggagagaggcctgtctttgggtttaggctttttttttttttttttttttgagacggagtcccgctctgtcgcccaggctggagtgcagcgggtttaggctttttaagggaccccctcccaatcagggcaacagagggatgcccaaggtgaccgccaacaccttcctggggggctgactccagggctcaggaggaagggaccagccttcttcgccaagagggggagccctagcatgcacttctgggctggctttacccaaatagtgaggcaccccaggtgtggagacctccctctccccactccaaacaccactgggtcagggggctgccagccagccacctccagcagcccaggcaggaagccggaaatgatgcagcccaaattcctcttggtggggtttcctgtaagtggggagccgcccagggcaggatcataaatgggctgatctgaggtctgtggtcctaccggagaagccaggcatggaaggctgactatatatccacggccaatggctccagagccctaagccatgggcagaccagatgtggtgagtgaccctggctatggcagtaaccaagaccaggatgcaggagtgtggtccaagggtttgcctggcactttcccccagcctgggggaggggttctccttctcctccaggtgacctgagaagaatggtaggcaaaggacactgtcctggtctgggcagccgctattggtgtcagctcatttctggatgacacagatgggacgcccaccctaaccattctgtctcctccctctgtgcaagtgcccttgggactacccagattgtagtttaaggtgaagggatccttgcgtcaagaagctccttggaccaaacctgggacggaaaggacaggaactgtaagggaactcgtcagccctccccctgcgcttctggctccaccggcagggtatgggtctgtatgtgtggagaggtagcaggcgtgatcctgggatcacgttaaccagtgccaaccccatggaggcctctactacggtgaattcctgccaccacctgaagccatcagtggcctccagggccagtaggtttgcacatacaggctagcctcaggcctccctcccctgagctaagggccagatctccactagactaagggaaaagcccacatcatgaaggcaggcgagagtagtccttggggtagagtcagaatggtggttacctctggggtgcacggactgggagggggtacttggaagccccctaaggtgatggaaatgttctataacatgcttgtctaacctgcagtccatatgcggcccaggcagctttgaatgtggcccaacacaaattcataaactttcttaaaacattatgagacttttttgtgactttattttttatttttatttttgcttgttttatttagctcaccagctatcattagtgttagcgtattttaggtgtggcccaagaaaattcttcttccaatgtggcccagggaagcaaaaagattggatacccttattctataacatgatcagagcagtagttacatgggtatacacacatgtaaaagcccatcaggatgaacactcaggtgcaggcattgacacacacaaattctacctccataagggaggaagaggagcccaacatttgtcccactctgcaatctacactatgaagagacaaatcagcctgtagcttgtcccgtaacatgtccccggccttgctcaccagagatacctacaggacaggcatcttgaggccttcactctcacccccagggttgccaaagtggaaaaggctgagatagaagcccatggggtgaggagaggcccttgactgagatcgtgtggcgaggtgggccaagcctaaggaaaggggaagatgcacattctccagggctccctgcccccttcctctcttggactccccaggcaggcaggaacacatacggtgcctgacgaggtggcacaagctgccagagcagccatgtcatgtccagctgcctagcaacacactcacacttgtcctgtgtgcccatgcccgggagcagagggaggatggggctctctggggacaggctgcatctcacctctgacctccatgaccccccaaattaaccaagcacaaaaagtccctggccccactcctgtggttaggactgcagggctcctatcataataaaagaagcctgtgaccctggggtggagcgatacaccatggggctggcactggatctggactccggactgctgggtaccctcatgcctctctgcctgagatgccacaggacccagaccaaacatgccgctgcatgccagggccagcatcctagggtccaggtgtgggatagtcccaagcagccagccagggtcctaacaagcagccaaacactcagggagtgcctgccatgtgctggacacctcgctgggtgctaggtgggctgatgagtaagactgtccacatcctccccaccccaccatcctcaccttctcaccaccttcctgacctctattgtgaatcaggggaaaggaggcatctggggcacaaattcctctgacagatgaggacctgggaggaggagctgggcaatccaacacatctgatgcccaccattcctccctgagcccactgggcatccagaggctgtggtcggacattcaacgcaacatacaaaggacaactgccttgctggtgctgcccttcacccctccaccccagaatcagaccacagattcggagatggcagccccccaaaaaccatttctactccaacttctttgcctctgaattgaggaagctgaggaccccacagtgaggaaagtcttgttgggattacagagtaagctgggaacaaaggcaacactaagccccagactcccccgattgggcgcctgctaagactctcctccacattccatgccatgcttaccccacggagttgtggaacagtggggagacatttataaggcaaggtgcatcctcagccctgccatccccagacctgcctgcagctcggggaacggagtcacagtttcttaggggtatggaccctcaaccccagggccctctaaaccatgataagcccctaggaggccttggtcataaccacctatggagtattttgtgcccaagccctgctaagtcatagttcccaaatactctagcttggcacccccagaaccaccagagcatctgtgaggctcaaccggtggggtcctgggcctgctcaaggggtggctgaaagttatgggcccacaaaccagcaccccatactctcactcttaatcatgcccacagccccgctagagttcacggacctccgcagcctgcccaggggcctaccagggagatagctcctttgctaaagaaagaatggatgtgggctagagcttccttcccaggccagctgcagagccccgtcactggctgtcctccctcatcagaagggagcagcctcttggatcattacccctgacttcctcagcaggcctggggggtttcactccagcccagtcctaactctgttaggaaaaggaagggaaccaccatgtaaatacagccaggagacaggccaggaagccagcaggatacggggaatctcggcacggcctcccacccatttctggccagactgggctaggggacagggaggggcccgcacccaggatagcttgatgccaagctcactttcccaagcaggccttaccggtgaacaggaacagcagggtccagccgagctgttcccagtcaccaccagcaggcctggggatgcctcccgagaagacacccgggtctagactggccctgaacgccaggcccggcaaggagcgctagccttaggaacccgaggcagggagtcctgggagtagccaccgctcatctgctcctgaggagacggtattcaggccccactggcgcatctgcccggccctctgctccttgccctccaccaccccggcaggcgtaccgaccacgcgagcagcaggtgcaagacgcgggggtggcactgagatgacataaaaccacactcgcccccacctcccaagccctgacggcctccgccacggccctcctgccaccccaggctggcgcttccgtcggatacagagatggaggtggaggagcagccagctgcccgcctccctcagaccgaggagcgggaggcggcgccgggaacgtccttcctcgctagtccacggcctccagggagcatgggcaccccaggccggccctcccgccaagggcgcagctccgcagtggccgaggcgggggcccagcctggaggccgcagccccccgccccgcccagccctccggccccgcacagcgctcttgccaggccccggcgcccgcccggcggcggcctggctgtgcggtcccgcccccggccccgccgcgcttacccggggcgctgcagtccgcacacacctccgctcgcggcccctttcgggacatcctcagcggcgacgcggccgcagccctctgggccagcgtggggggcgcgggcggcgggcccgggcggcggcggcggcccctgctgcccggcccggctccggcgaggccccggcgaggctccgcgcgcccggccaaccgtccgccccggggctggcccggaacccgccgtgcccgcctgcccgctcgccctcgggcgccctccgccccgcgccgccccgccgccgctcgcggctcctctctccgccccctgcgcggctcccggccgcttctgcaggaagcggcgcaggccctgcccacagggggaggggccgcacccccgccccgccgcgcgctgccggccgcgccccctagagaaaggaagcccgggcgcgggcaggagggggcgggggcgcttaaaggggccgcggcagatgcccggccccggcgggcagcgtggcctgcggccctggcctccgctgcagcgctcgcctggcccggaggcaatgtgagtcaccctcacagccccctccccttcactttccgcgtggggtggaccgggggacgctgggcccacggacggcgagggtggggattagggaagaaggacttggaggcccaagtcccgctccaggtcaaaggggctgtgccttggggtacccgtctatctctggttggggtgaggtgtgcgtccctgtcccgtaggtgtccacatctgtgtgtccaggggtgtgtgtgtatgtgtcacactcttgctgaatacgcccactgctaacaatatggacgcccaggtgccagaaaggtcaggcagtgtattcccctgcctccggactaaaaatatatctatctctccatgcatccttccatccagagaggagagaatctgggcggtttttaaagacctcccgaggagtgaccactgtgcctgtgtgcactcacatccacttgtcatccgccttacacacacccacggtgtttctgggccaccagaggtgtgtgtgtccagaaagggtgcatataacatagaggggccgtttcaggtgacggcctttcttcctggacttcacacgacgaggcaggcaaaggcaaggcaggtgagggacgtgggtgggctggggggcagggagcctaggtagaggccgcacatgagcgcagcccccgcactgagcatgcgcccccatacgcgtgtgccgcgcgtgtacccaacccccaatccctgcagcagcaaaaggcccgggcactctgcttgtggggagagggtagaggtccccagggccagacctgggggccaggtcagtggtgacaattgaggaggggttctccaagagtcagagactcctgcttgttaagatgggggcagtcctttggcaggggtgctcaagttggtcgattatcccaacggtgccagagcggcagtgatttgtgggtgggcaggctccttccctaggggagacaagtaatgctcatgagtcacaccacccgaaatacatgcaaagctgcctccatcgccttttgctgcggcccagattgacaagtttgtttgaaatcgcgatccatgggctttatttataattgcaccttaaaaaaatcttgcaggcctcccctccctcgacagccagccgctcagctggtggggcttttgcaagcaacgatacctagctggtgtgtaggggggagcaccacctgccgccccgagctgctctctcaccagagtccatgggcttggtggcctcagcgggaagggggtaaggggcggggggagtgagacgggaggagtggccaggcagcccgtgccaggcgctcagtccacgagcggtggccgcccgttcacccccgatcgacccccagctatggaatttcatttattaaatgtcgaggaggctgctggcagccctgccgcttggctgtctttgtttctccgctgtgtgggcgcgtctcgagcacgtggcagctgagagcgcgggccgaagcgcaagcgacctgggttcagtgtctaccgccgcctggcaaaaaaagaacacggccgcccaggggacagttccccacaatcgacaactccccacaatccatcctgaactccccctgtcctcggactcctgggctttgctggggaagaaggatgattcactctgcttacccctccaccccactccccatctcctggttggctcagagactacctgggagtggccctggcgcggacacatcgtccaaactttgtttcccccagccccgtcacagccaaacttctgggcctgggactggagataaaagggtttctggattcccccgtggagatgtcaccaccccaggaagcaggactgctacagtggaatcacacacaaggttcgaaaaacaatttaataaggaaatgcacaggcatgctcccggccactcctagatgcccctcaaccgcgccagccccctcccctgcactggctgcagccacgacactctgctgacccctggtggtgcaggcgggcagcggtcccgggcccccggagacgccagctggctcctcccaggcgggagaaaggggcgaggcagcccgctcctccctcatctcttcccgctggggcctggcaccacagggtgtggaggaggaaggagggaagaccacacaaagaaacctgagagagtttgcaagcttttgctggcacctcccacacaaacacttcttggattgttgttttaagtagggccggtgtggaatcccttattcctgccttgttctgaggtgggctcaagaaggcaccgtgcctggtcccgccacctgtctcggcccgcctggttgggggagggaggcgctgtttccagggcagtcattatccttagctcaccccaggaggtagtatctagattctcattttgaaggggagtggaccgagaaagtcggaaaaattaagcagtttgctcttttaaggtcaggcagttggagctattcgaactctggtctctctgacatcacagtcccctccctccagggactggtccaagcctcttggtccttccaggccttgcaattggcgcttgagaggccaattcaacttttaccacaccctctgcagggaccattctggaagtacctcttcaccctggggtcattcaggaaggagacagtctctggaatcagtcacttcccttcctgaagggccagctgggtggaggaacggagctgccacctgctgctttttctgtccaacctcactctggttcttgctggggacagtgtgcggggggaaagggaccatctttcccgcgttactggacattctgtttccaatgacatgtgtggaagatggagtttaattttctaacagggcagggaagactcctcagaaatgttccaggggccagacccctggctgctccaatgacccttggtactgatgccccacacctttctcaggagttcccaatcagacgctctcttctgggaatccggatccttcttcatggcccctgggacccaagctcaattctgaagaccacacctccaccccgtctcccaaacgctcgacctaggcccgtgcccccccacttccccagcaaaaggcaaaatgccagcgggggaggtgcgtcccagcccacctggcgtcagggccccgcccgcgtctgggccaggcctgactccccgcccactctcccacgagatccggggacagtgcagaccctcttcggccacctgccacccccagtttcacgaggcggactacaaaccccatgatgccgcggggctgagctgacaagctctacccggggcgcctggtccccttcctctctccccatcatccccacatccccgtatcccgcgccggccgctcgggctgagggccgggctatgcagctgtggggacccgggggctgcgggcgcgcgtccctgcggcggcgtccccggggcccgcgtcccgtgcgcccccgcgcccgctgcgggcgcctgctccctccgccgagcggcgtctttgtgtgcgggggtgtgggaggcgagcgcgagtccgcgcagcgccgccgagtgcccgctccctcccagggcgggtgggggcctctccgcgccgcccgccgccgccgcctcgcgaggacgcccgtcgcccgcgccgcccgcaccgcgccgggcgcgccgcccccgcccgccgccgctcgcacatgcccgagccgcagccccgcgagcaggcagcgccggccccccgccccgcggccccgggccccggctccggcgccgtccctcctccccggccgggcgccgcggccccggcatgaggagcgggcgatgatccccgccaacgcctccgccaggaaggggcccgagggcaagtatccgctgcactacctcgtgtggcacaaccgccaccgcgagctggagaaggaggtccgcgcgggccaggtaggagcgccttcggggcgccgcggggaccccgcggccgggcacgcccgtccggcctggggagggggtgcggcgcgggctgtcccgcctccctggcgagtttgcggcgcgtctttgtttgcggccgcggcttttgtgcttgttgaccgggaaagggtgatcccctccggccgggacgggcgggaccacacgtgtttcggactcacctagatgagagtagaggcctctgtgcccctcctccgccggggcagtgagggctgcagggaggggctgcgggctgtgtcggtgttccatgtggtgggagagtccgccccagccagttgagcggcgacacctcccgagtgagggtgcggaggtgggaaaggcttgcgtggggagggggccataggtcaagaatggggaagaggctgtgtcacactcccaggcaccccagccccacccagcgccctctccccaacggtgagcgctttctcttttagctctcaaactgggcagatccttggatctctcagagcccagccccagctcaggaacagggagtggagaaagaccctcttgggaggccccaagggccttgtccaggtgctgaaaagcgctctcctgccctctggtgctggggcctggtttctaggcgcagaggaagctgaggggccctggctgctggaaggacttgaggttctgcgcaccaggtgggctccctggtttctgctggtcagtaaggccacgtgggtcaccagctttgggctgggcagtggtctccagaaaacaggggaaggggggatgtcttctggccatgcttcaggatgtcttctggccatgcttcagaacaaaggcaggcacaggtcacagattgccacttctgcccttggcacccaggccacaggtaggcactcatggcagagatgaccccccgcctccagggtgggctgcaagagccagagctgggcccgggtcccatggcttgctgcaggctgagaaccccagttttggactgggtctgagaccttggggccatgggctgggggtggttagcgcagttgcccgctgtgggaatttaccttctgagggctgcttattgagtcatgagaagttcagtctgaggagctgtgcaatcgccaagggaagcatggaggtggagggcaggccatcggactgagcaggctgggggtcaggatgtgtctctgaagtcccacgctgagccagcccccaggcctgcatggcatccagctctgcatggcagtccctgtaaatatgcgagtgacctgtgcccgcaggcctctgggccggtctgggtggccacttcctgttacctgtgcctatgccagcactctccgagtttctcctcagactgaactcctcagaccctgtctttgtttatctatcataaaggcagtgctctgcagccacgagaagcctgttaaagagagtgggtcacagtgcccccaggaaacagatgaacaaacagggcatcaacccctgccctcaaggagtctctgttctggtgaagcaagtgtgaacaggaaattccagggtgatgtgcaaagcgctaagacatggccagccagcctctgctggctcttctctgctttccttccctgaaagcaaaagaagacaagcctcatgtgggaagaacttcccaggggtccaaggatcactaggcagaaggctgaatctccagaatgcctcagtcccactcccttgcctgagggtgggtggtccttttactgcagagactggagagaggcagaatgccctgggagaaaagacttctccagcaggcctctctgctgataatcctgaagtgggtggccatcttgctggggtaaggttggggtggggggcaccggagccgctgcaggtagaggtgttgggggctgctcatgtgtttctctctcccacccctctggctgcctcagaaacaaggtcccagattcacccctacccctgccccagtgagttaatgtctccttgaaatggacactgcctgtcctggatccaggccagggggaatatagggcactggtggaggttaacccttgttcaaccacagaggagccaggccagtcctctccttccctcaggcgtgccaaaaagaggaatgccactccgtgtaggtgggagagttccctagctgtctcccctctcgaggactggcccagagtgaggcttgtatccagatgtacactgcctactccccagggcaccaggctctgttttctgcaagggggacctggggacagccacctaacatcatgagaaaagcactgtggaaccctggcatcccagccaggggtccctggcctctagtccccctggtaccagccgccacagaaacagctcggctttcctcaagcactcaggagccaggtttccctggtcttggcttggcatagctgcctcttcttcactccaagaaagccccgcagaggccctccgtgggcaggcttggcagtgcagctggctgaggagggggccagcatggccaccttcagagcaggttaatgggctttgctcagccccaaattgctctgctggaggctggaagcagggagtgatgggcagataggaggtgcctggtgaagggaaggggcacccagcagtgctgtgatgccagcccggtgccctgcttgccgctatgcatgttctctgccaggtcgggggggacagggttgtaagccagggaatatgccagttcccccttgcctggcatggccagctgggcatggtcctggttctggagtcgtgagttcctggtgttccctggggtgggaacagggggaagggttagcctgtgcagctcccgtgggagggacatgtgtgggctgggcctggggagcaggactctgcccctggcaaccagaaccctgaagtgggcagattgtggtcccagagaatcattttccttctccctggggcgttctccaccgtgggcttgcttcctgctttccctgttcacccttctgacctagaggcaggggagatgggttgtggggcccaggatgtgcgaggagcacctcagacccctccctttgcctacactgggcagtcctggatgtggggcatcaccacagctggtaagctaggaagctcgggagagggagccacaaaccccagaaaccaaaaatcaatgtgttctgggatgagggggaggggctgcaagggcaggatgggaggggtgacatggagggagaagtccagggtgcggtccccacagcccgtggcctcctacgcagcttgaggatgcatcctgcctccctccccttgaatgagctcaggcagacctgcccctgcaccccacgctgggcaggagaggtcaagcaacgactacaccagactcctgccttcctcctcgtgggctggggaaggggctgagcaggcaccaccttgagcacaggctctgcgtccctcaccttcctcgcaagcactgtgtttagtccatacatgagatgtatgcttttcatacttcccttaacaaaaggattctgctcatgctaaaggagtttggaaagtaccctgctagtgcacatgggtgtgaggggtgttcctgtgcaaatacgcacacacacgttacacaggagtggactcctgcagggccagaaggcagctgggcatgcatgtgcttgtacacttaagggcacacgtgagtacctatgagcgtacgagtgtgtatctgtatggtaccagtgtgtactagagtgtggtgtgtgtgcctgagtggaggtagggaggctctctgcccagggacccccagctacaaaactccaaagactccaccttttgactccagctgaggcctgctgggataaggaatctccgttctcttggtggggagggctgggtgttgggtttcatgggaaaccttttcattccagcaattaaatagctagaggcctctgctgaggagaagctggaggcctctgctgaggagattaatgaattctcctacctgggcccagggcaaggtgccacttacactgcaggcggcactctgggcttgtggggagagctgctctggagcttggctgagtgtatggggttctgcatggggtgtatggggtgctgagccatccaggcctccctggggagtgctcctgaggtgtggggatggggaggagcaccctgcttgcaaggaagtgccagccgctctctggagcctggagctgaggcacctgatggggaggtggaggcagcatctggagccctgaggccaggcagcggcctgccagctccctagggtcttattagctgcagcggctgcggctgcagcatctggggcagggctgggaggcctggattgctcagcacttccccagtcagctcgggccctgtggccctctcccactcccgctgccgggctcaggaccccacccaggttgcaagccccggagtccagcccaaccaggattggacaagagtaaacaacactccccttctctgtgaggggccacagctcagaggccaacaggggccaggcccgctggtttttttgaggctcccagtatattgaaaaatgaagaaattccaggacaaggctataaaaattatataaataatcttaaattatttaaaatgtttcatttttgacaatggagttcatggtcatgctttaaaatatttaactgttgctagaagatgcgtaatgaaaagcagtgctccttgctccgcctctcccacctccccagcactctggactccttttgtcatttacctccctaattataaacaatatattgtttatactgccctctcccctccccttctccctccctccctcccttccctgcctccctccctttctctttctttcttcttcttttttttcttttttcatgagacagcgtctcactctgtcacccaggctggagtgcagtagtgtgatcacagctcagtgcagcctctgcctcccaggctcaggtgatcctcccatctcagcctcccaaggagctaggactacaggtggtgccaccatgcctggctaatttttgtatttttttttgtagagatggggtcttgccatgttgctcaggctggtctcgaactcctgagctcaagtgatccacctactttggcctcccaaagtgctgggattacagacgtgagccccccggcataaacaatatacttctgcaatgatttcttggttaattaccttcccctccttgtgccccctcagcctagtactctatgcatttgtctagcaaatatttatgtgccaggtgctgcctggggagtggggaaccagcagtgaacaaagcaggcagggacctggctgatggggcttctgttcgaggtgcaggaggtgctcaacaggcacttggacgggcagtggatagagccatagcagctgttacctcagatgggctgtcagggtgggcttttctaaggaggtgacatttgagcagcagcctgagtgaagggagggagaaagctttggggctctctggaggatcctggagaacgttccggggaaggccattggcgaagggtggagcaaatgagttcaaagagaagtctggggccattggattccctgctacctacgatggaaagccactggaagattttgaactaaagagtgtcaggacctgagtaacacttcacagggtgactttagctgccataggtgaggtggacaatagagcctggcaaccggggagcagcaaagaggcagtagggggctgccagtgagagatgggggggcaacagctgcaaggtagtggaaactgggcggcttctaggtctgttttggaggcagagcctacaagtttttctgatgggttagatgtggagggtgcgggaaaaagaagagatgtagacagttttaaagttggtttttttttccacctgaaaatgcagtaaatccaggtgatgtttactgtttatgggggcaggtgcagctgtccaggaatgcagaaaacaaggaaaagttaagaaagtcacttccagaatgaagaaggcaagagaaagggcaggagacgtcatggaaagccaggctgtcccattttgtttcatgaattcaatgatctttttatatttttcctgaggatgtaaattactgttttcccccaaagagttttcttttattccctgcatcaagagaatttcctctgggttcttagcatctaatttgtttttttttttttttttttttttttttttgatacggagtctcgctctgtcccccgcgctagagtgcagtggcgcaatctcggctcactgcaagctccgcctcccgggttcacaccattctcctgcctcagcctcccgagtagctgtgactacaggcgcccgccaccacgcccagctaattttttgtatttttagtagagacggggtttcaccgtgttagccaggatggtctcgatctcctgacctcgtgatccgcccacctcggcctcccaaagagctgggattacaggcgtgagccactgcacccagccgtcttagcatctaatttgtatgttttggtttatttcacatgggaagctttcatcaagtgtccagtttctcctggctgttgggtcatatttaagaatggggctggggagctcagggatgtgtgggtgctactgtaaggtgatcaggtggcaggctggcctgttcattgtagggtcaccagatgtctgtattctgaggtctttgggacaacttcctactcgggtagatagggtggtggtggtgtgacctggctgccagtggttcaggacccaggtagggaaggggctggggtttcacggatcactggctttcagcaccatacctcatcctctgctgtggccaatgctcctgagtccagagcatctcatgcccaatttctacaaagaataaacccctggtgtcctgtggtgaggaaggggggcatctcccagcttaatgaggctgggaaggggaccaggggatcctgaattgtaaccagcctccctgcactcagctctagcttcacctccacctctgccatccccattgcctgcaggtcctacctacacctttcaggggggctgggggtcacctggcttgctccttatgtggacgtttccctctgtggctgctttagtttcagcttcctctgctcccctaagtcagttgtgaggccccagccactttccatgttctaaagttgtgttgaagtttctcatctgctgacatctcttctctttattcttgtgggttttaaatattttactgacttttttttttttttttttttgagacagggtctggctttgttgcctaggctggagtgcagtgggatgatctctgctcactgcaacctctggctccctggctcaagggatcctcccacctcagcctcccagtagctgggacgataggcatgcaccaccacgcctggctaattttagtatttttttgtagcacagagtttcaccacattgcccacgctggtttcaaactcctgggctcaagtgatctgcccacctcggcctcccaaagcttacaggcatgagccactgcgcccagcctgacattctttttttttttttttgagacagagtctctctctgtcacccaggctggagtgcagtggtgcgatctctgttcactgcaacctccacctcccaggttcaagcgattcttgtgcctcagcctccctagtagctgggattacaggaatcccccaccacgcccagctaatttttgtatttttagtagagatggggtttcaccatgttggccaggctggtctcaaactcctgacctctggtgacctgcccgcctcggcctcccaaagtgctgggattacaggcatgagccactgtgcctggcctcctgacattcttatacatttaacattttttggcactcttcaatcctttgtacagattcaagtttctatctgggatcattttctttccacctgaagaactccctttaacatttcctgcacatctggcaataaattcccttagaatttgtttgtctgccaacatatttatttcttcttcagttttgaagaatattttcaccgggtatggaattctaggtcaataccagtcatactggattagagaaaaaaaaaaaaagaattctaggttgaaagtttttgtttttgtttttttcccccagcactttaaagatttcattatattgtttcctggcttacatagtttctgatgagaagaatatagtatttcctgtatctgttcttccatacataatggacctcatttctttgaatgcttttaggattttctttttaccactagttttcagcatttgattatgatggaccttggtgtagtttacttcgtgtttgtcttacttggggttcattgaatttcttggttcttggctttatcttggtattagtttccacaacaaattactacaaactaggtgggttaaaacaacaaatatttggccgggtgtggtggctcacgcctgtaatcccagcattttgggaggccgaggcgggcggatcacgaggtcaggagatcgagaccatgctggctaacacggtgaaaccccgtctctactaaaaatacaaaaaattagccgggcgtggtggtgggtgcctgtaatcccagctacttgggaggctgaggcaggagaatggcgtgaaccggggaagcggagcttacagtgagctgagatcacgccactgcactccagcctgggcgacagagtgagattccatctcaaaaaaaaaaaaaaaaaatttattctgtcacagttcgggagacataaatacaaatttgagatgttggcagggtggcagtccttccaaaggctctagggaagagtcctgccttgtctctttcagattctggtgactgggccacaaccctcttggcttgtggctgcagaactctagtctctgcctccgtcttcacatggccttcccacctctctgagtgtcttagaaagacacctgtcattggatttagggccccctgggtgatccaggattatttcatcttgagatccttaacttaattatgtctgcaaagacccttttttgaaataaggtctcattcataggctgtgagggtcagaatgtgatgtggacatgtcttaggaggggcaccattcttcaacccaccatagtagtttttatcaagtttggaaaaattttggacgttctttctttcttttattatttatttacttattttgaaatggagtctccctctgtcgcccaagctggagtgcagtgacacgatctcggctcattgcaacctccccttcccgggttcaagcgattctcctgcctcagcccccaagtagctgggactacaggtgcccaccaccacgcctggctaatttttgtatttttagtaaaaatggggtttcaccatattggccaggctggtctcaaactcctgatgttgtgatccacccgccttggcctcccaaagtactgggattacaggcgtgagccaccgcacccggcctatttctctaaatttgtcttatttgtcctacttctttattctgtcctttgggattccaatagatatatgttacaatgcttgataatgtcttacagattatgaggctccatagagacagggtcttgctctgttgcccaggctggagtgcagtggcgtgatcatagctcactgcagcctcgaactcctgggctcaagggatcctcctgcctcagcttcagaggagctgggactacagctgcttgccaccatgcccagctaatgtaaaagttgttttgttttgttttgttttgtttgtagagacagagtcttgctgtattgcctgggctggtcttaaactcctgaactcaagccaacctcccgccttggcctccaaaagtgctgggactatagaagcccagccaactttatttttcagtactgtttttctcctctgtgcttcagtttggaaagttctattgctgtcttcaaattcactgatttttaaattgtgcagtgtctaatctgctgttatttccattcagtgaatttttcatttcagttactgtacttactatctttagatggtccactgggttcttttttatacctctcattcctctcctcatgaacatctttttcatgtttttctttaaactcttgagtatattgagccatctatcatctttatcatttctgagttttgtttctatgaaattatttttctcctgattataggttatattttctttcttttttttttttttttgagatggagtctctctctctgttgcccaggctggagtgcaggggcgccatctcggctcactgcaagctcgatctcctgacctcgtgatccacccgcctcagcctcccaaaatgctgggattacaggctcacgtgagccaccgcaccctgcctataagttttattttcctactttttggcatatctagtaatttttaactgaattttggacattgtaaatatgatgttaagcatctggatttgttattgttctttaaagagtgttgggctttgttcaggcagactaggtaaattacttgcaaatcagtttgacctttttgaggcttttttttttgagacagagtcttgctctgtcacccaggcttgagtgcagtggggcaatctcagctcattgcagcctcaacctcctgggcttaagggatcctcctgcctcagtcactgagtagctgaggctacaggcacatgctaccatacctggctaattttttgtattttttgtagacatggggttttggtatgttgcccaggctggtcttgaactcctaggctcaagtgatctgcctgcctcagcctcccaaagtgctgggattagaggtgtgagccaccgtgcctggcctttgatgctaatttttctttttctttttcttttcttttcttttttttttttgagatggagtcttgctctgtcacccaggccagagtgtagtggtgcagtcttggctcactgcaacctccgcctcctgggttcaagtgattcttgtgcctcagcctcctgagtagctgggattacaggcacccatcaccaagcccggctaattttttgtatttttagtagagatgtggtttcgccattttggccaggctggtcttgaactcctgacctcaggtgatctgcccgcctccgcctcccaaagtgctgggattacaggcatgagccactgcacccggcctgaggctaatttttaatctgttagggtgggtctaggtgagccttttctctagggatagtttagctctactgctaaggcataacccttctgaggtctgattaaatatgcatctccactctaggaggctggagcttgattatctccttgcttttggtgagctctgagaatttaccattttattgctcctttttgtgtggtcttactgagtttcactatacacatgtgaagtttagtattcaggaagacttgaagagacccctatgcagatttctggagttttttgagtagtttactcttttccagaactgtgctctgctgcaacctttaataccttggcttccctgaatcctgtctccatcttctcaactcaggaagagcaccatgctctgctcgggcttcccctccttgaattacagtctggaatgttcctccaggcagaaatccagggatgttacagagctcaccttgttcattttccttacttcagggatcacagttctggacttctaaaaacagctatttctctttacatatattttctatatagagaaatatatatatatacacacacaaacacacacacacacacacatacacacacacatatatatatacacacacacgcatatgtatatatatatttgagacagcgtctcactctgttgcccagcctggagtgcagaggtgtgatgatacctcactgcagcctcaacctcccaggcttaagcgatcctcccacctcagcctctgagtagctgggactacaggcacaggccatcatacccggctaattcttttgtattttttgtagagatggggttttgccatattgcccaggctgatctctaactcctgggctcaagcaatccgccaacctttgcctcccaaattgctgggattacaggggtgagcctctgtgcccagccttcatatattttgcagcaataattttctcattgtttatggtggcagagtaatttcatttattatggtaggagtagaagcctttttactggcgttttaatcaagttcagagaagaggagggagttacatgcatgtggtcagttcactgttccttttttttttgagacggagttttgctcttgtcgcccaggctggagtgcagtggcatgatctcggctcactgcaacctccgcctcccgggttcaagcggttctcttgcctcagcctcctgattagctgggattacaggcatgggccaccacgcctggctaattttgtatttttagtagagatggggtttctccatgttgtcaggctggtctcgaactcccaacctcaggtgatctacccgcctcggcctcccaaagtgctgggattacaggcgtgagctaccgcgcctggcctgtcagttcactgttcttaaccagaagtcctagactctcgaaatatatttaaatacttatgcttaagaccgggcgtggtggctcacgcctgtaatcccaacactttgggaggccaaggcaggcgaatcacttgaggtcaggagttagagaccagcctgggcaacatatcaaaaccccgtctctactaaaatacaaaaattagcctggcatagtggtgctcgcctgtaatcccagctactcagaaggctgaggcacaagaatcgcttgaacctgggaggcggaagttgcaatgagccaagatggcaccactgcactctagcctgggtgacacagtgagactctgtctcaaaaaacaaacaaacaaacaaacaaacaaaacttacgtttaacaaacatgctttctaagccaggtgcaggggcttgtaatcccagctgcttgggaggctgaaacaggaggattgctcaagcctaggagtttgagaccagcctgggtgacatagtgagaccctgtctcaagtaaaaaaaaaaaaaaaaaaaaaaaaaaaaaaaatcttttgtctgggcactgcggctcacacctgtaatcccagcactttgggagcccgagccaggtggatcacctgaggtcaggagttcaagactagcctggccaacatggtgaaaacccatctctactaaaaatacaaaaaattagccagacgtgttggcgaatgtctgtaatcccagctacttgggaggctgaggcaggagaatcgcttgaacctgggagacggaggttacagcgagctgatatcacgtcattgtactccagcctagccaacagagtgagactccgtccccccaaaaaaaacacaaaaaaaaaccccaaaaaaagcttttatcacttttatcacacaacagaaatctcatgcaatgtaatcatgttattcacaaaattataggatttgtacaaattttaatgcatagtgtcccacaagcacaggacatggttgtgaaattgtattaataccatgaacttgttatttcattcctgtctgtgtattactgtaaccgtttgttaaacctcactcagtgataatgtcagtgatctaaattggtagctcttcctgaaggtggcctgggacccttagggtaggtctggtcccaggtgagctccttggccaacagcctctttgccaccccacttcagtcccaggcttattcttggcaggcaggccactgggccctggaggagaggacccagccaggggcccttggtggacaggaagggaggaagccctccctcttccagagttactttctgtcctgtcttctaagcccctttccatccacgtgtctgtctttccgttgctcatagtgtctgtctttccgttgcccatagtgtctgtctttccgttgccttgtgaggttggtgaggcagagcagccccagcagggggtgggggttgctgcctgctccagggctgtctggctccggagggctgcctccgacgtgactggggctttatcttccactcctcctcctcctccaggtggacatcgagcagctggatccccgcggccggactcccctgcacctggccaccacgctggggcaccttgagtgtgcccgtgtgctcctggcgcacggcgcagacgtgggcagggagaatcgcagcggctggacaggtgggcagccctgctcaccccagccccacagccggggcctccccagcatcatagacctatggttggctgaagggtcctgccctgtgaccttgcctcgccctcccccagtgctccaggaggctgtgagtacccgggacctggagctggtgcagctggtgcttcggtaccgggactaccagcgggtggtgaagcggctggcgggcatccccgtgctcctggagaagctgcgcaaggtgaggcccagcctctcagcctccacgggagcccttgagcccttctccagtgcagacttagcctctctccccttcgtcctccaggcccaggacttctacgtggagatgaaatgggagttcactagctggggtaagcgggctgcagcaggtcgcttctgggctctcccactttaggtcctgcgcttgctcccctgcctggaatgtgttctcatagttcttccggcggttccctctatgccttagctcagctcagggccaccgcctcagctaggcctttccagattgccccagatactgtcttgactccattattattctcttcactctgtcatgatttgcttactgtattcatgacctgccgctccttgttagaaggtaagctctgagagggcaggagtcctgtctttttcactgttgtattcccagtggctggaacactcagtaggtgtttcataaatatttgttgaaagaatggatgaaagagtgagtgagtgaattaacaaatgatggacactagggacttagtggtgacagaaacatgcccgtcccgacctcaggttgctcttctgtgtgagtatggtctacactggccagggagggggttttggaggagaggctgctctctcttcagttccctcccctgttcctggccacacggatcccaaaccccatgccctgagctggtccaggccgtgtaggccagaccagtcaaagccacctccaacctccgcttccaccagtgcccctggtgtccaagatctgccctagtgacacctacaaagtgtggaagagcggccagaacctgagggtagacaccacactcctgggctttgaccacatgacctggcagcgagggaaccgcagctttgtcttcaggggccaaggtcaggcaggcaggaagtggggcagggtggggacgatgggaggcagccccaggccacccctgatccccctgtgctgttccgtgtctggcagacacaagcgccgtggtcatggagattgaccacgaccgccgggtggtgtacacagagactctggcactggctgggcaggaccgggagctgctgctggctgctgctcagcccactgaggaacaggtgctgagccggcttaccgcgcccgtcgtcaccactcagcttgacaccaagaatatctcctttgagaggtgggtggacatggccttggtcacccttgagccagcccggtggggtgcctgcctcacctggaccactctgcttccccaggaacaagactggcatcctgggctggcgcagtgaaaagacggagatggtgaatgggtatgaagctaaggtgaggctgcagctcccagctgccagcccagctgcactcttgcctacagcaagctgtacaggggattctgacctcccttccccagccctggaggtacagaagcaatgcagcgtggtcaagcacttatatttgggttcaaggcacttctctggtgttttatatggatgtatggatgtatacacagggcacgtgcacacgcacacacacacacacatttattcctcacagcaaccctttctggtaggtgctgttctgttagtattcccattttacgcatgtttattgagtcctttccttggcatcccatttactcttcacaacaaccccaggaagtagggatgatcggtccattttatgatgaggaaatagaggcttagagtggttctgtgacctgtacaaggtcacacagctgttaagtggcagagttggggttcagatcctggctggcctgaccctagagccaggcctttatccctaaaaatgactgcctggctgggcatggtggctcatgcctgtaatcccagcgctttgggaggccgaggtgagcggatcacctgaggtcagttcgagaccagcctggctaacatggtgaaaccccgtctctactaacaatacaaaaaattagccgggtgtggtagcaggcgcctgtaatcccagctactcgggaggctgaggcaggagaattgcttgaacctgggaggcggagcttgcagtgtgcagcgatcccgccacagcactccagcctgggcaacagagcgagactccatctaaaaaaaaaaaaaaaaaaaggctctgcctgttactctgggacccctatgttgcccacgacatgaaagcaggaactaacaaatgccatgggttttgtgtgtggcatctcctctgaaagcctcccctgcttctgtagtctgggaaggcctctgtgctacccccaccagtgcatggaccatgctgttataactccattttattgtctccttatagagattgtaagtctcaggagggcagggatcatgtttggcttgtttactgtatccctgatgcctacctcaatgcctggcacataaaggctcctcaaaaaatgtttgttgaatgaataagtgaatgaatgaatgaatgaatgacctcatatattcacttacccaaaagcctgaagcagagtctctccaggaccctttgctacagggagtgttcccagtgcccttaggggtaagacacagggtaagaccagaactgcttatgagccctttcttcatctgtccccaggtgtatggggcatctaacgtggagctcatcacccgcacacggacagaacatctttcagaacagcacaagggcaaggtcaaaggtaatgaggcagagctggatggggagaggtgttgcaggactgcgggaaccagctcccacttcagtgcttccatcagtattcccactggcatcctagcaagaggctggatgctttattcaggccgatagatttcaattcaggtgccaagccctaaggatgggtagtggctgcctagagtactaagaagtttctaaggactcatctgggttcagtggagagccatgctgcaagtgattactaatgttgctgttgaatttgggagaggagagaaatgccatgtatgccatttattggccattctagtctagtgggacatatcctaggtagaaagtcaggggaccttgccacagattctgtatgcccattgatgccacacctgattctctgggtaccagataccgtgtccgaggtgaaaaagcataatttctacctcacaggggaacaacatgaaatcatgcctatggaagtgcctgaagcaaacacacacacgcacatgcacaccccacagtgcctgccggggcaggcgttttactgtccagggtcaccgagctggagaggagcacttttggaagttgcttctgacctctaggccttccttttagtgttttaagctgtgctcacagaggccctggcccctggtccttgaagcactcagtccccttcaggtgaaggtgcctgagtatgtggttgggtgagcaggccccaccccaggaaccggcctcctccctaggtcttgggtgctgtcacctctgatgaggtgcccaggtgtgtgtggagttgcggtgtcctctgagatgccacatttcttgtaggctgtaagacacctttgcagtccttcctgggaatcgctgagcagcacgggggcccccaaaatggggtgagtgtgtgcaggggtacccgtaagtggagggatgtggatgtggctcaggaggaggcttgggaagcgtcctgcttagcatggcctatgtggacctcctttccacaatgcccaaggccatgtcagcgccacactggcagaggggacagcttgggggccttgtgacaacaaatgagttggcctggcattaggaactgaggggagctcctgggcccctccccatgtggtacagaccctgatcactcagactctgagccaagccaaccccactgccatcactgcagaagaatacttcaaccccaactttgagctgggcaaccgtgatatgggccgccccatggaactgaccaccaagacacagaagtgaggcccctgccggtgctgggaaggtggggggccggggctccaggagatgctgggaggccatggcttcctgcagtgtcccttaccccttgggatctggtgggggcaggttcaaggccaagctgtggctgtgtgaggagcatcccctgtccctgtgtgagcaggtggcccccatcattgacctcatggccgtcagcaatgcgctttttgccaagctccgggacttcatcaccctgcgtctgcctcctggcttcccagttaagattggtgagaccgcacggccatttctcctgagcccgtggcgggccgaccggggtttagatgaggtcggggtggggctgaggctgaggtgtgaggggctgagtggtggcgcctaaaggtttcctcatcctcagaaatcccgatcttccacatcctcaacgcccgcatcaccttcgggaacctcaacggctgcgacgaaccggtgccatcggtgcgaggcagccccagcagcgagacgccttccccaggcagcgactcctccagcgtcagcagctccagctccacgagtgaggccccccgcgagaacgcctgcccctcggctctccccggggtgggtgggaggggcgcgcccggccgtgcctgacccagcccccgcgcccccagcctcctgccgcggctgcgagatctccccagcgttgttcgaggccccgcgcggctacagcatgatgggcggccagcgggaggcggcgacccgggacgacgacgacgacctgctgcaattcgccatccagcagagcctgcttgaggcgggcagtgagtatgaccaggtgcgtctccgcgggcgcgcggggccacgggactccgcgccgccacggctaacgcccacgcctccccgcaggtcaccatctgggaggcgctaaccaacagcaagccaggcacccaccccatgtcctacgagggtcgccgacaggacaggtcagtgcccgctgggccggagagaatcctccggagaggatcctgtctcccctaagccaggacacagccggagaacccgcggggccctcggcagggaccctcctggtatcgggatggcttctgccaccactcctgcctccgaggcggcaggcaggggtcagggatccaggcttcaccgcggagttcagactctccccaggcattgacggggagaacttggtagggtctgggctccgccacgaccaggtgggggccaggacgccgcgggactgaccgcctccactagagggtggtggccgcgggccgccctggagcctccacgccgtgtcccggccccggccggtgggtgggtgcgcccgggagcccgcgacattccttccccacccccaggagcgccccgcccacgccgcagcgccagcctgcgcccccggcgtcagtgcccagccctcggcccagctcagggccaggttccggcggccacgtgttccggagctacgacgagcagctgcggctggcgatggaactgtcggcgcaggagcaggaggagaggcggcggcgcgcgcgccaggaggaggaggagctggagcgcatcctgaggctctcactgaccgagcagtagcgccccctgccgggaccctcgccagcgccacgcgcgccacgcccagggccaggagccagacaaaccccggcctgcgcgcctgcagagcggcggctggagactggagccaccgcctcgcgggtgcagcagcacagcaggcacggttcggggagggattcggcatggccgcggggtaccttcccaggccagggccctggaggcaactggcacggcctggtccccctgctttgctgtattctgattccccaacccgctcccctgggctcagatctgtcctgtcctagggcggagccaggcggtcctgagggggagatgaatccttagaggagcgctgtccctatcccttgctccttctggccggtccgcatttctgttcactaaccccactccaggacactgcccctgaagcctttgcatctctgctcttcactcctggggggcagctgagctccccgcgtgctgtgtcactgctttgttccagacacaaaccagcacgtctagggcccagcccctcccccaccccggcatttcagcgtcaagtgcacttagcggggtacccggctcccccagcccccacacccgtcctgggtctcagggtggttccagcttctccttgggcagccagaagttggagtcccatcccccaaggcacatttttttttttttttttttgtgatcagggagtgtgtccaacgtagccccctggcctgtgcaagccctgactccctcatggtgcctcggagagtggggagcatattgggctggggtaagcactagacccaagtagactggacacaaagggctcgcccagggccctggcgccacccccaccccttcccaccagctgctgctagcctctgtggttgtacatcccacttgcccccacacggagactgactctaaaacccttcatccaatggtgctaacccccggctctcccctgccccacctcacccacccagagaagcacagaccccgccaggggcaggggcccaccgcacacccttgtcccgggcctgtctgggactggccttcccggctcagccagtgaggctcagaagggacacaaagagggatggaagaaaagaacaaagagaaactgttcctcccacccccttccctgatgccaggggcaccagactgattctgaggcacaaataaaagaggcttcataccggaggcttttgctacctaactttacttggggggaacgcctacggtgtgggttggggtccttctgaacctcagagtggagagagctctagggtaagaggctgcctgatggaccctgagcccaggagtgcatcgccaggtctcccaggagcctgggggtagcatttgcagaggctgggggtctcgttcccctcactcccacccatgcaggaggcacagactgaacgcttagtaaaatatttcattcagtacgtcttgtttttctgagagaggcaacggcagagggttgggggcagtgtgtgtgtatttgtgatgaacctaactcctcatgccagttctctcgagatttcttcgcgggggctgccgcgaggaagcagccctcgcccctgtcggtggaaagaaggaagagagttctctaccacagaccgctgtgggtgtagccactgggtccggctctgcagcaaacgggttgtgtatgtgtctgcagaactggggtgacgcccatctggtttaccgctcagggtgatggaatccagtgagctgattaggagaagcgctgtcattttccccagcctgggggtacccatcaaatcgccacccgtttgaggtcaagctcaggctccaataaccccaagcatcacgctaatactaagcactttccctgccctgggcggaggacaaagggggacaccacctcgccgtgcagcaccattgctgagccccccaggttaccccaggcctccctaggccagctccagccgagtcccagacgaggctcgcagtccagcctccgctggagcgacgtgggtctcccctaagctccaagagttctggtctcccgcgaggggcggagttccctccccagtcccgcccccgggcccagcccaagaaggcggggtccggagttcgggactaaaagccggggcggggccgagcttgtgcgccccgccccgctccgcctgcctggcgcgcggggctagtccgtgccgtccaccagctcgcacagcatgttctccagagccgtgatgcgctgctcctgggcctgcacccgctcgcggagggccttgatctcttccagcagcgtctccagggtgtgctgctgctggggcggaggacagagaggccgtgtcgtataggggcggttgggggagatgtagattgggccagagtgcagcagggccgatcttaccgacaagggggcgtcgctggccgactggctgcggcgggggccggagggcgggcgcacgtccaggatgttgcgcttcgtgacccggagctcgcggtgcttggggggcacatagccgtccctcagcgaaatgagcacgggttcggcgtcctggccggatagccattcgtccgcttctagggccggctccgggcctggcgtatccgggtacagatcgtcctggaagaggtctgactgcgggggtgggtggacaggaggacttgcgtgagagggtgcggggcttgctccgctcccttccgcctcgtagccctgcccaacccttctcccggcccctcaccttgcggggcacagtcatgatgataggttcacactttctttcgtgtagcttgtagaacctataagggagcagggttcagcaccctcgcagacttccacgtccttaacttctcctgtctaagaccaagggggttggaggccaacacttgctcagcgcctaccatgcatattgcacattacacacattattggttctgcaataaaacaccctgatggtgtgttcaccatcatcttatagatgaggaaactgaagttgagaatgtaaggctagtgagcggtgggtctggcactgaaacagagctgtcttatccccccgccccgcttttccaaagcactgcattactggggaagccccgtggctaggacccgacatgagtgggggacagaggcgggtaggtgttcaggaggggccaaggctgctgaccgggcgatctcacacttgctgacatccagtccccttttgggcatgaaacccatgccccgctgcggctctttgctgctgaacgtgttcaggtagtgcacgaaaggcggctcgtcggtaatctcaaagtaccgaatgctgctgtcgccctgcaaaatcagtcggttcaggggcgcgcccggacaaggccctccacatctccatccagtgccctgttctccctgcccggccgtgagcaccttgccacacaggtagacgatgctggagtcgggatcgtaaaagggcaataggaccccgttgcttgtgtccatctcctgcagtgccactggctcctcgaagttgttctgcccgagcacaggaggcgtgaccagccctgccccaccctcccgtgctacttcgggacccccagaagcccctttacgcttcctggccttcccaaaccctatgccccaaacctctagtgaccagagttgcaggcccctcccctgggcacatctctcctcctcccctgcgcacatagctcctcctcccctgcacatatacccgctgcgcgccgcatgcagtcacagcaaaccacccccagggactcggcatcaccaggtgggggcgccagcgcaggatccttcacgcgacgcagcaaaactgggcagaggggtgggtgtgagaatggcaggcgctgcagaggtggcagcagccttcagtcctgtccaggtgggcatgccctgcgggtggggggcgcctggccactctcccgtgatgccagtccccgaggcacacaccccaagcctccagctgcgttaccgggtcccacaggcccagctctcgctggctcatgcgggtgaagcccgtggtgaagatatggccctggcgcgtgaagacggcccgcatgggcctcatcccctcgtgggccgcaaacctctcctggggggagggggagacagggagggacatcacccagctgcctgccctgaggagcatggagggatgagcaaccagcttgctgacttgggtgtccggggtggaggagcggatgcggggaagagacaaatggggcctaagcactcagcttcctgcggggccacgtctggcccctgacctggagagcatccgggcctggagagagcaggaggcacgcggctctcagccgatcccgaacccttaagcgcgctcaaaggccgatccctagagcaggggtgtctgctggctccccggagtcgcagcgaggcttttcccgaatgggagctccccgctccgctctggcctcttgggcgccagccacagcccgggaaggcgctcccggcagacccagagaaggagcgagctagcgcgcccggcgcggcctggcctaccgggtcccagagcgcgagttgccgctcactcatcctgctgaagccggtgctgagcagcttcccgtctgcggtgaagacagcccgcagcgggcgggcgccctcgtgaggccgggcttgctcctgctcgccgggttagtgggttagagcgccccggcgccagccccgaccgctctcggcgcgcttgctccacgcagacatgcacgcggcccacgcacccgcaccccaggttagacttgaggctggcgaggccagggccgccgccctcccagggcatccggctgggataagcaacgcgcgagggttgccccatcccccgcccagcgggtccacaaggagaaagggccagccctcgagccagtgtcaggccccagaccctggaagatgcgtctgggtgccggctgagaggagaggggtccaggagctcaggtttcatgcaggttctggtgggaggatggagtttccagcttctcccctcctcaatcccaaagcgaggagcccttctctgagcttctgagatgcaagggaggggagggaacaggagccgggcagagaattgcaggctgggggcttacttagggcagagacctgtggttgcagagacgggggaagggggctagtctctggagcagggatgcgacaggtgaaagccgggaccaggggctctgataatggtgggtacaagggtgctgacagctggccactggtcaaggggttctggggagtggccaggccaggcactcaccgccaccacttggccttttctggggtcaatgatgcgcaaggtcttgtccttgcaggtggtggctagcaggctaccgttgctgttccagcacacactgtggatgacgtctgggtgcatatcatccaggctcagcagcacctccccggtgcccacattccagatgatgatcacattgtcaccacctgcccagagtggccaggcatggtcacctgggtcccacctttgccaccacccacccatctatgggggacccctccttagcccccagacctgcactgagcaggacattcctggcagtagggtgccaggagaggatgcccacacgcttggagtggccctcaagtgtgatgataggttccgtaatgttgcgcatgggggtatagtctggaatctgccacacctgggtaggaagaaaaggtatatggtgggtggaatgaggagccaccctgtccctccactccttccctacctttttttttaaccctactggctctcttgagtggtaagggtcaaatacagggcaagatgtggtggtgcatgcctagaacagaagcagctgggagccaggagggggcactgccagctctccagagacctcccattcactccagcagggagacttcagagcactgccctgctgctctccaggcaccaagttggccatggctataattagtcctaagcagtgcatcctgggagggggtgggcatgtagctaaaaatagtccaggagctgggcagggcagggccctgggacccagcacctcccttattaccacccttagcaccttccccagcacaggtgaggcagccttccctgctcccctgctcaactgcccagcagtagccacctggctcctaccatgatggtggtgtcgtctgaggcactggcgataacgttgtcattgtgtggacaccagtcaatatccagcacaggggcagtgtgcccagtgaccagtgggtagttcttatc

SEQ ID NO: 2 - DNA, 34993 bp, Artificial Sequence
  C to T (bis1)
ggataagaattttttttaattagaaggtaatttttaggttttttttttttaaggatttttattaaagtttttaggaaaattgaggagattttgagttaggggtttagtttgagttttgtttatagtaagtgatttttattgaggtatgaaaataggaagtaaaggagagaggtttgtttttgggtttaggttttttttttttttttttttttgagacggagtttcgttttgtcgtttaggttggagtgtagcgggtttaggttttttaagggatttttttttaattagggtaatagagggatgtttaaggtgatcgttaatatttttttggggggttgattttagggtttaggaggaagggattagtttttttcgttaagagggggagttttagtatgtatttttgggttggttttatttaaatagtgaggtattttaggtgtggagatttttttttttttattttaaatattattgggttagggggttgttagttagttatttttagtagtttaggtaggaagtcggaaatgatgtagtttaaattttttttggtggggttttttgtaagtggggagtcgtttagggtaggattataaatgggttgatttgaggtttgtggttttatcggagaagttaggtatggaaggttgattatatatttacggttaatggttttagagttttaagttatgggtagattagatgtggtgagtgattttggttatggtagtaattaagattaggatgtaggagtgtggtttaagggtttgtttggtatttttttttagtttgggggaggggtttttttttttttttaggtgatttgagaagaatggtaggtaaaggatattgttttggtttgggtagtcgttattggtgttagtttatttttggatgatatagatgggacgtttattttaattattttgttttttttttttgtgtaagtgtttttgggattatttagattgtagtttaaggtgaagggatttttgcgttaagaagttttttggattaaatttgggacggaaaggataggaattgtaagggaattcgttagttttttttttgcgtttttggttttatcggtagggtatgggtttgtatgtgtggagaggtagtaggcgtgattttgggattacgttaattagtgttaattttatggaggtttttattacggtgaatttttgttattatttgaagttattagtggtttttagggttagtaggtttgtatatataggttagttttaggttttttttttttgagttaagggttagatttttattagattaagggaaaagtttatattatgaaggtaggcgagagtagtttttggggtagagttagaatggtggttatttttggggtgtacggattgggagggggtatttggaagttttttaaggtgatggaaatgttttataatatgtttgtttaatttgtagtttatatgcggtttaggtagttttgaatgtggtttaatataaatttataaatttttttaaaatattatgagatttttttgtgattttattttttatttttatttttgtttgttttatttagtttattagttattattagtgttagcgtattttaggtgtggtttaagaaaattttttttttaatgtggtttagggaagtaaaaagattggatatttttattttataatatgattagagtagtagttatatgggtatatatatatgtaaaagtttattaggatgaatatttaggtgtaggtattgatatatataaattttatttttataagggaggaagaggagtttaatatttgttttattttgtaatttatattatgaagagataaattagtttgtagtttgtttcgtaatatgttttcggttttgtttattagagatatttataggataggtattttgaggtttttatttttatttttagggttgttaaagtggaaaaggttgagatagaagtttatggggtgaggagaggtttttgattgagatcgtgtggcgaggtgggttaagtttaaggaaaggggaagatgtatattttttagggttttttgtttttttttttttttggattttttaggtaggtaggaatatatacggtgtttgacgaggtggtataagttgttagagtagttatgttatgtttagttgtttagtaatatatttatatttgttttgtgtgtttatgttcgggagtagagggaggatggggttttttggggataggttgtattttatttttgatttttatgattttttaaattaattaagtataaaaagtttttggttttatttttgtggttaggattgtagggtttttattataataaaagaagtttgtgattttggggtggagcgatatattatggggttggtattggatttggatttcggattgttgggtatttttatgtttttttgtttgagatgttataggatttagattaaatatgtcgttgtatgttagggttagtattttagggtttaggtgtgggatagttttaagtagttagttagggttttaataagtagttaaatatttagggagtgtttgttatgtgttggatatttcgttgggtgttaggtgggttgatgagtaagattgtttatattttttttattttattatttttatttttttattatttttttgatttttattgtgaattaggggaaaggaggtatttggggtataaatttttttgatagatgaggatttgggaggaggagttgggtaatttaatatatttgatgtttattatttttttttgagtttattgggtatttagaggttgtggtcggatatttaacgtaatatataaaggataattgttttgttggtgttgttttttatttttttattttagaattagattatagattcggagatggtagttttttaaaaattatttttattttaatttttttgtttttgaattgaggaagttgaggattttatagtgaggaaagttttgttgggattatagagtaagttgggaataaaggtaatattaagttttagattttttcgattgggcgtttgttaagatttttttttatattttatgttatgtttattttacggagttgtggaatagtggggagatatttataaggtaaggtgtatttttagttttgttatttttagatttgtttgtagttcggggaacggagttatagttttttaggggtatggatttttaattttagggttttttaaattatgataagtttttaggaggttttggttataattatttatggagtattttgtgtttaagttttgttaagttatagtttttaaatattttagtttggtatttttagaattattagagtatttgtgaggtttaatcggtggggttttgggtttgtttaaggggtggttgaaagttatgggtttataaattagtattttatatttttatttttaattatgtttatagtttcgttagagtttacggattttcgtagtttgtttaggggtttattagggagatagtttttttgttaaagaaagaatggatgtgggttagagttttttttttaggttagttgtagagtttcgttattggttgtttttttttattagaagggagtagttttttggattattatttttgatttttttagtaggtttggggggttttattttagtttagttttaattttgttaggaaaaggaagggaattattatgtaaatatagttaggagataggttaggaagttagtaggatacggggaatttcggtacggttttttatttatttttggttagattgggttaggggatagggaggggttcgtatttaggatagtttgatgttaagtttatttttttaagtaggttttatcggtgaataggaatagtagggtttagtcgagttgtttttagttattattagtaggtttggggatgtttttcgagaagatattcgggtttagattggttttgaacgttaggttcggtaaggagcgttagttttaggaattcgaggtagggagttttgggagtagttatcgtttatttgtttttgaggagacggtatttaggttttattggcgtatttgttcggttttttgttttttgttttttattatttcggtaggcgtatcgattacgcgagtagtaggtgtaagacgcgggggtggtattgagatgatataaaattatattcgtttttattttttaagttttgacggttttcgttacggtttttttgttattttaggttggcgttttcgtcggatatagagatggaggtggaggagtagttagttgttcgttttttttagatcgaggagcgggaggcggcgtcgggaacgttttttttcgttagtttacggtttttagggagtatgggtattttaggtcggttttttcgttaagggcgtagtttcgtagtggtcgaggcgggggtttagtttggaggtcgtagtttttcgtttcgtttagtttttcggtttcgtatagcgtttttgttaggtttcggcgttcgttcggcggcggtttggttgtgcggtttcgttttcggtttcgtcgcgtttattcggggcgttgtagttcgtatatattttcgttcgcggtttttttcgggatatttttagcggcgacgcggtcgtagttttttgggttagcgtggggggcgcgggcggcgggttcgggcggcggcggcggtttttgttgttcggttcggtttcggcgaggtttcggcgaggtttcgcgcgttcggttaatcgttcgtttcggggttggttcggaattcgtcgtgttcgtttgttcgttcgttttcgggcgtttttcgtttcgcgtcgtttcgtcgtcgttcgcggttttttttttcgttttttgcgcggttttcggtcgtttttgtaggaagcggcgtaggttttgtttatagggggaggggtcgtattttcgtttcgtcgcgcgttgtcggtcgcgttttttagagaaaggaagttcgggcgcgggtaggagggggcgggggcgtttaaaggggtcgcggtagatgttcggtttcggcgggtagcgtggtttgcggttttggttttcgttgtagcgttcgtttggttcggaggtaatgtgagttatttttatagtttttttttttttatttttcgcgtggggtggatcgggggacgttgggtttacggacggcgagggtggggattagggaagaaggatttggaggtttaagtttcgttttaggttaaaggggttgtgttttggggtattcgtttatttttggttggggtgaggtgtgcgtttttgtttcgtaggtgtttatatttgtgtgtttaggggtgtgtgtgtatgtgttatatttttgttgaatacgtttattgttaataatatggacgtttaggtgttagaaaggttaggtagtgtatttttttgttttcggattaaaaatatatttatttttttatgtatttttttatttagagaggagagaatttgggcggtttttaaagatttttcgaggagtgattattgtgtttgtgtgtatttatatttatttgttattcgttttatatatatttacggtgtttttgggttattagaggtgtgtgtgtttagaaagggtgtatataatatagaggggtcgttttaggtgacggtttttttttttggattttatacgacgaggtaggtaaaggtaaggtaggtgagggacgtgggtgggttggggggtagggagtttaggtagaggtcgtatatgagcgtagttttcgtattgagtatgcgtttttatacgcgtgtgtcgcgcgtgtatttaatttttaatttttgtagtagtaaaaggttcgggtattttgtttgtggggagagggtagaggtttttagggttagatttgggggttaggttagtggtgataattgaggaggggttttttaagagttagagatttttgtttgttaagatgggggtagttttttggtaggggtgtttaagttggtcgattattttaacggtgttagagcggtagtgatttgtgggtgggtaggttttttttttaggggagataagtaatgtttatgagttatattattcgaaatatatgtaaagttgtttttatcgttttttgttgcggtttagattgataagtttgtttgaaatcgcgatttatgggttttatttataattgtattttaaaaaaattttgtaggttttttttttttcgatagttagtcgtttagttggtggggtttttgtaagtaacgatatttagttggtgtgtaggggggagtattatttgtcgtttcgagttgtttttttattagagtttatgggtttggtggttttagcgggaagggggtaaggggcggggggagtgagacgggaggagtggttaggtagttcgtgttaggcgtttagtttacgagcggtggtcgttcgtttattttcgatcgatttttagttatggaattttatttattaaatgtcgaggaggttgttggtagttttgtcgtttggttgtttttgttttttcgttgtgtgggcgcgtttcgagtacgtggtagttgagagcgcgggtcgaagcgtaagcgatttgggtttagtgtttatcgtcgtttggtaaaaaaagaatacggtcgtttaggggatagttttttataatcgataattttttataatttattttgaattttttttgttttcggatttttgggttttgttggggaagaaggatgatttattttgtttatttttttattttattttttattttttggttggtttagagattatttgggagtggttttggcgcggatatatcgtttaaattttgttttttttagtttcgttatagttaaatttttgggtttgggattggagataaaagggtttttggattttttcgtggagatgttattattttaggaagtaggattgttatagtggaattatatataaggttcgaaaaataatttaataaggaaatgtataggtatgttttcggttatttttagatgttttttaatcgcgttagtttttttttttgtattggttgtagttacgatattttgttgatttttggtggtgtaggcgggtagcggtttcgggttttcggagacgttagttggttttttttaggcgggagaaaggggcgaggtagttcgttttttttttattttttttcgttggggtttggtattatagggtgtggaggaggaaggagggaagattatataaagaaatttgagagagtttgtaagtttttgttggtattttttatataaatattttttggattgttgttttaagtagggtcggtgtggaattttttatttttgttttgttttgaggtgggtttaagaaggtatcgtgtttggtttcgttatttgtttcggttcgtttggttgggggagggaggcgttgtttttagggtagttattatttttagtttattttaggaggtagtatttagatttttattttgaaggggagtggatcgagaaagtcggaaaaattaagtagtttgtttttttaaggttaggtagttggagttattcgaattttggtttttttgatattatagttttttttttttagggattggtttaagttttttggtttttttaggttttgtaattggcgtttgagaggttaatttaatttttattatattttttgtagggattattttggaagtatttttttattttggggttatttaggaaggagatagtttttggaattagttatttttttttttgaagggttagttgggtggaggaacggagttgttatttgttgttttttttgtttaattttattttggtttttgttggggatagtgtgcggggggaaagggattatttttttcgcgttattggatattttgtttttaatgatatgtgtggaagatggagtttaattttttaatagggtagggaagattttttagaaatgttttaggggttagatttttggttgttttaatgatttttggtattgatgttttatattttttttaggagtttttaattagacgtttttttttgggaattcggatttttttttatggtttttgggatttaagtttaattttgaagattatatttttatttcgttttttaaacgttcgatttaggttcgtgtttttttatttttttagtaaaaggtaaaatgttagcgggggaggtgcgttttagtttatttggcgttagggtttcgttcgcgtttgggttaggtttgatttttcgtttatttttttacgagattcggggatagtgtagatttttttcggttatttgttatttttagttttacgaggcggattataaattttatgatgtcgcggggttgagttgataagttttattcggggcgtttggttttttttttttttttttattatttttatattttcgtatttcgcgtcggtcgttcgggttgagggtcgggttatgtagttgtggggattcgggggttgcgggcgcgcgtttttgcggcggcgttttcggggttcgcgtttcgtgcgttttcgcgttcgttgcgggcgtttgtttttttcgtcgagcggcgtttttgtgtgcgggggtgtgggaggcgagcgcgagttcgcgtagcgtcgtcgagtgttcgtttttttttagggcgggtgggggttttttcgcgtcgttcgtcgtcgtcgtttcgcgaggacgttcgtcgttcgcgtcgttcgtatcgcgtcgggcgcgtcgttttcgttcgtcgtcgttcgtatatgttcgagtcgtagtttcgcgagtaggtagcgtcggtttttcgtttcgcggtttcgggtttcggtttcggcgtcgtttttttttttcggtcgggcgtcgcggtttcggtatgaggagcgggcgatgattttcgttaacgttttcgttaggaaggggttcgagggtaagtattcgttgtattatttcgtgtggtataatcgttatcgcgagttggagaaggaggttcgcgcgggttaggtaggagcgttttcggggcgtcgcggggatttcgcggtcgggtacgttcgttcggtttggggagggggtgcggcgcgggttgtttcgtttttttggcgagtttgcggcgcgtttttgtttgcggtcgcggtttttgtgtttgttgatcgggaaagggtgatttttttcggtcgggacgggcgggattatacgtgtttcggatttatttagatgagagtagaggtttttgtgtttttttttcgtcggggtagtgagggttgtagggaggggttgcgggttgtgtcggtgttttatgtggtgggagagttcgttttagttagttgagcggcgatatttttcgagtgagggtgcggaggtgggaaaggtttgcgtggggagggggttataggttaagaatggggaagaggttgtgttatatttttaggtattttagttttatttagcgttttttttttaacggtgagcgtttttttttttagtttttaaattgggtagatttttggattttttagagtttagttttagtttaggaatagggagtggagaaagatttttttgggaggttttaagggttttgtttaggtgttgaaaagcgtttttttgttttttggtgttggggtttggtttttaggcgtagaggaagttgaggggttttggttgttggaaggatttgaggttttgcgtattaggtgggttttttggtttttgttggttagtaaggttacgtgggttattagttttgggttgggtagtggtttttagaaaataggggaaggggggatgttttttggttatgttttaggatgttttttggttatgttttagaataaaggtaggtataggttatagattgttatttttgtttttggtatttaggttataggtaggtatttatggtagagatgatttttcgtttttagggtgggttgtaagagttagagttgggttcgggttttatggtttgttgtaggttgagaattttagttttggattgggtttgagattttggggttatgggttgggggtggttagcgtagttgttcgttgtgggaatttattttttgagggttgtttattgagttatgagaagtttagtttgaggagttgtgtaatcgttaagggaagtatggaggtggagggtaggttatcggattgagtaggttgggggttaggatgtgtttttgaagttttacgttgagttagtttttaggtttgtatggtatttagttttgtatggtagtttttgtaaatatgcgagtgatttgtgttcgtaggtttttgggtcggtttgggtggttattttttgttatttgtgtttatgttagtatttttcgagtttttttttagattgaattttttagattttgtttttgtttatttattataaaggtagtgttttgtagttacgagaagtttgttaaagagagtgggttatagtgtttttaggaaatagatgaataaatagggtattaatttttgtttttaaggagtttttgttttggtgaagtaagtgtgaataggaaattttagggtgatgtgtaaagcgttaagatatggttagttagtttttgttggtttttttttgttttttttttttgaaagtaaaagaagataagttttatgtgggaagaattttttaggggtttaaggattattaggtagaaggttgaatttttagaatgttttagttttatttttttgtttgagggtgggtggtttttttattgtagagattggagagaggtagaatgttttgggagaaaagatttttttagtaggtttttttgttgataattttgaagtgggtggttattttgttggggtaaggttggggtggggggtatcggagtcgttgtaggtagaggtgttgggggttgtttatgtgttttttttttttatttttttggttgttttagaaataaggttttagatttatttttatttttgttttagtgagttaatgtttttttgaaatggatattgtttgttttggatttaggttagggggaatatagggtattggtggaggttaatttttgtttaattatagaggagttaggttagtttttttttttttttaggcgtgttaaaaagaggaatgttatttcgtgtaggtgggagagttttttagttgttttttttttcgaggattggtttagagtgaggtttgtatttagatgtatattgtttattttttagggtattaggttttgttttttgtaagggggatttggggatagttatttaatattatgagaaaagtattgtggaattttggtattttagttaggggtttttggtttttagtttttttggtattagtcgttatagaaatagttcggttttttttaagtatttaggagttaggtttttttggttttggtttggtatagttgttttttttttattttaagaaagtttcgtagaggtttttcgtgggtaggtttggtagtgtagttggttgaggagggggttagtatggttatttttagagtaggttaatgggttttgtttagttttaaattgttttgttggaggttggaagtagggagtgatgggtagataggaggtgtttggtgaagggaaggggtatttagtagtgttgtgatgttagttcggtgttttgtttgtcgttatgtatgttttttgttaggtcgggggggatagggttgtaagttagggaatatgttagtttttttttgtttggtatggttagttgggtatggttttggttttggagtcgtgagtttttggtgttttttggggtgggaatagggggaagggttagtttgtgtagttttcgtgggagggatatgtgtgggttgggtttggggagtaggattttgtttttggtaattagaattttgaagtgggtagattgtggttttagagaattattttttttttttttggggcgttttttatcgtgggtttgttttttgttttttttgtttatttttttgatttagaggtaggggagatgggttgtggggtttaggatgtgcgaggagtattttagatttttttttttgtttatattgggtagttttggatgtggggtattattatagttggtaagttaggaagttcgggagagggagttataaattttagaaattaaaaattaatgtgttttgggatgagggggaggggttgtaagggtaggatgggaggggtgatatggagggagaagtttagggtgcggtttttatagttcgtggttttttacgtagtttgaggatgtattttgtttttttttttttgaatgagtttaggtagatttgtttttgtattttacgttgggtaggagaggttaagtaacgattatattagatttttgttttttttttcgtgggttggggaaggggttgagtaggtattattttgagtataggttttgcgttttttatttttttcgtaagtattgtgtttagtttatatatgagatgtatgttttttatattttttttaataaaaggattttgtttatgttaaaggagtttggaaagtattttgttagtgtatatgggtgtgaggggtgtttttgtgtaaatacgtatatatacgttatataggagtggatttttgtagggttagaaggtagttgggtatgtatgtgtttgtatatttaagggtatacgtgagtatttatgagcgtacgagtgtgtatttgtatggtattagtgtgtattagagtgtggtgtgtgtgtttgagtggaggtagggaggttttttgtttagggatttttagttataaaattttaaagattttattttttgattttagttgaggtttgttgggataaggaattttcgtttttttggtggggagggttgggtgttgggttttatgggaaatttttttattttagtaattaaatagttagaggtttttgttgaggagaagttggaggtttttgttgaggagattaatgaatttttttatttgggtttagggtaaggtgttatttatattgtaggcggtattttgggtttgtggggagagttgttttggagtttggttgagtgtatggggttttgtatggggtgtatggggtgttgagttatttaggtttttttggggagtgtttttgaggtgtggggatggggaggagtattttgtttgtaaggaagtgttagtcgttttttggagtttggagttgaggtatttgatggggaggtggaggtagtatttggagttttgaggttaggtagcggtttgttagttttttagggttttattagttgtagcggttgcggttgtagtatttggggtagggttgggaggtttggattgtttagtatttttttagttagttcgggttttgtggtttttttttattttcgttgtcgggtttaggattttatttaggttgtaagtttcggagtttagtttaattaggattggataagagtaaataatattttttttttttgtgaggggttatagtttagaggttaataggggttaggttcgttggtttttttgaggtttttagtatattgaaaaatgaagaaattttaggataaggttataaaaattatataaataattttaaattatttaaaatgttttatttttgataatggagtttatggttatgttttaaaatatttaattgttgttagaagatgcgtaatgaaaagtagtgttttttgtttcgttttttttatttttttagtattttggattttttttgttatttatttttttaattataaataatatattgtttatattgttttttttttttttttttttttttttttttttttttttttgttttttttttttttttttttttttttttttttttttttttttttttatgagatagcgttttattttgttatttaggttggagtgtagtagtgtgattatagtttagtgtagtttttgttttttaggtttaggtgatttttttattttagttttttaaggagttaggattataggtggtgttattatgtttggttaatttttgtatttttttttgtagagatggggttttgttatgttgtttaggttggtttcgaatttttgagtttaagtgatttatttattttggttttttaaagtgttgggattatagacgtgagtttttcggtataaataatatatttttgtaatgattttttggttaattatttttttttttttgtgtttttttagtttagtattttatgtatttgtttagtaaatatttatgtgttaggtgttgtttggggagtggggaattagtagtgaataaagtaggtagggatttggttgatggggtttttgttcgaggtgtaggaggtgtttaataggtatttggacgggtagtggatagagttatagtagttgttattttagatgggttgttagggtgggtttttttaaggaggtgatatttgagtagtagtttgagtgaagggagggagaaagttttggggttttttggaggattttggagaacgtttcggggaaggttattggcgaagggtggagtaaatgagtttaaagagaagtttggggttattggattttttgttatttacgatggaaagttattggaagattttgaattaaagagtgttaggatttgagtaatattttatagggtgattttagttgttataggtgaggtggataatagagtttggtaatcggggagtagtaaagaggtagtagggggttgttagtgagagatgggggggtaatagttgtaaggtagtggaaattgggcggtttttaggtttgttttggaggtagagtttataagtttttttgatgggttagatgtggagggtgcgggaaaaagaagagatgtagatagttttaaagttggtttttttttttatttgaaaatgtagtaaatttaggtgatgtttattgtttatgggggtaggtgtagttgtttaggaatgtagaaaataaggaaaagttaagaaagttatttttagaatgaagaaggtaagagaaagggtaggagacgttatggaaagttaggttgttttattttgttttatgaatttaatgatttttttatattttttttgaggatgtaaattattgtttttttttaaagagtttttttttattttttgtattaagagaattttttttgggtttttagtatttaatttgtttttttttttttttttttttttttttttgatacggagtttcgttttgtttttcgcgttagagtgtagtggcgtaatttcggtttattgtaagtttcgtttttcgggtttatattatttttttgttttagtttttcgagtagttgtgattataggcgttcgttattacgtttagttaattttttgtatttttagtagagacggggttttatcgtgttagttaggatggtttcgattttttgatttcgtgattcgtttatttcggttttttaaagagttgggattataggcgtgagttattgtatttagtcgttttagtatttaatttgtatgttttggtttattttatatgggaagtttttattaagtgtttagttttttttggttgttgggttatatttaagaatggggttggggagtttagggatgtgtgggtgttattgtaaggtgattaggtggtaggttggtttgtttattgtagggttattagatgtttgtattttgaggtttttgggataattttttattcgggtagatagggtggtggtggtgtgatttggttgttagtggtttaggatttaggtagggaaggggttggggttttacggattattggtttttagtattatattttattttttgttgtggttaatgtttttgagtttagagtattttatgtttaatttttataaagaataaatttttggtgttttgtggtgaggaaggggggtattttttagtttaatgaggttgggaaggggattaggggattttgaattgtaattagtttttttgtatttagttttagttttatttttatttttgttatttttattgtttgtaggttttatttatattttttaggggggttgggggttatttggtttgttttttatgtggacgtttttttttgtggttgttttagttttagttttttttgtttttttaagttagttgtgaggttttagttattttttatgttttaaagttgtgttgaagttttttatttgttgatattttttttttttatttttgtgggttttaaatattttattgatttttttttttttttttttttgagatagggtttggttttgttgtttaggttggagtgtagtgggatgatttttgtttattgtaatttttggttttttggtttaagggatttttttattttagttttttagtagttgggacgataggtatgtattattacgtttggttaattttagtatttttttgtagtatagagttttattatattgtttacgttggttttaaatttttgggtttaagtgatttgtttatttcggttttttaaagtttataggtatgagttattgcgtttagtttgatattttttttttttttttttgagatagagtttttttttgttatttaggttggagtgtagtggtgcgatttttgtttattgtaatttttattttttaggtttaagcgatttttgtgttttagtttttttagtagttgggattataggaattttttattacgtttagttaatttttgtatttttagtagagatggggttttattatgttggttaggttggttttaaatttttgatttttggtgatttgttcgtttcggttttttaaagtgttgggattataggtatgagttattgtgtttggttttttgatatttttatatatttaatattttttggtattttttaattttttgtatagatttaagtttttatttgggattattttttttttatttgaagaattttttttaatattttttgtatatttggtaataaatttttttagaatttgtttgtttgttaatatatttattttttttttagttttgaagaatatttttatcgggtatggaattttaggttaatattagttatattggattagagaaaaaaaaaaaaagaattttaggttgaaagtttttgtttttgttttttttttttagtattttaaagattttattatattgttttttggtttatatagtttttgatgagaagaatatagtattttttgtatttgtttttttatatataatggattttatttttttgaatgtttttaggattttttttttattattagtttttagtatttgattatgatggattttggtgtagtttatttcgtgtttgttttatttggggtttattgaattttttggtttttggttttattttggtattagtttttataataaattattataaattaggtgggttaaaataataaatatttggtcgggtgtggtggtttacgtttgtaattttagtattttgggaggtcgaggcgggcggattacgaggttaggagatcgagattatgttggttaatacggtgaaatttcgtttttattaaaaatataaaaaattagtcgggcgtggtggtgggtgtttgtaattttagttatttgggaggttgaggtaggagaatggcgtgaatcggggaagcggagtttatagtgagttgagattacgttattgtattttagtttgggcgatagagtgagattttattttaaaaaaaaaaaaaaaaaatttattttgttatagttcgggagatataaatataaatttgagatgttggtagggtggtagtttttttaaaggttttagggaagagttttgttttgttttttttagattttggtgattgggttataatttttttggtttgtggttgtagaattttagtttttgttttcgtttttatatggtttttttatttttttgagtgttttagaaagatatttgttattggatttagggttttttgggtgatttaggattattttattttgagatttttaatttaattatgtttgtaaagatttttttttgaaataaggttttatttataggttgtgagggttagaatgtgatgtggatatgttttaggaggggtattattttttaatttattatagtagtttttattaagtttggaaaaattttggacgtttttttttttttttattatttatttatttattttgaaatggagtttttttttgtcgtttaagttggagtgtagtgatacgatttcggtttattgtaatttttttttttcgggtttaagcgatttttttgttttagtttttaagtagttgggattataggtgtttattattacgtttggttaatttttgtatttttagtaaaaatggggttttattatattggttaggttggttttaaatttttgatgttgtgatttattcgttttggttttttaaagtattgggattataggcgtgagttatcgtattcggtttatttttttaaatttgttttatttgttttatttttttattttgttttttgggattttaatagatatatgttataatgtttgataatgttttatagattatgaggttttatagagatagggttttgttttgttgtttaggttggagtgtagtggcgtgattatagtttattgtagtttcgaatttttgggtttaagggatttttttgttttagttttagaggagttgggattatagttgtttgttattatgtttagttaatgtaaaagttgttttgttttgttttgttttgtttgtagagatagagttttgttgtattgtttgggttggttttaaatttttgaatttaagttaatttttcgttttggtttttaaaagtgttgggattatagaagtttagttaattttattttttagtattgttttttttttttgtgttttagtttggaaagttttattgttgtttttaaatttattgatttttaaattgtgtagtgtttaatttgttgttatttttatttagtgaattttttattttagttattgtatttattatttttagatggtttattgggtttttttttatattttttatttttttttttatgaatattttttttatgtttttttttaaatttttgagtatattgagttatttattatttttattatttttgagttttgtttttatgaaattattttttttttgattataggttatatttttttttttttttttttttttttgagatggagtttttttttttgttgtttaggttggagtgtaggggcgttatttcggtttattgtaagttcgattttttgatttcgtgatttattcgttttagttttttaaaatgttgggattataggtttacgtgagttatcgtattttgtttataagttttatttttttattttttggtatatttagtaatttttaattgaattttggatattgtaaatatgatgttaagtatttggatttgttattgttttttaaagagtgttgggttttgtttaggtagattaggtaaattatttgtaaattagtttgatttttttgaggtttttttttttgagatagagttttgttttgttatttaggtttgagtgtagtggggtaattttagtttattgtagttttaattttttgggtttaagggatttttttgttttagttattgagtagttgaggttataggtatatgttattatatttggttaattttttgtattttttgtagatatggggttttggtatgttgtttaggttggttttgaatttttaggtttaagtgatttgtttgttttagttttttaaagtgttgggattagaggtgtgagttatcgtgtttggtttttgatgttaattttttttttttttttttttttttttttttttttttttttgagatggagttttgttttgttatttaggttagagtgtagtggtgtagttttggtttattgtaattttcgttttttgggtttaagtgatttttgtgttttagttttttgagtagttgggattataggtatttattattaagttcggttaattttttgtatttttagtagagatgtggtttcgttattttggttaggttggttttgaatttttgattttaggtgatttgttcgttttcgttttttaaagtgttgggattataggtatgagttattgtattcggtttgaggttaatttttaatttgttagggtgggtttaggtgagttttttttttagggatagtttagttttattgttaaggtataatttttttgaggtttgattaaatatgtatttttattttaggaggttggagtttgattatttttttgtttttggtgagttttgagaatttattattttattgtttttttttgtgtggttttattgagttttattatatatatgtgaagtttagtatttaggaagatttgaagagatttttatgtagatttttggagttttttgagtagtttatttttttttagaattgtgttttgttgtaatttttaatattttggtttttttgaattttgtttttatttttttaatttaggaagagtattatgttttgttcgggttttttttttttgaattatagtttggaatgtttttttaggtagaaatttagggatgttatagagtttattttgtttattttttttattttagggattatagttttggatttttaaaaatagttatttttttttatatatattttttatatagagaaatatatatatatatatatataaatatatatatatatatatatatatatatatatatatatatatatatatacgtatatgtatatatatatttgagatagcgttttattttgttgtttagtttggagtgtagaggtgtgatgatattttattgtagttttaattttttaggtttaagcgatttttttattttagtttttgagtagttgggattataggtataggttattatattcggttaatttttttgtattttttgtagagatggggttttgttatattgtttaggttgatttttaatttttgggtttaagtaattcgttaatttttgttttttaaattgttgggattataggggtgagtttttgtgtttagtttttatatattttgtagtaataatttttttattgtttatggtggtagagtaattttatttattatggtaggagtagaagtttttttattggcgttttaattaagtttagagaagaggagggagttatatgtatgtggttagtttattgttttttttttttttgagacggagttttgtttttgtcgtttaggttggagtgtagtggtatgatttcggtttattgtaattttcgtttttcgggtttaagcggtttttttgttttagttttttgattagttgggattataggtatgggttattacgtttggttaattttgtatttttagtagagatggggtttttttatgttgttaggttggtttcgaatttttaattttaggtgatttattcgtttcggttttttaaagtgttgggattataggcgtgagttatcgcgtttggtttgttagtttattgtttttaattagaagttttagattttcgaaatatatttaaatatttatgtttaagatcgggcgtggtggtttacgtttgtaattttaatattttgggaggttaaggtaggcgaattatttgaggttaggagttagagattagtttgggtaatatattaaaatttcgtttttattaaaatataaaaattagtttggtatagtggtgttcgtttgtaattttagttatttagaaggttgaggtataagaatcgtttgaatttgggaggcggaagttgtaatgagttaagatggtattattgtattttagtttgggtgatatagtgagattttgttttaaaaaataaataaataaataaataaataaaatttacgtttaataaatatgttttttaagttaggtgtaggggtttgtaattttagttgtttgggaggttgaaataggaggattgtttaagtttaggagtttgagattagtttgggtgatatagtgagattttgttttaagtaaaaaaaaaaaaaaaaaaaaaaaaaaaaaaaattttttgtttgggtattgcggtttatatttgtaattttagtattttgggagttcgagttaggtggattatttgaggttaggagtttaagattagtttggttaatatggtgaaaatttatttttattaaaaatataaaaaattagttagacgtgttggcgaatgtttgtaattttagttatttgggaggttgaggtaggagaatcgtttgaatttgggagacggaggttatagcgagttgatattacgttattgtattttagtttagttaatagagtgagatttcgtttttttaaaaaaaatataaaaaaaaattttaaaaaaagtttttattatttttattatataatagaaattttatgtaatgtaattatgttatttataaaattataggatttgtataaattttaatgtatagtgttttataagtataggatatggttgtgaaattgtattaatattatgaatttgttattttatttttgtttgtgtattattgtaatcgtttgttaaattttatttagtgataatgttagtgatttaaattggtagttttttttgaaggtggtttgggatttttagggtaggtttggttttaggtgagttttttggttaatagtttttttgttattttattttagttttaggtttatttttggtaggtaggttattgggttttggaggagaggatttagttaggggtttttggtggataggaagggaggaagtttttttttttttagagttattttttgttttgttttttaagtttttttttatttacgtgtttgttttttcgttgtttatagtgtttgttttttcgttgtttatagtgtttgttttttcgttgttttgtgaggttggtgaggtagagtagttttagtagggggtgggggttgttgtttgttttagggttgtttggtttcggagggttgttttcgacgtgattggggttttattttttattttttttttttttttaggtggatatcgagtagttggattttcgcggtcggatttttttgtatttggttattacgttggggtattttgagtgtgttcgtgtgtttttggcgtacggcgtagacgtgggtagggagaatcgtagcggttggataggtgggtagttttgtttattttagttttatagtcggggtttttttagtattatagatttatggttggttgaagggttttgttttgtgattttgtttcgtttttttttagtgttttaggaggttgtgagtattcgggatttggagttggtgtagttggtgtttcggtatcgggattattagcgggtggtgaagcggttggcgggtattttcgtgtttttggagaagttgcgtaaggtgaggtttagttttttagtttttacgggagtttttgagtttttttttagtgtagatttagtttttttttttttcgttttttaggtttaggatttttacgtggagatgaaatgggagtttattagttggggtaagcgggttgtagtaggtcgtttttgggtttttttattttaggttttgcgtttgtttttttgtttggaatgtgtttttatagttttttcggcggttttttttatgttttagtttagtttagggttatcgttttagttaggtttttttagattgttttagatattgttttgattttattattattttttttattttgttatgatttgtttattgtatttatgatttgtcgttttttgttagaaggtaagttttgagagggtaggagttttgttttttttattgttgtatttttagtggttggaatatttagtaggtgttttataaatatttgttgaaagaatggatgaaagagtgagtgagtgaattaataaatgatggatattagggatttagtggtgatagaaatatgttcgtttcgattttaggttgtttttttgtgtgagtatggtttatattggttagggagggggttttggaggagaggttgttttttttttagtttttttttttgtttttggttatacggattttaaattttatgttttgagttggtttaggtcgtgtaggttagattagttaaagttatttttaattttcgtttttattagtgtttttggtgtttaagatttgttttagtgatatttataaagtgtggaagagcggttagaatttgagggtagatattatatttttgggttttgattatatgatttggtagcgagggaatcgtagttttgtttttaggggttaaggttaggtaggtaggaagtggggtagggtggggacgatgggaggtagttttaggttatttttgatttttttgtgttgtttcgtgtttggtagatataagcgtcgtggttatggagattgattacgatcgtcgggtggtgtatatagagattttggtattggttgggtaggatcgggagttgttgttggttgttgtttagtttattgaggaataggtgttgagtcggtttatcgcgttcgtcgttattatttagtttgatattaagaatattttttttgagaggtgggtggatatggttttggttatttttgagttagttcggtggggtgtttgttttatttggattattttgtttttttaggaataagattggtattttgggttggcgtagtgaaaagacggagatggtgaatgggtatgaagttaaggtgaggttgtagtttttagttgttagtttagttgtatttttgtttatagtaagttgtataggggattttgattttttttttttagttttggaggtatagaagtaatgtagcgtggttaagtatttatatttgggtttaaggtatttttttggtgttttatatggatgtatggatgtatatatagggtacgtgtatacgtatatatatatatatatttattttttatagtaattttttttggtaggtgttgttttgttagtatttttattttacgtatgtttattgagttttttttttggtattttatttattttttataataattttaggaagtagggatgatcggtttattttatgatgaggaaatagaggtttagagtggttttgtgatttgtataaggttatatagttgttaagtggtagagttggggtttagattttggttggtttgattttagagttaggtttttatttttaaaaatgattgtttggttgggtatggtggtttatgtttgtaattttagcgttttgggaggtcgaggtgagcggattatttgaggttagttcgagattagtttggttaatatggtgaaatttcgtttttattaataatataaaaaattagtcgggtgtggtagtaggcgtttgtaattttagttattcgggaggttgaggtaggagaattgtttgaatttgggaggcggagtttgtagtgtgtagcgatttcgttatagtattttagtttgggtaatagagcgagattttatttaaaaaaaaaaaaaaaaaaaggttttgtttgttattttgggatttttatgttgtttacgatatgaaagtaggaattaataaatgttatgggttttgtgtgtggtattttttttgaaagttttttttgtttttgtagtttgggaaggtttttgtgttatttttattagtgtatggattatgttgttataattttattttattgtttttttatagagattgtaagttttaggagggtagggattatgtttggtttgtttattgtatttttgatgtttattttaatgtttggtatataaaggttttttaaaaaatgtttgttgaatgaataagtgaatgaatgaatgaatgaatgattttatatatttatttatttaaaagtttgaagtagagtttttttaggattttttgttatagggagtgtttttagtgtttttaggggtaagatatagggtaagattagaattgtttatgagttttttttttatttgtttttaggtgtatggggtatttaacgtggagtttattattcgtatacggatagaatattttttagaatagtataagggtaaggttaaaggtaatgaggtagagttggatggggagaggtgttgtaggattgcgggaattagtttttattttagtgtttttattagtatttttattggtattttagtaagaggttggatgttttatttaggtcgatagattttaatttaggtgttaagttttaaggatgggtagtggttgtttagagtattaagaagtttttaaggatttatttgggtttagtggagagttatgttgtaagtgattattaatgttgttgttgaatttgggagaggagagaaatgttatgtatgttatttattggttattttagtttagtgggatatattttaggtagaaagttaggggattttgttatagattttgtatgtttattgatgttatatttgattttttgggtattagatatcgtgttcgaggtgaaaaagtataatttttattttataggggaataatatgaaattatgtttatggaagtgtttgaagtaaatatatatacgtatatgtatattttatagtgtttgtcggggtaggcgttttattgtttagggttatcgagttggagaggagtatttttggaagttgtttttgatttttaggttttttttttagtgttttaagttgtgtttatagaggttttggtttttggtttttgaagtatttagttttttttaggtgaaggtgtttgagtatgtggttgggtgagtaggttttattttaggaatcggttttttttttaggttttgggtgttgttatttttgatgaggtgtttaggtgtgtgtggagttgcggtgttttttgagatgttatattttttgtaggttgtaagatatttttgtagttttttttgggaatcgttgagtagtacgggggtttttaaaatggggtgagtgtgtgtaggggtattcgtaagtggagggatgtggatgtggtttaggaggaggtttgggaagcgttttgtttagtatggtttatgtggattttttttttataatgtttaaggttatgttagcgttatattggtagaggggatagtttgggggttttgtgataataaatgagttggtttggtattaggaattgaggggagtttttgggtttttttttatgtggtatagattttgattatttagattttgagttaagttaattttattgttattattgtagaagaatattttaattttaattttgagttgggtaatcgtgatatgggtcgttttatggaattgattattaagatatagaagtgaggtttttgtcggtgttgggaaggtggggggtcggggttttaggagatgttgggaggttatggttttttgtagtgttttttattttttgggatttggtgggggtaggtttaaggttaagttgtggttgtgtgaggagtattttttgtttttgtgtgagtaggtggtttttattattgattttatggtcgttagtaatgcgttttttgttaagtttcgggattttattattttgcgtttgttttttggttttttagttaagattggtgagatcgtacggttattttttttgagttcgtggcgggtcgatcggggtttagatgaggtcggggtggggttgaggttgaggtgtgaggggttgagtggtggcgtttaaaggtttttttatttttagaaatttcgattttttatatttttaacgttcgtattattttcgggaattttaacggttgcgacgaatcggtgttatcggtgcgaggtagttttagtagcgagacgttttttttaggtagcgatttttttagcgttagtagttttagttttacgagtgaggtttttcgcgagaacgtttgtttttcggtttttttcggggtgggtgggaggggcgcgttcggtcgtgtttgatttagttttcgcgtttttagttttttgtcgcggttgcgagatttttttagcgttgttcgaggtttcgcgcggttatagtatgatgggcggttagcgggaggcggcgattcgggacgacgacgacgatttgttgtaattcgttatttagtagagtttgtttgaggcgggtagtgagtatgattaggtgcgttttcgcgggcgcgcggggttacgggatttcgcgtcgttacggttaacgtttacgttttttcgtaggttattatttgggaggcgttaattaatagtaagttaggtatttattttatgttttacgagggtcgtcgataggataggttagtgttcgttgggtcggagagaatttttcggagaggattttgttttttttaagttaggatatagtcggagaattcgcggggttttcggtagggatttttttggtatcgggatggtttttgttattatttttgttttcgaggcggtaggtaggggttagggatttaggttttatcgcggagtttagattttttttaggtattgacggggagaatttggtagggtttgggtttcgttacgattaggtgggggttaggacgtcgcgggattgatcgtttttattagagggtggtggtcgcgggtcgttttggagtttttacgtcgtgtttcggtttcggtcggtgggtgggtgcgttcgggagttcgcgatattttttttttatttttaggagcgtttcgtttacgtcgtagcgttagtttgcgttttcggcgttagtgtttagttttcggtttagtttagggttaggtttcggcggttacgtgtttcggagttacgacgagtagttgcggttggcgatggaattgtcggcgtaggagtaggaggagaggcggcggcgcgcgcgttaggaggaggaggagttggagcgtattttgaggtttttattgatcgagtagtagcgttttttgtcgggattttcgttagcgttacgcgcgttacgtttagggttaggagttagataaatttcggtttgcgcgtttgtagagcggcggttggagattggagttatcgtttcgcgggtgtagtagtatagtaggtacggttcggggagggattcggtatggtcgcggggtatttttttaggttagggttttggaggtaattggtacggtttggtttttttgttttgttgtattttgattttttaattcgtttttttgggtttagatttgttttgttttagggcggagttaggcggttttgagggggagatgaatttttagaggagcgttgtttttattttttgttttttttggtcggttcgtatttttgtttattaattttattttaggatattgtttttgaagtttttgtatttttgttttttatttttggggggtagttgagtttttcgcgtgttgtgttattgttttgttttagatataaattagtacgtttagggtttagttttttttttatttcggtattttagcgttaagtgtatttagcggggtattcggtttttttagtttttatattcgttttgggttttagggtggttttagtttttttttgggtagttagaagttggagttttattttttaaggtatatttttttttttttttttttgtgattagggagtgtgtttaacgtagttttttggtttgtgtaagttttgatttttttatggtgtttcggagagtggggagtatattgggttggggtaagtattagatttaagtagattggatataaagggttcgtttagggttttggcgttatttttatttttttttattagttgttgttagtttttgtggttgtatattttatttgtttttatacggagattgattttaaaattttttatttaatggtgttaattttcggtttttttttgttttattttatttatttagagaagtatagatttcgttaggggtaggggtttatcgtatatttttgtttcgggtttgtttgggattggttttttcggtttagttagtgaggtttagaagggatataaagagggatggaagaaaagaataaagagaaattgttttttttatttttttttttgatgttaggggtattagattgattttgaggtataaataaaagaggttttatatcggaggtttttgttatttaattttatttggggggaacgtttacggtgtgggttggggtttttttgaattttagagtggagagagttttagggtaagaggttgtttgatggattttgagtttaggagtgtatcgttaggttttttaggagtttgggggtagtatttgtagaggttgggggtttcgttttttttatttttatttatgtaggaggtatagattgaacgtttagtaaaatattttatttagtacgttttgtttttttgagagaggtaacggtagagggttgggggtagtgtgtgtgtatttgtgatgaatttaattttttatgttagttttttcgagattttttcgcgggggttgtcgcgaggaagtagttttcgtttttgtcggtggaaagaaggaagagagttttttattatagatcgttgtgggtgtagttattgggttcggttttgtagtaaacgggttgtgtatgtgtttgtagaattggggtgacgtttatttggtttatcgtttagggtgatggaatttagtgagttgattaggagaagcgttgttattttttttagtttgggggtatttattaaatcgttattcgtttgaggttaagtttaggttttaataattttaagtattacgttaatattaagtattttttttgttttgggcggaggataaagggggatattatttcgtcgtgtagtattattgttgagttttttaggttattttaggtttttttaggttagttttagtcgagttttagacgaggttcgtagtttagttttcgttggagcgacgtgggttttttttaagttttaagagttttggtttttcgcgaggggcggagttttttttttagtttcgttttcgggtttagtttaagaaggcggggttcggagttcgggattaaaagtcggggcggggtcgagtttgtgcgtttcgtttcgtttcgtttgtttggcgcgcggggttagttcgtgtcgtttattagttcgtatagtatgttttttagagtcgtgatgcgttgtttttgggtttgtattcgttcgcggagggttttgattttttttagtagcgtttttagggtgtgttgttgttggggcggaggatagagaggtcgtgtcgtataggggcggttgggggagatgtagattgggttagagtgtagtagggtcgattttatcgataagggggcgtcgttggtcgattggttgcggcgggggtcggagggcgggcgtacgtttaggatgttgcgtttcgtgattcggagttcgcggtgtttggggggtatatagtcgttttttagcgaaatgagtacgggttcggcgttttggtcggatagttattcgttcgtttttagggtcggtttcgggtttggcgtattcgggtatagatcgttttggaagaggtttgattgcgggggtgggtggataggaggatttgcgtgagagggtgcggggtttgtttcgttttttttcgtttcgtagttttgtttaatttttttttcggttttttattttgcggggtatagttatgatgataggtttatattttttttcgtgtagtttgtagaatttataagggagtagggtttagtattttcgtagatttttacgtttttaattttttttgtttaagattaagggggttggaggttaatatttgtttagcgtttattatgtatattgtatattatatatattattggttttgtaataaaatattttgatggtgtgtttattattattttatagatgaggaaattgaagttgagaatgtaaggttagtgagcggtgggtttggtattgaaatagagttgttttattttttcgtttcgtttttttaaagtattgtattattggggaagtttcgtggttaggattcgatatgagtgggggatagaggcgggtaggtgtttaggaggggttaaggttgttgatcgggcgattttatatttgttgatatttagtttttttttgggtatgaaatttatgtttcgttgcggttttttgttgttgaacgtgtttaggtagtgtacgaaaggcggttcgtcggtaattttaaagtatcgaatgttgttgtcgttttgtaaaattagtcggtttaggggcgcgttcggataaggttttttatatttttatttagtgttttgttttttttgttcggtcgtgagtattttgttatataggtagacgatgttggagtcgggatcgtaaaagggtaataggatttcgttgtttgtgtttattttttgtagtgttattggtttttcgaagttgttttgttcgagtataggaggcgtgattagttttgttttattttttcgtgttatttcgggatttttagaagtttttttacgttttttggtttttttaaattttatgttttaaatttttagtgattagagttgtaggttttttttttgggtatattttttttttttttttgcgtatatagtttttttttttttgtatatatattcgttgcgcgtcgtatgtagttatagtaaattatttttagggattcggtattattaggtgggggcgttagcgtaggattttttacgcgacgtagtaaaattgggtagaggggtgggtgtgagaatggtaggcgttgtagaggtggtagtagtttttagttttgtttaggtgggtatgttttgcgggtggggggcgtttggttattttttcgtgatgttagttttcgaggtatatattttaagtttttagttgcgttatcgggttttataggtttagttttcgttggtttatgcgggtgaagttcgtggtgaagatatggttttggcgcgtgaagacggttcgtatgggttttattttttcgtgggtcgtaaattttttttggggggagggggagatagggagggatattatttagttgtttgttttgaggagtatggagggatgagtaattagtttgttgatttgggtgttcggggtggaggagcggatgcggggaagagataaatggggtttaagtatttagttttttgcggggttacgtttggtttttgatttggagagtattcgggtttggagagagtaggaggtacgcggtttttagtcgatttcgaatttttaagcgcgtttaaaggtcgatttttagagtaggggtgtttgttggtttttcggagtcgtagcgaggtttttttcgaatgggagtttttcgtttcgttttggttttttgggcgttagttatagttcgggaaggcgttttcggtagatttagagaaggagcgagttagcgcgttcggcgcggtttggtttatcgggttttagagcgcgagttgtcgtttatttattttgttgaagtcggtgttgagtagtttttcgtttgcggtgaagatagttcgtagcgggcgggcgttttcgtgaggtcgggtttgtttttgttcgtcgggttagtgggttagagcgtttcggcgttagtttcgatcgttttcggcgcgtttgttttacgtagatatgtacgcggtttacgtattcgtattttaggttagatttgaggttggcgaggttagggtcgtcgtttttttagggtattcggttgggataagtaacgcgcgagggttgttttatttttcgtttagcgggtttataaggagaaagggttagttttcgagttagtgttaggttttagattttggaagatgcgtttgggtgtcggttgagaggagaggggtttaggagtttaggttttatgtaggttttggtgggaggatggagtttttagttttttttttttttaattttaaagcgaggagtttttttttgagtttttgagatgtaagggaggggagggaataggagtcgggtagagaattgtaggttgggggtttatttagggtagagatttgtggttgtagagacgggggaagggggttagtttttggagtagggatgcgataggtgaaagtcgggattaggggttttgataatggtgggtataagggtgttgatagttggttattggttaaggggttttggggagtggttaggttaggtatttatcgttattatttggttttttttggggttaatgatgcgtaaggttttgtttttgtaggtggtggttagtaggttatcgttgttgttttagtatatattgtggatgacgtttgggtgtatattatttaggtttagtagtattttttcggtgtttatattttagatgatgattatattgttattatttgtttagagtggttaggtatggttatttgggttttatttttgttattatttatttatttatgggggatttttttttagtttttagatttgtattgagtaggatatttttggtagtagggtgttaggagaggatgtttatacgtttggagtggtttttaagtgtgatgataggtttcgtaatgttgcgtatgggggtatagtttggaatttgttatatttgggtaggaagaaaaggtatatggtgggtggaatgaggagttattttgtttttttattttttttttatttttttttttaattttattggtttttttgagtggtaagggttaaatatagggtaagatgtggtggtgtatgtttagaatagaagtagttgggagttaggagggggtattgttagttttttagagattttttatttattttagtagggagattttagagtattgttttgttgttttttaggtattaagttggttatggttataattagttttaagtagtgtattttgggagggggtgggtatgtagttaaaaatagtttaggagttgggtagggtagggttttgggatttagtattttttttattattatttttagtattttttttagtataggtgaggtagttttttttgtttttttgtttaattgtttagtagtagttatttggtttttattatgatggtggtgtcgtttgaggtattggcgataacgttgttattgtgtggatattagttaatatttagtataggggtagtgtgtttagtgattagtgggtagtttttatt

SEQ ID NO: 3 - DNA, 34993 bp, Artificial Sequence
  rc C to T (bis1)
aataaaaactacccactaatcactaaacacactacccctatactaaatattaactaatatccacacaataacaacgttatcgccaatacctcaaacgacaccaccatcataataaaaaccaaataactactactaaacaattaaacaaaaaaacaaaaaaaactacctcacctatactaaaaaaaatactaaaaataataataaaaaaaatactaaatcccaaaaccctaccctacccaactcctaaactatttttaactacatacccaccccctcccaaaatacactacttaaaactaattataaccataaccaacttaatacctaaaaaacaacaaaacaatactctaaaatctccctactaaaataaataaaaaatctctaaaaaactaacaataccccctcctaactcccaactacttctattctaaacatacaccaccacatcttaccctatatttaacccttaccactcaaaaaaaccaataaaattaaaaaaaaaaataaaaaaaaaataaaaaaacaaaataactcctcattccacccaccatataccttttcttcctacccaaatataacaaattccaaactatacccccatacgcaacattacgaaacctatcatcacacttaaaaaccactccaaacgtataaacatcctctcctaacaccctactaccaaaaatatcctactcaatacaaatctaaaaactaaaaaaaaatcccccataaataaataaataataacaaaaataaaacccaaataaccatacctaaccactctaaacaaataataacaatataatcatcatctaaaatataaacaccgaaaaaatactactaaacctaaataatatacacccaaacgtcatccacaatatatactaaaacaacaacgataacctactaaccaccacctacaaaaacaaaaccttacgcatcattaaccccaaaaaaaaccaaataataacgataaatacctaacctaaccactccccaaaaccccttaaccaataaccaactatcaacacccttatacccaccattatcaaaacccctaatcccgactttcacctatcgcatccctactccaaaaactaacccccttcccccgtctctacaaccacaaatctctaccctaaataaacccccaacctacaattctctacccgactcctattccctcccctcccttacatctcaaaaactcaaaaaaaaactcctcgctttaaaattaaaaaaaaaaaaaactaaaaactccatcctcccaccaaaacctacataaaacctaaactcctaaacccctctcctctcaaccgacacccaaacgcatcttccaaaatctaaaacctaacactaactcgaaaactaaccctttctccttataaacccgctaaacgaaaaataaaacaaccctcgcgcgttacttatcccaaccgaataccctaaaaaaacgacgaccctaacctcgccaacctcaaatctaacctaaaatacgaatacgtaaaccgcgtacatatctacgtaaaacaaacgcgccgaaaacgatcgaaactaacgccgaaacgctctaacccactaacccgacgaacaaaaacaaacccgacctcacgaaaacgcccgcccgctacgaactatcttcaccgcaaacgaaaaactactcaacaccgacttcaacaaaataaataaacgacaactcgcgctctaaaacccgataaaccaaaccgcgccgaacgcgctaactcgctccttctctaaatctaccgaaaacgccttcccgaactataactaacgcccaaaaaaccaaaacgaaacgaaaaactcccattcgaaaaaaacctcgctacgactccgaaaaaccaacaaacacccctactctaaaaatcgacctttaaacgcgcttaaaaattcgaaatcgactaaaaaccgcgtacctcctactctctccaaacccgaatactctccaaatcaaaaaccaaacgtaaccccgcaaaaaactaaatacttaaaccccatttatctcttccccgcatccgctcctccaccccgaacacccaaatcaacaaactaattactcatccctccatactcctcaaaacaaacaactaaataatatccctccctatctccccctccccccaaaaaaaatttacgacccacgaaaaaataaaacccatacgaaccgtcttcacgcgccaaaaccatatcttcaccacgaacttcacccgcataaaccaacgaaaactaaacctataaaacccgataacgcaactaaaaacttaaaatatatacctcgaaaactaacatcacgaaaaaataaccaaacgccccccacccgcaaaacatacccacctaaacaaaactaaaaactactaccacctctacaacgcctaccattctcacacccacccctctacccaattttactacgtcgcgtaaaaaatcctacgctaacgcccccacctaataataccgaatccctaaaaataatttactataactacatacgacgcgcaacgaatatatatacaaaaaaaaaaaaactatatacgcaaaaaaaaaaaaaaaatatacccaaaaaaaaaacctacaactctaatcactaaaaatttaaaacataaaatttaaaaaaaccaaaaaacgtaaaaaaacttctaaaaatcccgaaataacacgaaaaaataaaacaaaactaatcacgcctcctatactcgaacaaaacaacttcgaaaaaccaataacactacaaaaaataaacacaaacaacgaaatcctattacccttttacgatcccgactccaacatcgtctacctatataacaaaatactcacgaccgaacaaaaaaaacaaaacactaaataaaaatataaaaaaccttatccgaacgcgcccctaaaccgactaattttacaaaacgacaacaacattcgatactttaaaattaccgacgaaccgcctttcgtacactacctaaacacgttcaacaacaaaaaaccgcaacgaaacataaatttcatacccaaaaaaaaactaaatatcaacaaatataaaatcgcccgatcaacaaccttaacccctcctaaacacctacccgcctctatcccccactcatatcgaatcctaaccacgaaacttccccaataatacaatactttaaaaaaacgaaacgaaaaaataaaacaactctatttcaataccaaacccaccgctcactaaccttacattctcaacttcaatttcctcatctataaaataataataaacacaccatcaaaatattttattacaaaaccaataatatatataatatacaatatacataataaacgctaaacaaatattaacctccaacccccttaatcttaaacaaaaaaaattaaaaacgtaaaaatctacgaaaatactaaaccctactcccttataaattctacaaactacacgaaaaaaaatataaacctatcatcataactataccccgcaaaataaaaaaccgaaaaaaaaattaaacaaaactacgaaacgaaaaaaaacgaaacaaaccccgcaccctctcacgcaaatcctcctatccacccacccccgcaatcaaacctcttccaaaacgatctatacccgaatacgccaaacccgaaaccgaccctaaaaacgaacgaataactatccgaccaaaacgccgaacccgtactcatttcgctaaaaaacgactatataccccccaaacaccgcgaactccgaatcacgaaacgcaacatcctaaacgtacgcccgccctccgacccccgccgcaaccaatcgaccaacgacgcccccttatcgataaaatcgaccctactacactctaacccaatctacatctcccccaaccgcccctatacgacacgacctctctatcctccgccccaacaacaacacaccctaaaaacgctactaaaaaaaatcaaaaccctccgcgaacgaatacaaacccaaaaacaacgcatcacgactctaaaaaacatactatacgaactaataaacgacacgaactaaccccgcgcgccaaacaaacgaaacgaaacgaaacgcacaaactcgaccccgccccgacttttaatcccgaactccgaaccccgccttcttaaactaaacccgaaaacgaaactaaaaaaaaaactccgcccctcgcgaaaaaccaaaactcttaaaacttaaaaaaaacccacgtcgctccaacgaaaactaaactacgaacctcgtctaaaactcgactaaaactaacctaaaaaaacctaaaataacctaaaaaactcaacaataatactacacgacgaaataatatccccctttatcctccgcccaaaacaaaaaaaatacttaatattaacgtaatacttaaaattattaaaacctaaacttaacctcaaacgaataacgatttaataaatacccccaaactaaaaaaaataacaacgcttctcctaatcaactcactaaattccatcaccctaaacgataaaccaaataaacgtcaccccaattctacaaacacatacacaacccgtttactacaaaaccgaacccaataactacacccacaacgatctataataaaaaactctcttccttctttccaccgacaaaaacgaaaactacttcctcgcgacaacccccgcgaaaaaatctcgaaaaaactaacataaaaaattaaattcatcacaaatacacacacactacccccaaccctctaccgttacctctctcaaaaaaacaaaacgtactaaataaaatattttactaaacgttcaatctatacctcctacataaataaaaataaaaaaaacgaaacccccaacctctacaaatactacccccaaactcctaaaaaacctaacgatacactcctaaactcaaaatccatcaaacaacctcttaccctaaaactctctccactctaaaattcaaaaaaaccccaacccacaccgtaaacgttccccccaaataaaattaaataacaaaaacctccgatataaaacctcttttatttatacctcaaaatcaatctaatacccctaacatcaaaaaaaaaaataaaaaaaacaatttctctttattcttttcttccatccctctttatatcccttctaaacctcactaactaaaccgaaaaaaccaatcccaaacaaacccgaaacaaaaatatacgataaacccctacccctaacgaaatctatacttctctaaataaataaaataaaacaaaaaaaaaccgaaaattaacaccattaaataaaaaattttaaaatcaatctccgtataaaaacaaataaaatatacaaccacaaaaactaacaacaactaataaaaaaaaataaaaataacgccaaaaccctaaacgaaccctttatatccaatctacttaaatctaatacttaccccaacccaatatactccccactctccgaaacaccataaaaaaatcaaaacttacacaaaccaaaaaactacgttaaacacactccctaatcacaaaaaaaaaaaaaaaaaaatataccttaaaaaataaaactccaacttctaactacccaaaaaaaaactaaaaccaccctaaaacccaaaacgaatataaaaactaaaaaaaccgaataccccgctaaatacacttaacgctaaaataccgaaataaaaaaaaaactaaaccctaaacgtactaatttatatctaaaacaaaacaataacacaacacgcgaaaaactcaactaccccccaaaaataaaaaacaaaaatacaaaaacttcaaaaacaatatcctaaaataaaattaataaacaaaaatacgaaccgaccaaaaaaaacaaaaaataaaaacaacgctcctctaaaaattcatctccccctcaaaaccgcctaactccgccctaaaacaaaacaaatctaaacccaaaaaaacgaattaaaaaatcaaaatacaacaaaacaaaaaaaccaaaccgtaccaattacctccaaaaccctaacctaaaaaaataccccgcgaccataccgaatccctccccgaaccgtacctactatactactacacccgcgaaacgataactccaatctccaaccgccgctctacaaacgcgcaaaccgaaatttatctaactcctaaccctaaacgtaacgcgcgtaacgctaacgaaaatcccgacaaaaaacgctactactcgatcaataaaaacctcaaaatacgctccaactcctcctcctcctaacgcgcgcgccgccgcctctcctcctactcctacgccgacaattccatcgccaaccgcaactactcgtcgtaactccgaaacacgtaaccgccgaaacctaaccctaaactaaaccgaaaactaaacactaacgccgaaaacgcaaactaacgctacgacgtaaacgaaacgctcctaaaaataaaaaaaaaatatcgcgaactcccgaacgcacccacccaccgaccgaaaccgaaacacgacgtaaaaactccaaaacgacccgcgaccaccaccctctaataaaaacgatcaatcccgcgacgtcctaacccccacctaatcgtaacgaaacccaaaccctaccaaattctccccgtcaatacctaaaaaaaatctaaactccgcgataaaacctaaatccctaacccctacctaccgcctcgaaaacaaaaataataacaaaaaccatcccgataccaaaaaaatccctaccgaaaaccccgcgaattctccgactatatcctaacttaaaaaaaacaaaatcctctccgaaaaattctctccgacccaacgaacactaacctatcctatcgacgaccctcgtaaaacataaaataaatacctaacttactattaattaacgcctcccaaataataacctacgaaaaaacgtaaacgttaaccgtaacgacgcgaaatcccgtaaccccgcgcgcccgcgaaaacgcacctaatcatactcactacccgcctcaaacaaactctactaaataacgaattacaacaaatcgtcgtcgtcgtcccgaatcgccgcctcccgctaaccgcccatcatactataaccgcgcgaaacctcgaacaacgctaaaaaaatctcgcaaccgcgacaaaaaactaaaaacgcgaaaactaaatcaaacacgaccgaacgcgcccctcccacccaccccgaaaaaaaccgaaaaacaaacgttctcgcgaaaaacctcactcgtaaaactaaaactactaacgctaaaaaaatcgctacctaaaaaaaacgtctcgctactaaaactacctcgcaccgataacaccgattcgtcgcaaccgttaaaattcccgaaaataatacgaacgttaaaaatataaaaaatcgaaatttctaaaaataaaaaaacctttaaacgccaccactcaacccctcacacctcaacctcaaccccaccccgacctcatctaaaccccgatcgacccgccacgaactcaaaaaaaataaccgtacgatctcaccaatcttaactaaaaaaccaaaaaacaaacgcaaaataataaaatcccgaaacttaacaaaaaacgcattactaacgaccataaaatcaataataaaaaccacctactcacacaaaaacaaaaaatactcctcacacaaccacaacttaaccttaaacctacccccaccaaatcccaaaaaataaaaaacactacaaaaaaccataacctcccaacatctcctaaaaccccgaccccccaccttcccaacaccgacaaaaacctcacttctatatcttaataatcaattccataaaacgacccatatcacgattacccaactcaaaattaaaattaaaatattcttctacaataataacaataaaattaacttaactcaaaatctaaataatcaaaatctataccacataaaaaaaaacccaaaaactcccctcaattcctaataccaaaccaactcatttattatcacaaaacccccaaactatcccctctaccaatataacgctaacataaccttaaacattataaaaaaaaaatccacataaaccatactaaacaaaacgcttcccaaacctcctcctaaaccacatccacatccctccacttacgaatacccctacacacactcaccccattttaaaaacccccgtactactcaacgattcccaaaaaaaactacaaaaatatcttacaacctacaaaaaatataacatctcaaaaaacaccgcaactccacacacacctaaacacctcatcaaaaataacaacacccaaaacctaaaaaaaaaaccgattcctaaaataaaacctactcacccaaccacatactcaaacaccttcacctaaaaaaaactaaatacttcaaaaaccaaaaaccaaaacctctataaacacaacttaaaacactaaaaaaaaaacctaaaaatcaaaaacaacttccaaaaatactcctctccaactcgataaccctaaacaataaaacgcctaccccgacaaacactataaaatatacatatacgtatatatatttacttcaaacacttccataaacataatttcatattattcccctataaaataaaaattatactttttcacctcgaacacgatatctaatacccaaaaaatcaaatataacatcaataaacatacaaaatctataacaaaatcccctaactttctacctaaaatatatcccactaaactaaaataaccaataaataacatacataacatttctctcctctcccaaattcaacaacaacattaataatcacttacaacataactctccactaaacccaaataaatccttaaaaacttcttaatactctaaacaaccactacccatccttaaaacttaacacctaaattaaaatctatcgacctaaataaaacatccaacctcttactaaaataccaataaaaatactaataaaaacactaaaataaaaactaattcccgcaatcctacaacacctctccccatccaactctacctcattacctttaaccttacccttatactattctaaaaaatattctatccgtatacgaataataaactccacgttaaataccccatacacctaaaaacaaataaaaaaaaaactcataaacaattctaatcttaccctatatcttacccctaaaaacactaaaaacactccctataacaaaaaatcctaaaaaaactctacttcaaacttttaaataaataaatatataaaatcattcattcattcattcattcacttattcattcaacaaacattttttaaaaaacctttatataccaaacattaaaataaacatcaaaaatacaataaacaaaccaaacataatccctaccctcctaaaacttacaatctctataaaaaaacaataaaataaaattataacaacataatccatacactaataaaaataacacaaaaaccttcccaaactacaaaaacaaaaaaaactttcaaaaaaaataccacacacaaaacccataacatttattaattcctactttcatatcgtaaacaacataaaaatcccaaaataacaaacaaaacctttttttttttttttttttaaataaaatctcgctctattacccaaactaaaatactataacgaaatcgctacacactacaaactccgcctcccaaattcaaacaattctcctacctcaacctcccgaataactaaaattacaaacgcctactaccacacccgactaattttttatattattaataaaaacgaaatttcaccatattaaccaaactaatctcgaactaacctcaaataatccgctcacctcgacctcccaaaacgctaaaattacaaacataaaccaccatacccaaccaaacaatcatttttaaaaataaaaacctaactctaaaatcaaaccaaccaaaatctaaaccccaactctaccacttaacaactatataaccttatacaaatcacaaaaccactctaaacctctatttcctcatcataaaataaaccgatcatccctacttcctaaaattattataaaaaataaataaaataccaaaaaaaaaactcaataaacatacgtaaaataaaaatactaacaaaacaacacctaccaaaaaaaattactataaaaaataaatatatatatatatatacgtatacacgtaccctatatatacatccatacatccatataaaacaccaaaaaaataccttaaacccaaatataaatacttaaccacgctacattacttctatacctccaaaactaaaaaaaaaaaatcaaaatcccctatacaacttactataaacaaaaatacaactaaactaacaactaaaaactacaacctcaccttaacttcatacccattcaccatctccgtcttttcactacgccaacccaaaataccaatcttattcctaaaaaaacaaaataatccaaataaaacaaacaccccaccgaactaactcaaaaataaccaaaaccatatccacccacctctcaaaaaaaatattcttaatatcaaactaaataataacgacgaacgcgataaaccgactcaacacctattcctcaataaactaaacaacaaccaacaacaactcccgatcctacccaaccaataccaaaatctctatatacaccacccgacgatcgtaatcaatctccataaccacgacgcttatatctaccaaacacgaaacaacacaaaaaaatcaaaaataacctaaaactacctcccatcgtccccaccctaccccacttcctacctacctaaccttaacccctaaaaacaaaactacgattccctcgctaccaaatcatataatcaaaacccaaaaatataatatctaccctcaaattctaaccgctcttccacactttataaatatcactaaaacaaatcttaaacaccaaaaacactaataaaaacgaaaattaaaaataactttaactaatctaacctacacgacctaaaccaactcaaaacataaaatttaaaatccgtataaccaaaaacaaaaaaaaaaactaaaaaaaaaacaacctctcctccaaaaccccctccctaaccaatataaaccatactcacacaaaaaaacaacctaaaatcgaaacgaacatatttctatcaccactaaatccctaatatccatcatttattaattcactcactcactctttcatccattctttcaacaaatatttataaaacacctactaaatattccaaccactaaaaatacaacaataaaaaaaacaaaactcctaccctctcaaaacttaccttctaacaaaaaacgacaaatcataaatacaataaacaaatcataacaaaataaaaaaaataataataaaatcaaaacaatatctaaaacaatctaaaaaaacctaactaaaacgataaccctaaactaaactaaaacataaaaaaaaccgccgaaaaaactataaaaacacattccaaacaaaaaaacaaacgcaaaacctaaaataaaaaaacccaaaaacgacctactacaacccgcttaccccaactaataaactcccatttcatctccacgtaaaaatcctaaacctaaaaaacgaaaaaaaaaaaaactaaatctacactaaaaaaaaactcaaaaactcccgtaaaaactaaaaaactaaacctcaccttacgcaacttctccaaaaacacgaaaatacccgccaaccgcttcaccacccgctaataatcccgataccgaaacaccaactacaccaactccaaatcccgaatactcacaacctcctaaaacactaaaaaaaaacgaaacaaaatcacaaaacaaaacccttcaaccaaccataaatctataatactaaaaaaaccccgactataaaactaaaataaacaaaactacccacctatccaaccgctacgattctccctacccacgtctacgccgtacgccaaaaacacacgaacacactcaaaataccccaacgtaataaccaaatacaaaaaaatccgaccgcgaaaatccaactactcgatatccacctaaaaaaaaaaaaaaaataaaaaataaaaccccaatcacgtcgaaaacaaccctccgaaaccaaacaaccctaaaacaaacaacaacccccaccccctactaaaactactctacctcaccaacctcacaaaacaacgaaaaaacaaacactataaacaacgaaaaaacaaacactataaacaacgaaaaaacaaacacgtaaataaaaaaaaacttaaaaaacaaaacaaaaaataactctaaaaaaaaaaaaacttcctcccttcctatccaccaaaaacccctaactaaatcctctcctccaaaacccaataacctacctaccaaaaataaacctaaaactaaaataaaataacaaaaaaactattaaccaaaaaactcacctaaaaccaaacctaccctaaaaatcccaaaccaccttcaaaaaaaactaccaatttaaatcactaacattatcactaaataaaatttaacaaacgattacaataatacacaaacaaaaataaaataacaaattcataatattaatacaatttcacaaccatatcctatacttataaaacactatacattaaaatttatacaaatcctataattttataaataacataattacattacataaaatttctattatataataaaaataataaaaactttttttaaaatttttttttatattttttttaaaaaaacgaaatctcactctattaactaaactaaaatacaataacgtaatatcaactcgctataacctccgtctcccaaattcaaacgattctcctacctcaacctcccaaataactaaaattacaaacattcgccaacacgtctaactaattttttatatttttaataaaaataaattttcaccatattaaccaaactaatcttaaactcctaacctcaaataatccacctaactcgaactcccaaaatactaaaattacaaatataaaccgcaatacccaaacaaaaaattttttttttttttttttttttttttttttttacttaaaacaaaatctcactatatcacccaaactaatctcaaactcctaaacttaaacaatcctcctatttcaacctcccaaacaactaaaattacaaacccctacacctaacttaaaaaacatatttattaaacgtaaattttatttatttatttatttatttattttttaaaacaaaatctcactatatcacccaaactaaaatacaataataccatcttaactcattacaacttccgcctcccaaattcaaacgattcttatacctcaaccttctaaataactaaaattacaaacgaacaccactataccaaactaatttttatattttaataaaaacgaaattttaatatattacccaaactaatctctaactcctaacctcaaataattcgcctaccttaacctcccaaaatattaaaattacaaacgtaaaccaccacgcccgatcttaaacataaatatttaaatatatttcgaaaatctaaaacttctaattaaaaacaataaactaacaaaccaaacgcgataactcacgcctataatcccaacactttaaaaaaccgaaacgaataaatcacctaaaattaaaaattcgaaaccaacctaacaacataaaaaaaccccatctctactaaaaatacaaaattaaccaaacgtaataacccatacctataatcccaactaatcaaaaaactaaaacaaaaaaaccgcttaaacccgaaaaacgaaaattacaataaaccgaaatcataccactacactccaacctaaacgacaaaaacaaaactccgtctcaaaaaaaaaaaaaacaataaactaaccacatacatataactccctcctcttctctaaacttaattaaaacgccaataaaaaaacttctactcctaccataataaataaaattactctaccaccataaacaataaaaaaattattactacaaaatatataaaaactaaacacaaaaactcacccctataatcccaacaatttaaaaaacaaaaattaacgaattacttaaacccaaaaattaaaaatcaacctaaacaatataacaaaaccccatctctacaaaaaatacaaaaaaattaaccgaatataataacctatacctataatcccaactactcaaaaactaaaataaaaaaatcgcttaaacctaaaaaattaaaactacaataaaatatcatcacacctctacactccaaactaaacaacaaaataaaacgctatctcaaatatatatatacatatacgtatatatatatatatatatatatatatatatatatatatatatatatatttatatatatatatatatatatttctctatataaaaaatatatataaaaaaaaataactatttttaaaaatccaaaactataatccctaaaataaaaaaaataaacaaaataaactctataacatccctaaatttctacctaaaaaaacattccaaactataattcaaaaaaaaaaaacccgaacaaaacataatactcttcctaaattaaaaaaataaaaacaaaattcaaaaaaaccaaaatattaaaaattacaacaaaacacaattctaaaaaaaaataaactactcaaaaaactccaaaaatctacataaaaatctcttcaaatcttcctaaatactaaacttcacatatatataataaaactcaataaaaccacacaaaaaaaaacaataaaataataaattctcaaaactcaccaaaaacaaaaaaataatcaaactccaacctcctaaaataaaaatacatatttaatcaaacctcaaaaaaattataccttaacaataaaactaaactatccctaaaaaaaaaactcacctaaacccaccctaacaaattaaaaattaacctcaaaccgaatacaataactcatacctataatcccaacactttaaaaaacgaaaacgaacaaatcacctaaaatcaaaaattcaaaaccaacctaaccaaaataacgaaaccacatctctactaaaaatacaaaaaattaaccgaacttaataataaatacctataatcccaactactcaaaaaactaaaacacaaaaatcacttaaacccaaaaaacgaaaattacaataaaccaaaactacaccactacactctaacctaaataacaaaacaaaactccatctcaaaaaaaaaaaaaaaaaaaaaaaaaaaaaaaaaaaaaaaattaacatcaaaaaccaaacacgataactcacacctctaatcccaacactttaaaaaactaaaacaaacaaatcacttaaacctaaaaattcaaaaccaacctaaacaacataccaaaaccccatatctacaaaaaatacaaaaaattaaccaaatataataacatatacctataacctcaactactcaataactaaaacaaaaaaatcccttaaacccaaaaaattaaaactacaataaactaaaattaccccactacactcaaacctaaataacaaaacaaaactctatctcaaaaaaaaaaacctcaaaaaaatcaaactaatttacaaataatttacctaatctacctaaacaaaacccaacactctttaaaaaacaataacaaatccaaatacttaacatcatatttacaatatccaaaattcaattaaaaattactaaatataccaaaaaataaaaaaataaaacttataaacaaaatacgataactcacgtaaacctataatcccaacattttaaaaaactaaaacgaataaatcacgaaatcaaaaaatcgaacttacaataaaccgaaataacgcccctacactccaacctaaacaacaaaaaaaaaaactccatctcaaaaaaaaaaaaaaaaaaaaaaaaatataacctataatcaaaaaaaaaataatttcataaaaacaaaactcaaaaataataaaaataataaataactcaatatactcaaaaatttaaaaaaaaacataaaaaaaatattcataaaaaaaaaaataaaaaatataaaaaaaaacccaataaaccatctaaaaataataaatacaataactaaaataaaaaattcactaaataaaaataacaacaaattaaacactacacaatttaaaaatcaataaatttaaaaacaacaataaaactttccaaactaaaacacaaaaaaaaaaaacaatactaaaaaataaaattaactaaacttctataatcccaacacttttaaaaaccaaaacgaaaaattaacttaaattcaaaaatttaaaaccaacccaaacaatacaacaaaactctatctctacaaacaaaacaaaacaaaacaaaacaacttttacattaactaaacataataacaaacaactataatcccaactcctctaaaactaaaacaaaaaaatcccttaaacccaaaaattcgaaactacaataaactataatcacgccactacactccaacctaaacaacaaaacaaaaccctatctctataaaacctcataatctataaaacattatcaaacattataacatatatctattaaaatcccaaaaaacaaaataaaaaaataaaacaaataaaacaaatttaaaaaaataaaccgaatacgataactcacgcctataatcccaatactttaaaaaaccaaaacgaataaatcacaacatcaaaaatttaaaaccaacctaaccaatataataaaaccccatttttactaaaaatacaaaaattaaccaaacgtaataataaacacctataatcccaactacttaaaaactaaaacaaaaaaatcgcttaaacccgaaaaaaaaaaattacaataaaccgaaatcgtatcactacactccaacttaaacgacaaaaaaaaactccatttcaaaataaataaataaataataaaaaaaaaaaaaaacgtccaaaatttttccaaacttaataaaaactactataataaattaaaaaataatacccctcctaaaacatatccacatcacattctaaccctcacaacctataaataaaaccttatttcaaaaaaaaatctttacaaacataattaaattaaaaatctcaaaataaaataatcctaaatcacccaaaaaaccctaaatccaataacaaatatctttctaaaacactcaaaaaaataaaaaaaccatataaaaacgaaaacaaaaactaaaattctacaaccacaaaccaaaaaaattataacccaatcaccaaaatctaaaaaaaacaaaacaaaactcttccctaaaacctttaaaaaaactaccaccctaccaacatctcaaatttatatttatatctcccgaactataacaaaataaattttttttttttttttttaaaataaaatctcactctatcgcccaaactaaaatacaataacgtaatctcaactcactataaactccgcttccccgattcacgccattctcctacctcaacctcccaaataactaaaattacaaacacccaccaccacgcccgactaattttttatatttttaataaaaacgaaatttcaccgtattaaccaacataatctcgatctcctaacctcgtaatccgcccgcctcgacctcccaaaatactaaaattacaaacgtaaaccaccacacccgaccaaatatttattattttaacccacctaatttataataatttattataaaaactaataccaaaataaaaccaaaaaccaaaaaattcaataaaccccaaataaaacaaacacgaaataaactacaccaaaatccatcataatcaaatactaaaaactaataataaaaaaaaaatcctaaaaacattcaaaaaaataaaatccattatatataaaaaaacaaatacaaaaaatactatattcttctcatcaaaaactatataaaccaaaaaacaatataataaaatctttaaaatactaaaaaaaaaaaacaaaaacaaaaactttcaacctaaaattctttttttttttttctctaatccaatataactaatattaacctaaaattccatacccgataaaaatattcttcaaaactaaaaaaaaaataaatatattaacaaacaaacaaattctaaaaaaatttattaccaaatatacaaaaaatattaaaaaaaattcttcaaataaaaaaaaaataatcccaaataaaaacttaaatctatacaaaaaattaaaaaataccaaaaaatattaaatatataaaaatatcaaaaaaccaaacacaataactcatacctataatcccaacactttaaaaaaccgaaacgaacaaatcaccaaaaatcaaaaatttaaaaccaacctaaccaacataataaaaccccatctctactaaaaatacaaaaattaactaaacgtaataaaaaattcctataatcccaactactaaaaaaactaaaacacaaaaatcgcttaaacctaaaaaataaaaattacaataaacaaaaatcgcaccactacactccaacctaaataacaaaaaaaaactctatctcaaaaaaaaaaaaaaaaaatatcaaactaaacgcaataactcatacctataaactttaaaaaaccgaaataaacaaatcacttaaacccaaaaatttaaaaccaacgtaaacaatataataaaactctatactacaaaaaaatactaaaattaaccaaacgtaataatacatacctatcgtcccaactactaaaaaactaaaataaaaaaatcccttaaaccaaaaaaccaaaaattacaataaacaaaaatcatcccactacactccaacctaaacaacaaaaccaaaccctatctcaaaaaaaaaaaaaaaaaaaaatcaataaaatatttaaaacccacaaaaataaaaaaaaaaaatatcaacaaataaaaaacttcaacacaactttaaaacataaaaaataactaaaacctcacaactaacttaaaaaaacaaaaaaaactaaaactaaaacaaccacaaaaaaaaacgtccacataaaaaacaaaccaaataacccccaacccccctaaaaaatataaataaaacctacaaacaataaaaataacaaaaataaaaataaaactaaaactaaatacaaaaaaactaattacaattcaaaatcccctaatccccttcccaacctcattaaactaaaaaataccccccttcctcaccacaaaacaccaaaaatttattctttataaaaattaaacataaaatactctaaactcaaaaacattaaccacaacaaaaaataaaatataatactaaaaaccaataatccgtaaaaccccaaccccttccctacctaaatcctaaaccactaacaaccaaatcacaccaccaccaccctatctacccgaataaaaaattatcccaaaaacctcaaaatacaaacatctaataaccctacaataaacaaaccaacctaccacctaatcaccttacaataacacccacacatccctaaactccccaaccccattcttaaatataacccaacaaccaaaaaaaactaaacacttaataaaaacttcccatataaaataaaccaaaacatacaaattaaatactaaaacgactaaatacaataactcacgcctataatcccaactctttaaaaaaccgaaataaacgaatcacgaaatcaaaaaatcgaaaccatcctaactaacacgataaaaccccgtctctactaaaaatacaaaaaattaactaaacgtaataacgaacgcctataatcacaactactcgaaaaactaaaacaaaaaaataatataaacccgaaaaacgaaacttacaataaaccgaaattacgccactacactctaacgcgaaaaacaaaacgaaactccgtatcaaaaaaaaaaaaaaaaaaaaaaaaaaaaacaaattaaatactaaaaacccaaaaaaaattctcttaatacaaaaaataaaaaaaaactctttaaaaaaaaacaataatttacatcctcaaaaaaaatataaaaaaatcattaaattcataaaacaaaataaaacaacctaactttccataacgtctcctaccctttctcttaccttcttcattctaaaaataactttcttaacttttccttattttctacattcctaaacaactacacctacccccataaacaataaacatcacctaaatttactacattttcaaataaaaaaaaaaaccaactttaaaactatctacatctcttctttttcccgcaccctccacatctaacccatcaaaaaaacttataaactctacctccaaaacaaacctaaaaaccgcccaatttccactaccttacaactattacccccccatctctcactaacaaccccctactacctctttactactccccgattaccaaactctattatccacctcacctataacaactaaaatcaccctataaaatattactcaaatcctaacactctttaattcaaaatcttccaataactttccatcgtaaataacaaaaaatccaataaccccaaacttctctttaaactcatttactccacccttcgccaataaccttccccgaaacgttctccaaaatcctccaaaaaaccccaaaactttctccctcccttcactcaaactactactcaaatatcacctccttaaaaaaacccaccctaacaacccatctaaaataacaactactataactctatccactacccgtccaaatacctattaaacacctcctacacctcgaacaaaaaccccatcaaccaaatccctacctactttattcactactaattccccactccccaaacaacacctaacacataaatatttactaaacaaatacataaaatactaaactaaaaaaacacaaaaaaaaaaaaataattaaccaaaaaatcattacaaaaatatattatttataccgaaaaactcacgtctataatcccaacactttaaaaaaccaaaataaataaatcacttaaactcaaaaattcgaaaccaacctaaacaacataacaaaaccccatctctacaaaaaaaaatacaaaaattaaccaaacataataacaccacctataatcctaactccttaaaaaactaaaataaaaaaatcacctaaacctaaaaaacaaaaactacactaaactataatcacactactacactccaacctaaataacaaaataaaacgctatctcataaaaaaaaaaaaaaaaaaaaaaaaaaaaaaaaaaaaaaaaaaaaaacaaaaaaaaaaaaaaaaaaaaaaaaaaaaaaaaaaaaaaaacaatataaacaatatattatttataattaaaaaaataaataacaaaaaaaatccaaaatactaaaaaaataaaaaaaacgaaacaaaaaacactacttttcattacgcatcttctaacaacaattaaatattttaaaacataaccataaactccattatcaaaaataaaacattttaaataatttaaaattatttatataatttttataaccttatcctaaaatttcttcatttttcaatatactaaaaacctcaaaaaaaccaacgaacctaacccctattaacctctaaactataacccctcacaaaaaaaaaaaatattatttactcttatccaatcctaattaaactaaactccgaaacttacaacctaaataaaatcctaaacccgacaacgaaaataaaaaaaaaccacaaaacccgaactaactaaaaaaatactaaacaatccaaacctcccaaccctaccccaaatactacaaccgcaaccgctacaactaataaaaccctaaaaaactaacaaaccgctacctaacctcaaaactccaaatactacctccacctccccatcaaatacctcaactccaaactccaaaaaacgactaacacttccttacaaacaaaatactcctccccatccccacacctcaaaaacactccccaaaaaaacctaaataactcaacaccccatacaccccatacaaaaccccatacactcaaccaaactccaaaacaactctccccacaaacccaaaataccgcctacaatataaataacaccttaccctaaacccaaataaaaaaattcattaatctcctcaacaaaaacctccaacttctcctcaacaaaaacctctaactatttaattactaaaataaaaaaatttcccataaaacccaacacccaaccctccccaccaaaaaaacgaaaattccttatcccaacaaacctcaactaaaatcaaaaaataaaatctttaaaattttataactaaaaatccctaaacaaaaaacctccctacctccactcaaacacacacaccacactctaatacacactaataccatacaaatacacactcgtacgctcataaatactcacgtatacccttaaatatacaaacacatacatacccaactaccttctaaccctacaaaaatccactcctatataacgtatatatacgtatttacacaaaaacacccctcacacccatatacactaacaaaatactttccaaactcctttaacataaacaaaatccttttattaaaaaaaatataaaaaacatacatctcatatataaactaaacacaatacttacgaaaaaaataaaaaacgcaaaacctatactcaaaataatacctactcaaccccttccccaacccacgaaaaaaaaaacaaaaatctaatataatcgttacttaacctctcctacccaacgtaaaatacaaaaacaaatctacctaaactcattcaaaaaaaaaaaaacaaaatacatcctcaaactacgtaaaaaaccacgaactataaaaaccgcaccctaaacttctccctccatatcacccctcccatcctacccttacaacccctccccctcatcccaaaacacattaatttttaatttctaaaatttataactccctctcccgaacttcctaacttaccaactataataataccccacatccaaaactacccaatataaacaaaaaaaaaaatctaaaatactcctcgcacatcctaaaccccacaacccatctcccctacctctaaatcaaaaaaataaacaaaaaaaacaaaaaacaaacccacgataaaaaacgccccaaaaaaaaaaaaaataattctctaaaaccacaatctacccacttcaaaattctaattaccaaaaacaaaatcctactccccaaacccaacccacacatatccctcccacgaaaactacacaaactaacccttccccctattcccaccccaaaaaacaccaaaaactcacgactccaaaaccaaaaccatacccaactaaccataccaaacaaaaaaaaactaacatattccctaacttacaaccctatcccccccgacctaacaaaaaacatacataacgacaaacaaaacaccgaactaacatcacaacactactaaataccccttcccttcaccaaacacctcctatctacccatcactccctacttccaacctccaacaaaacaatttaaaactaaacaaaacccattaacctactctaaaaataaccatactaaccccctcctcaaccaactacactaccaaacctacccacgaaaaacctctacgaaactttcttaaaataaaaaaaaaacaactataccaaaccaaaaccaaaaaaacctaactcctaaatacttaaaaaaaaccgaactatttctataacgactaataccaaaaaaactaaaaaccaaaaacccctaactaaaataccaaaattccacaatacttttctcataatattaaataactatccccaaatcccccttacaaaaaacaaaacctaataccctaaaaaataaacaatatacatctaaatacaaacctcactctaaaccaatcctcgaaaaaaaaaacaactaaaaaactctcccacctacacgaaataacattcctctttttaacacgcctaaaaaaaaaaaaaaactaacctaactcctctataattaaacaaaaattaacctccaccaataccctatattccccctaacctaaatccaaaacaaacaatatccatttcaaaaaaacattaactcactaaaacaaaaataaaaataaatctaaaaccttatttctaaaacaaccaaaaaaataaaaaaaaaaaacacataaacaacccccaacacctctacctacaacgactccgataccccccaccccaaccttaccccaacaaaataaccacccacttcaaaattatcaacaaaaaaacctactaaaaaaatcttttctcccaaaacattctacctctctccaatctctacaataaaaaaaccacccaccctcaaacaaaaaaataaaactaaaacattctaaaaattcaaccttctacctaataatccttaaacccctaaaaaattcttcccacataaaacttatcttcttttactttcaaaaaaaaaaaacaaaaaaaaaccaacaaaaactaactaaccatatcttaacgctttacacatcaccctaaaatttcctattcacacttacttcaccaaaacaaaaactccttaaaaacaaaaattaataccctatttattcatctatttcctaaaaacactataacccactctctttaacaaacttctcgtaactacaaaacactacctttataataaataaacaaaaacaaaatctaaaaaattcaatctaaaaaaaaactcgaaaaatactaacataaacacaaataacaaaaaataaccacccaaaccgacccaaaaacctacgaacacaaatcactcgcatatttacaaaaactaccatacaaaactaaataccatacaaacctaaaaactaactcaacgtaaaacttcaaaaacacatcctaacccccaacctactcaatccgataacctaccctccacctccatacttcccttaacgattacacaactcctcaaactaaacttctcataactcaataaacaaccctcaaaaaataaattcccacaacgaacaactacgctaaccacccccaacccataaccccaaaatctcaaacccaatccaaaactaaaattctcaacctacaacaaaccataaaacccgaacccaactctaactcttacaacccaccctaaaaacgaaaaatcatctctaccataaatacctacctataacctaaataccaaaaacaaaaataacaatctataacctatacctacctttattctaaaacataaccaaaaaacatcctaaaacataaccaaaaaacatccccccttcccctattttctaaaaaccactacccaacccaaaactaataacccacgtaaccttactaaccaacaaaaaccaaaaaacccacctaatacgcaaaacctcaaatccttccaacaaccaaaacccctcaacttcctctacgcctaaaaaccaaaccccaacaccaaaaaacaaaaaaacgcttttcaacacctaaacaaaacccttaaaacctcccaaaaaaatctttctccactccctattcctaaactaaaactaaactctaaaaaatccaaaaatctacccaatttaaaaactaaaaaaaaaaacgctcaccgttaaaaaaaaaacgctaaataaaactaaaatacctaaaaatataacacaacctcttccccattcttaacctataaccccctccccacgcaaacctttcccacctccgcaccctcactcgaaaaatatcgccgctcaactaactaaaacgaactctcccaccacataaaacaccgacacaacccgcaacccctccctacaaccctcactaccccgacgaaaaaaaaacacaaaaacctctactctcatctaaataaatccgaaacacgtataatcccgcccgtcccgaccgaaaaaaatcaccctttcccgatcaacaaacacaaaaaccgcgaccgcaaacaaaaacgcgccgcaaactcgccaaaaaaacgaaacaacccgcgccgcaccccctccccaaaccgaacgaacgtacccgaccgcgaaatccccgcgacgccccgaaaacgctcctacctaacccgcgcgaacctccttctccaactcgcgataacgattataccacacgaaataatacaacgaatacttaccctcgaaccccttcctaacgaaaacgttaacgaaaatcatcgcccgctcctcataccgaaaccgcgacgcccgaccgaaaaaaaaaaacgacgccgaaaccgaaacccgaaaccgcgaaacgaaaaaccgacgctacctactcgcgaaactacgactcgaacatatacgaacgacgacgaacgaaaacgacgcgcccgacgcgatacgaacgacgcgaacgacgaacgtcctcgcgaaacgacgacgacgaacgacgcgaaaaaacccccacccgccctaaaaaaaaacgaacactcgacgacgctacgcgaactcgcgctcgcctcccacacccccgcacacaaaaacgccgctcgacgaaaaaaacaaacgcccgcaacgaacgcgaaaacgcacgaaacgcgaaccccgaaaacgccgccgcaaaaacgcgcgcccgcaacccccgaatccccacaactacataacccgaccctcaacccgaacgaccgacgcgaaatacgaaaatataaaaataataaaaaaaaaaaaaaaaaaccaaacgccccgaataaaacttatcaactcaaccccgcgacatcataaaatttataatccgcctcgtaaaactaaaaataacaaataaccgaaaaaaatctacactatccccgaatctcgtaaaaaaataaacgaaaaatcaaacctaacccaaacgcgaacgaaaccctaacgccaaataaactaaaacgcacctcccccgctaacattttaccttttactaaaaaaataaaaaaacacgaacctaaatcgaacgtttaaaaaacgaaataaaaatataatcttcaaaattaaacttaaatcccaaaaaccataaaaaaaaatccgaattcccaaaaaaaaacgtctaattaaaaactcctaaaaaaaatataaaacatcaataccaaaaatcattaaaacaaccaaaaatctaacccctaaaacatttctaaaaaatcttccctaccctattaaaaaattaaactccatcttccacacatatcattaaaaacaaaatatccaataacgcgaaaaaaataatccctttccccccgcacactatccccaacaaaaaccaaaataaaattaaacaaaaaaaacaacaaataacaactccgttcctccacccaactaacccttcaaaaaaaaaaataactaattccaaaaactatctccttcctaaataaccccaaaataaaaaaatacttccaaaataatccctacaaaaaatataataaaaattaaattaacctctcaaacgccaattacaaaacctaaaaaaaccaaaaaacttaaaccaatccctaaaaaaaaaaaactataatatcaaaaaaaccaaaattcgaataactccaactacctaaccttaaaaaaacaaactacttaatttttccgactttctcgatccactccccttcaaaataaaaatctaaatactacctcctaaaataaactaaaaataataactaccctaaaaacaacgcctccctcccccaaccaaacgaaccgaaacaaataacgaaaccaaacacgataccttcttaaacccacctcaaaacaaaacaaaaataaaaaattccacaccgaccctacttaaaacaacaatccaaaaaatatttatataaaaaataccaacaaaaacttacaaactctctcaaatttctttatataatcttccctccttcctcctccacaccctataataccaaaccccaacgaaaaaaaataaaaaaaaaacgaactacctcgcccctttctcccgcctaaaaaaaaccaactaacgtctccgaaaacccgaaaccgctacccgcctacaccaccaaaaatcaacaaaatatcgtaactacaaccaatacaaaaaaaaaaactaacgcgattaaaaaacatctaaaaataaccgaaaacatacctatacatttccttattaaattatttttcgaaccttatatataattccactataacaatcctacttcctaaaataataacatctccacgaaaaaatccaaaaacccttttatctccaatcccaaacccaaaaatttaactataacgaaactaaaaaaaacaaaatttaaacgatatatccgcgccaaaaccactcccaaataatctctaaaccaaccaaaaaataaaaaataaaataaaaaaataaacaaaataaatcatccttcttccccaacaaaacccaaaaatccgaaaacaaaaaaaattcaaaataaattataaaaaattatcgattataaaaaactatcccctaaacgaccgtattctttttttaccaaacgacgataaacactaaacccaaatcgcttacgcttcgacccgcgctctcaactaccacgtactcgaaacgcgcccacacaacgaaaaaacaaaaacaaccaaacgacaaaactaccaacaacctcctcgacatttaataaataaaattccataactaaaaatcgatcgaaaataaacgaacgaccaccgctcgtaaactaaacgcctaacacgaactacctaaccactcctcccgtctcactccccccgccccttacccccttcccgctaaaaccaccaaacccataaactctaataaaaaaacaactcgaaacgacaaataatactcccccctacacaccaactaaatatcgttacttacaaaaaccccaccaactaaacgactaactatcgaaaaaaaaaaaacctacaaaatttttttaaaatacaattataaataaaacccataaatcgcgatttcaaacaaacttatcaatctaaaccgcaacaaaaaacgataaaaacaactttacatatatttcgaataatataactcataaacattacttatctcccctaaaaaaaaaacctacccacccacaaatcactaccgctctaacaccgttaaaataatcgaccaacttaaacacccctaccaaaaaactacccccatcttaacaaacaaaaatctctaactcttaaaaaacccctcctcaattatcaccactaacctaacccccaaatctaaccctaaaaacctctaccctctccccacaaacaaaatacccgaaccttttactactacaaaaattaaaaattaaatacacgcgcgacacacgcgtataaaaacgcatactcaatacgaaaactacgctcatatacgacctctacctaaactccctaccccccaacccacccacgtccctcacctaccttacctttacctacctcgtcgtataaaatccaaaaaaaaaaaccgtcacctaaaacgacccctctatattatatacaccctttctaaacacacacacctctaataacccaaaaacaccgtaaatatatataaaacgaataacaaataaatataaatacacacaaacacaataatcactcctcgaaaaatctttaaaaaccgcccaaattctctcctctctaaataaaaaaatacataaaaaaataaatatatttttaatccgaaaacaaaaaaatacactacctaacctttctaacacctaaacgtccatattattaacaataaacgtattcaacaaaaatataacacatacacacacacccctaaacacacaaatataaacacctacgaaacaaaaacgcacacctcaccccaaccaaaaataaacgaataccccaaaacacaacccctttaacctaaaacgaaacttaaacctccaaatccttcttccctaatccccaccctcgccgtccgtaaacccaacgtcccccgatccaccccacgcgaaaaataaaaaaaaaaaaactataaaaataactcacattacctccgaaccaaacgaacgctacaacgaaaaccaaaaccgcaaaccacgctacccgccgaaaccgaacatctaccgcgacccctttaaacgcccccgccccctcctacccgcgcccgaacttcctttctctaaaaaacgcgaccgacaacgcgcgacgaaacgaaaatacgacccctccccctataaacaaaacctacgccgcttcctacaaaaacgaccgaaaaccgcgcaaaaaacgaaaaaaaaaaccgcgaacgacgacgaaacgacgcgaaacgaaaaacgcccgaaaacgaacgaacaaacgaacacgacgaattccgaaccaaccccgaaacgaacgattaaccgaacgcgcgaaacctcgccgaaacctcgccgaaaccgaaccgaacaacaaaaaccgccgccgccgcccgaacccgccgcccgcgccccccacgctaacccaaaaaactacgaccgcgtcgccgctaaaaatatcccgaaaaaaaccgcgaacgaaaatatatacgaactacaacgccccgaataaacgcgacgaaaccgaaaacgaaaccgcacaaccaaaccgccgccgaacgaacgccgaaacctaacaaaaacgctatacgaaaccgaaaaactaaacgaaacgaaaaactacgacctccaaactaaacccccgcctcgaccactacgaaactacgcccttaacgaaaaaaccgacctaaaatacccatactccctaaaaaccgtaaactaacgaaaaaaaacgttcccgacgccgcctcccgctcctcgatctaaaaaaaacgaacaactaactactcctccacctccatctctatatccgacgaaaacgccaacctaaaataacaaaaaaaccgtaacgaaaaccgtcaaaacttaaaaaataaaaacgaatataattttatatcatctcaataccacccccgcgtcttacacctactactcgcgtaatcgatacgcctaccgaaataataaaaaacaaaaaacaaaaaaccgaacaaatacgccaataaaacctaaataccgtctcctcaaaaacaaataaacgataactactcccaaaactccctacctcgaattcctaaaactaacgctccttaccgaacctaacgttcaaaaccaatctaaacccgaatatcttctcgaaaaacatccccaaacctactaataataactaaaaacaactcgactaaaccctactattcctattcaccgataaaacctacttaaaaaaataaacttaacatcaaactatcctaaatacgaacccctccctatcccctaacccaatctaaccaaaaataaataaaaaaccgtaccgaaattccccgtatcctactaacttcctaacctatctcctaactatatttacataataattcccttccttttcctaacaaaattaaaactaaactaaaataaaaccccccaaacctactaaaaaaatcaaaaataataatccaaaaaactactcccttctaataaaaaaaaacaaccaataacgaaactctacaactaacctaaaaaaaaaactctaacccacatccattctttctttaacaaaaaaactatctccctaataaacccctaaacaaactacgaaaatccgtaaactctaacgaaactataaacataattaaaaataaaaatataaaatactaatttataaacccataactttcaaccaccccttaaacaaacccaaaaccccaccgattaaacctcacaaatactctaataattctaaaaataccaaactaaaatatttaaaaactataacttaacaaaacttaaacacaaaatactccataaataattataaccaaaacctcctaaaaacttatcataatttaaaaaaccctaaaattaaaaatccatacccctaaaaaactataactccgttccccgaactacaaacaaatctaaaaataacaaaactaaaaatacaccttaccttataaatatctccccactattccacaactccgtaaaataaacataacataaaatataaaaaaaaatcttaacaaacgcccaatcgaaaaaatctaaaacttaatattacctttattcccaacttactctataatcccaacaaaactttcctcactataaaatcctcaacttcctcaattcaaaaacaaaaaaattaaaataaaaataatttttaaaaaactaccatctccgaatctataatctaattctaaaataaaaaaataaaaaacaacaccaacaaaacaattatcctttatatattacgttaaatatccgaccacaacctctaaatacccaataaactcaaaaaaaaataataaacatcaaatatattaaattacccaactcctcctcccaaatcctcatctatcaaaaaaatttataccccaaatacctcctttcccctaattcacaataaaaatcaaaaaaataataaaaaaataaaaataataaaataaaaaaaatataaacaatcttactcatcaacccacctaacacccaacgaaatatccaacacataacaaacactccctaaatatttaactacttattaaaaccctaactaactacttaaaactatcccacacctaaaccctaaaatactaaccctaacatacaacgacatatttaatctaaatcctataacatctcaaacaaaaaaacataaaaatacccaacaatccgaaatccaaatccaataccaaccccataatatatcgctccaccccaaaatcacaaacttcttttattataataaaaaccctacaatcctaaccacaaaaataaaaccaaaaactttttatacttaattaatttaaaaaatcataaaaatcaaaaataaaatacaacctatccccaaaaaaccccatcctccctctactcccgaacataaacacacaaaacaaatataaatatattactaaacaactaaacataacataactactctaacaacttataccacctcgtcaaacaccgtatatattcctacctacctaaaaaatccaaaaaaaaaaaaaaacaaaaaaccctaaaaaatatacatcttcccctttccttaaacttaacccacctcgccacacgatctcaatcaaaaacctctcctcaccccataaacttctatctcaaccttttccactttaacaaccctaaaaataaaaataaaaacctcaaaatacctatcctataaatatctctaataaacaaaaccgaaaacatattacgaaacaaactacaaactaatttatctcttcataatataaattacaaaataaaacaaatattaaactcctcttcctcccttataaaaataaaatttatatatatcaatacctacacctaaatattcatcctaataaacttttacatatatatatacccatataactactactctaatcatattataaaataaaaatatccaatctttttacttccctaaaccacattaaaaaaaaaattttcttaaaccacacctaaaatacgctaacactaataataactaataaactaaataaaacaaacaaaaataaaaataaaaaataaaatcacaaaaaaatctcataatattttaaaaaaatttataaatttatattaaaccacattcaaaactacctaaaccgcatataaactacaaattaaacaaacatattataaaacatttccatcaccttaaaaaacttccaaataccccctcccaatccgtacaccccaaaaataaccaccattctaactctaccccaaaaactactctcgcctaccttcataatataaacttttcccttaatctaataaaaatctaacccttaactcaaaaaaaaaaaacctaaaactaacctatatatacaaacctactaaccctaaaaaccactaataacttcaaataataacaaaaattcaccgtaataaaaacctccataaaattaacactaattaacgtaatcccaaaatcacgcctactacctctccacacatacaaacccataccctaccgataaaaccaaaaacgcaaaaaaaaaactaacgaattcccttacaattcctatcctttccgtcccaaatttaatccaaaaaacttcttaacgcaaaaatcccttcaccttaaactacaatctaaataatcccaaaaacacttacacaaaaaaaaaaaacaaaataattaaaataaacgtcccatctatatcatccaaaaataaactaacaccaataacgactacccaaaccaaaacaatatcctttacctaccattcttctcaaatcacctaaaaaaaaaaaaaaacccctcccccaaactaaaaaaaaataccaaacaaacccttaaaccacactcctacatcctaatcttaattactaccataaccaaaatcactcaccacatctaatctacccataacttaaaactctaaaaccattaaccgtaaatatataatcaaccttccatacctaacttctccgataaaaccacaaacctcaaatcaacccatttataatcctaccctaaacgactccccacttacaaaaaaccccaccaaaaaaaatttaaactacatcatttccgacttcctacctaaactactaaaaataactaactaacaaccccctaacccaataatatttaaaataaaaaaaaaaaaatctccacacctaaaatacctcactatttaaataaaaccaacccaaaaatacatactaaaactccccctcttaacgaaaaaaactaatcccttcctcctaaaccctaaaatcaaccccccaaaaaaatattaacgatcaccttaaacatccctctattaccctaattaaaaaaaaatcccttaaaaaacctaaacccgctacactccaacctaaacgacaaaacgaaactccgtctcaaaaaaaaaaaaaaaaaaaaaacctaaacccaaaaacaaacctctctcctttacttcctattttcatacctcaataaaaatcacttactataaacaaaactcaaactaaacccctaactcaaaatctcctcaattttcctaaaaactttaataaaaatccttaaaaaaaaaaaacctaaaaattaccttctaattaaaaaaaattcttatcc

SEQ ID NO: 4 - DNA, 34993 bp, Artificial Sequence
  G to A (bis2 rc)
aaataaaaatctctcccaactaaaaaacaattctcaaacctttcccctctaaaaacttccaccaaaattcccaaaaaaattaaaaaaactctaaatcaaaaacccaacctaaactctacccacaacaaataacccccactaaaacataaaaacaaaaaataaaaaaaaaaaacctatctttaaatttaaactttttttttttttttttttttaaaacgaaatcccgctctatcgcccaaactaaaatacaacgaatttaaactttttaaaaaaccccctcccaatcaaaacaacaaaaaaatacccaaaataaccgccaacaccttcctaaaaaactaactccaaaactcaaaaaaaaaaaaccaaccttcttcgccaaaaaaaaaaaccctaacatacacttctaaactaactttacccaaataataaaacaccccaaatataaaaacctccctctccccactccaaacaccactaaatcaaaaaactaccaaccaaccacctccaacaacccaaacaaaaaaccgaaaataatacaacccaaattcctcttaataaaatttcctataaataaaaaaccgcccaaaacaaaatcataaataaactaatctaaaatctataatcctaccgaaaaaaccaaacataaaaaactaactatatatccacgaccaataactccaaaaccctaaaccataaacaaaccaaatataataaataaccctaactataacaataaccaaaaccaaaatacaaaaatataatccaaaaatttacctaacactttcccccaacctaaaaaaaaaattctccttctcctccaaataacctaaaaaaaataataaacaaaaaacactatcctaatctaaacaaccgctattaatatcaactcatttctaaataacacaaataaaacgcccaccctaaccattctatctcctccctctatacaaatacccttaaaactacccaaattataatttaaaataaaaaaatccttacgtcaaaaaactccttaaaccaaacctaaaacgaaaaaaacaaaaactataaaaaaactcgtcaaccctccccctacgcttctaactccaccgacaaaatataaatctatatatataaaaaaataacaaacgtaatcctaaaatcacgttaaccaataccaaccccataaaaacctctactacgataaattcctaccaccacctaaaaccatcaataacctccaaaaccaataaatttacacatacaaactaacctcaaacctccctcccctaaactaaaaaccaaatctccactaaactaaaaaaaaaacccacatcataaaaacaaacgaaaataatccttaaaataaaatcaaaataataattacctctaaaatacacgaactaaaaaaaaatacttaaaaaccccctaaaataataaaaatattctataacatacttatctaacctacaatccatatacgacccaaacaactttaaatataacccaacacaaattcataaactttcttaaaacattataaaacttttttataactttattttttatttttatttttacttattttatttaactcaccaactatcattaatattaacgtattttaaatataacccaaaaaaattcttcttccaatataacccaaaaaaacaaaaaaattaaatacccttattctataacataatcaaaacaataattacataaatatacacacatataaaaacccatcaaaataaacactcaaatacaaacattaacacacacaaattctacctccataaaaaaaaaaaaaaaacccaacatttatcccactctacaatctacactataaaaaaacaaatcaacctataacttatcccgtaacatatccccgaccttactcaccaaaaatacctacaaaacaaacatcttaaaaccttcactctcacccccaaaattaccaaaataaaaaaaactaaaataaaaacccataaaataaaaaaaaacccttaactaaaatcgtataacgaaataaaccaaacctaaaaaaaaaaaaaaatacacattctccaaaactccctacccccttcctctcttaaactccccaaacaaacaaaaacacatacgatacctaacgaaataacacaaactaccaaaacaaccatatcatatccaactacctaacaacacactcacacttatcctatatacccatacccgaaaacaaaaaaaaaataaaactctctaaaaacaaactacatctcacctctaacctccataaccccccaaattaaccaaacacaaaaaatccctaaccccactcctataattaaaactacaaaactcctatcataataaaaaaaacctataaccctaaaataaaacgatacaccataaaactaacactaaatctaaactccgaactactaaataccctcatacctctctacctaaaataccacaaaacccaaaccaaacataccgctacataccaaaaccaacatcctaaaatccaaatataaaataatcccaaacaaccaaccaaaatcctaacaaacaaccaaacactcaaaaaatacctaccatatactaaacacctcgctaaatactaaataaactaataaataaaactatccacatcctccccaccccaccatcctcaccttctcaccaccttcctaacctctattataaatcaaaaaaaaaaaaacatctaaaacacaaattcctctaacaaataaaaacctaaaaaaaaaaactaaacaatccaacacatctaatacccaccattcctccctaaacccactaaacatccaaaaactataatcgaacattcaacgcaacatacaaaaaacaactaccttactaatactacccttcacccctccaccccaaaatcaaaccacaaattcgaaaataacaaccccccaaaaaccatttctactccaacttctttacctctaaattaaaaaaactaaaaaccccacaataaaaaaaatcttattaaaattacaaaataaactaaaaacaaaaacaacactaaaccccaaactcccccgattaaacgcctactaaaactctcctccacattccataccatacttaccccacgaaattataaaacaataaaaaaacatttataaaacaaaatacatcctcaaccctaccatccccaaacctacctacaactcgaaaaacgaaatcacaatttcttaaaaatataaaccctcaaccccaaaaccctctaaaccataataaacccctaaaaaaccttaatcataaccacctataaaatattttatacccaaaccctactaaatcataattcccaaatactctaacttaacacccccaaaaccaccaaaacatctataaaactcaaccgataaaatcctaaacctactcaaaaaataactaaaaattataaacccacaaaccaacaccccatactctcactcttaatcatacccacaaccccgctaaaattcacgaacctccgcaacctacccaaaaacctaccaaaaaaataactcctttactaaaaaaaaaataaatataaactaaaacttccttcccaaaccaactacaaaaccccgtcactaactatcctccctcatcaaaaaaaaacaacctcttaaatcattacccctaacttcctcaacaaacctaaaaaatttcactccaacccaatcctaactctattaaaaaaaaaaaaaaaaccaccatataaatacaaccaaaaaacaaaccaaaaaaccaacaaaatacgaaaaatctcgacacgacctcccacccatttctaaccaaactaaactaaaaaacaaaaaaaaacccgcacccaaaataacttaataccaaactcactttcccaaacaaaccttaccgataaacaaaaacaacaaaatccaaccgaactattcccaatcaccaccaacaaacctaaaaatacctcccgaaaaaacacccgaatctaaactaaccctaaacgccaaacccgacaaaaaacgctaaccttaaaaacccgaaacaaaaaatcctaaaaataaccaccgctcatctactcctaaaaaaacgatattcaaaccccactaacgcatctacccgaccctctactccttaccctccaccaccccgacaaacgtaccgaccacgcgaacaacaaatacaaaacgcgaaaataacactaaaataacataaaaccacactcgcccccacctcccaaaccctaacgacctccgccacgaccctcctaccaccccaaactaacgcttccgtcgaatacaaaaataaaaataaaaaaacaaccaactacccgcctccctcaaaccgaaaaacgaaaaacgacgccgaaaacgtccttcctcgctaatccacgacctccaaaaaacataaacaccccaaaccgaccctcccgccaaaaacgcaactccgcaataaccgaaacgaaaacccaacctaaaaaccgcaaccccccgccccgcccaaccctccgaccccgcacaacgctcttaccaaaccccgacgcccgcccgacgacgacctaactatacgatcccgcccccgaccccgccgcgcttacccgaaacgctacaatccgcacacacctccgctcgcgacccctttcgaaacatcctcaacgacgacgcgaccgcaaccctctaaaccaacgtaaaaaacgcgaacgacgaacccgaacgacgacgacgacccctactacccgacccgactccgacgaaaccccgacgaaactccgcgcgcccgaccaaccgtccgccccgaaactaacccgaaacccgccgtacccgcctacccgctcgccctcgaacgccctccgccccgcgccgccccgccgccgctcgcgactcctctctccgccccctacgcgactcccgaccgcttctacaaaaaacgacgcaaaccctacccacaaaaaaaaaaaccgcacccccgccccgccgcgcgctaccgaccgcgccccctaaaaaaaaaaaacccgaacgcgaacaaaaaaaaacgaaaacgcttaaaaaaaccgcgacaaatacccgaccccgacgaacaacgtaacctacgaccctaacctccgctacaacgctcgcctaacccgaaaacaatataaatcaccctcacaaccccctccccttcactttccgcgtaaaataaaccgaaaaacgctaaacccacgaacgacgaaaataaaaattaaaaaaaaaaaacttaaaaacccaaatcccgctccaaatcaaaaaaactataccttaaaatacccgtctatctctaattaaaataaaatatacgtccctatcccgtaaatatccacatctatatatccaaaaatatatatatatatatcacactcttactaaatacgcccactactaacaatataaacgcccaaataccaaaaaaatcaaacaatatattcccctacctccgaactaaaaatatatctatctctccatacatccttccatccaaaaaaaaaaaaatctaaacgatttttaaaaacctcccgaaaaataaccactatacctatatacactcacatccacttatcatccgccttacacacacccacgatatttctaaaccaccaaaaatatatatatccaaaaaaaatacatataacataaaaaaaccgtttcaaataacgacctttcttcctaaacttcacacgacgaaacaaacaaaaacaaaacaaataaaaaacgtaaataaactaaaaaacaaaaaacctaaataaaaaccgcacataaacgcaacccccgcactaaacatacgcccccatacgcgtataccgcgcgtatacccaacccccaatccctacaacaacaaaaaacccgaacactctacttataaaaaaaaaataaaaatccccaaaaccaaacctaaaaaccaaatcaataataacaattaaaaaaaaattctccaaaaatcaaaaactcctacttattaaaataaaaacaatcctttaacaaaaatactcaaattaatcgattatcccaacgataccaaaacgacaataatttataaataaacaaactccttccctaaaaaaaacaaataatactcataaatcacaccacccgaaatacatacaaaactacctccatcgccttttactacgacccaaattaacaaatttatttaaaatcgcgatccataaactttatttataattacaccttaaaaaaatcttacaaacctcccctccctcgacaaccaaccgctcaactaataaaacttttacaaacaacgatacctaactaatatataaaaaaaaacaccacctaccgccccgaactactctctcaccaaaatccataaacttaataacctcaacgaaaaaaaaataaaaaacgaaaaaaataaaacgaaaaaaataaccaaacaacccgtaccaaacgctcaatccacgaacgataaccgcccgttcacccccgatcgacccccaactataaaatttcatttattaaatatcgaaaaaactactaacaaccctaccgcttaactatctttatttctccgctatataaacgcgtctcgaacacgtaacaactaaaaacgcgaaccgaaacgcaaacgacctaaattcaatatctaccgccgcctaacaaaaaaaaaacacgaccgcccaaaaaacaattccccacaatcgacaactccccacaatccatcctaaactccccctatcctcgaactcctaaactttactaaaaaaaaaaaataattcactctacttacccctccaccccactccccatctcctaattaactcaaaaactacctaaaaataaccctaacgcgaacacatcgtccaaactttatttcccccaaccccgtcacaaccaaacttctaaacctaaaactaaaaataaaaaaatttctaaattcccccgtaaaaatatcaccaccccaaaaaacaaaactactacaataaaatcacacacaaaattcgaaaaacaatttaataaaaaaatacacaaacatactcccgaccactcctaaatacccctcaaccgcgccaaccccctcccctacactaactacaaccacgacactctactaacccctaataatacaaacgaacaacgatcccgaacccccgaaaacgccaactaactcctcccaaacgaaaaaaaaaaacgaaacaacccgctcctccctcatctcttcccgctaaaacctaacaccacaaaatataaaaaaaaaaaaaaaaaaaaccacacaaaaaaacctaaaaaaatttacaaacttttactaacacctcccacacaaacacttcttaaattattattttaaataaaaccgatataaaatcccttattcctaccttattctaaaataaactcaaaaaaacaccgtacctaatcccgccacctatctcgacccgcctaattaaaaaaaaaaaacgctatttccaaaacaatcattatccttaactcaccccaaaaaataatatctaaattctcattttaaaaaaaaataaaccgaaaaaatcgaaaaaattaaacaatttactcttttaaaatcaaacaattaaaactattcgaactctaatctctctaacatcacaatcccctccctccaaaaactaatccaaacctcttaatccttccaaaccttacaattaacgcttaaaaaaccaattcaacttttaccacaccctctacaaaaaccattctaaaaatacctcttcaccctaaaatcattcaaaaaaaaaacaatctctaaaatcaatcacttcccttcctaaaaaaccaactaaataaaaaaacgaaactaccacctactactttttctatccaacctcactctaattcttactaaaaacaatatacgaaaaaaaaaaaaccatctttcccgcgttactaaacattctatttccaataacatatataaaaaataaaatttaattttctaacaaaacaaaaaaaactcctcaaaaatattccaaaaaccaaacccctaactactccaataacccttaatactaataccccacacctttctcaaaaattcccaatcaaacgctctcttctaaaaatccgaatccttcttcataacccctaaaacccaaactcaattctaaaaaccacacctccaccccgtctcccaaacgctcgacctaaacccgtacccccccacttccccaacaaaaaacaaaataccaacgaaaaaaatacgtcccaacccacctaacgtcaaaaccccgcccgcgtctaaaccaaacctaactccccgcccactctcccacgaaatccgaaaacaatacaaaccctcttcgaccacctaccacccccaatttcacgaaacgaactacaaaccccataataccgcgaaactaaactaacaaactctacccgaaacgcctaatccccttcctctctccccatcatccccacatccccgtatcccgcgccgaccgctcgaactaaaaaccgaactatacaactataaaaacccgaaaactacgaacgcgcgtccctacgacgacgtccccgaaacccgcgtcccgtacgcccccgcgcccgctacgaacgcctactccctccgccgaacgacgtctttatatacgaaaatataaaaaacgaacgcgaatccgcgcaacgccgccgaatacccgctccctcccaaaacgaataaaaacctctccgcgccgcccgccgccgccgcctcgcgaaaacgcccgtcgcccgcgccgcccgcaccgcgccgaacgcgccgcccccgcccgccgccgctcgcacatacccgaaccgcaaccccgcgaacaaacaacgccgaccccccgccccgcgaccccgaaccccgactccgacgccgtccctcctccccgaccgaacgccgcgaccccgacataaaaaacgaacgataatccccgccaacgcctccgccaaaaaaaaacccgaaaacaaatatccgctacactacctcgtataacacaaccgccaccgcgaactaaaaaaaaaaatccgcgcgaaccaaataaaaacgccttcgaaacgccgcgaaaaccccgcgaccgaacacgcccgtccgacctaaaaaaaaaatacgacgcgaactatcccgcctccctaacgaatttacgacgcgtctttatttacgaccgcgacttttatacttattaaccgaaaaaaaataatcccctccgaccgaaacgaacgaaaccacacgtatttcgaactcacctaaataaaaataaaaacctctatacccctcctccgccgaaacaataaaaactacaaaaaaaaactacgaactatatcgatattccatataataaaaaaatccgccccaaccaattaaacgacgacacctcccgaataaaaatacgaaaataaaaaaaacttacgtaaaaaaaaaaccataaatcaaaaataaaaaaaaaactatatcacactcccaaacaccccaaccccacccaacgccctctccccaacgataaacgctttctcttttaactctcaaactaaacaaatccttaaatctctcaaaacccaaccccaactcaaaaacaaaaaataaaaaaaaaccctcttaaaaaaccccaaaaaccttatccaaatactaaaaaacgctctcctaccctctaatactaaaacctaatttctaaacgcaaaaaaaactaaaaaaccctaactactaaaaaaacttaaaattctacgcaccaaataaactccctaatttctactaatcaataaaaccacgtaaatcaccaactttaaactaaacaataatctccaaaaaacaaaaaaaaaaaaaatatcttctaaccatacttcaaaatatcttctaaccatacttcaaaacaaaaacaaacacaaatcacaaattaccacttctacccttaacacccaaaccacaaataaacactcataacaaaaataaccccccgcctccaaaataaactacaaaaaccaaaactaaacccgaatcccataacttactacaaactaaaaaccccaattttaaactaaatctaaaaccttaaaaccataaactaaaaataattaacgcaattacccgctataaaaatttaccttctaaaaactacttattaaatcataaaaaattcaatctaaaaaactatacaatcgccaaaaaaaacataaaaataaaaaacaaaccatcgaactaaacaaactaaaaatcaaaatatatctctaaaatcccacgctaaaccaacccccaaacctacataacatccaactctacataacaatccctataaatatacgaataacctatacccgcaaacctctaaaccgatctaaataaccacttcctattacctatacctataccaacactctccgaatttctcctcaaactaaactcctcaaaccctatctttatttatctatcataaaaacaatactctacaaccacgaaaaacctattaaaaaaaataaatcacaatacccccaaaaaacaaataaacaaacaaaacatcaacccctaccctcaaaaaatctctattctaataaaacaaatataaacaaaaaattccaaaataatatacaaaacgctaaaacataaccaaccaacctctactaactcttctctactttccttccctaaaaacaaaaaaaaacaaacctcatataaaaaaaacttcccaaaaatccaaaaatcactaaacaaaaaactaaatctccaaaatacctcaatcccactcccttacctaaaaataaataatccttttactacaaaaactaaaaaaaaacaaaataccctaaaaaaaaaaacttctccaacaaacctctctactaataatcctaaaataaataaccatcttactaaaataaaattaaaataaaaaacaccgaaaccgctacaaataaaaatattaaaaactactcatatatttctctctcccacccctctaactacctcaaaaacaaaatcccaaattcacccctacccctaccccaataaattaatatctccttaaaataaacactacctatcctaaatccaaaccaaaaaaaatataaaacactaataaaaattaacccttattcaaccacaaaaaaaccaaaccaatcctctccttccctcaaacgtaccaaaaaaaaaaataccactccgtataaataaaaaaattccctaactatctcccctctcgaaaactaacccaaaataaaacttatatccaaatatacactacctactccccaaaacaccaaactctattttctacaaaaaaaacctaaaaacaaccacctaacatcataaaaaaaacactataaaaccctaacatcccaaccaaaaatccctaacctctaatccccctaataccaaccgccacaaaaacaactcgactttcctcaaacactcaaaaaccaaatttccctaatcttaacttaacataactacctcttcttcactccaaaaaaaccccgcaaaaaccctccgtaaacaaacttaacaatacaactaactaaaaaaaaaaccaacataaccaccttcaaaacaaattaataaactttactcaaccccaaattactctactaaaaactaaaaacaaaaaataataaacaaataaaaaatacctaataaaaaaaaaaaacacccaacaatactataataccaacccgataccctacttaccgctatacatattctctaccaaatcgaaaaaaacaaaattataaaccaaaaaatataccaattcccccttacctaacataaccaactaaacataatcctaattctaaaatcgtaaattcctaatattccctaaaataaaaacaaaaaaaaaaattaacctatacaactcccgtaaaaaaaacatatataaactaaacctaaaaaacaaaactctacccctaacaaccaaaaccctaaaataaacaaattataatcccaaaaaatcattttccttctccctaaaacgttctccaccgtaaacttacttcctactttccctattcacccttctaacctaaaaacaaaaaaaataaattataaaacccaaaatatacgaaaaacacctcaaacccctccctttacctacactaaacaatcctaaatataaaacatcaccacaactaataaactaaaaaactcgaaaaaaaaaaccacaaaccccaaaaaccaaaaatcaatatattctaaaataaaaaaaaaaaactacaaaaacaaaataaaaaaaataacataaaaaaaaaaatccaaaatacgatccccacaacccgtaacctcctacgcaacttaaaaatacatcctacctccctccccttaaataaactcaaacaaacctacccctacaccccacgctaaacaaaaaaaatcaaacaacgactacaccaaactcctaccttcctcctcgtaaactaaaaaaaaaactaaacaaacaccaccttaaacacaaactctacgtccctcaccttcctcgcaaacactatatttaatccatacataaaatatatacttttcatacttcccttaacaaaaaaattctactcatactaaaaaaatttaaaaaataccctactaatacacataaatataaaaaatattcctatacaaatacgcacacacacgttacacaaaaataaactcctacaaaaccaaaaaacaactaaacatacatatacttatacacttaaaaacacacgtaaatacctataaacgtacgaatatatatctatataataccaatatatactaaaatataatatatatacctaaataaaaataaaaaaactctctacccaaaaacccccaactacaaaactccaaaaactccaccttttaactccaactaaaacctactaaaataaaaaatctccgttctcttaataaaaaaaactaaatattaaatttcataaaaaaccttttcattccaacaattaaataactaaaaacctctactaaaaaaaaactaaaaacctctactaaaaaaattaataaattctcctacctaaacccaaaacaaaataccacttacactacaaacgacactctaaacttataaaaaaaactactctaaaacttaactaaatatataaaattctacataaaatatataaaatactaaaccatccaaacctccctaaaaaatactcctaaaatataaaaataaaaaaaaacaccctacttacaaaaaaataccaaccgctctctaaaacctaaaactaaaacacctaataaaaaaataaaaacaacatctaaaaccctaaaaccaaacaacgacctaccaactccctaaaatcttattaactacaacgactacgactacaacatctaaaacaaaactaaaaaacctaaattactcaacacttccccaatcaactcgaaccctataaccctctcccactcccgctaccgaactcaaaaccccacccaaattacaaaccccgaaatccaacccaaccaaaattaaacaaaaataaacaacactccccttctctataaaaaaccacaactcaaaaaccaacaaaaaccaaacccgctaatttttttaaaactcccaatatattaaaaaataaaaaaattccaaaacaaaactataaaaattatataaataatcttaaattatttaaaatatttcatttttaacaataaaattcataatcatactttaaaatatttaactattactaaaaaatacgtaataaaaaacaatactccttactccgcctctcccacctccccaacactctaaactccttttatcatttacctccctaattataaacaatatattatttatactaccctctcccctccccttctccctccctccctcccttccctacctccctccctttctctttctttcttcttcttttttttcttttttcataaaacaacgtctcactctatcacccaaactaaaatacaataatataatcacaactcaatacaacctctacctcccaaactcaaataatcctcccatctcaacctcccaaaaaactaaaactacaaataataccaccatacctaactaatttttatatttttttttataaaaataaaatcttaccatattactcaaactaatctcgaactcctaaactcaaataatccacctactttaacctcccaaaatactaaaattacaaacgtaaaccccccgacataaacaatatacttctacaataatttcttaattaattaccttcccctccttataccccctcaacctaatactctatacatttatctaacaaatatttatataccaaatactacctaaaaaataaaaaaccaacaataaacaaaacaaacaaaaacctaactaataaaacttctattcgaaatacaaaaaatactcaacaaacacttaaacgaacaataaataaaaccataacaactattacctcaaataaactatcaaaataaacttttctaaaaaaataacatttaaacaacaacctaaataaaaaaaaaaaaaaaactttaaaactctctaaaaaatcctaaaaaacgttccgaaaaaaaccattaacgaaaaataaaacaaataaattcaaaaaaaaatctaaaaccattaaattccctactacctacgataaaaaaccactaaaaaattttaaactaaaaaatatcaaaacctaaataacacttcacaaaataactttaactaccataaataaaataaacaataaaacctaacaaccgaaaaacaacaaaaaaacaataaaaaactaccaataaaaaataaaaaaacaacaactacaaaataataaaaactaaacgacttctaaatctattttaaaaacaaaacctacaaatttttctaataaattaaatataaaaaatacgaaaaaaaaaaaaaatataaacaattttaaaattaatttttttttccacctaaaaatacaataaatccaaataatatttactatttataaaaacaaatacaactatccaaaaatacaaaaaacaaaaaaaaattaaaaaaatcacttccaaaataaaaaaaacaaaaaaaaaaacaaaaaacgtcataaaaaaccaaactatcccattttatttcataaattcaataatctttttatatttttcctaaaaatataaattactattttcccccaaaaaattttcttttattccctacatcaaaaaaatttcctctaaattcttaacatctaatttatttttttttttttttttttttttttttttaatacgaaatctcgctctatcccccgcgctaaaatacaataacgcaatctcgactcactacaaactccgcctcccgaattcacaccattctcctacctcaacctcccgaataactataactacaaacgcccgccaccacgcccaactaattttttatatttttaataaaaacgaaatttcaccgtattaaccaaaataatctcgatctcctaacctcgtaatccgcccacctcgacctcccaaaaaactaaaattacaaacgtaaaccactacacccaaccgtcttaacatctaatttatatattttaatttatttcacataaaaaactttcatcaaatatccaatttctcctaactattaaatcatatttaaaaataaaactaaaaaactcaaaaatatataaatactactataaaataatcaaataacaaactaacctattcattataaaatcaccaaatatctatattctaaaatctttaaaacaacttcctactcgaataaataaaataataataatataacctaactaccaataattcaaaacccaaataaaaaaaaaactaaaatttcacgaatcactaactttcaacaccatacctcatcctctactataaccaatactcctaaatccaaaacatctcatacccaatttctacaaaaaataaacccctaatatcctataataaaaaaaaaaaacatctcccaacttaataaaactaaaaaaaaaaccaaaaaatcctaaattataaccaacctccctacactcaactctaacttcacctccacctctaccatccccattacctacaaatcctacctacacctttcaaaaaaactaaaaatcacctaacttactccttatataaacgtttccctctataactactttaatttcaacttcctctactcccctaaatcaattataaaaccccaaccactttccatattctaaaattatattaaaatttctcatctactaacatctcttctctttattcttataaattttaaatattttactaacttttttttttttttttttttaaaacaaaatctaactttattacctaaactaaaatacaataaaataatctctactcactacaacctctaactccctaactcaaaaaatcctcccacctcaacctcccaataactaaaacgataaacatacaccaccacgcctaactaattttaatatttttttataacacaaaatttcaccacattacccacgctaatttcaaactcctaaactcaaataatctacccacctcgacctcccaaaacttacaaacataaaccactacgcccaacctaacattctttttttttttttttaaaacaaaatctctctctatcacccaaactaaaatacaataatacgatctctattcactacaacctccacctcccaaattcaaacgattcttatacctcaacctccctaataactaaaattacaaaaatcccccaccacgcccaactaatttttatatttttaataaaaataaaatttcaccatattaaccaaactaatctcaaactcctaacctctaataacctacccgcctcgacctcccaaaatactaaaattacaaacataaaccactatacctaacctcctaacattcttatacatttaacattttttaacactcttcaatcctttatacaaattcaaatttctatctaaaatcattttctttccacctaaaaaactccctttaacatttcctacacatctaacaataaattcccttaaaatttatttatctaccaacatatttatttcttcttcaattttaaaaaatattttcaccgaatataaaattctaaatcaataccaatcatactaaattaaaaaaaaaaaaaaaaaaaattctaaattaaaaatttttatttttatttttttcccccaacactttaaaaatttcattatattatttcctaacttacataatttctaataaaaaaaatataatatttcctatatctattcttccatacataataaacctcatttctttaaatacttttaaaattttctttttaccactaattttcaacatttaattataataaaccttaatataatttacttcgtatttatcttacttaaaattcattaaatttcttaattcttaactttatcttaatattaatttccacaacaaattactacaaactaaataaattaaaacaacaaatatttaaccgaatataataactcacgcctataatcccaacattttaaaaaaccgaaacgaacgaatcacgaaatcaaaaaatcgaaaccatactaactaacacgataaaaccccgtctctactaaaaatacaaaaaattaaccgaacgtaataataaatacctataatcccaactacttaaaaaactaaaacaaaaaaataacgtaaaccgaaaaaacgaaacttacaataaactaaaatcacgccactacactccaacctaaacgacaaaataaaattccatctcaaaaaaaaaaaaaaaaaatttattctatcacaattcgaaaaacataaatacaaatttaaaatattaacaaaataacaatccttccaaaaactctaaaaaaaaatcctaccttatctctttcaaattctaataactaaaccacaaccctcttaacttataactacaaaactctaatctctacctccgtcttcacataaccttcccacctctctaaatatcttaaaaaaacacctatcattaaatttaaaaccccctaaataatccaaaattatttcatcttaaaatccttaacttaattatatctacaaaaacccttttttaaaataaaatctcattcataaactataaaaatcaaaatataatataaacatatcttaaaaaaaacaccattcttcaacccaccataataatttttatcaaatttaaaaaaattttaaacgttctttctttcttttattatttatttacttattttaaaataaaatctccctctatcgcccaaactaaaatacaataacacgatctcgactcattacaacctccccttcccgaattcaaacgattctcctacctcaacccccaaataactaaaactacaaatacccaccaccacgcctaactaatttttatatttttaataaaaataaaatttcaccatattaaccaaactaatctcaaactcctaatattataatccacccgccttaacctcccaaaatactaaaattacaaacgtaaaccaccgcacccgacctatttctctaaatttatcttatttatcctacttctttattctatcctttaaaattccaataaatatatattacaatacttaataatatcttacaaattataaaactccataaaaacaaaatcttactctattacccaaactaaaatacaataacgtaatcataactcactacaacctcgaactcctaaactcaaaaaatcctcctacctcaacttcaaaaaaactaaaactacaactacttaccaccatacccaactaatataaaaattattttattttattttattttatttataaaaacaaaatcttactatattacctaaactaatcttaaactcctaaactcaaaccaacctcccgccttaacctccaaaaatactaaaactataaaaacccaaccaactttatttttcaatactatttttctcctctatacttcaatttaaaaaattctattactatcttcaaattcactaatttttaaattatacaatatctaatctactattatttccattcaataaatttttcatttcaattactatacttactatctttaaataatccactaaattcttttttatacctctcattcctctcctcataaacatctttttcatatttttctttaaactcttaaatatattaaaccatctatcatctttatcatttctaaattttatttctataaaattatttttctcctaattataaattatattttctttcttttttttttttttttaaaataaaatctctctctctattacccaaactaaaatacaaaaacgccatctcgactcactacaaactcgatctcctaacctcgtaatccacccgcctcaacctcccaaaatactaaaattacaaactcacgtaaaccaccgcaccctacctataaattttattttcctactttttaacatatctaataatttttaactaaattttaaacattataaatataatattaaacatctaaatttattattattctttaaaaaatattaaactttattcaaacaaactaaataaattacttacaaatcaatttaacctttttaaaacttttttttttaaaacaaaatcttactctatcacccaaacttaaatacaataaaacaatctcaactcattacaacctcaacctcctaaacttaaaaaatcctcctacctcaatcactaaataactaaaactacaaacacatactaccatacctaactaattttttatattttttataaacataaaattttaatatattacccaaactaatcttaaactcctaaactcaaataatctacctacctcaacctcccaaaatactaaaattaaaaatataaaccaccgtacctaacctttaatactaatttttctttttctttttcttttcttttcttttttttttttaaaataaaatcttactctatcacccaaaccaaaatataataatacaatcttaactcactacaacctccgcctcctaaattcaaataattcttatacctcaacctcctaaataactaaaattacaaacacccatcaccaaacccgactaattttttatatttttaataaaaatataatttcgccattttaaccaaactaatcttaaactcctaacctcaaataatctacccgcctccgcctcccaaaatactaaaattacaaacataaaccactacacccgacctaaaactaatttttaatctattaaaataaatctaaataaaccttttctctaaaaataatttaactctactactaaaacataacccttctaaaatctaattaaatatacatctccactctaaaaaactaaaacttaattatctccttacttttaataaactctaaaaatttaccattttattactcctttttatataatcttactaaatttcactatacacatataaaatttaatattcaaaaaaacttaaaaaaacccctatacaaatttctaaaattttttaaataatttactcttttccaaaactatactctactacaacctttaataccttaacttccctaaatcctatctccatcttctcaactcaaaaaaaacaccatactctactcgaacttcccctccttaaattacaatctaaaatattcctccaaacaaaaatccaaaaatattacaaaactcaccttattcattttccttacttcaaaaatcacaattctaaacttctaaaaacaactatttctctttacatatattttctatataaaaaaatatatatatatacacacacaaacacacacacacacacacatacacacacacatatatatatacacacacacgcatatatatatatatatttaaaacaacgtctcactctattacccaacctaaaatacaaaaatataataatacctcactacaacctcaacctcccaaacttaaacgatcctcccacctcaacctctaaataactaaaactacaaacacaaaccatcatacccgactaattcttttatattttttataaaaataaaattttaccatattacccaaactaatctctaactcctaaactcaaacaatccgccaacctttacctcccaaattactaaaattacaaaaataaacctctatacccaaccttcatatattttacaacaataattttctcattatttataataacaaaataatttcatttattataataaaaataaaaacctttttactaacgttttaatcaaattcaaaaaaaaaaaaaaaattacatacatataatcaattcactattccttttttttttaaaacgaaattttactcttatcgcccaaactaaaatacaataacataatctcgactcactacaacctccgcctcccgaattcaaacgattctcttacctcaacctcctaattaactaaaattacaaacataaaccaccacgcctaactaattttatatttttaataaaaataaaatttctccatattatcaaactaatctcgaactcccaacctcaaataatctacccgcctcgacctcccaaaatactaaaattacaaacgtaaactaccgcgcctaacctatcaattcactattcttaaccaaaaatcctaaactctcgaaatatatttaaatacttatacttaaaaccgaacgtaataactcacgcctataatcccaacactttaaaaaaccaaaacaaacgaatcacttaaaatcaaaaattaaaaaccaacctaaacaacatatcaaaaccccgtctctactaaaatacaaaaattaacctaacataataatactcgcctataatcccaactactcaaaaaactaaaacacaaaaatcgcttaaacctaaaaaacgaaaattacaataaaccaaaataacaccactacactctaacctaaataacacaataaaactctatctcaaaaaacaaacaaacaaacaaacaaacaaaacttacgtttaacaaacatactttctaaaccaaatacaaaaacttataatcccaactacttaaaaaactaaaacaaaaaaattactcaaacctaaaaatttaaaaccaacctaaataacataataaaaccctatctcaaataaaaaaaaaaaaaaaaaaaaaaaaaaaaaaaatcttttatctaaacactacgactcacacctataatcccaacactttaaaaacccgaaccaaataaatcacctaaaatcaaaaattcaaaactaacctaaccaacataataaaaacccatctctactaaaaatacaaaaaattaaccaaacgtattaacgaatatctataatcccaactacttaaaaaactaaaacaaaaaaatcgcttaaacctaaaaaacgaaaattacaacgaactaatatcacgtcattatactccaacctaaccaacaaaataaaactccgtccccccaaaaaaaacacaaaaaaaaaccccaaaaaaaacttttatcacttttatcacacaacaaaaatctcatacaatataatcatattattcacaaaattataaaatttatacaaattttaatacataatatcccacaaacacaaaacataattataaaattatattaataccataaacttattatttcattcctatctatatattactataaccgtttattaaacctcactcaataataatatcaataatctaaattaataactcttcctaaaaataacctaaaacccttaaaataaatctaatcccaaataaactccttaaccaacaacctctttaccaccccacttcaatcccaaacttattcttaacaaacaaaccactaaaccctaaaaaaaaaaacccaaccaaaaacccttaataaacaaaaaaaaaaaaaaccctccctcttccaaaattactttctatcctatcttctaaacccctttccatccacgtatctatctttccgttactcataatatctatctttccgttacccataatatctatctttccgttaccttataaaattaataaaacaaaacaaccccaacaaaaaataaaaattactacctactccaaaactatctaactccgaaaaactacctccgacgtaactaaaactttatcttccactcctcctcctcctccaaataaacatcgaacaactaaatccccgcgaccgaactcccctacacctaaccaccacgctaaaacaccttaaatatacccgtatactcctaacgcacgacgcaaacgtaaacaaaaaaaatcgcaacgactaaacaaataaacaaccctactcaccccaaccccacaaccgaaacctccccaacatcataaacctataattaactaaaaaatcctaccctataaccttacctcgccctcccccaatactccaaaaaactataaatacccgaaacctaaaactaatacaactaatacttcgataccgaaactaccaacgaataataaaacgactaacgaacatccccgtactcctaaaaaaactacgcaaaataaaacccaacctctcaacctccacgaaaacccttaaacccttctccaatacaaacttaacctctctccccttcgtcctccaaacccaaaacttctacgtaaaaataaaataaaaattcactaactaaaataaacgaactacaacaaatcgcttctaaactctcccactttaaatcctacgcttactcccctacctaaaatatattctcataattcttccgacgattccctctataccttaactcaactcaaaaccaccgcctcaactaaacctttccaaattaccccaaatactatcttaactccattattattctcttcactctatcataatttacttactatattcataacctaccgctccttattaaaaaataaactctaaaaaaacaaaaatcctatctttttcactattatattcccaataactaaaacactcaataaatatttcataaatatttattaaaaaaataaataaaaaaataaataaataaattaacaaataataaacactaaaaacttaataataacaaaaacatacccgtcccgacctcaaattactcttctatataaatataatctacactaaccaaaaaaaaaattttaaaaaaaaaactactctctcttcaattccctcccctattcctaaccacacgaatcccaaaccccataccctaaactaatccaaaccgtataaaccaaaccaatcaaaaccacctccaacctccgcttccaccaatacccctaatatccaaaatctaccctaataacacctacaaaatataaaaaaacgaccaaaacctaaaaataaacaccacactcctaaactttaaccacataacctaacaacgaaaaaaccgcaactttatcttcaaaaaccaaaatcaaacaaacaaaaaataaaacaaaataaaaacgataaaaaacaaccccaaaccacccctaatccccctatactattccgtatctaacaaacacaaacgccgtaatcataaaaattaaccacgaccgccgaataatatacacaaaaactctaacactaactaaacaaaaccgaaaactactactaactactactcaacccactaaaaaacaaatactaaaccgacttaccgcgcccgtcgtcaccactcaacttaacaccaaaaatatctcctttaaaaaataaataaacataaccttaatcacccttaaaccaacccgataaaatacctacctcacctaaaccactctacttccccaaaaacaaaactaacatcctaaactaacgcaataaaaaaacgaaaataataaataaatataaaactaaaataaaactacaactcccaactaccaacccaactacactcttacctacaacaaactatacaaaaaattctaacctcccttccccaaccctaaaaatacaaaaacaatacaacgtaatcaaacacttatatttaaattcaaaacacttctctaatattttatataaatatataaatatatacacaaaacacgtacacacgcacacacacacacacatttattcctcacaacaaccctttctaataaatactattctattaatattcccattttacgcatatttattaaatcctttccttaacatcccatttactcttcacaacaaccccaaaaaataaaaataatcgatccattttataataaaaaaataaaaacttaaaataattctataacctatacaaaatcacacaactattaaataacaaaattaaaattcaaatcctaactaacctaaccctaaaaccaaacctttatccctaaaaataactacctaactaaacataataactcatacctataatcccaacgctttaaaaaaccgaaataaacgaatcacctaaaatcaattcgaaaccaacctaactaacataataaaaccccgtctctactaacaatacaaaaaattaaccgaatataataacaaacgcctataatcccaactactcgaaaaactaaaacaaaaaaattacttaaacctaaaaaacgaaacttacaatatacaacgatcccgccacaacactccaacctaaacaacaaaacgaaactccatctaaaaaaaaaaaaaaaaaaaaactctacctattactctaaaacccctatattacccacgacataaaaacaaaaactaacaaataccataaattttatatataacatctcctctaaaaacctcccctacttctataatctaaaaaaacctctatactacccccaccaatacataaaccatactattataactccattttattatctccttataaaaattataaatctcaaaaaaacaaaaatcatatttaacttatttactatatccctaatacctacctcaatacctaacacataaaaactcctcaaaaaatatttattaaataaataaataaataaataaataaataaataacctcatatattcacttacccaaaaacctaaaacaaaatctctccaaaaccctttactacaaaaaatattcccaatacccttaaaaataaaacacaaaataaaaccaaaactacttataaaccctttcttcatctatccccaaatatataaaacatctaacgtaaaactcatcacccgcacacgaacaaaacatctttcaaaacaacacaaaaacaaaatcaaaaataataaaacaaaactaaataaaaaaaaatattacaaaactacgaaaaccaactcccacttcaatacttccatcaatattcccactaacatcctaacaaaaaactaaatactttattcaaaccgataaatttcaattcaaataccaaaccctaaaaataaataataactacctaaaatactaaaaaatttctaaaaactcatctaaattcaataaaaaaccatactacaaataattactaatattactattaaatttaaaaaaaaaaaaaaataccatatataccatttattaaccattctaatctaataaaacatatcctaaataaaaaatcaaaaaaccttaccacaaattctatatacccattaataccacacctaattctctaaataccaaataccgtatccgaaataaaaaaacataatttctacctcacaaaaaaacaacataaaatcatacctataaaaatacctaaaacaaacacacacacgcacatacacaccccacaatacctaccgaaacaaacgttttactatccaaaatcaccgaactaaaaaaaaacacttttaaaaattacttctaacctctaaaccttccttttaatattttaaactatactcacaaaaaccctaacccctaatccttaaaacactcaatccccttcaaataaaaatacctaaatatataattaaataaacaaaccccaccccaaaaaccgacctcctccctaaatcttaaatactatcacctctaataaaatacccaaatatatataaaattacgatatcctctaaaataccacatttcttataaactataaaacacctttacaatccttcctaaaaatcgctaaacaacacgaaaacccccaaaataaaataaatatatacaaaaatacccgtaaataaaaaaatataaatataactcaaaaaaaaacttaaaaaacgtcctacttaacataacctatataaacctcctttccacaatacccaaaaccatatcaacgccacactaacaaaaaaaacaacttaaaaaccttataacaacaaataaattaacctaacattaaaaactaaaaaaaactcctaaacccctccccatataatacaaaccctaatcactcaaactctaaaccaaaccaaccccactaccatcactacaaaaaaatacttcaaccccaactttaaactaaacaaccgtaatataaaccgccccataaaactaaccaccaaaacacaaaaataaaacccctaccgatactaaaaaaataaaaaaccgaaactccaaaaaatactaaaaaaccataacttcctacaatatcccttaccccttaaaatctaataaaaacaaattcaaaaccaaactataactatataaaaaacatcccctatccctatataaacaaataacccccatcattaacctcataaccgtcaacaatacgctttttaccaaactccgaaacttcatcaccctacgtctacctcctaacttcccaattaaaattaataaaaccgcacgaccatttctcctaaacccgtaacgaaccgaccgaaatttaaataaaatcgaaataaaactaaaactaaaatataaaaaactaaataataacgcctaaaaatttcctcatcctcaaaaatcccgatcttccacatcctcaacgcccgcatcaccttcgaaaacctcaacgactacgacgaaccgataccatcgatacgaaacaaccccaacaacgaaacgccttccccaaacaacgactcctccaacgtcaacaactccaactccacgaataaaaccccccgcgaaaacgcctacccctcgactctccccgaaataaataaaaaaaacgcgcccgaccgtacctaacccaacccccgcgcccccaacctcctaccgcgactacgaaatctccccaacgttattcgaaaccccgcgcgactacaacataataaacgaccaacgaaaaacgacgacccgaaacgacgacgacgacctactacaattcgccatccaacaaaacctacttaaaacgaacaataaatataaccaaatacgtctccgcgaacgcgcgaaaccacgaaactccgcgccgccacgactaacgcccacgcctccccgcaaatcaccatctaaaaaacgctaaccaacaacaaaccaaacacccaccccatatcctacgaaaatcgccgacaaaacaaatcaatacccgctaaaccgaaaaaaatcctccgaaaaaaatcctatctcccctaaaccaaaacacaaccgaaaaacccgcgaaaccctcgacaaaaaccctcctaatatcgaaataacttctaccaccactcctacctccgaaacgacaaacaaaaatcaaaaatccaaacttcaccgcgaaattcaaactctccccaaacattaacgaaaaaaacttaataaaatctaaactccgccacgaccaaataaaaaccaaaacgccgcgaaactaaccgcctccactaaaaaataataaccgcgaaccgccctaaaacctccacgccgtatcccgaccccgaccgataaataaatacgcccgaaaacccgcgacattccttccccacccccaaaaacgccccgcccacgccgcaacgccaacctacgcccccgacgtcaatacccaaccctcgacccaactcaaaaccaaattccgacgaccacgtattccgaaactacgacgaacaactacgactaacgataaaactatcgacgcaaaaacaaaaaaaaaaacgacgacgcgcgcgccaaaaaaaaaaaaaactaaaacgcatcctaaaactctcactaaccgaacaataacgccccctaccgaaaccctcgccaacgccacgcgcgccacgcccaaaaccaaaaaccaaacaaaccccgacctacgcgcctacaaaacgacgactaaaaactaaaaccaccgcctcgcgaatacaacaacacaacaaacacgattcgaaaaaaaattcgacataaccgcgaaataccttcccaaaccaaaaccctaaaaacaactaacacgacctaatccccctactttactatattctaattccccaacccgctcccctaaactcaaatctatcctatcctaaaacgaaaccaaacgatcctaaaaaaaaaataaatccttaaaaaaacgctatccctatcccttactccttctaaccgatccgcatttctattcactaaccccactccaaaacactacccctaaaacctttacatctctactcttcactcctaaaaaacaactaaactccccgcgtactatatcactactttattccaaacacaaaccaacacgtctaaaacccaacccctcccccaccccgacatttcaacgtcaaatacacttaacgaaatacccgactcccccaacccccacacccgtcctaaatctcaaaataattccaacttctccttaaacaaccaaaaattaaaatcccatcccccaaaacacatttttttttttttttttttataatcaaaaaatatatccaacgtaaccccctaacctatacaaaccctaactccctcataatacctcgaaaaataaaaaacatattaaactaaaataaacactaaacccaaataaactaaacacaaaaaactcgcccaaaaccctaacgccacccccaccccttcccaccaactactactaacctctataattatacatcccacttacccccacacgaaaactaactctaaaacccttcatccaataatactaacccccgactctcccctaccccacctcacccacccaaaaaaacacaaaccccgccaaaaacaaaaacccaccgcacacccttatcccgaacctatctaaaactaaccttcccgactcaaccaataaaactcaaaaaaaacacaaaaaaaaataaaaaaaaaaaacaaaaaaaaactattcctcccacccccttccctaataccaaaaacaccaaactaattctaaaacacaaataaaaaaaacttcataccgaaaacttttactacctaactttacttaaaaaaaacgcctacgatataaattaaaatccttctaaacctcaaaataaaaaaaactctaaaataaaaaactacctaataaaccctaaacccaaaaatacatcgccaaatctcccaaaaacctaaaaataacatttacaaaaactaaaaatctcgttcccctcactcccacccatacaaaaaacacaaactaaacgcttaataaaatatttcattcaatacgtcttatttttctaaaaaaaacaacgacaaaaaattaaaaacaatatatatatatttataataaacctaactcctcataccaattctctcgaaatttcttcgcgaaaactaccgcgaaaaaacaaccctcgcccctatcgataaaaaaaaaaaaaaaaattctctaccacaaaccgctataaatataaccactaaatccgactctacaacaaacgaattatatatatatctacaaaactaaaataacgcccatctaatttaccgctcaaaataataaaatccaataaactaattaaaaaaaacgctatcattttccccaacctaaaaatacccatcaaatcgccacccgtttaaaatcaaactcaaactccaataaccccaaacatcacgctaatactaaacactttccctaccctaaacgaaaaacaaaaaaaaacaccacctcgccgtacaacaccattactaaaccccccaaattaccccaaacctccctaaaccaactccaaccgaatcccaaacgaaactcgcaatccaacctccgctaaaacgacgtaaatctcccctaaactccaaaaattctaatctcccgcgaaaaacgaaattccctccccaatcccgcccccgaacccaacccaaaaaaacgaaatccgaaattcgaaactaaaaaccgaaacgaaaccgaacttatacgccccgccccgctccgcctacctaacgcgcgaaactaatccgtaccgtccaccaactcgcacaacatattctccaaaaccgtaatacgctactcctaaacctacacccgctcgcgaaaaaccttaatctcttccaacaacgtctccaaaatatactactactaaaacgaaaaacaaaaaaaccgtatcgtataaaaacgattaaaaaaaatataaattaaaccaaaatacaacaaaaccgatcttaccgacaaaaaaacgtcgctaaccgactaactacgacgaaaaccgaaaaacgaacgcacgtccaaaatattacgcttcgtaacccgaaactcgcgatacttaaaaaacacataaccgtccctcaacgaaataaacacgaattcgacgtcctaaccgaataaccattcgtccgcttctaaaaccgactccgaacctaacgtatccgaatacaaatcgtcctaaaaaaaatctaactacgaaaataaataaacaaaaaaacttacgtaaaaaaatacgaaacttactccgctcccttccgcctcgtaaccctacccaacccttctcccgacccctcaccttacgaaacacaatcataataataaattcacactttctttcgtataacttataaaacctataaaaaaacaaaattcaacaccctcgcaaacttccacgtccttaacttctcctatctaaaaccaaaaaaattaaaaaccaacacttactcaacgcctaccatacatattacacattacacacattattaattctacaataaaacaccctaataatatattcaccatcatcttataaataaaaaaactaaaattaaaaatataaaactaataaacgataaatctaacactaaaacaaaactatcttatccccccgccccgcttttccaaaacactacattactaaaaaaaccccgtaactaaaacccgacataaataaaaaacaaaaacgaataaatattcaaaaaaaaccaaaactactaaccgaacgatctcacacttactaacatccaatccccttttaaacataaaacccataccccgctacgactctttactactaaacgtattcaaataatacacgaaaaacgactcgtcgataatctcaaaataccgaatactactatcgccctacaaaatcaatcgattcaaaaacgcgcccgaacaaaaccctccacatctccatccaataccctattctccctacccgaccgtaaacaccttaccacacaaataaacgatactaaaatcgaaatcgtaaaaaaacaataaaaccccgttacttatatccatctcctacaataccactaactcctcgaaattattctacccgaacacaaaaaacgtaaccaaccctaccccaccctcccgtactacttcgaaacccccaaaaacccctttacgcttcctaaccttcccaaaccctataccccaaacctctaataaccaaaattacaaacccctcccctaaacacatctctcctcctcccctacgcacataactcctcctcccctacacatatacccgctacgcgccgcatacaatcacaacaaaccacccccaaaaactcgacatcaccaaataaaaacgccaacgcaaaatccttcacgcgacgcaacaaaactaaacaaaaaaataaatataaaaataacaaacgctacaaaaataacaacaaccttcaatcctatccaaataaacataccctacgaataaaaaacgcctaaccactctcccgtaataccaatccccgaaacacacaccccaaacctccaactacgttaccgaatcccacaaacccaactctcgctaactcatacgaataaaacccgtaataaaaatataaccctaacgcgtaaaaacgacccgcataaacctcatcccctcgtaaaccgcaaacctctcctaaaaaaaaaaaaaaacaaaaaaaaacatcacccaactacctaccctaaaaaacataaaaaaataaacaaccaacttactaacttaaatatccgaaataaaaaaacgaatacgaaaaaaaaacaaataaaacctaaacactcaacttcctacgaaaccacgtctaacccctaacctaaaaaacatccgaacctaaaaaaaacaaaaaacacgcgactctcaaccgatcccgaacccttaaacgcgctcaaaaaccgatccctaaaacaaaaatatctactaactccccgaaatcgcaacgaaacttttcccgaataaaaactccccgctccgctctaacctcttaaacgccaaccacaacccgaaaaaacgctcccgacaaacccaaaaaaaaaacgaactaacgcgcccgacgcgacctaacctaccgaatcccaaaacgcgaattaccgctcactcatcctactaaaaccgatactaaacaacttcccgtctacgataaaaacaacccgcaacgaacgaacgccctcgtaaaaccgaacttactcctactcgccgaattaataaattaaaacgccccgacgccaaccccgaccgctctcgacgcgcttactccacgcaaacatacacgcgacccacgcacccgcaccccaaattaaacttaaaactaacgaaaccaaaaccgccgccctcccaaaacatccgactaaaataaacaacgcgcgaaaattaccccatcccccgcccaacgaatccacaaaaaaaaaaaaccaaccctcgaaccaatatcaaaccccaaaccctaaaaaatacgtctaaataccgactaaaaaaaaaaaaatccaaaaactcaaatttcatacaaattctaataaaaaaataaaatttccaacttctcccctcctcaatcccaaaacgaaaaacccttctctaaacttctaaaatacaaaaaaaaaaaaaaaacaaaaaccgaacaaaaaattacaaactaaaaacttacttaaaacaaaaacctataattacaaaaacgaaaaaaaaaaactaatctctaaaacaaaaatacgacaaataaaaaccgaaaccaaaaactctaataataataaatacaaaaatactaacaactaaccactaatcaaaaaattctaaaaaataaccaaaccaaacactcaccgccaccacttaaccttttctaaaatcaataatacgcaaaatcttatccttacaaataataactaacaaactaccgttactattccaacacacactataaataacgtctaaatacatatcatccaaactcaacaacacctccccgatacccacattccaaataataatcacattatcaccacctacccaaaataaccaaacataatcacctaaatcccacctttaccaccacccacccatctataaaaaacccctccttaacccccaaacctacactaaacaaaacattcctaacaataaaataccaaaaaaaaatacccacacgcttaaaataaccctcaaatataataataaattccgtaatattacgcataaaaatataatctaaaatctaccacacctaaataaaaaaaaaaaatatataataaataaaataaaaaaccaccctatccctccactccttccctacctttttttttaaccctactaactctcttaaataataaaaatcaaatacaaaacaaaatataataatacatacctaaaacaaaaacaactaaaaaccaaaaaaaaacactaccaactctccaaaaacctcccattcactccaacaaaaaaacttcaaaacactaccctactactctccaaacaccaaattaaccataactataattaatcctaaacaatacatcctaaaaaaaaataaacatataactaaaaataatccaaaaactaaacaaaacaaaaccctaaaacccaacacctcccttattaccacccttaacaccttccccaacacaaataaaacaaccttccctactcccctactcaactacccaacaataaccacctaactcctaccataataataatatcgtctaaaacactaacgataacgttatcattatataaacaccaatcaatatccaacacaaaaacaatatacccaataaccaataaataattcttatc

SEQ ID NO: 5 - DNA, 34993 bp, Artificial Sequence
  G to A (bis2 rc) rc
gataagaattatttattggttattgggtatattgtttttgtgttggatattgattggtgtttatataatgataacgttatcgttagtgttttagacgatattattattatggtaggagttaggtggttattgttgggtagttgagtaggggagtagggaaggttgttttatttgtgttggggaaggtgttaagggtggtaataagggaggtgttgggttttagggttttgttttgtttagtttttggattatttttagttatatgtttatttttttttaggatgtattgtttaggattaattatagttatggttaatttggtgtttggagagtagtagggtagtgttttgaagtttttttgttggagtgaatgggaggtttttggagagttggtagtgtttttttttggtttttagttgtttttgttttaggtatgtattattatattttgttttgtatttgatttttattatttaagagagttagtagggttaaaaaaaaaggtagggaaggagtggagggatagggtggttttttattttatttattatatattttttttttttatttaggtgtggtagattttagattatatttttatgcgtaatattacggaatttattattatatttgagggttattttaagcgtgtgggtatttttttttggtattttattgttaggaatgttttgtttagtgtaggtttgggggttaaggaggggttttttatagatgggtgggtggtggtaaaggtgggatttaggtgattatgtttggttattttgggtaggtggtgataatgtgattattatttggaatgtgggtatcggggaggtgttgttgagtttggatgatatgtatttagacgttatttatagtgtgtgttggaatagtaacggtagtttgttagttattatttgtaaggataagattttgcgtattattgattttagaaaaggttaagtggtggcggtgagtgtttggtttggttattttttagaattttttgattagtggttagttgttagtatttttgtatttattattattagagtttttggtttcggtttttatttgtcgtatttttgttttagagattagtttttttttttcgtttttgtaattataggtttttgttttaagtaagtttttagtttgtaattttttgttcggtttttgttttttttttttttttgtattttagaagtttagagaagggtttttcgttttgggattgaggaggggagaagttggaaattttatttttttattagaatttgtatgaaatttgagtttttggatttttttttttttagtcggtatttagacgtattttttagggtttggggtttgatattggttcgagggttggttttttttttttgtggattcgttgggcgggggatggggtaattttcgcgcgttgtttattttagtcggatgttttgggagggcggcggttttggtttcgttagttttaagtttaatttggggtgcgggtgcgtgggtcgcgtgtatgtttgcgtggagtaagcgcgtcgagagcggtcggggttggcgtcggggcgttttaatttattaattcggcgagtaggagtaagttcggttttacgagggcgttcgttcgttgcgggttgtttttatcgtagacgggaagttgtttagtatcggttttagtaggatgagtgagcggtaattcgcgttttgggattcggtaggttaggtcgcgtcgggcgcgttagttcgttttttttttgggtttgtcgggagcgttttttcgggttgtggttggcgtttaagaggttagagcggagcggggagtttttattcgggaaaagtttcgttgcgatttcggggagttagtagatatttttgttttagggatcggtttttgagcgcgtttaagggttcgggatcggttgagagtcgcgtgttttttgttttttttaggttcggatgttttttaggttaggggttagacgtggtttcgtaggaagttgagtgtttaggttttatttgtttttttttcgtattcgtttttttatttcggatatttaagttagtaagttggttgtttatttttttatgttttttagggtaggtagttgggtgatgtttttttttgtttttttttttttttaggagaggtttgcggtttacgaggggatgaggtttatgcgggtcgtttttacgcgttagggttatatttttattacgggttttattcgtatgagttagcgagagttgggtttgtgggattcggtaacgtagttggaggtttggggtgtgtgtttcggggattggtattacgggagagtggttaggcgttttttattcgtagggtatgtttatttggataggattgaaggttgttgttatttttgtagcgtttgttatttttatatttatttttttgtttagttttgttgcgtcgcgtgaaggattttgcgttggcgtttttatttggtgatgtcgagtttttgggggtggtttgttgtgattgtatgcggcgcgtagcgggtatatgtgtaggggaggaggagttatgtgcgtaggggaggaggagagatgtgtttaggggaggggtttgtaattttggttattagaggtttggggtatagggtttgggaaggttaggaagcgtaaaggggtttttgggggtttcgaagtagtacgggagggtggggtagggttggttacgttttttgtgttcgggtagaataatttcgaggagttagtggtattgtaggagatggatataagtaacggggttttattgtttttttacgatttcgattttagtatcgtttatttgtgtggtaaggtgtttacggtcgggtagggagaatagggtattggatggagatgtggagggttttgttcgggcgcgtttttgaatcgattgattttgtagggcgatagtagtattcggtattttgagattatcgacgagtcgtttttcgtgtattatttgaatacgtttagtagtaaagagtcgtagcggggtatgggttttatgtttaaaaggggattggatgttagtaagtgtgagatcgttcggttagtagttttggttttttttgaatatttattcgtttttgttttttatttatgtcgggttttagttacggggtttttttagtaatgtagtgttttggaaaagcggggcggggggataagatagttttgttttagtgttagatttatcgtttattagttttatatttttaattttagtttttttatttataagatgatggtgaatatattattagggtgttttattgtagaattaataatgtgtgtaatgtgtaatatgtatggtaggcgttgagtaagtgttggtttttaatttttttggttttagataggagaagttaaggacgtggaagtttgcgagggtgttgaattttgtttttttataggttttataagttatacgaaagaaagtgtgaatttattattatgattgtgtttcgtaaggtgaggggtcgggagaagggttgggtagggttacgaggcggaagggagcggagtaagtttcgtatttttttacgtaagtttttttgtttatttattttcgtagttagattttttttaggacgatttgtattcggatacgttaggttcggagtcggttttagaagcggacgaatggttattcggttaggacgtcgaattcgtgtttatttcgttgagggacggttatgtgttttttaagtatcgcgagtttcgggttacgaagcgtaatattttggacgtgcgttcgtttttcggttttcgtcgtagttagtcggttagcgacgtttttttgtcggtaagatcggttttgttgtattttggtttaatttatattttttttaatcgtttttatacgatacggtttttttgtttttcgttttagtagtagtatattttggagacgttgttggaagagattaaggtttttcgcgagcgggtgtaggtttaggagtagcgtattacggttttggagaatatgttgtgcgagttggtggacggtacggattagtttcgcgcgttaggtaggcggagcggggcggggcgtataagttcggtttcgtttcggtttttagtttcgaatttcggatttcgtttttttgggttgggttcgggggcgggattggggagggaatttcgtttttcgcgggagattagaatttttggagtttaggggagatttacgtcgttttagcggaggttggattgcgagtttcgtttgggattcggttggagttggtttagggaggtttggggtaatttggggggtttagtaatggtgttgtacggcgaggtggtgtttttttttgtttttcgtttagggtagggaaagtgtttagtattagcgtgatgtttggggttattggagtttgagtttgattttaaacgggtggcgatttgatgggtatttttaggttggggaaaatgatagcgttttttttaattagtttattggattttattattttgagcggtaaattagatgggcgttattttagttttgtagatatatatataattcgtttgttgtagagtcggatttagtggttatatttatagcggtttgtggtagagaatttttttttttttttttatcgataggggcgagggttgttttttcgcggtagttttcgcgaagaaatttcgagagaattggtatgaggagttaggtttattataaatatatatatattgtttttaattttttgtcgttgttttttttagaaaaataagacgtattgaatgaaatattttattaagcgtttagtttgtgttttttgtatgggtgggagtgaggggaacgagatttttagtttttgtaaatgttatttttaggtttttgggagatttggcgatgtatttttgggtttagggtttattaggtagttttttattttagagttttttttattttgaggtttagaaggattttaatttatatcgtaggcgttttttttaagtaaagttaggtagtaaaagttttcggtatgaagttttttttatttgtgttttagaattagtttggtgtttttggtattagggaagggggtgggaggaatagtttttttttgttttttttttttatttttttttgtgttttttttgagttttattggttgagtcgggaaggttagttttagataggttcgggataagggtgtgcggtgggtttttgtttttggcggggtttgtgtttttttgggtgggtgaggtggggtaggggagagtcgggggttagtattattggatgaagggttttagagttagttttcgtgtgggggtaagtgggatgtataattatagaggttagtagtagttggtgggaaggggtgggggtggcgttagggttttgggcgagttttttgtgtttagtttatttgggtttagtgtttattttagtttaatatgttttttatttttcgaggtattatgagggagttagggtttgtataggttagggggttacgttggatatattttttgattataaaaaaaaaaaaaaaaaaatgtgttttgggggatgggattttaatttttggttgtttaaggagaagttggaattattttgagatttaggacgggtgtgggggttgggggagtcgggtatttcgttaagtgtatttgacgttgaaatgtcggggtgggggaggggttgggttttagacgtgttggtttgtgtttggaataaagtagtgatatagtacgcggggagtttagttgttttttaggagtgaagagtagagatgtaaaggttttaggggtagtgttttggagtggggttagtgaatagaaatgcggatcggttagaaggagtaagggatagggatagcgtttttttaaggatttattttttttttaggatcgtttggtttcgttttaggataggatagatttgagtttaggggagcgggttggggaattagaatatagtaaagtagggggattaggtcgtgttagttgtttttagggttttggtttgggaaggtatttcgcggttatgtcgaattttttttcgaatcgtgtttgttgtgttgttgtattcgcgaggcggtggttttagtttttagtcgtcgttttgtaggcgcgtaggtcggggtttgtttggtttttggttttgggcgtggcgcgcgtggcgttggcgagggtttcggtagggggcgttattgttcggttagtgagagttttaggatgcgttttagttttttttttttttggcgcgcgcgtcgtcgtttttttttttgtttttgcgtcgatagttttatcgttagtcgtagttgttcgtcgtagtttcggaatacgtggtcgtcggaatttggttttgagttgggtcgagggttgggtattgacgtcgggggcgtaggttggcgttgcggcgtgggcggggcgtttttgggggtggggaaggaatgtcgcgggttttcgggcgtatttatttatcggtcggggtcgggatacggcgtggaggttttagggcggttcgcggttattattttttagtggaggcggttagtttcgcggcgttttggtttttatttggtcgtggcggagtttagattttattaagtttttttcgttaatgtttggggagagtttgaatttcgcggtgaagtttggatttttgatttttgtttgtcgtttcggaggtaggagtggtggtagaagttatttcgatattaggagggtttttgtcgagggtttcgcgggtttttcggttgtgttttggtttaggggagataggatttttttcggaggatttttttcggtttagcgggtattgatttgttttgtcggcgattttcgtaggatatggggtgggtgtttggtttgttgttggttagcgttttttagatggtgatttgcggggaggcgtgggcgttagtcgtggcggcgcggagtttcgtggtttcgcgcgttcgcggagacgtatttggttatatttattgttcgttttaagtaggttttgttggatggcgaattgtagtaggtcgtcgtcgtcgtttcgggtcgtcgtttttcgttggtcgtttattatgttgtagtcgcgcggggtttcgaataacgttggggagatttcgtagtcgcggtaggaggttgggggcgcgggggttgggttaggtacggtcgggcgcgttttttttatttatttcggggagagtcgaggggtaggcgttttcgcggggggttttattcgtggagttggagttgttgacgttggaggagtcgttgtttggggaaggcgtttcgttgttggggttgtttcgtatcgatggtatcggttcgtcgtagtcgttgaggttttcgaaggtgatgcgggcgttgaggatgtggaagatcgggatttttgaggatgaggaaatttttaggcgttattatttagttttttatattttagttttagttttatttcgattttatttaaatttcggtcggttcgttacgggtttaggagaaatggtcgtgcggttttattaattttaattgggaagttaggaggtagacgtagggtgatgaagtttcggagtttggtaaaaagcgtattgttgacggttatgaggttaatgatgggggttatttgtttatatagggataggggatgttttttatatagttatagtttggttttgaatttgtttttattagattttaaggggtaagggatattgtaggaagttatggttttttagtattttttggagtttcggttttttatttttttagtatcggtaggggttttatttttgtgttttggtggttagttttatggggcggtttatattacggttgtttagtttaaagttggggttgaagtatttttttgtagtgatggtagtggggttggtttggtttagagtttgagtgattagggtttgtattatatggggaggggtttaggagttttttttagtttttaatgttaggttaatttatttgttgttataaggtttttaagttgttttttttgttagtgtggcgttgatatggttttgggtattgtggaaaggaggtttatataggttatgttaagtaggacgttttttaagtttttttttgagttatatttatatttttttatttacgggtatttttgtatatatttattttattttgggggttttcgtgttgtttagcgatttttaggaaggattgtaaaggtgttttatagtttataagaaatgtggtattttagaggatatcgtaattttatatatatttgggtattttattagaggtgatagtatttaagatttagggaggaggtcggtttttggggtggggtttgtttatttaattatatatttaggtatttttatttgaaggggattgagtgttttaaggattaggggttagggtttttgtgagtatagtttaaaatattaaaaggaaggtttagaggttagaagtaatttttaaaagtgtttttttttagttcggtgattttggatagtaaaacgtttgtttcggtaggtattgtggggtgtgtatgtgcgtgtgtgtgtttgttttaggtatttttataggtatgattttatgttgtttttttgtgaggtagaaattatgtttttttatttcggatacggtatttggtatttagagaattaggtgtggtattaatgggtatatagaatttgtggtaaggttttttgattttttatttaggatatgttttattagattagaatggttaataaatggtatatatggtatttttttttttttttaaatttaatagtaatattagtaattatttgtagtatggttttttattgaatttagatgagtttttagaaattttttagtattttaggtagttattatttatttttagggtttggtatttgaattgaaatttatcggtttgaataaagtatttagttttttgttaggatgttagtgggaatattgatggaagtattgaagtgggagttggttttcgtagttttgtaatatttttttttatttagttttgttttattatttttgattttgtttttgtgttgttttgaaagatgttttgttcgtgtgcgggtgatgagttttacgttagatgttttatatatttggggatagatgaagaaagggtttataagtagttttggttttattttgtgttttatttttaagggtattgggaatattttttgtagtaaagggttttggagagattttgttttaggtttttgggtaagtgaatatatgaggttatttatttatttatttatttatttatttatttaataaatattttttgaggagtttttatgtgttaggtattgaggtaggtattagggatatagtaaataagttaaatatgatttttgtttttttgagatttataatttttataaggagataataaaatggagttataatagtatggtttatgtattggtgggggtagtatagaggtttttttagattatagaagtaggggaggtttttagaggagatgttatatataaaatttatggtatttgttagtttttgtttttatgtcgtgggtaatataggggttttagagtaataggtagagtttttttttttttttttttttagatggagtttcgttttgttgtttaggttggagtgttgtggcgggatcgttgtatattgtaagtttcgttttttaggtttaagtaatttttttgttttagtttttcgagtagttgggattataggcgtttgttattatattcggttaattttttgtattgttagtagagacggggttttattatgttagttaggttggtttcgaattgattttaggtgattcgtttatttcggttttttaaagcgttgggattataggtatgagttattatgtttagttaggtagttatttttagggataaaggtttggttttagggttaggttagttaggatttgaattttaattttgttatttaatagttgtgtgattttgtataggttatagaattattttaagtttttatttttttattataaaatggatcgattatttttattttttggggttgttgtgaagagtaaatgggatgttaaggaaaggatttaataaatatgcgtaaaatgggaatattaatagaatagtatttattagaaagggttgttgtgaggaataaatgtgtgtgtgtgtgtgcgtgtgtacgtgttttgtgtatatatttatatatttatataaaatattagagaagtgttttgaatttaaatataagtgtttgattacgttgtattgtttttgtatttttagggttggggaagggaggttagaattttttgtatagtttgttgtaggtaagagtgtagttgggttggtagttgggagttgtagttttattttagttttatatttatttattattttcgtttttttattgcgttagtttaggatgttagttttgtttttggggaagtagagtggtttaggtgaggtaggtattttatcgggttggtttaagggtgattaaggttatgtttatttattttttaaaggagatatttttggtgttaagttgagtggtgacgacgggcgcggtaagtcggtttagtatttgttttttagtgggttgagtagtagttagtagtagttttcggttttgtttagttagtgttagagtttttgtgtatattattcggcggtcgtggttaatttttatgattacggcgtttgtgtttgttagatacggaatagtatagggggattaggggtggtttggggttgttttttatcgtttttattttgttttattttttgtttgtttgattttggtttttgaagataaagttgcggttttttcgttgttaggttatgtggttaaagtttaggagtgtggtgtttatttttaggttttggtcgtttttttatattttgtaggtgttattagggtagattttggatattaggggtattggtggaagcggaggttggaggtggttttgattggtttggtttatacggtttggattagtttagggtatggggtttgggattcgtgtggttaggaataggggagggaattgaagagagagtagttttttttttaaaattttttttttggttagtgtagattatatttatatagaagagtaatttgaggtcgggacgggtatgtttttgttattattaagtttttagtgtttattatttgttaatttatttatttatttttttatttatttttttaataaatatttatgaaatatttattgagtgttttagttattgggaatataatagtgaaaaagataggatttttgtttttttagagtttattttttaataaggagcggtaggttatgaatatagtaagtaaattatgatagagtgaagagaataataatggagttaagatagtatttggggtaatttggaaaggtttagttgaggcggtggttttgagttgagttaaggtatagagggaatcgtcggaagaattatgagaatatattttaggtaggggagtaagcgtaggatttaaagtgggagagtttagaagcgatttgttgtagttcgtttattttagttagtgaatttttattttatttttacgtagaagttttgggtttggaggacgaaggggagagaggttaagtttgtattggagaagggtttaagggttttcgtggaggttgagaggttgggttttattttgcgtagtttttttaggagtacggggatgttcgttagtcgttttattattcgttggtagtttcggtatcgaagtattagttgtattagttttaggtttcgggtatttatagttttttggagtattgggggagggcgaggtaaggttatagggtaggattttttagttaattataggtttatgatgttggggaggtttcggttgtggggttggggtgagtagggttgtttatttgtttagtcgttgcgattttttttgtttacgtttgcgtcgtgcgttaggagtatacgggtatatttaaggtgttttagcgtggtggttaggtgtaggggagttcggtcgcggggatttagttgttcgatgtttatttggaggaggaggaggagtggaagataaagttttagttacgtcggaggtagtttttcggagttagatagttttggagtaggtagtaatttttattttttgttggggttgttttgttttattaattttataaggtaacggaaagatagatattatgggtaacggaaagatagatattatgagtaacggaaagatagatacgtggatggaaaggggtttagaagataggatagaaagtaattttggaagagggagggttttttttttttttgtttattaagggtttttggttgggtttttttttttagggtttagtggtttgtttgttaagaataagtttgggattgaagtggggtggtaaagaggttgttggttaaggagtttatttgggattagatttattttaagggttttaggttatttttaggaagagttattaatttagattattgatattattattgagtgaggtttaataaacggttatagtaatatatagataggaatgaaataataagtttatggtattaatataattttataattatgttttgtgtttgtgggatattatgtattaaaatttgtataaattttataattttgtgaataatatgattatattgtatgagatttttgttgtgtgataaaagtgataaaagttttttttggggtttttttttgtgttttttttggggggacggagttttattttgttggttaggttggagtataatgacgtgatattagttcgttgtaattttcgttttttaggtttaagcgatttttttgttttagttttttaagtagttgggattatagatattcgttaatacgtttggttaattttttgtatttttagtagagatgggtttttattatgttggttaggttagttttgaatttttgattttaggtgatttatttggttcgggtttttaaagtgttgggattataggtgtgagtcgtagtgtttagataaaagattttttttttttttttttttttttttttttttatttgagatagggttttattatgttatttaggttggttttaaatttttaggtttgagtaatttttttgttttagttttttaagtagttgggattataagtttttgtatttggtttagaaagtatgtttgttaaacgtaagttttgtttgtttgtttgtttgtttgttttttgagatagagttttattgtgttatttaggttagagtgtagtggtgttattttggtttattgtaattttcgttttttaggtttaagcgatttttgtgttttagttttttgagtagttgggattataggcgagtattattatgttaggttaatttttgtattttagtagagacggggttttgatatgttgtttaggttggtttttaatttttgattttaagtgattcgtttgttttggttttttaaagtgttgggattataggcgtgagttattacgttcggttttaagtataagtatttaaatatatttcgagagtttaggatttttggttaagaatagtgaattgataggttaggcgcggtagtttacgtttgtaattttagtattttgggaggtcgaggcgggtagattatttgaggttgggagttcgagattagtttgataatatggagaaattttatttttattaaaaatataaaattagttaggcgtggtggtttatgtttgtaattttagttaattaggaggttgaggtaagagaatcgtttgaattcgggaggcggaggttgtagtgagtcgagattatgttattgtattttagtttgggcgataagagtaaaatttcgttttaaaaaaaaaaggaatagtgaattgattatatgtatgtaattttttttttttttttgaatttgattaaaacgttagtaaaaaggtttttatttttattataataaatgaaattattttgttattataaataatgagaaaattattgttgtaaaatatatgaaggttgggtatagaggtttatttttgtaattttagtaatttgggaggtaaaggttggcggattgtttgagtttaggagttagagattagtttgggtaatatggtaaaattttatttttataaaaaatataaaagaattagtcgggtatgatggtttgtgtttgtagttttagttatttagaggttgaggtgggaggatcgtttaagtttgggaggttgaggttgtagtgaggtattattatatttttgtattttaggttgggtaatagagtgagacgttgttttaaatatatatatatatatgcgtgtgtgtgtatatatatatgtgtgtgtgtatgtgtgtgtgtgtgtgtgtttgtgtgtgtatatatatatatttttttatatagaaaatatatgtaaagagaaatagttgtttttagaagtttagaattgtgatttttgaagtaaggaaaatgaataaggtgagttttgtaatatttttggatttttgtttggaggaatattttagattgtaatttaaggaggggaagttcgagtagagtatggtgttttttttgagttgagaagatggagataggatttagggaagttaaggtattaaaggttgtagtagagtatagttttggaaaagagtaaattatttaaaaaattttagaaatttgtataggggtttttttaagtttttttgaatattaaattttatatgtgtatagtgaaatttagtaagattatataaaaaggagtaataaaatggtaaatttttagagtttattaaaagtaaggagataattaagttttagttttttagagtggagatgtatatttaattagattttagaagggttatgttttagtagtagagttaaattatttttagagaaaaggtttatttagatttattttaatagattaaaaattagttttaggtcgggtgtagtggtttatgtttgtaattttagtattttgggaggcggaggcgggtagattatttgaggttaggagtttaagattagtttggttaaaatggcgaaattatatttttattaaaaatataaaaaattagtcgggtttggtgatgggtgtttgtaattttagttatttaggaggttgaggtataagaattatttgaatttaggaggcggaggttgtagtgagttaagattgtattattatattttggtttgggtgatagagtaagattttattttaaaaaaaaaaaagaaaagaaaagaaaaagaaaaagaaaaattagtattaaaggttaggtacggtggtttatatttttaattttagtattttgggaggttgaggtaggtagattatttgagtttaggagtttaagattagtttgggtaatatattaaaattttatgtttataaaaaatataaaaaattagttaggtatggtagtatgtgtttgtagttttagttatttagtgattgaggtaggaggattttttaagtttaggaggttgaggttgtaatgagttgagattgttttattgtatttaagtttgggtgatagagtaagattttgttttaaaaaaaaaagttttaaaaaggttaaattgatttgtaagtaatttatttagtttgtttgaataaagtttaatattttttaaagaataataataaatttagatgtttaatattatatttataatgtttaaaatttagttaaaaattattagatatgttaaaaagtaggaaaataaaatttataggtagggtgcggtggtttacgtgagtttgtaattttagtattttgggaggttgaggcgggtggattacgaggttaggagatcgagtttgtagtgagtcgagatggcgtttttgtattttagtttgggtaatagagagagagattttattttaaaaaaaaaaaaaaaagaaagaaaatataatttataattaggagaaaaataattttatagaaataaaatttagaaatgataaagatgatagatggtttaatatatttaagagtttaaagaaaaatatgaaaaagatgtttatgaggagaggaatgagaggtataaaaaagaatttagtggattatttaaagatagtaagtatagtaattgaaatgaaaaatttattgaatggaaataatagtagattagatattgtataatttaaaaattagtgaatttgaagatagtaatagaattttttaaattgaagtatagaggagaaaaatagtattgaaaaataaagttggttgggtttttatagttttagtatttttggaggttaaggcgggaggttggtttgagtttaggagtttaagattagtttaggtaatatagtaagattttgtttttataaataaaataaaataaaataaaataatttttatattagttgggtatggtggtaagtagttgtagttttagtttttttgaagttgaggtaggaggattttttgagtttaggagttcgaggttgtagtgagttatgattacgttattgtattttagtttgggtaatagagtaagattttgtttttatggagttttataatttgtaagatattattaagtattgtaatatatatttattggaattttaaaggatagaataaagaagtaggataaataagataaatttagagaaataggtcgggtgcggtggtttacgtttgtaattttagtattttgggaggttaaggcgggtggattataatattaggagtttgagattagtttggttaatatggtgaaattttatttttattaaaaatataaaaattagttaggcgtggtggtgggtatttgtagttttagttatttgggggttgaggtaggagaatcgtttgaattcgggaaggggaggttgtaatgagtcgagatcgtgttattgtattttagtttgggcgatagagggagattttattttaaaataagtaaataaataataaaagaaagaaagaacgtttaaaatttttttaaatttgataaaaattattatggtgggttgaagaatggtgttttttttaagatatgtttatattatattttgatttttatagtttatgaatgagattttattttaaaaaagggtttttgtagatataattaagttaaggattttaagatgaaataattttggattatttagggggttttaaatttaatgataggtgtttttttaagatatttagagaggtgggaaggttatgtgaagacggaggtagagattagagttttgtagttataagttaagagggttgtggtttagttattagaatttgaaagagataaggtaggatttttttttagagtttttggaaggattgttattttgttaatattttaaatttgtatttatgtttttcgaattgtgatagaataaattttttttttttttttttgagatggaattttattttgtcgtttaggttggagtgtagtggcgtgattttagtttattgtaagtttcgttttttcggtttacgttatttttttgttttagttttttaagtagttgggattataggtatttattattacgttcggttaattttttgtatttttagtagagacggggttttatcgtgttagttagtatggtttcgattttttgatttcgtgattcgttcgtttcggttttttaaaatgttgggattataggcgtgagttattatattcggttaaatatttgttgttttaatttatttagtttgtagtaatttgttgtggaaattaatattaagataaagttaagaattaagaaatttaatgaattttaagtaagataaatacgaagtaaattatattaaggtttattataattaaatgttgaaaattagtggtaaaaagaaaattttaaaagtatttaaagaaatgaggtttattatgtatggaagaatagatataggaaatattatattttttttattagaaattatgtaagttaggaaataatataatgaaatttttaaagtgttgggggaaaaaaataaaaataaaaatttttaatttagaattttttttttttttttttttaatttagtatgattggtattgatttagaattttatattcggtgaaaatattttttaaaattgaagaagaaataaatatgttggtagataaataaattttaagggaatttattgttagatgtgtaggaaatgttaaagggagttttttaggtggaaagaaaatgattttagatagaaatttgaatttgtataaaggattgaagagtgttaaaaaatgttaaatgtataagaatgttaggaggttaggtatagtggtttatgtttgtaattttagtattttgggaggtcgaggcgggtaggttattagaggttaggagtttgagattagtttggttaatatggtgaaattttatttttattaaaaatataaaaattagttgggcgtggtgggggatttttgtaattttagttattagggaggttgaggtataagaatcgtttgaatttgggaggtggaggttgtagtgaatagagatcgtattattgtattttagtttgggtgatagagagagattttgttttaaaaaaaaaaaaaaagaatgttaggttgggcgtagtggtttatgtttgtaagttttgggaggtcgaggtgggtagattatttgagtttaggagtttgaaattagcgtgggtaatgtggtgaaattttgtgttataaaaaaatattaaaattagttaggcgtggtggtgtatgtttatcgttttagttattgggaggttgaggtgggaggattttttgagttagggagttagaggttgtagtgagtagagattattttattgtattttagtttaggtaataaagttagattttgttttaaaaaaaaaaaaaaaaaaaagttagtaaaatatttaaaatttataagaataaagagaagagatgttagtagatgagaaattttaatataattttagaatatggaaagtggttggggttttataattgatttaggggagtagaggaagttgaaattaaagtagttatagagggaaacgtttatataaggagtaagttaggtgatttttagtttttttgaaaggtgtaggtaggatttgtaggtaatggggatggtagaggtggaggtgaagttagagttgagtgtagggaggttggttataatttaggattttttggttttttttttagttttattaagttgggagatgttttttttttttattataggatattaggggtttattttttgtagaaattgggtatgagatgttttggatttaggagtattggttatagtagaggatgaggtatggtgttgaaagttagtgattcgtgaaattttagttttttttttatttgggttttgaattattggtagttaggttatattattattattttatttattcgagtaggaagttgttttaaagattttagaatatagatatttggtgattttataatgaataggttagtttgttatttgattattttatagtagtatttatatatttttgagttttttagttttatttttaaatatgatttaatagttaggagaaattggatatttgatgaaagttttttatgtgaaataaattaaaatatataaattagatgttaagacggttgggtgtagtggtttacgtttgtaattttagttttttgggaggtcgaggtgggcggattacgaggttaggagatcgagattattttggttaatacggtgaaatttcgtttttattaaaaatataaaaaattagttgggcgtggtggcgggcgtttgtagttatagttattcgggaggttgaggtaggagaatggtgtgaattcgggaggcggagtttgtagtgagtcgagattgcgttattgtattttagcgcgggggatagagcgagatttcgtattaaaaaaaaaaaaaaaaaaaaaaaaaaaaataaattagatgttaagaatttagaggaaatttttttgatgtagggaataaaagaaaattttttgggggaaaatagtaatttatatttttaggaaaaatataaaaagattattgaatttatgaaataaaatgggatagtttggttttttatgacgttttttgtttttttttttgttttttttattttggaagtgatttttttaatttttttttgttttttgtatttttggatagttgtatttgtttttataaatagtaaatattatttggatttattgtatttttaggtggaaaaaaaaattaattttaaaattgtttatattttttttttttttcgtattttttatatttaatttattagaaaaatttgtaggttttgtttttaaaatagatttagaagtcgtttagtttttattattttgtagttgttgtttttttattttttattggtagttttttattgtttttttgttgtttttcggttgttaggttttattgtttattttatttatggtagttaaagttattttgtgaagtgttatttaggttttgatattttttagtttaaaattttttagtggttttttatcgtaggtagtagggaatttaatggttttagatttttttttgaatttatttgttttatttttcgttaatggtttttttcggaacgttttttaggattttttagagagttttaaagttttttttttttttttatttaggttgttgtttaaatgttatttttttagaaaagtttattttgatagtttatttgaggtaatagttgttatggttttatttattgttcgtttaagtgtttgttgagtattttttgtatttcgaatagaagttttattagttaggtttttgtttgttttgtttattgttggttttttattttttaggtagtatttggtatataaatatttgttagataaatgtatagagtattaggttgagggggtataaggaggggaaggtaattaattaagaaattattgtagaagtatattgtttatgtcggggggtttacgtttgtaattttagtattttgggaggttaaagtaggtggattatttgagtttaggagttcgagattagtttgagtaatatggtaagattttatttttataaaaaaaaatataaaaattagttaggtatggtggtattatttgtagttttagttttttgggaggttgagatgggaggattatttgagtttgggaggtagaggttgtattgagttgtgattatattattgtattttagtttgggtgatagagtgagacgttgttttatgaaaaaagaaaaaaaagaagaagaaagaaagagaaagggagggaggtagggaagggagggagggagggagaaggggaggggagagggtagtataaataatatattgtttataattagggaggtaaatgataaaaggagtttagagtgttggggaggtgggagaggcggagtaaggagtattgttttttattacgtattttttagtaatagttaaatattttaaagtatgattatgaattttattgttaaaaatgaaatattttaaataatttaagattatttatataatttttatagttttgttttggaatttttttattttttaatatattgggagttttaaaaaaattagcgggtttggtttttgttggtttttgagttgtggttttttatagagaaggggagtgttgtttatttttgtttaattttggttgggttggatttcggggtttgtaatttgggtggggttttgagttcggtagcgggagtgggagagggttatagggttcgagttgattggggaagtgttgagtaatttaggttttttagttttgttttagatgttgtagtcgtagtcgttgtagttaataagattttagggagttggtaggtcgttgtttggttttagggttttagatgttgtttttatttttttattaggtgttttagttttaggttttagagagcggttggtatttttttgtaagtagggtgtttttttttatttttatattttaggagtattttttagggaggtttggatggtttagtattttatatattttatgtagaattttatatatttagttaagttttagagtagttttttttataagtttagagtgtcgtttgtagtgtaagtggtattttgttttgggtttaggtaggagaatttattaatttttttagtagaggtttttagtttttttttagtagaggtttttagttatttaattgttggaatgaaaaggttttttatgaaatttaatatttagttttttttattaagagaacggagattttttattttagtaggttttagttggagttaaaaggtggagtttttggagttttgtagttgggggtttttgggtagagagtttttttatttttatttaggtatatatattatattttagtatatattggtattatatagatatatattcgtacgtttataggtatttacgtgtgtttttaagtgtataagtatatgtatgtttagttgttttttggttttgtaggagtttatttttgtgtaacgtgtgtgtgcgtatttgtataggaatattttttatatttatgtgtattagtagggtattttttaaatttttttagtatgagtagaatttttttgttaagggaagtatgaaaagtatatattttatgtatggattaaatatagtgtttgcgaggaaggtgagggacgtagagtttgtgtttaaggtggtgtttgtttagttttttttttagtttacgaggaggaaggtaggagtttggtgtagtcgttgtttgattttttttgtttagcgtggggtgtaggggtaggtttgtttgagtttatttaaggggagggaggtaggatgtatttttaagttgcgtaggaggttacgggttgtggggatcgtattttggatttttttttttatgttattttttttattttgtttttgtagttttttttttttattttagaatatattgatttttggtttttggggtttgtggttttttttttcgagttttttagtttattagttgtggtgatgttttatatttaggattgtttagtgtaggtaaagggaggggtttgaggtgtttttcgtatattttgggttttataatttattttttttgtttttaggttagaagggtgaatagggaaagtaggaagtaagtttacggtggagaacgttttagggagaaggaaaatgattttttgggattataatttgtttattttagggttttggttgttaggggtagagttttgttttttaggtttagtttatatatgttttttttacgggagttgtataggttaatttttttttttgtttttattttagggaatattaggaatttacgattttagaattaggattatgtttagttggttatgttaggtaagggggaattggtatattttttggtttataattttgtttttttcgatttggtagagaatatgtatagcggtaagtagggtatcgggttggtattatagtattgttgggtgttttttttttttattaggtattttttatttgtttattattttttgtttttagtttttagtagagtaatttggggttgagtaaagtttattaatttgttttgaaggtggttatgttggttttttttttagttagttgtattgttaagtttgtttacggagggtttttgcggggtttttttggagtgaagaagaggtagttatgttaagttaagattagggaaatttggtttttgagtgtttgaggaaagtcgagttgtttttgtggcggttggtattagggggattagaggttagggatttttggttgggatgttagggttttatagtgttttttttatgatgttaggtggttgtttttaggttttttttgtagaaaatagagtttggtgttttggggagtaggtagtgtatatttggatataagttttattttgggttagttttcgagaggggagatagttagggaatttttttatttatacggagtggtatttttttttttggtacgtttgagggaaggagaggattggtttggtttttttgtggttgaataagggttaatttttattagtgttttatattttttttggtttggatttaggataggtagtgtttattttaaggagatattaatttattggggtaggggtaggggtgaatttgggattttgtttttgaggtagttagaggggtgggagagagaaatatatgagtagtttttaatatttttatttgtagcggtttcggtgttttttattttaattttattttagtaagatggttatttattttaggattattagtagagaggtttgttggagaagtttttttttttagggtattttgtttttttttagtttttgtagtaaaaggattatttatttttaggtaagggagtgggattgaggtattttggagatttagttttttgtttagtgatttttggatttttgggaagttttttttatatgaggtttgtttttttttgtttttagggaaggaaagtagagaagagttagtagaggttggttggttatgttttagcgttttgtatattattttggaattttttgtttatatttgttttattagaatagagattttttgagggtaggggttgatgttttgtttgtttatttgttttttgggggtattgtgatttattttttttaataggtttttcgtggttgtagagtattgtttttatgatagataaataaagatagggtttgaggagtttagtttgaggagaaattcggagagtgttggtataggtataggtaataggaagtggttatttagatcggtttagaggtttgcgggtataggttattcgtatatttatagggattgttatgtagagttggatgttatgtaggtttgggggttggtttagcgtgggattttagagatatattttgatttttagtttgtttagttcgatggtttgttttttatttttatgttttttttggcgattgtatagttttttagattgaattttttatgatttaataagtagtttttagaaggtaaatttttatagcgggtaattgcgttaattatttttagtttatggttttaaggttttagatttagtttaaaattggggtttttagtttgtagtaagttatgggattcgggtttagttttggtttttgtagtttattttggaggcggggggttatttttgttatgagtgtttatttgtggtttgggtgttaagggtagaagtggtaatttgtgatttgtgtttgtttttgttttgaagtatggttagaagatattttgaagtatggttagaagatattttttttttttttgttttttggagattattgtttagtttaaagttggtgatttacgtggttttattgattagtagaaattagggagtttatttggtgcgtagaattttaagtttttttagtagttagggttttttagttttttttgcgtttagaaattaggttttagtattagagggtaggagagcgttttttagtatttggataaggtttttggggttttttaagagggtttttttttattttttgtttttgagttggggttgggttttgagagatttaaggatttgtttagtttgagagttaaaagagaaagcgtttatcgttggggagagggcgttgggtggggttggggtgtttgggagtgtgatatagttttttttttatttttgatttatggttttttttttacgtaagttttttttattttcgtatttttattcgggaggtgtcgtcgtttaattggttggggcggatttttttattatatggaatatcgatatagttcgtagtttttttttgtagtttttattgtttcggcggaggaggggtatagaggtttttatttttatttaggtgagttcgaaatacgtgtggtttcgttcgtttcggtcggaggggattattttttttcggttaataagtataaaagtcgcggtcgtaaataaagacgcgtcgtaaattcgttagggaggcgggatagttcgcgtcgtattttttttttaggtcggacgggcgtgttcggtcgcggggttttcgcggcgtttcgaaggcgtttttatttggttcgcgcggatttttttttttagttcgcggtggcggttgtgttatacgaggtagtgtagcggatatttgttttcgggtttttttttggcggaggcgttggcggggattatcgttcgttttttatgtcggggtcgcggcgttcggtcggggaggagggacggcgtcggagtcggggttcggggtcgcggggcggggggtcggcgttgtttgttcgcggggttgcggttcgggtatgtgcgagcggcggcgggcgggggcggcgcgttcggcgcggtgcgggcggcgcgggcgacgggcgttttcgcgaggcggcggcggcgggcggcgcggagaggtttttattcgttttgggagggagcgggtattcggcggcgttgcgcggattcgcgttcgttttttatattttcgtatataaagacgtcgttcggcggagggagtaggcgttcgtagcgggcgcgggggcgtacgggacgcgggtttcggggacgtcgtcgtagggacgcgcgttcgtagttttcgggtttttatagttgtatagttcggtttttagttcgagcggtcggcgcgggatacggggatgtggggatgatggggagagaggaaggggattaggcgtttcgggtagagtttgttagtttagtttcgcggtattatggggtttgtagttcgtttcgtgaaattgggggtggtaggtggtcgaagagggtttgtattgttttcggatttcgtgggagagtgggcggggagttaggtttggtttagacgcgggcggggttttgacgttaggtgggttgggacgtatttttttcgttggtattttgttttttgttggggaagtgggggggtacgggtttaggtcgagcgtttgggagacggggtggaggtgtggtttttagaattgagtttgggttttaggggttatgaagaaggattcggatttttagaagagagcgtttgattgggaatttttgagaaaggtgtggggtattagtattaagggttattggagtagttaggggtttggtttttggaatatttttgaggagttttttttgttttgttagaaaattaaattttattttttatatatgttattggaaatagaatgtttagtaacgcgggaaagatggttttttttttttcgtatattgtttttagtaagaattagagtgaggttggatagaaaaagtagtaggtggtagtttcgtttttttatttagttggttttttaggaagggaagtgattgattttagagattgttttttttttgaatgattttagggtgaagaggtatttttagaatggtttttgtagagggtgtggtaaaagttgaattggttttttaagcgttaattgtaaggtttggaaggattaagaggtttggattagtttttggagggaggggattgtgatgttagagagattagagttcgaatagttttaattgtttgattttaaaagagtaaattgtttaattttttcgattttttcggtttatttttttttaaaatgagaatttagatattattttttggggtgagttaaggataatgattgttttggaaatagcgttttttttttttaattaggcgggtcgagataggtggcgggattaggtacggtgtttttttgagtttattttagaataaggtaggaataagggattttatatcggttttatttaaaataataatttaagaagtgtttgtgtgggaggtgttagtaaaagtttgtaaatttttttaggtttttttgtgtggttttttttttttttttttttatattttgtggtgttaggttttagcgggaagagatgagggaggagcgggttgtttcgtttttttttttcgtttgggaggagttagttggcgttttcgggggttcgggatcgttgttcgtttgtattattaggggttagtagagtgtcgtggttgtagttagtgtaggggagggggttggcgcggttgaggggtatttaggagtggtcgggagtatgtttgtgtatttttttattaaattgtttttcgaattttgtgtgtgattttattgtagtagttttgttttttggggtggtgatatttttacgggggaatttagaaatttttttatttttagttttaggtttagaagtttggttgtgacggggttgggggaaataaagtttggacgatgtgttcgcgttagggttatttttaggtagtttttgagttaattaggagatggggagtggggtggaggggtaagtagagtgaattattttttttttttagtaaagtttaggagttcgaggatagggggagtttaggatggattgtggggagttgtcgattgtggggaattgttttttgggcggtcgtgttttttttttgttaggcggcggtagatattgaatttaggtcgtttgcgtttcggttcgcgtttttagttgttacgtgttcgagacgcgtttatatagcggagaaataaagatagttaagcggtagggttgttagtagttttttcgatatttaataaatgaaattttatagttgggggtcgatcgggggtgaacgggcggttatcgttcgtggattgagcgtttggtacgggttgtttggttatttttttcgttttatttttttcgttttttatttttttttcgttgaggttattaagtttatggattttggtgagagagtagttcggggcggtaggtggtgtttttttttatatattagttaggtatcgttgtttgtaaaagttttattagttgagcggttggttgtcgagggaggggaggtttgtaagatttttttaaggtgtaattataaataaagtttatggatcgcgattttaaataaatttgttaatttgggtcgtagtaaaaggcgatggaggtagttttgtatgtatttcgggtggtgtgatttatgagtattatttgttttttttagggaaggagtttgtttatttataaattattgtcgttttggtatcgttgggataatcgattaatttgagtatttttgttaaaggattgtttttattttaataagtaggagtttttgatttttggagaatttttttttaattgttattattgatttggtttttaggtttggttttggggatttttattttttttttataagtagagtgttcgggttttttgttgttgtagggattgggggttgggtatacgcgcggtatacgcgtatgggggcgtatgtttagtgcgggggttgcgtttatgtgcggtttttatttaggttttttgttttttagtttatttacgttttttatttgttttgtttttgtttgtttcgtcgtgtgaagtttaggaagaaaggtcgttatttgaaacggtttttttatgttatatgtattttttttggatatatatatttttggtggtttagaaatatcgtgggtgtgtgtaaggcggatgataagtggatgtgagtgtatataggtatagtggttatttttcgggaggtttttaaaaatcgtttagatttttttttttttggatggaaggatgtatggagagatagatatatttttagttcggaggtaggggaatatattgtttgatttttttggtatttgggcgtttatattgttagtagtgggcgtatttagtaagagtgtgatatatatatatatatttttggatatatagatgtggatatttacgggatagggacgtatattttattttaattagagatagacgggtattttaaggtatagtttttttgatttggagcgggatttgggtttttaagttttttttttttaatttttattttcgtcgttcgtgggtttagcgtttttcggtttattttacgcggaaagtgaaggggagggggttgtgagggtgatttatattgttttcgggttaggcgagcgttgtagcggaggttagggtcgtaggttacgttgttcgtcggggtcgggtatttgtcgcggtttttttaagcgttttcgtttttttttgttcgcgttcgggttttttttttttagggggcgcggtcggtagcgcgcggcggggcgggggtgcggtttttttttttgtgggtagggtttgcgtcgttttttgtagaagcggtcgggagtcgcgtagggggcggagagaggagtcgcgagcggcggcggggcggcgcggggcggagggcgttcgagggcgagcgggtaggcgggtacggcgggtttcgggttagtttcggggcggacggttggtcgggcgcgcggagtttcgtcggggtttcgtcggagtcgggtcgggtagtaggggtcgtcgtcgtcgttcgggttcgtcgttcgcgttttttacgttggtttagagggttgcggtcgcgtcgtcgttgaggatgtttcgaaaggggtcgcgagcggaggtgtgtgcggattgtagcgtttcgggtaagcgcggcggggtcgggggcgggatcgtatagttaggtcgtcgtcgggcgggcgtcggggtttggtaagagcgttgtgcggggtcggagggttgggcggggcggggggttgcggtttttaggttgggttttcgtttcggttattgcggagttgcgtttttggcgggagggtcggtttggggtgtttatgttttttggaggtcgtggattagcgaggaaggacgttttcggcgtcgtttttcgtttttcggtttgagggaggcgggtagttggttgtttttttatttttatttttgtattcgacggaagcgttagtttggggtggtaggagggtcgtggcggaggtcgttagggtttgggaggtgggggcgagtgtggttttatgttattttagtgttattttcgcgttttgtatttgttgttcgcgtggtcggtacgtttgtcggggtggtggagggtaaggagtagagggtcgggtagatgcgttagtggggtttgaatatcgtttttttaggagtagatgagcggtggttatttttaggattttttgtttcgggtttttaaggttagcgttttttgtcgggtttggcgtttagggttagtttagattcgggtgttttttcgggaggtatttttaggtttgttggtggtgattgggaatagttcggttggattttgttgtttttgtttatcggtaaggtttgtttgggaaagtgagtttggtattaagttattttgggtgcgggtttttttttgttttttagtttagtttggttagaaatgggtgggaggtcgtgtcgagatttttcgtattttgttggttttttggtttgttttttggttgtatttatatggtggttttttttttttttttaatagagttaggattgggttggagtgaaattttttaggtttgttgaggaagttaggggtaatgatttaagaggttgtttttttttgatgagggaggatagttagtgacggggttttgtagttggtttgggaaggaagttttagtttatatttattttttttttagtaaaggagttatttttttggtaggtttttgggtaggttgcggaggttcgtgaattttagcggggttgtgggtatgattaagagtgagagtatggggtgttggtttgtgggtttataatttttagttattttttgagtaggtttaggattttatcggttgagttttatagatgttttggtggttttgggggtgttaagttagagtatttgggaattatgatttagtagggtttgggtataaaatattttataggtggttatgattaaggttttttaggggtttattatggtttagagggttttggggttgagggtttatatttttaagaaattgtgatttcgtttttcgagttgtaggtaggtttggggatggtagggttgaggatgtattttgttttataaatgtttttttattgttttataatttcgtggggtaagtatggtatggaatgtggaggagagttttagtaggcgtttaatcgggggagtttggggtttagtgttgtttttgtttttagtttattttgtaattttaataagattttttttattgtggggtttttagtttttttaatttagaggtaaagaagttggagtagaaatggtttttggggggttgttattttcgaatttgtggtttgattttggggtggaggggtgaagggtagtattagtaaggtagttgttttttgtatgttgcgttgaatgttcgattatagtttttggatgtttagtgggtttagggaggaatggtgggtattagatgtgttggattgtttagtttttttttttaggtttttatttgttagaggaatttgtgttttagatgtttttttttttttgatttataatagaggttaggaaggtggtgagaaggtgaggatggtggggtggggaggatgtggatagttttatttattagtttatttagtatttagcgaggtgtttagtatatggtaggtattttttgagtgtttggttgtttgttaggattttggttggttgtttgggattattttatatttggattttaggatgttggttttggtatgtagcggtatgtttggtttgggttttgtggtattttaggtagagaggtatgagggtatttagtagttcggagtttagatttagtgttagttttatggtgtatcgttttattttagggttataggttttttttattatgataggagttttgtagttttaattataggagtggggttagggattttttgtgtttggttaatttggggggttatggaggttagaggtgagatgtagtttgtttttagagagttttattttttttttgttttcgggtatgggtatataggataagtgtgagtgtgttgttaggtagttggatatgatatggttgttttggtagtttgtgttatttcgttaggtatcgtatgtgtttttgtttgtttggggagtttaagagaggaagggggtagggagttttggagaatgtgtatttttttttttttttaggtttggtttatttcgttatacgattttagttaagggtttttttttattttatgggtttttattttagttttttttattttggtaattttgggggtgagagtgaaggttttaagatgtttgttttgtaggtatttttggtgagtaaggtcggggatatgttacgggataagttataggttgatttgtttttttatagtgtagattgtagagtgggataaatgttgggttttttttttttttttatggaggtagaatttgtgtgtgttaatgtttgtatttgagtgtttattttgatgggtttttatatgtgtgtatatttatgtaattattgttttgattatgttatagaataagggtatttaatttttttgtttttttgggttatattggaagaagaatttttttgggttatatttaaaatacgttaatattaatgatagttggtgagttaaataaaataagtaaaaataaaaataaaaaataaagttataaaaaagttttataatgttttaagaaagtttatgaatttgtgttgggttatatttaaagttgtttgggtcgtatatggattgtaggttagataagtatgttatagaatatttttattattttagggggtttttaagtatttttttttagttcgtgtattttagaggtaattattattttgattttattttaaggattattttcgtttgtttttatgatgtgggttttttttttagtttagtggagatttggtttttagtttaggggagggaggtttgaggttagtttgtatgtgtaaatttattggttttggaggttattgatggttttaggtggtggtaggaatttatcgtagtagaggtttttatggggttggtattggttaacgtgattttaggattacgtttgttatttttttatatatatagatttatattttgtcggtggagttagaagcgtagggggagggttgacgagtttttttatagtttttgtttttttcgttttaggtttggtttaaggagttttttgacgtaaggatttttttattttaaattataatttgggtagttttaagggtatttgtatagagggaggagatagaatggttagggtgggcgttttatttgtgttatttagaaatgagttgatattaatagcggttgtttagattaggatagtgttttttgtttattattttttttaggttatttggaggagaaggagaattttttttttaggttgggggaaagtgttaggtaaatttttggattatatttttgtattttggttttggttattgttatagttagggttatttattatatttggtttgtttatggtttagggttttggagttattggtcgtggatatatagttagttttttatgtttggttttttcggtaggattatagattttagattagtttatttatgattttgttttgggcggttttttatttataggaaattttattaagaggaatttgggttgtattattttcggttttttgtttgggttgttggaggtggttggttggtagttttttgatttagtggtgtttggagtggggagagggaggtttttatatttggggtgttttattatttgggtaaagttagtttagaagtgtatgttagggtttttttttttggcgaagaaggttggttttttttttttgagttttggagttagttttttaggaaggtgttggcggttattttgggtatttttttgttgttttgattgggagggggttttttaaaaagtttaaattcgttgtattttagtttgggcgatagagcgggatttcgttttaaaaaaaaaaaaaaaaaaaaagtttaaatttaaagataggttttttttttttattttttgtttttatgttttagtgggggttatttgttgtgggtagagtttaggttgggtttttgatttagagtttttttaatttttttgggaattttggtggaagtttttagaggggaaaggtttgagaattgttttttagttgggagagatttttattt

SEQ ID NO: 6 - DNA, 24993 bp, Homo sapiens
gcttaaaggggccgcggcagatgcccggccccggcgggcagcgtggcctgcggccctggcctccgctgcagcgctcgcctggcccggaggcaatgtgagtcaccctcacagccccctccccttcactttccgcgtggggtggaccgggggacgctgggcccacggacggcgagggtggggattagggaagaaggacttggaggcccaagtcccgctccaggtcaaaggggctgtgccttggggtacccgtctatctctggttggggtgaggtgtgcgtccctgtcccgtaggtgtccacatctgtgtgtccaggggtgtgtgtgtatgtgtcacactcttgctgaatacgcccactgctaacaatatggacgcccaggtgccagaaaggtcaggcagtgtattcccctgcctccggactaaaaatatatctatctctccatgcatccttccatccagagaggagagaatctgggcggtttttaaagacctcccgaggagtgaccactgtgcctgtgtgcactcacatccacttgtcatccgccttacacacacccacggtgtttctgggccaccagaggtgtgtgtgtccagaaagggtgcatataacatagaggggccgtttcaggtgacggcctttcttcctggacttcacacgacgaggcaggcaaaggcaaggcaggtgagggacgtgggtgggctggggggcagggagcctaggtagaggccgcacatgagcgcagcccccgcactgagcatgcgcccccatacgcgtgtgccgcgcgtgtacccaacccccaatccctgcagcagcaaaaggcccgggcactctgcttgtggggagagggtagaggtccccagggccagacctgggggccaggtcagtggtgacaattgaggaggggttctccaagagtcagagactcctgcttgttaagatgggggcagtcctttggcaggggtgctcaagttggtcgattatcccaacggtgccagagcggcagtgatttgtgggtgggcaggctccttccctaggggagacaagtaatgctcatgagtcacaccacccgaaatacatgcaaagctgcctccatcgccttttgctgcggcccagattgacaagtttgtttgaaatcgcgatccatgggctttatttataattgcaccttaaaaaaatcttgcaggcctcccctccctcgacagccagccgctcagctggtggggcttttgcaagcaacgatacctagctggtgtgtaggggggagcaccacctgccgccccgagctgctctctcaccagagtccatgggcttggtggcctcagcgggaagggggtaaggggcggggggagtgagacgggaggagtggccaggcagcccgtgccaggcgctcagtccacgagcggtggccgcccgttcacccccgatcgacccccagctatggaatttcatttattaaatgtcgaggaggctgctggcagccctgccgcttggctgtctttgtttctccgctgtgtgggcgcgtctcgagcacgtggcagctgagagcgcgggccgaagcgcaagcgacctgggttcagtgtctaccgccgcctggcaaaaaaagaacacggccgcccaggggacagttccccacaatcgacaactccccacaatccatcctgaactccccctgtcctcggactcctgggctttgctggggaagaaggatgattcactctgcttacccctccaccccactccccatctcctggttggctcagagactacctgggagtggccctggcgcggacacatcgtccaaactttgtttcccccagccccgtcacagccaaacttctgggcctgggactggagataaaagggtttctggattcccccgtggagatgtcaccaccccaggaagcaggactgctacagtggaatcacacacaaggttcgaaaaacaatttaataaggaaatgcacaggcatgctcccggccactcctagatgcccctcaaccgcgccagccccctcccctgcactggctgcagccacgacactctgctgacccctggtggtgcaggcgggcagcggtcccgggcccccggagacgccagctggctcctcccaggcgggagaaaggggcgaggcagcccgctcctccctcatctcttcccgctggggcctggcaccacagggtgtggaggaggaaggagggaagaccacacaaagaaacctgagagagtttgcaagcttttgctggcacctcccacacaaacacttcttggattgttgttttaagtagggccggtgtggaatcccttattcctgccttgttctgaggtgggctcaagaaggcaccgtgcctggtcccgccacctgtctcggcccgcctggttgggggagggaggcgctgtttccagggcagtcattatccttagctcaccccaggaggtagtatctagattctcattttgaaggggagtggaccgagaaagtcggaaaaattaagcagtttgctcttttaaggtcaggcagttggagctattcgaactctggtctctctgacatcacagtcccctccctccagggactggtccaagcctcttggtccttccaggccttgcaattggcgcttgagaggccaattcaacttttaccacaccctctgcagggaccattctggaagtacctcttcaccctggggtcattcaggaaggagacagtctctggaatcagtcacttcccttcctgaagggccagctgggtggaggaacggagctgccacctgctgctttttctgtccaacctcactctggttcttgctggggacagtgtgcggggggaaagggaccatctttcccgcgttactggacattctgtttccaatgacatgtgtggaagatggagtttaattttctaacagggcagggaagactcctcagaaatgttccaggggccagacccctggctgctccaatgacccttggtactgatgccccacacctttctcaggagttcccaatcagacgctctcttctgggaatccggatccttcttcatggcccctgggacccaagctcaattctgaagaccacacctccaccccgtctcccaaacgctcgacctaggcccgtgcccccccacttccccagcaaaaggcaaaatgccagcgggggaggtgcgtcccagcccacctggcgtcagggccccgcccgcgtctgggccaggcctgactccccgcccactctcccacgagatccggggacagtgcagaccctcttcggccacctgccacccccagtttcacgaggcggactacaaaccccatgatgccgcggggctgagctgacaagctctacccggggcgcctggtccccttcctctctccccatcatccccacatccccgtatcccgcgccggccgctcgggctgagggccgggctatgcagctgtggggacccgggggctgcgggcgcgcgtccctgcggcggcgtccccggggcccgcgtcccgtgcgcccccgcgcccgctgcgggcgcctgctccctccgccgagcggcgtctttgtgtgcgggggtgtgggaggcgagcgcgagtccgcgcagcgccgccgagtgcccgctccctcccagggcgggtgggggcctctccgcgccgcccgccgccgccgcctcgcgaggacgcccgtcgcccgcgccgcccgcaccgcgccgggcgcgccgcccccgcccgccgccgctcgcacatgcccgagccgcagccccgcgagcaggcagcgccggccccccgccccgcggccccgggccccggctccggcgccgtccctcctccccggccgggcgccgcggccccggcatgaggagcgggcgatgatccccgccaacgcctccgccaggaaggggcccgagggcaagtatccgctgcactacctcgtgtggcacaaccgccaccgcgagctggagaaggaggtccgcgcgggccaggtaggagcgccttcggggcgccgcggggaccccgcggccgggcacgcccgtccggcctggggagggggtgcggcgcgggctgtcccgcctccctggcgagtttgcggcgcgtctttgtttgcggccgcggcttttgtgcttgttgaccgggaaagggtgatcccctccggccgggacgggcgggaccacacgtgtttcggactcacctagatgagagtagaggcctctgtgcccctcctccgccggggcagtgagggctgcagggaggggctgcgggctgtgtcggtgttccatgtggtgggagagtccgccccagccagttgagcggcgacacctcccgagtgagggtgcggaggtgggaaaggcttgcgtggggagggggccataggtcaagaatggggaagaggctgtgtcacactcccaggcaccccagccccacccagcgccctctccccaacggtgagcgctttctcttttagctctcaaactgggcagatccttggatctctcagagcccagccccagctcaggaacagggagtggagaaagaccctcttgggaggccccaagggccttgtccaggtgctgaaaagcgctctcctgccctctggtgctggggcctggtttctaggcgcagaggaagctgaggggccctggctgctggaaggacttgaggttctgcgcaccaggtgggctccctggtttctgctggtcagtaaggccacgtgggtcaccagctttgggctgggcagtggtctccagaaaacaggggaaggggggatgtcttctggccatgcttcaggatgtcttctggccatgcttcagaacaaaggcaggcacaggtcacagattgccacttctgcccttggcacccaggccacaggtaggcactcatggcagagatgaccccccgcctccagggtgggctgcaagagccagagctgggcccgggtcccatggcttgctgcaggctgagaaccccagttttggactgggtctgagaccttggggccatgggctgggggtggttagcgcagttgcccgctgtgggaatttaccttctgagggctgcttattgagtcatgagaagttcagtctgaggagctgtgcaatcgccaagggaagcatggaggtggagggcaggccatcggactgagcaggctgggggtcaggatgtgtctctgaagtcccacgctgagccagcccccaggcctgcatggcatccagctctgcatggcagtccctgtaaatatgcgagtgacctgtgcccgcaggcctctgggccggtctgggtggccacttcctgttacctgtgcctatgccagcactctccgagtttctcctcagactgaactcctcagaccctgtctttgtttatctatcataaaggcagtgctctgcagccacgagaagcctgttaaagagagtgggtcacagtgcccccaggaaacagatgaacaaacagggcatcaacccctgccctcaaggagtctctgttctggtgaagcaagtgtgaacaggaaattccagggtgatgtgcaaagcgctaagacatggccagccagcctctgctggctcttctctgctttccttccctgaaagcaaaagaagacaagcctcatgtgggaagaacttcccaggggtccaaggatcactaggcagaaggctgaatctccagaatgcctcagtcccactcccttgcctgagggtgggtggtccttttactgcagagactggagagaggcagaatgccctgggagaaaagacttctccagcaggcctctctgctgataatcctgaagtgggtggccatcttgctggggtaaggttggggtggggggcaccggagccgctgcaggtagaggtgttgggggctgctcatgtgtttctctctcccacccctctggctgcctcagaaacaaggtcccagattcacccctacccctgccccagtgagttaatgtctccttgaaatggacactgcctgtcctggatccaggccagggggaatatagggcactggtggaggttaacccttgttcaaccacagaggagccaggccagtcctctccttccctcaggcgtgccaaaaagaggaatgccactccgtgtaggtgggagagttccctagctgtctcccctctcgaggactggcccagagtgaggcttgtatccagatgtacactgcctactccccagggcaccaggctctgttttctgcaagggggacctggggacagccacctaacatcatgagaaaagcactgtggaaccctggcatcccagccaggggtccctggcctctagtccccctggtaccagccgccacagaaacagctcggctttcctcaagcactcaggagccaggtttccctggtcttggcttggcatagctgcctcttcttcactccaagaaagccccgcagaggccctccgtgggcaggcttggcagtgcagctggctgaggagggggccagcatggccaccttcagagcaggttaatgggctttgctcagccccaaattgctctgctggaggctggaagcagggagtgatgggcagataggaggtgcctggtgaagggaaggggcacccagcagtgctgtgatgccagcccggtgccctgcttgccgctatgcatgttctctgccaggtcgggggggacagggttgtaagccagggaatatgccagttcccccttgcctggcatggccagctgggcatggtcctggttctggagtcgtgagttcctggtgttccctggggtgggaacagggggaagggttagcctgtgcagctcccgtgggagggacatgtgtgggctgggcctggggagcaggactctgcccctggcaaccagaaccctgaagtgggcagattgtggtcccagagaatcattttccttctccctggggcgttctccaccgtgggcttgcttcctgctttccctgttcacccttctgacctagaggcaggggagatgggttgtggggcccaggatgtgcgaggagcacctcagacccctccctttgcctacactgggcagtcctggatgtggggcatcaccacagctggtaagctaggaagctcgggagagggagccacaaaccccagaaaccaaaaatcaatgtgttctgggatgagggggaggggctgcaagggcaggatgggaggggtgacatggagggagaagtccagggtgcggtccccacagcccgtggcctcctacgcagcttgaggatgcatcctgcctccctccccttgaatgagctcaggcagacctgcccctgcaccccacgctgggcaggagaggtcaagcaacgactacaccagactcctgccttcctcctcgtgggctggggaaggggctgagcaggcaccaccttgagcacaggctctgcgtccctcaccttcctcgcaagcactgtgtttagtccatacatgagatgtatgcttttcatacttcccttaacaaaaggattctgctcatgctaaaggagtttggaaagtaccctgctagtgcacatgggtgtgaggggtgttcctgtgcaaatacgcacacacacgttacacaggagtggactcctgcagggccagaaggcagctgggcatgcatgtgcttgtacacttaagggcacacgtgagtacctatgagcgtacgagtgtgtatctgtatggtaccagtgtgtactagagtgtggtgtgtgtgcctgagtggaggtagggaggctctctgcccagggacccccagctacaaaactccaaagactccaccttttgactccagctgaggcctgctgggataaggaatctccgttctcttggtggggagggctgggtgttgggtttcatgggaaaccttttcattccagcaattaaatagctagaggcctctgctgaggagaagctggaggcctctgctgaggagattaatgaattctcctacctgggcccagggcaaggtgccacttacactgcaggcggcactctgggcttgtggggagagctgctctggagcttggctgagtgtatggggttctgcatggggtgtatggggtgctgagccatccaggcctccctggggagtgctcctgaggtgtggggatggggaggagcaccctgcttgcaaggaagtgccagccgctctctggagcctggagctgaggcacctgatggggaggtggaggcagcatctggagccctgaggccaggcagcggcctgccagctccctagggtcttattagctgcagcggctgcggctgcagcatctggggcagggctgggaggcctggattgctcagcacttccccagtcagctcgggccctgtggccctctcccactcccgctgccgggctcaggaccccacccaggttgcaagccccggagtccagcccaaccaggattggacaagagtaaacaacactccccttctctgtgaggggccacagctcagaggccaacaggggccaggcccgctggtttttttgaggctcccagtatattgaaaaatgaagaaattccaggacaaggctataaaaattatataaataatcttaaattatttaaaatgtttcatttttgacaatggagttcatggtcatgctttaaaatatttaactgttgctagaagatgcgtaatgaaaagcagtgctccttgctccgcctctcccacctccccagcactctggactccttttgtcatttacctccctaattataaacaatatattgtttatactgccctctcccctccccttctccctccctccctcccttccctgcctccctccctttctctttctttcttcttcttttttttcttttttcatgagacagcgtctcactctgtcacccaggctggagtgcagtagtgtgatcacagctcagtgcagcctctgcctcccaggctcaggtgatcctcccatctcagcctcccaaggagctaggactacaggtggtgccaccatgcctggctaatttttgtatttttttttgtagagatggggtcttgccatgttgctcaggctggtctcgaactcctgagctcaagtgatccacctactttggcctcccaaagtgctgggattacagacgtgagccccccggcataaacaatatacttctgcaatgatttcttggttaattaccttcccctccttgtgccccctcagcctagtactctatgcatttgtctagcaaatatttatgtgccaggtgctgcctggggagtggggaaccagcagtgaacaaagcaggcagggacctggctgatggggcttctgttcgaggtgcaggaggtgctcaacaggcacttggacgggcagtggatagagccatagcagctgttacctcagatgggctgtcagggtgggcttttctaaggaggtgacatttgagcagcagcctgagtgaagggagggagaaagctttggggctctctggaggatcctggagaacgttccggggaaggccattggcgaagggtggagcaaatgagttcaaagagaagtctggggccattggattccctgctacctacgatggaaagccactggaagattttgaactaaagagtgtcaggacctgagtaacacttcacagggtgactttagctgccataggtgaggtggacaatagagcctggcaaccggggagcagcaaagaggcagtagggggctgccagtgagagatgggggggcaacagctgcaaggtagtggaaactgggcggcttctaggtctgttttggaggcagagcctacaagtttttctgatgggttagatgtggagggtgcgggaaaaagaagagatgtagacagttttaaagttggtttttttttccacctgaaaatgcagtaaatccaggtgatgtttactgtttatgggggcaggtgcagctgtccaggaatgcagaaaacaaggaaaagttaagaaagtcacttccagaatgaagaaggcaagagaaagggcaggagacgtcatggaaagccaggctgtcccattttgtttcatgaattcaatgatctttttatatttttcctgaggatgtaaattactgttttcccccaaagagttttcttttattccctgcatcaagagaatttcctctgggttcttagcatctaatttgtttttttttttttttttttttttttttttgatacggagtctcgctctgtcccccgcgctagagtgcagtggcgcaatctcggctcactgcaagctccgcctcccgggttcacaccattctcctgcctcagcctcccgagtagctgtgactacaggcgcccgccaccacgcccagctaattttttgtatttttagtagagacggggtttcaccgtgttagccaggatggtctcgatctcctgacctcgtgatccgcccacctcggcctcccaaagagctgggattacaggcgtgagccactgcacccagccgtcttagcatctaatttgtatgttttggtttatttcacatgggaagctttcatcaagtgtccagtttctcctggctgttgggtcatatttaagaatggggctggggagctcagggatgtgtgggtgctactgtaaggtgatcaggtggcaggctggcctgttcattgtagggtcaccagatgtctgtattctgaggtctttgggacaacttcctactcgggtagatagggtggtggtggtgtgacctggctgccagtggttcaggacccaggtagggaaggggctggggtttcacggatcactggctttcagcaccatacctcatcctctgctgtggccaatgctcctgagtccagagcatctcatgcccaatttctacaaagaataaacccctggtgtcctgtggtgaggaaggggggcatctcccagcttaatgaggctgggaaggggaccaggggatcctgaattgtaaccagcctccctgcactcagctctagcttcacctccacctctgccatccccattgcctgcaggtcctacctacacctttcaggggggctgggggtcacctggcttgctccttatgtggacgtttccctctgtggctgctttagtttcagcttcctctgctcccctaagtcagttgtgaggccccagccactttccatgttctaaagttgtgttgaagtttctcatctgctgacatctcttctctttattcttgtgggttttaaatattttactgacttttttttttttttttttttgagacagggtctggctttgttgcctaggctggagtgcagtgggatgatctctgctcactgcaacctctggctccctggctcaagggatcctcccacctcagcctcccagtagctgggacgataggcatgcaccaccacgcctggctaattttagtatttttttgtagcacagagtttcaccacattgcccacgctggtttcaaactcctgggctcaagtgatctgcccacctcggcctcccaaagcttacaggcatgagccactgcgcccagcctgacattctttttttttttttttgagacagagtctctctctgtcacccaggctggagtgcagtggtgcgatctctgttcactgcaacctccacctcccaggttcaagcgattcttgtgcctcagcctccctagtagctgggattacaggaatcccccaccacgcccagctaatttttgtatttttagtagagatggggtttcaccatgttggccaggctggtctcaaactcctgacctctggtgacctgcccgcctcggcctcccaaagtgctgggattacaggcatgagccactgtgcctggcctcctgacattcttatacatttaacattttttggcactcttcaatcctttgtacagattcaagtttctatctgggatcattttctttccacctgaagaactccctttaacatttcctgcacatctggcaataaattcccttagaatttgtttgtctgccaacatatttatttcttcttcagttttgaagaatattttcaccgggtatggaattctaggtcaataccagtcatactggattagagaaaaaaaaaaaaagaattctaggttgaaagtttttgtttttgtttttttcccccagcactttaaagatttcattatattgtttcctggcttacatagtttctgatgagaagaatatagtatttcctgtatctgttcttccatacataatggacctcatttctttgaatgcttttaggattttctttttaccactagttttcagcatttgattatgatggaccttggtgtagtttacttcgtgtttgtcttacttggggttcattgaatttcttggttcttggctttatcttggtattagtttccacaacaaattactacaaactaggtgggttaaaacaacaaatatttggccgggtgtggtggctcacgcctgtaatcccagcattttgggaggccgaggcgggcggatcacgaggtcaggagatcgagaccatgctggctaacacggtgaaaccccgtctctactaaaaatacaaaaaattagccgggcgtggtggtgggtgcctgtaatcccagctacttgggaggctgaggcaggagaatggcgtgaaccggggaagcggagcttacagtgagctgagatcacgccactgcactccagcctgggcgacagagtgagattccatctcaaaaaaaaaaaaaaaaaatttattctgtcacagttcgggagacataaatacaaatttgagatgttggcagggtggcagtccttccaaaggctctagggaagagtcctgccttgtctctttcagattctggtgactgggccacaaccctcttggcttgtggctgcagaactctagtctctgcctccgtcttcacatggccttcccacctctctgagtgtcttagaaagacacctgtcattggatttagggccccctgggtgatccaggattatttcatcttgagatccttaacttaattatgtctgcaaagacccttttttgaaataaggtctcattcataggctgtgagggtcagaatgtgatgtggacatgtcttaggaggggcaccattcttcaacccaccatagtagtttttatcaagtttggaaaaattttggacgttctttctttcttttattatttatttacttattttgaaatggagtctccctctgtcgcccaagctggagtgcagtgacacgatctcggctcattgcaacctccccttcccgggttcaagcgattctcctgcctcagcccccaagtagctgggactacaggtgcccaccaccacgcctggctaatttttgtatttttagtaaaaatggggtttcaccatattggccaggctggtctcaaactcctgatgttgtgatccacccgccttggcctcccaaagtactgggattacaggcgtgagccaccgcacccggcctatttctctaaatttgtcttatttgtcctacttctttattctgtcctttgggattccaatagatatatgttacaatgcttgataatgtcttacagattatgaggctccatagagacagggtcttgctctgttgcccaggctggagtgcagtggcgtgatcatagctcactgcagcctcgaactcctgggctcaagggatcctcctgcctcagcttcagaggagctgggactacagctgcttgccaccatgcccagctaatgtaaaagttgttttgttttgttttgttttgtttgtagagacagagtcttgctgtattgcctgggctggtcttaaactcctgaactcaagccaacctcccgccttggcctccaaaagtgctgggactatagaagcccagccaactttatttttcagtactgtttttctcctctgtgcttcagtttggaaagttctattgctgtcttcaaattcactgatttttaaattgtgcagtgtctaatctgctgttatttccattcagtgaatttttcatttcagttactgtacttactatctttagatggtccactgggttcttttttatacctctcattcctctcctcatgaacatctttttcatgtttttctttaaactcttgagtatattgagccatctatcatctttatcatttctgagttttgtttctatgaaattatttttctcctgattataggttatattttctttcttttttttttttttttgagatggagtctctctctctgttgcccaggctggagtgcaggggcgccatctcggctcactgcaagctcgatctcctgacctcgtgatccacccgcctcagcctcccaaaatgctgggattacaggctcacgtgagccaccgcaccctgcctataagttttattttcctactttttggcatatctagtaatttttaactgaattttggacattgtaaatatgatgttaagcatctggatttgttattgttctttaaagagtgttgggctttgttcaggcagactaggtaaattacttgcaaatcagtttgacctttttgaggcttttttttttgagacagagtcttgctctgtcacccaggcttgagtgcagtggggcaatctcagctcattgcagcctcaacctcctgggcttaagggatcctcctgcctcagtcactgagtagctgaggctacaggcacatgctaccatacctggctaattttttgtattttttgtagacatggggttttggtatgttgcccaggctggtcttgaactcctaggctcaagtgatctgcctgcctcagcctcccaaagtgctgggattagaggtgtgagccaccgtgcctggcctttgatgctaatttttctttttctttttcttttcttttcttttttttttttgagatggagtcttgctctgtcacccaggccagagtgtagtggtgcagtcttggctcactgcaacctccgcctcctgggttcaagtgattcttgtgcctcagcctcctgagtagctgggattacaggcacccatcaccaagcccggctaattttttgtatttttagtagagatgtggtttcgccattttggccaggctggtcttgaactcctgacctcaggtgatctgcccgcctccgcctcccaaagtgctgggattacaggcatgagccactgcacccggcctgaggctaatttttaatctgttagggtgggtctaggtgagccttttctctagggatagtttagctctactgctaaggcataacccttctgaggtctgattaaatatgcatctccactctaggaggctggagcttgattatctccttgcttttggtgagctctgagaatttaccattttattgctcctttttgtgtggtcttactgagtttcactatacacatgtgaagtttagtattcaggaagacttgaagagacccctatgcagatttctggagttttttgagtagtttactcttttccagaactgtgctctgctgcaacctttaataccttggcttccctgaatcctgtctccatcttctcaactcaggaagagcaccatgctctgctcgggcttcccctccttgaattacagtctggaatgttcctccaggcagaaatccagggatgttacagagctcaccttgttcattttccttacttcagggatcacagttctggacttctaaaaacagctatttctctttacatatattttctatatagagaaatatatatatatacacacacaaacacacacacacacacacatacacacacacatatatatatacacacacacgcatatgtatatatatatttgagacagcgtctcactctgttgcccagcctggagtgcagaggtgtgatgatacctcactgcagcctcaacctcccaggcttaagcgatcctcccacctcagcctctgagtagctgggactacaggcacaggccatcatacccggctaattcttttgtattttttgtagagatggggttttgccatattgcccaggctgatctctaactcctgggctcaagcaatccgccaacctttgcctcccaaattgctgggattacaggggtgagcctctgtgcccagccttcatatattttgcagcaataattttctcattgtttatggtggcagagtaatttcatttattatggtaggagtagaagcctttttactggcgttttaatcaagttcagagaagaggagggagttacatgcatgtggtcagttcactgttccttttttttttgagacggagttttgctcttgtcgcccaggctggagtgcagtggcatgatctcggctcactgcaacctccgcctcccgggttcaagcggttctcttgcctcagcctcctgattagctgggattacaggcatgggccaccacgcctggctaattttgtatttttagtagagatggggtttctccatgttgtcaggctggtctcgaactcccaacctcaggtgatctacccgcctcggcctcccaaagtgctgggattacaggcgtgagctaccgcgcctggcctgtcagttcactgttcttaaccagaagtcctagactctcgaaatatatttaaatacttatgcttaagaccgggcgtggtggctcacgcctgtaatcccaacactttgggaggccaaggcaggcgaatcacttgaggtcaggagttagagaccagcctgggcaacatatcaaaaccccgtctctactaaaatacaaaaattagcctggcatagtggtgctcgcctgtaatcccagctactcagaaggctgaggcacaagaatcgcttgaacctgggaggcggaagttgcaatgagccaagatggcaccactgcactctagcctgggtgacacagtgagactctgtctcaaaaaacaaacaaacaaacaaacaaacaaaacttacgtttaacaaacatgctttctaagccaggtgcaggggcttgtaatcccagctgcttgggaggctgaaacaggaggattgctcaagcctaggagtttgagaccagcctgggtgacatagtgagaccctgtctcaagtaaaaaaaaaaaaaaaaaaaaaaaaaaaaaaaatcttttgtctgggcactgcggctcacacctgtaatcccagcactttgggagcccgagccaggtggatcacctgaggtcaggagttcaagactagcctggccaacatggtgaaaacccatctctactaaaaatacaaaaaattagccagacgtgttggcgaatgtctgtaatcccagctacttgggaggctgaggcaggagaatcgcttgaacctgggagacggaggttacagcgagctgatatcacgtcattgtactccagcctagccaacagagtgagactccgtccccccaaaaaaaacacaaaaaaaaaccccaaaaaaagcttttatcacttttatcacacaacagaaatctcatgcaatgtaatcatgttattcacaaaattataggatttgtacaaattttaatgcatagtgtcccacaagcacaggacatggttgtgaaattgtattaataccatgaacttgttatttcattcctgtctgtgtattactgtaaccgtttgttaaacctcactcagtgataatgtcagtgatctaaattggtagctcttcctgaaggtggcctgggacccttagggtaggtctggtcccaggtgagctccttggccaacagcctctttgccaccccacttcagtcccaggcttattcttggcaggcaggccactgggccctggaggagaggacccagccaggggcccttggtggacaggaagggaggaagccctccctcttccagagttactttctgtcctgtcttctaagcccctttccatccacgtgtctgtctttccgttgctcatagtgtctgtctttccgttgcccatagtgtctgtctttccgttgccttgtgaggttggtgaggcagagcagccccagcagggggtgggggttgctgcctgctccagggctgtctggctccggagggctgcctccgacgtgactggggctttatcttccactcctcctcctcctccaggtggacatcgagcagctggatccccgcggccggactcccctgcacctggccaccacgctggggcaccttgagtgtgcccgtgtgctcctggcgcacggcgcagacgtgggcagggagaatcgcagcggctggacaggtgggcagccctgctcaccccagccccacagccggggcctccccagcatcatagacctatggttggctgaagggtcctgccctgtgaccttgcctcgccctcccccagtgctccaggaggctgtgagtacccgggacctggagctggtgcagctggtgcttcggtaccgggactaccagcgggtggtgaagcggctggcgggcatccccgtgctcctggagaagctgcgcaaggtgaggcccagcctctcagcctccacgggagcccttgagcccttctccagtgcagacttagcctctctccccttcgtcctccaggcccaggacttctacgtggagatgaaatgggagttcactagctggggtaagcgggctgcagcaggtcgcttctgggctctcccactttaggtcctgcgcttgctcccctgcctggaatgtgttctcatagttcttccggcggttccctctatgccttagctcagctcagggccaccgcctcagctaggcctttccagattgccccagatactgtcttgactccattattattctcttcactctgtcatgatttgcttactgtattcatgacctgccgctccttgttagaaggtaagctctgagagggcaggagtcctgtctttttcactgttgtattcccagtggctggaacactcagtaggtgtttcataaatatttgttgaaagaatggatgaaagagtgagtgagtgaattaacaaatgatggacactagggacttagtggtgacagaaacatgcccgtcccgacctcaggttgctcttctgtgtgagtatggtctacactggccagggagggggttttggaggagaggctgctctctcttcagttccctcccctgttcctggccacacggatcccaaaccccatgccctgagctggtccaggccgtgtaggccagaccagtcaaagccacctccaacctccgcttccaccagtgcccctggtgtccaagatctgccctagtgacacctacaaagtgtggaagagcggccagaacctgagggtagacaccacactcctgggctttgaccacatgacctggcagcgagggaaccgcagctttgtcttcaggggccaaggtcaggcaggcaggaagtggggcagggtggggacgatgggaggcagccccaggccacccctgatccccctgtgctgttccgtgtctggcagacacaagcgccgtggtcatggagattgaccacgaccgccgggtggtgtacacagagactctggcactggctgggcaggaccgggagctgctgctggctgctgctcagcccactgaggaacaggtgctgagccggcttaccgcgcccgtcgtcaccactcagcttgacaccaagaatatctcctttgagaggtgggtggacatggccttggtcacccttgagccagcccggtggggtgcctgcctcacctggaccactctgcttccccaggaacaagactggcatcctgggctggcgcagtgaaaagacggagatggtgaatgggtatgaagctaaggtgaggctgcagctcccagctgccagcccagctgcactcttgcctacagcaagctgtacaggggattctgacctcccttccccagccctggaggtacagaagcaatgcagcgtggtcaagcacttatatttgggttcaaggcacttctctggtgttttatatggatgtatggatgtatacacagggcacgtgcacacgcacacacacacacacatttattcctcacagcaaccctttctggtaggtgctgttctgttagtattcccattttacgcatgtttattgagtcctttccttggcatcccatttactcttcacaacaaccccaggaagtagggatgatcggtccattttatgatgaggaaatagaggcttagagtggttctgtgacctgtacaaggtcacacagctgttaagtggcagagttggggttcagatcctggctggcctgaccctagagccaggcctttatccctaaaaatgactgcctggctgggcatggtggctcatgcctgtaatcccagcgctttgggaggccgaggtgagcggatcacctgaggtcagttcgagaccagcctggctaacatggtgaaaccccgtctctactaacaatacaaaaaattagccgggtgtggtagcaggcgcctgtaatcccagctactcgggaggctgaggcaggagaattgcttgaacctgggaggcggagcttgcagtgtgcagcgatcccgccacagcactccagcctgggcaacagagcgagactccatctaaaaaaaaaaaaaaaaaaaggctctgcctgttactctgggacccctatgttgcccacgacatgaaagcaggaactaacaaatgccatgggttttgtgtgtggcatctcctctgaaagcctcccctgcttctgtagtctgggaaggcctctgtgctacccccaccagtgcatggaccatgctgttataactccattttattgtctccttatagagattgtaagtctcaggagggcagggatcatgtttggcttgtttactgtatccctgatgcctacctcaatgcctggcacataaaggctcctcaaaaaatgtttgttgaatgaataagtgaatgaatgaatgaatgaatgacctcatatattcacttacccaaaagcctgaagcagagtctctccaggaccctttgctacagggagtgttcccagtgcccttaggggtaagacacagggtaagaccagaactgcttatgagccctttcttcatctgtccccaggtgtatggggcatctaacgtggagctcatcacccgcacacggacagaacatctttcagaacagcacaagggcaaggtcaaaggtaatgaggcagagctggatggggagaggtgttgcaggactgcgggaaccagctcccacttcagtgcttccatcagtattcccactggcatcctagcaagaggctggatgctttattcaggccgatagatttcaattcaggtgccaagccctaaggatgggtagtggctgcctagagtactaagaagtttctaaggactcatctgggttcagtggagagccatgctgcaagtgattactaatgttgctgttgaatttgggagaggagagaaatgccatgtatgccatttattggccattctagtctagtgggacatatcctaggtagaaagtcaggggaccttgccacagattctgtatgcccattgatgccacacctgattctctgggtaccagataccgtgtccgaggtgaaaaagcataatttctacctcacaggggaacaacatgaaatcatgcctatggaagtgcctgaagcaaacacacacacgcacatgcacaccccacagtgcctgccggggcaggcgttttactgtccagggtcaccgagctggagaggagcacttttggaagttgcttctgacctctaggccttccttttagtgttttaagctgtgctcacagaggccctggcccctggtccttgaagcactcagtccccttcaggtgaaggtgcctgagtatgtggttgggtgagcaggccccaccccaggaaccggcctcctccctaggtcttgggtgctgtcacctctgatgaggtgcccaggtgtgtgtggagttgcggtgtcctctgagatgccacatttcttgtaggctgtaagacacctttgcagtccttcctgggaatcgctgagcagcacgggggcccccaaaatggggtgagtgtgtgcaggggtacccgtaagtggagggatgtggatgtggctcaggaggaggcttgggaagcgtcctgcttagcatggcctatgtggacctcctttccacaatgcccaaggccatgtcagcgccacactggcagaggggacagcttgggggccttgtgacaacaaatgagttggcctggcattaggaactgaggggagctcctgggcccctccccatgtggtacagaccctgatcactcagactctgagccaagccaaccccactgccatcactgcagaagaatacttcaaccccaactttgagctgggcaaccgtgatatgggccgccccatggaactgaccaccaagacacagaagtgaggcccctgccggtgctgggaaggtggggggccggggctccaggagatgctgggaggccatggcttcctgcagtgtcccttaccccttgggatctggtgggggcaggttcaaggccaagctgtggctgtgtgaggagcatcccctgtccctgtgtgagcaggtggcccccatcattgacctcatggccgtcagcaatgcgctttttgccaagctccgggacttcatcaccctgcgtctgcctcctggcttcccagttaagattggtgagaccgcacggccatttctcctgagcccgtggcgggccgaccggggtttagatgaggtcggggtggggctgaggctgaggtgtgaggggctgagtggtggcgcctaaaggtttcctcatcctcagaaatcccgatcttccacatcctcaacgcccgcatcaccttcgggaacctcaacggctgcgacgaaccggtgccatcggtgcgaggcagccccagcagcgagacgccttccccaggcagcgactcctccagcgtcagcagctccagctccacgagtgaggccccccgcgagaacgcctgcccctcggctctccccggggtgggtgggaggggcgcgcccggccgtgcctgacccagcccccgcgcccccagcctcctgccgcggctgcgagatctccccagcgttgttcgaggccccgcgcggctacagcatgatgggcggccagcgggaggcggcgacccgggacgacgacgacgacctgctgcaattcgccatccagcagagcctgcttgaggcgggcagtgagtatgaccaggtgcgtctccgcgggcgcgcggggccacgggactccgcgccgccacggctaacgcccacgcctccccgcaggtcaccatctgggaggcgctaaccaacagcaagccaggcacccaccccatgtcctacgagggtcgccgacaggacaggtcagtgcccgctgggccggagagaatcctccggagaggatcctgtctcccctaagccaggacacagccggagaacccgcggggccctcggcagggaccctcctggtatcgggatggcttctgccaccactcctgcctccgaggcggcaggcaggggtcagggatccaggcttcaccgcggagttcagactctccccaggcattgacggggagaacttggtagggtctgggctccgccacgaccaggtgggggccaggacgccgcgggactgaccgcctccactagagggtggtggccgcgggccgccctggagcctccacgccgtgtcccggccccggccggtgggtgggtgcgcccgggagcccgcgacattccttccccacccccaggagcgccccgcccacgccgcagcgccagcctgcgcccccggcgtcagtgcccagccctcggcccagctcagggccaggttccggcggccacgtgttccggagctacgacgagcagctgcggctggcgatggaactgtcggcgcaggagcaggaggagaggcggcggcgcgcgcgccaggaggaggaggagctggagcgcatcctgaggctctcactgaccgagcagtagcgccccctgccgggaccctcgccagcgccacgcgcgccacgcccagggccaggagccagacaaaccccggcctgcgcgcctgcagagcggcggctggagactggagccaccgcctcgcgggtgcagcagcacagcaggcacggttcggggagggattcggcatggccgcggggtaccttcccaggccagggccctggaggcaactggcacggcctggtccccctgctttgctgtattctgattccccaacccgctcccctgggctcagatctgtcctgtcctagggcggagccaggcggtcctgagggggagatgaatccttagaggagcgctgtccctatcccttgctccttctggccggtccgcatttctgttcactaaccccactccaggacactgcccctgaagcctttgcatctctgctcttcactcctggggggcagctgagctccccgcgtgctgtgtcactgctttgttccagacacaaaccagcacgtctagggcccagcccctcccccaccccggcatttcagcgtcaagtgcacttagcggggtacccggctcccccagcccccacacccgtcctgggtctcagggtggttccagcttctccttgggcagccagaagttggagtcccatcccccaaggcacatttttttttttttttttttgtgatcagggagtgtgtccaacgtagccccctggcctgtgcaagccctgactccctcatggtgcctcggagagtggggagcatattgggctggggtaagcactagacccaagtagactggacacaaagggctcgcccagggccctggcgccacccccaccccttcccaccagctgctgctagcctctgtggttgtacatcccacttgcccccacacggagactgactctaaaacccttcatccaatggtgctaacccccggctctcccctgccccacctcacccacccagagaagcacagaccccgccaggggcaggggcccaccgcacacccttgtcccgggcctgtctgggactggccttcccggctcagccagtgaggctcagaagggacacaaagagggatggaagaaaagaacaaagagaaactgttcctcccacccccttccctgatgccaggggcaccagactgattctgaggcacaaataaaagaggcttcataccgga

SEQ ID NO: 7 - DNA, 24993 bp, Artificial Sequence
  C to T (bis1)
gtttaaaggggtcgcggtagatgttcggtttcggcgggtagcgtggtttgcggttttggttttcgttgtagcgttcgtttggttcggaggtaatgtgagttatttttatagtttttttttttttatttttcgcgtggggtggatcgggggacgttgggtttacggacggcgagggtggggattagggaagaaggatttggaggtttaagtttcgttttaggttaaaggggttgtgttttggggtattcgtttatttttggttggggtgaggtgtgcgtttttgtttcgtaggtgtttatatttgtgtgtttaggggtgtgtgtgtatgtgttatatttttgttgaatacgtttattgttaataatatggacgtttaggtgttagaaaggttaggtagtgtatttttttgttttcggattaaaaatatatttatttttttatgtatttttttatttagagaggagagaatttgggcggtttttaaagatttttcgaggagtgattattgtgtttgtgtgtatttatatttatttgttattcgttttatatatatttacggtgtttttgggttattagaggtgtgtgtgtttagaaagggtgtatataatatagaggggtcgttttaggtgacggtttttttttttggattttatacgacgaggtaggtaaaggtaaggtaggtgagggacgtgggtgggttggggggtagggagtttaggtagaggtcgtatatgagcgtagttttcgtattgagtatgcgtttttatacgcgtgtgtcgcgcgtgtatttaatttttaatttttgtagtagtaaaaggttcgggtattttgtttgtggggagagggtagaggtttttagggttagatttgggggttaggttagtggtgataattgaggaggggttttttaagagttagagatttttgtttgttaagatgggggtagttttttggtaggggtgtttaagttggtcgattattttaacggtgttagagcggtagtgatttgtgggtgggtaggttttttttttaggggagataagtaatgtttatgagttatattattcgaaatatatgtaaagttgtttttatcgttttttgttgcggtttagattgataagtttgtttgaaatcgcgatttatgggttttatttataattgtattttaaaaaaattttgtaggttttttttttttcgatagttagtcgtttagttggtggggtttttgtaagtaacgatatttagttggtgtgtaggggggagtattatttgtcgtttcgagttgtttttttattagagtttatgggtttggtggttttagcgggaagggggtaaggggcggggggagtgagacgggaggagtggttaggtagttcgtgttaggcgtttagtttacgagcggtggtcgttcgtttattttcgatcgatttttagttatggaattttatttattaaatgtcgaggaggttgttggtagttttgtcgtttggttgtttttgttttttcgttgtgtgggcgcgtttcgagtacgtggtagttgagagcgcgggtcgaagcgtaagcgatttgggtttagtgtttatcgtcgtttggtaaaaaaagaatacggtcgtttaggggatagttttttataatcgataattttttataatttattttgaattttttttgttttcggatttttgggttttgttggggaagaaggatgatttattttgtttatttttttattttattttttattttttggttggtttagagattatttgggagtggttttggcgcggatatatcgtttaaattttgttttttttagtttcgttatagttaaatttttgggtttgggattggagataaaagggtttttggattttttcgtggagatgttattattttaggaagtaggattgttatagtggaattatatataaggttcgaaaaataatttaataaggaaatgtataggtatgttttcggttatttttagatgttttttaatcgcgttagtttttttttttgtattggttgtagttacgatattttgttgatttttggtggtgtaggcgggtagcggtttcgggttttcggagacgttagttggttttttttaggcgggagaaaggggcgaggtagttcgttttttttttattttttttcgttggggtttggtattatagggtgtggaggaggaaggagggaagattatataaagaaatttgagagagtttgtaagtttttgttggtattttttatataaatattttttggattgttgttttaagtagggtcggtgtggaattttttatttttgttttgttttgaggtgggtttaagaaggtatcgtgtttggtttcgttatttgtttcggttcgtttggttgggggagggaggcgttgtttttagggtagttattatttttagtttattttaggaggtagtatttagatttttattttgaaggggagtggatcgagaaagtcggaaaaattaagtagtttgtttttttaaggttaggtagttggagttattcgaattttggtttttttgatattatagttttttttttttagggattggtttaagttttttggtttttttaggttttgtaattggcgtttgagaggttaatttaatttttattatattttttgtagggattattttggaagtatttttttattttggggttatttaggaaggagatagtttttggaattagttatttttttttttgaagggttagttgggtggaggaacggagttgttatttgttgttttttttgtttaattttattttggtttttgttggggatagtgtgcggggggaaagggattatttttttcgcgttattggatattttgtttttaatgatatgtgtggaagatggagtttaattttttaatagggtagggaagattttttagaaatgttttaggggttagatttttggttgttttaatgatttttggtattgatgttttatattttttttaggagtttttaattagacgtttttttttgggaattcggatttttttttatggtttttgggatttaagtttaattttgaagattatatttttatttcgttttttaaacgttcgatttaggttcgtgtttttttatttttttagtaaaaggtaaaatgttagcgggggaggtgcgttttagtttatttggcgttagggtttcgttcgcgtttgggttaggtttgatttttcgtttatttttttacgagattcggggatagtgtagatttttttcggttatttgttatttttagttttacgaggcggattataaattttatgatgtcgcggggttgagttgataagttttattcggggcgtttggttttttttttttttttttattatttttatattttcgtatttcgcgtcggtcgttcgggttgagggtcgggttatgtagttgtggggattcgggggttgcgggcgcgcgtttttgcggcggcgttttcggggttcgcgtttcgtgcgttttcgcgttcgttgcgggcgtttgtttttttcgtcgagcggcgtttttgtgtgcgggggtgtgggaggcgagcgcgagttcgcgtagcgtcgtcgagtgttcgtttttttttagggcgggtgggggttttttcgcgtcgttcgtcgtcgtcgtttcgcgaggacgttcgtcgttcgcgtcgttcgtatcgcgtcgggcgcgtcgttttcgttcgtcgtcgttcgtatatgttcgagtcgtagtttcgcgagtaggtagcgtcggtttttcgtttcgcggtttcgggtttcggtttcggcgtcgtttttttttttcggtcgggcgtcgcggtttcggtatgaggagcgggcgatgattttcgttaacgttttcgttaggaaggggttcgagggtaagtattcgttgtattatttcgtgtggtataatcgttatcgcgagttggagaaggaggttcgcgcgggttaggtaggagcgttttcggggcgtcgcggggatttcgcggtcgggtacgttcgttcggtttggggagggggtgcggcgcgggttgtttcgtttttttggcgagtttgcggcgcgtttttgtttgcggtcgcggtttttgtgtttgttgatcgggaaagggtgatttttttcggtcgggacgggcgggattatacgtgtttcggatttatttagatgagagtagaggtttttgtgtttttttttcgtcggggtagtgagggttgtagggaggggttgcgggttgtgtcggtgttttatgtggtgggagagttcgttttagttagttgagcggcgatatttttcgagtgagggtgcggaggtgggaaaggtttgcgtggggagggggttataggttaagaatggggaagaggttgtgttatatttttaggtattttagttttatttagcgttttttttttaacggtgagcgtttttttttttagtttttaaattgggtagatttttggattttttagagtttagttttagtttaggaatagggagtggagaaagatttttttgggaggttttaagggttttgtttaggtgttgaaaagcgtttttttgttttttggtgttggggtttggtttttaggcgtagaggaagttgaggggttttggttgttggaaggatttgaggttttgcgtattaggtgggttttttggtttttgttggttagtaaggttacgtgggttattagttttgggttgggtagtggtttttagaaaataggggaaggggggatgttttttggttatgttttaggatgttttttggttatgttttagaataaaggtaggtataggttatagattgttatttttgtttttggtatttaggttataggtaggtatttatggtagagatgatttttcgtttttagggtgggttgtaagagttagagttgggttcgggttttatggtttgttgtaggttgagaattttagttttggattgggtttgagattttggggttatgggttgggggtggttagcgtagttgttcgttgtgggaatttattttttgagggttgtttattgagttatgagaagtttagtttgaggagttgtgtaatcgttaagggaagtatggaggtggagggtaggttatcggattgagtaggttgggggttaggatgtgtttttgaagttttacgttgagttagtttttaggtttgtatggtatttagttttgtatggtagtttttgtaaatatgcgagtgatttgtgttcgtaggtttttgggtcggtttgggtggttattttttgttatttgtgtttatgttagtatttttcgagtttttttttagattgaattttttagattttgtttttgtttatttattataaaggtagtgttttgtagttacgagaagtttgttaaagagagtgggttatagtgtttttaggaaatagatgaataaatagggtattaatttttgtttttaaggagtttttgttttggtgaagtaagtgtgaataggaaattttagggtgatgtgtaaagcgttaagatatggttagttagtttttgttggtttttttttgttttttttttttgaaagtaaaagaagataagttttatgtgggaagaattttttaggggtttaaggattattaggtagaaggttgaatttttagaatgttttagttttatttttttgtttgagggtgggtggtttttttattgtagagattggagagaggtagaatgttttgggagaaaagatttttttagtaggtttttttgttgataattttgaagtgggtggttattttgttggggtaaggttggggtggggggtatcggagtcgttgtaggtagaggtgttgggggttgtttatgtgttttttttttttatttttttggttgttttagaaataaggttttagatttatttttatttttgttttagtgagttaatgtttttttgaaatggatattgtttgttttggatttaggttagggggaatatagggtattggtggaggttaatttttgtttaattatagaggagttaggttagtttttttttttttttaggcgtgttaaaaagaggaatgttatttcgtgtaggtgggagagttttttagttgttttttttttcgaggattggtttagagtgaggtttgtatttagatgtatattgtttattttttagggtattaggttttgttttttgtaagggggatttggggatagttatttaatattatgagaaaagtattgtggaattttggtattttagttaggggtttttggtttttagtttttttggtattagtcgttatagaaatagttcggttttttttaagtatttaggagttaggtttttttggttttggtttggtatagttgttttttttttattttaagaaagtttcgtagaggtttttcgtgggtaggtttggtagtgtagttggttgaggagggggttagtatggttatttttagagtaggttaatgggttttgtttagttttaaattgttttgttggaggttggaagtagggagtgatgggtagataggaggtgtttggtgaagggaaggggtatttagtagtgttgtgatgttagttcggtgttttgtttgtcgttatgtatgttttttgttaggtcgggggggatagggttgtaagttagggaatatgttagtttttttttgtttggtatggttagttgggtatggttttggttttggagtcgtgagtttttggtgttttttggggtgggaatagggggaagggttagtttgtgtagttttcgtgggagggatatgtgtgggttgggtttggggagtaggattttgtttttggtaattagaattttgaagtgggtagattgtggttttagagaattattttttttttttttggggcgttttttatcgtgggtttgttttttgttttttttgtttatttttttgatttagaggtaggggagatgggttgtggggtttaggatgtgcgaggagtattttagatttttttttttgtttatattgggtagttttggatgtggggtattattatagttggtaagttaggaagttcgggagagggagttataaattttagaaattaaaaattaatgtgttttgggatgagggggaggggttgtaagggtaggatgggaggggtgatatggagggagaagtttagggtgcggtttttatagttcgtggttttttacgtagtttgaggatgtattttgtttttttttttttgaatgagtttaggtagatttgtttttgtattttacgttgggtaggagaggttaagtaacgattatattagatttttgttttttttttcgtgggttggggaaggggttgagtaggtattattttgagtataggttttgcgttttttatttttttcgtaagtattgtgtttagtttatatatgagatgtatgttttttatattttttttaataaaaggattttgtttatgttaaaggagtttggaaagtattttgttagtgtatatgggtgtgaggggtgtttttgtgtaaatacgtatatatacgttatataggagtggatttttgtagggttagaaggtagttgggtatgtatgtgtttgtatatttaagggtatacgtgagtatttatgagcgtacgagtgtgtatttgtatggtattagtgtgtattagagtgtggtgtgtgtgtttgagtggaggtagggaggttttttgtttagggatttttagttataaaattttaaagattttattttttgattttagttgaggtttgttgggataaggaattttcgtttttttggtggggagggttgggtgttgggttttatgggaaatttttttattttagtaattaaatagttagaggtttttgttgaggagaagttggaggtttttgttgaggagattaatgaatttttttatttgggtttagggtaaggtgttatttatattgtaggcggtattttgggtttgtggggagagttgttttggagtttggttgagtgtatggggttttgtatggggtgtatggggtgttgagttatttaggtttttttggggagtgtttttgaggtgtggggatggggaggagtattttgtttgtaaggaagtgttagtcgttttttggagtttggagttgaggtatttgatggggaggtggaggtagtatttggagttttgaggttaggtagcggtttgttagttttttagggttttattagttgtagcggttgcggttgtagtatttggggtagggttgggaggtttggattgtttagtatttttttagttagttcgggttttgtggtttttttttattttcgttgtcgggtttaggattttatttaggttgtaagtttcggagtttagtttaattaggattggataagagtaaataatattttttttttttgtgaggggttatagtttagaggttaataggggttaggttcgttggtttttttgaggtttttagtatattgaaaaatgaagaaattttaggataaggttataaaaattatataaataattttaaattatttaaaatgttttatttttgataatggagtttatggttatgttttaaaatatttaattgttgttagaagatgcgtaatgaaaagtagtgttttttgtttcgttttttttatttttttagtattttggattttttttgttatttatttttttaattataaataatatattgtttatattgttttttttttttttttttttttttttttttttttttttttgttttttttttttttttttttttttttttttttttttttttttttttatgagatagcgttttattttgttatttaggttggagtgtagtagtgtgattatagtttagtgtagtttttgttttttaggtttaggtgatttttttattttagttttttaaggagttaggattataggtggtgttattatgtttggttaatttttgtatttttttttgtagagatggggttttgttatgttgtttaggttggtttcgaatttttgagtttaagtgatttatttattttggttttttaaagtgttgggattatagacgtgagtttttcggtataaataatatatttttgtaatgattttttggttaattatttttttttttttgtgtttttttagtttagtattttatgtatttgtttagtaaatatttatgtgttaggtgttgtttggggagtggggaattagtagtgaataaagtaggtagggatttggttgatggggtttttgttcgaggtgtaggaggtgtttaataggtatttggacgggtagtggatagagttatagtagttgttattttagatgggttgttagggtgggtttttttaaggaggtgatatttgagtagtagtttgagtgaagggagggagaaagttttggggttttttggaggattttggagaacgtttcggggaaggttattggcgaagggtggagtaaatgagtttaaagagaagtttggggttattggattttttgttatttacgatggaaagttattggaagattttgaattaaagagtgttaggatttgagtaatattttatagggtgattttagttgttataggtgaggtggataatagagtttggtaatcggggagtagtaaagaggtagtagggggttgttagtgagagatgggggggtaatagttgtaaggtagtggaaattgggcggtttttaggtttgttttggaggtagagtttataagtttttttgatgggttagatgtggagggtgcgggaaaaagaagagatgtagatagttttaaagttggtttttttttttatttgaaaatgtagtaaatttaggtgatgtttattgtttatgggggtaggtgtagttgtttaggaatgtagaaaataaggaaaagttaagaaagttatttttagaatgaagaaggtaagagaaagggtaggagacgttatggaaagttaggttgttttattttgttttatgaatttaatgatttttttatattttttttgaggatgtaaattattgtttttttttaaagagtttttttttattttttgtattaagagaattttttttgggtttttagtatttaatttgtttttttttttttttttttttttttttttgatacggagtttcgttttgtttttcgcgttagagtgtagtggcgtaatttcggtttattgtaagtttcgtttttcgggtttatattatttttttgttttagtttttcgagtagttgtgattataggcgttcgttattacgtttagttaattttttgtatttttagtagagacggggttttatcgtgttagttaggatggtttcgattttttgatttcgtgattcgtttatttcggttttttaaagagttgggattataggcgtgagttattgtatttagtcgttttagtatttaatttgtatgttttggtttattttatatgggaagtttttattaagtgtttagttttttttggttgttgggttatatttaagaatggggttggggagtttagggatgtgtgggtgttattgtaaggtgattaggtggtaggttggtttgtttattgtagggttattagatgtttgtattttgaggtttttgggataattttttattcgggtagatagggtggtggtggtgtgatttggttgttagtggtttaggatttaggtagggaaggggttggggttttacggattattggtttttagtattatattttattttttgttgtggttaatgtttttgagtttagagtattttatgtttaatttttataaagaataaatttttggtgttttgtggtgaggaaggggggtattttttagtttaatgaggttgggaaggggattaggggattttgaattgtaattagtttttttgtatttagttttagttttatttttatttttgttatttttattgtttgtaggttttatttatattttttaggggggttgggggttatttggtttgttttttatgtggacgtttttttttgtggttgttttagttttagttttttttgtttttttaagttagttgtgaggttttagttattttttatgttttaaagttgtgttgaagttttttatttgttgatattttttttttttatttttgtgggttttaaatattttattgatttttttttttttttttttttgagatagggtttggttttgttgtttaggttggagtgtagtgggatgatttttgtttattgtaatttttggttttttggtttaagggatttttttattttagttttttagtagttgggacgataggtatgtattattacgtttggttaattttagtatttttttgtagtatagagttttattatattgtttacgttggttttaaatttttgggtttaagtgatttgtttatttcggttttttaaagtttataggtatgagttattgcgtttagtttgatattttttttttttttttttgagatagagtttttttttgttatttaggttggagtgtagtggtgcgatttttgtttattgtaatttttattttttaggtttaagcgatttttgtgttttagtttttttagtagttgggattataggaattttttattacgtttagttaatttttgtatttttagtagagatggggttttattatgttggttaggttggttttaaatttttgatttttggtgatttgttcgtttcggttttttaaagtgttgggattataggtatgagttattgtgtttggttttttgatatttttatatatttaatattttttggtattttttaattttttgtatagatttaagtttttatttgggattattttttttttatttgaagaattttttttaatattttttgtatatttggtaataaatttttttagaatttgtttgtttgttaatatatttattttttttttagttttgaagaatatttttatcgggtatggaattttaggttaatattagttatattggattagagaaaaaaaaaaaaagaattttaggttgaaagtttttgtttttgttttttttttttagtattttaaagattttattatattgttttttggtttatatagtttttgatgagaagaatatagtattttttgtatttgtttttttatatataatggattttatttttttgaatgtttttaggattttttttttattattagtttttagtatttgattatgatggattttggtgtagtttatttcgtgtttgttttatttggggtttattgaattttttggtttttggttttattttggtattagtttttataataaattattataaattaggtgggttaaaataataaatatttggtcgggtgtggtggtttacgtttgtaattttagtattttgggaggtcgaggcgggcggattacgaggttaggagatcgagattatgttggttaatacggtgaaatttcgtttttattaaaaatataaaaaattagtcgggcgtggtggtgggtgtttgtaattttagttatttgggaggttgaggtaggagaatggcgtgaatcggggaagcggagtttatagtgagttgagattacgttattgtattttagtttgggcgatagagtgagattttattttaaaaaaaaaaaaaaaaaatttattttgttatagttcgggagatataaatataaatttgagatgttggtagggtggtagtttttttaaaggttttagggaagagttttgttttgttttttttagattttggtgattgggttataatttttttggtttgtggttgtagaattttagtttttgttttcgtttttatatggtttttttatttttttgagtgttttagaaagatatttgttattggatttagggttttttgggtgatttaggattattttattttgagatttttaatttaattatgtttgtaaagatttttttttgaaataaggttttatttataggttgtgagggttagaatgtgatgtggatatgttttaggaggggtattattttttaatttattatagtagtttttattaagtttggaaaaattttggacgtttttttttttttttattatttatttatttattttgaaatggagtttttttttgtcgtttaagttggagtgtagtgatacgatttcggtttattgtaatttttttttttcgggtttaagcgatttttttgttttagtttttaagtagttgggattataggtgtttattattacgtttggttaatttttgtatttttagtaaaaatggggttttattatattggttaggttggttttaaatttttgatgttgtgatttattcgttttggttttttaaagtattgggattataggcgtgagttatcgtattcggtttatttttttaaatttgttttatttgttttatttttttattttgttttttgggattttaatagatatatgttataatgtttgataatgttttatagattatgaggttttatagagatagggttttgttttgttgtttaggttggagtgtagtggcgtgattatagtttattgtagtttcgaatttttgggtttaagggatttttttgttttagttttagaggagttgggattatagttgtttgttattatgtttagttaatgtaaaagttgttttgttttgttttgttttgtttgtagagatagagttttgttgtattgtttgggttggttttaaatttttgaatttaagttaatttttcgttttggtttttaaaagtgttgggattatagaagtttagttaattttattttttagtattgttttttttttttgtgttttagtttggaaagttttattgttgtttttaaatttattgatttttaaattgtgtagtgtttaatttgttgttatttttatttagtgaattttttattttagttattgtatttattatttttagatggtttattgggtttttttttatattttttatttttttttttatgaatattttttttatgtttttttttaaatttttgagtatattgagttatttattatttttattatttttgagttttgtttttatgaaattattttttttttgattataggttatatttttttttttttttttttttttttgagatggagtttttttttttgttgtttaggttggagtgtaggggcgttatttcggtttattgtaagttcgattttttgatttcgtgatttattcgttttagttttttaaaatgttgggattataggtttacgtgagttatcgtattttgtttataagttttatttttttattttttggtatatttagtaatttttaattgaattttggatattgtaaatatgatgttaagtatttggatttgttattgttttttaaagagtgttgggttttgtttaggtagattaggtaaattatttgtaaattagtttgatttttttgaggtttttttttttgagatagagttttgttttgttatttaggtttgagtgtagtggggtaattttagtttattgtagttttaattttttgggtttaagggatttttttgttttagttattgagtagttgaggttataggtatatgttattatatttggttaattttttgtattttttgtagatatggggttttggtatgttgtttaggttggttttgaatttttaggtttaagtgatttgtttgttttagttttttaaagtgttgggattagaggtgtgagttatcgtgtttggtttttgatgttaattttttttttttttttttttttttttttttttttttttttgagatggagttttgttttgttatttaggttagagtgtagtggtgtagttttggtttattgtaattttcgttttttgggtttaagtgatttttgtgttttagttttttgagtagttgggattataggtatttattattaagttcggttaattttttgtatttttagtagagatgtggtttcgttattttggttaggttggttttgaatttttgattttaggtgatttgttcgttttcgttttttaaagtgttgggattataggtatgagttattgtattcggtttgaggttaatttttaatttgttagggtgggtttaggtgagttttttttttagggatagtttagttttattgttaaggtataatttttttgaggtttgattaaatatgtatttttattttaggaggttggagtttgattatttttttgtttttggtgagttttgagaatttattattttattgtttttttttgtgtggttttattgagttttattatatatatgtgaagtttagtatttaggaagatttgaagagatttttatgtagatttttggagttttttgagtagtttatttttttttagaattgtgttttgttgtaatttttaatattttggtttttttgaattttgtttttatttttttaatttaggaagagtattatgttttgttcgggttttttttttttgaattatagtttggaatgtttttttaggtagaaatttagggatgttatagagtttattttgtttattttttttattttagggattatagttttggatttttaaaaatagttatttttttttatatatattttttatatagagaaatatatatatatatatatataaatatatatatatatatatatatatatatatatatatatatatatatatacgtatatgtatatatatatttgagatagcgttttattttgttgtttagtttggagtgtagaggtgtgatgatattttattgtagttttaattttttaggtttaagcgatttttttattttagtttttgagtagttgggattataggtataggttattatattcggttaatttttttgtattttttgtagagatggggttttgttatattgtttaggttgatttttaatttttgggtttaagtaattcgttaatttttgttttttaaattgttgggattataggggtgagtttttgtgtttagtttttatatattttgtagtaataatttttttattgtttatggtggtagagtaattttatttattatggtaggagtagaagtttttttattggcgttttaattaagtttagagaagaggagggagttatatgtatgtggttagtttattgttttttttttttttgagacggagttttgtttttgtcgtttaggttggagtgtagtggtatgatttcggtttattgtaattttcgtttttcgggtttaagcggtttttttgttttagttttttgattagttgggattataggtatgggttattacgtttggttaattttgtatttttagtagagatggggtttttttatgttgttaggttggtttcgaatttttaattttaggtgatttattcgtttcggttttttaaagtgttgggattataggcgtgagttatcgcgtttggtttgttagtttattgtttttaattagaagttttagattttcgaaatatatttaaatatttatgtttaagatcgggcgtggtggtttacgtttgtaattttaatattttgggaggttaaggtaggcgaattatttgaggttaggagttagagattagtttgggtaatatattaaaatttcgtttttattaaaatataaaaattagtttggtatagtggtgttcgtttgtaattttagttatttagaaggttgaggtataagaatcgtttgaatttgggaggcggaagttgtaatgagttaagatggtattattgtattttagtttgggtgatatagtgagattttgttttaaaaaataaataaataaataaataaataaaatttacgtttaataaatatgttttttaagttaggtgtaggggtttgtaattttagttgtttgggaggttgaaataggaggattgtttaagtttaggagtttgagattagtttgggtgatatagtgagattttgttttaagtaaaaaaaaaaaaaaaaaaaaaaaaaaaaaaaattttttgtttgggtattgcggtttatatttgtaattttagtattttgggagttcgagttaggtggattatttgaggttaggagtttaagattagtttggttaatatggtgaaaatttatttttattaaaaatataaaaaattagttagacgtgttggcgaatgtttgtaattttagttatttgggaggttgaggtaggagaatcgtttgaatttgggagacggaggttatagcgagttgatattacgttattgtattttagtttagttaatagagtgagatttcgtttttttaaaaaaaatataaaaaaaaattttaaaaaaagtttttattatttttattatataatagaaattttatgtaatgtaattatgttatttataaaattataggatttgtataaattttaatgtatagtgttttataagtataggatatggttgtgaaattgtattaatattatgaatttgttattttatttttgtttgtgtattattgtaatcgtttgttaaattttatttagtgataatgttagtgatttaaattggtagttttttttgaaggtggtttgggatttttagggtaggtttggttttaggtgagttttttggttaatagtttttttgttattttattttagttttaggtttatttttggtaggtaggttattgggttttggaggagaggatttagttaggggtttttggtggataggaagggaggaagtttttttttttttagagttattttttgttttgttttttaagtttttttttatttacgtgtttgttttttcgttgtttatagtgtttgttttttcgttgtttatagtgtttgttttttcgttgttttgtgaggttggtgaggtagagtagttttagtagggggtgggggttgttgtttgttttagggttgtttggtttcggagggttgttttcgacgtgattggggttttattttttattttttttttttttttaggtggatatcgagtagttggattttcgcggtcggatttttttgtatttggttattacgttggggtattttgagtgtgttcgtgtgtttttggcgtacggcgtagacgtgggtagggagaatcgtagcggttggataggtgggtagttttgtttattttagttttatagtcggggtttttttagtattatagatttatggttggttgaagggttttgttttgtgattttgtttcgtttttttttagtgttttaggaggttgtgagtattcgggatttggagttggtgtagttggtgtttcggtatcgggattattagcgggtggtgaagcggttggcgggtattttcgtgtttttggagaagttgcgtaaggtgaggtttagttttttagtttttacgggagtttttgagtttttttttagtgtagatttagtttttttttttttcgttttttaggtttaggatttttacgtggagatgaaatgggagtttattagttggggtaagcgggttgtagtaggtcgtttttgggtttttttattttaggttttgcgtttgtttttttgtttggaatgtgtttttatagttttttcggcggttttttttatgttttagtttagtttagggttatcgttttagttaggtttttttagattgttttagatattgttttgattttattattattttttttattttgttatgatttgtttattgtatttatgatttgtcgttttttgttagaaggtaagttttgagagggtaggagttttgttttttttattgttgtatttttagtggttggaatatttagtaggtgttttataaatatttgttgaaagaatggatgaaagagtgagtgagtgaattaataaatgatggatattagggatttagtggtgatagaaatatgttcgtttcgattttaggttgtttttttgtgtgagtatggtttatattggttagggagggggttttggaggagaggttgttttttttttagtttttttttttgtttttggttatacggattttaaattttatgttttgagttggtttaggtcgtgtaggttagattagttaaagttatttttaattttcgtttttattagtgtttttggtgtttaagatttgttttagtgatatttataaagtgtggaagagcggttagaatttgagggtagatattatatttttgggttttgattatatgatttggtagcgagggaatcgtagttttgtttttaggggttaaggttaggtaggtaggaagtggggtagggtggggacgatgggaggtagttttaggttatttttgatttttttgtgttgtttcgtgtttggtagatataagcgtcgtggttatggagattgattacgatcgtcgggtggtgtatatagagattttggtattggttgggtaggatcgggagttgttgttggttgttgtttagtttattgaggaataggtgttgagtcggtttatcgcgttcgtcgttattatttagtttgatattaagaatattttttttgagaggtgggtggatatggttttggttatttttgagttagttcggtggggtgtttgttttatttggattattttgtttttttaggaataagattggtattttgggttggcgtagtgaaaagacggagatggtgaatgggtatgaagttaaggtgaggttgtagtttttagttgttagtttagttgtatttttgtttatagtaagttgtataggggattttgattttttttttttagttttggaggtatagaagtaatgtagcgtggttaagtatttatatttgggtttaaggtatttttttggtgttttatatggatgtatggatgtatatatagggtacgtgtatacgtatatatatatatatatttattttttatagtaattttttttggtaggtgttgttttgttagtatttttattttacgtatgtttattgagttttttttttggtattttatttattttttataataattttaggaagtagggatgatcggtttattttatgatgaggaaatagaggtttagagtggttttgtgatttgtataaggttatatagttgttaagtggtagagttggggtttagattttggttggtttgattttagagttaggtttttatttttaaaaatgattgtttggttgggtatggtggtttatgtttgtaattttagcgttttgggaggtcgaggtgagcggattatttgaggttagttcgagattagtttggttaatatggtgaaatttcgtttttattaataatataaaaaattagtcgggtgtggtagtaggcgtttgtaattttagttattcgggaggttgaggtaggagaattgtttgaatttgggaggcggagtttgtagtgtgtagcgatttcgttatagtattttagtttgggtaatagagcgagattttatttaaaaaaaaaaaaaaaaaaaggttttgtttgttattttgggatttttatgttgtttacgatatgaaagtaggaattaataaatgttatgggttttgtgtgtggtattttttttgaaagttttttttgtttttgtagtttgggaaggtttttgtgttatttttattagtgtatggattatgttgttataattttattttattgtttttttatagagattgtaagttttaggagggtagggattatgtttggtttgtttattgtatttttgatgtttattttaatgtttggtatataaaggttttttaaaaaatgtttgttgaatgaataagtgaatgaatgaatgaatgaatgattttatatatttatttatttaaaagtttgaagtagagtttttttaggattttttgttatagggagtgtttttagtgtttttaggggtaagatatagggtaagattagaattgtttatgagttttttttttatttgtttttaggtgtatggggtatttaacgtggagtttattattcgtatacggatagaatattttttagaatagtataagggtaaggttaaaggtaatgaggtagagttggatggggagaggtgttgtaggattgcgggaattagtttttattttagtgtttttattagtatttttattggtattttagtaagaggttggatgttttatttaggtcgatagattttaatttaggtgttaagttttaaggatgggtagtggttgtttagagtattaagaagtttttaaggatttatttgggtttagtggagagttatgttgtaagtgattattaatgttgttgttgaatttgggagaggagagaaatgttatgtatgttatttattggttattttagtttagtgggatatattttaggtagaaagttaggggattttgttatagattttgtatgtttattgatgttatatttgattttttgggtattagatatcgtgttcgaggtgaaaaagtataatttttattttataggggaataatatgaaattatgtttatggaagtgtttgaagtaaatatatatacgtatatgtatattttatagtgtttgtcggggtaggcgttttattgtttagggttatcgagttggagaggagtatttttggaagttgtttttgatttttaggttttttttttagtgttttaagttgtgtttatagaggttttggtttttggtttttgaagtatttagttttttttaggtgaaggtgtttgagtatgtggttgggtgagtaggttttattttaggaatcggttttttttttaggttttgggtgttgttatttttgatgaggtgtttaggtgtgtgtggagttgcggtgttttttgagatgttatattttttgtaggttgtaagatatttttgtagttttttttgggaatcgttgagtagtacgggggtttttaaaatggggtgagtgtgtgtaggggtattcgtaagtggagggatgtggatgtggtttaggaggaggtttgggaagcgttttgtttagtatggtttatgtggattttttttttataatgtttaaggttatgttagcgttatattggtagaggggatagtttgggggttttgtgataataaatgagttggtttggtattaggaattgaggggagtttttgggtttttttttatgtggtatagattttgattatttagattttgagttaagttaattttattgttattattgtagaagaatattttaattttaattttgagttgggtaatcgtgatatgggtcgttttatggaattgattattaagatatagaagtgaggtttttgtcggtgttgggaaggtggggggtcggggttttaggagatgttgggaggttatggttttttgtagtgttttttattttttgggatttggtgggggtaggtttaaggttaagttgtggttgtgtgaggagtattttttgtttttgtgtgagtaggtggtttttattattgattttatggtcgttagtaatgcgttttttgttaagtttcgggattttattattttgcgtttgttttttggttttttagttaagattggtgagatcgtacggttattttttttgagttcgtggcgggtcgatcggggtttagatgaggtcggggtggggttgaggttgaggtgtgaggggttgagtggtggcgtttaaaggtttttttatttttagaaatttcgattttttatatttttaacgttcgtattattttcgggaattttaacggttgcgacgaatcggtgttatcggtgcgaggtagttttagtagcgagacgttttttttaggtagcgatttttttagcgttagtagttttagttttacgagtgaggtttttcgcgagaacgtttgtttttcggtttttttcggggtgggtgggaggggcgcgttcggtcgtgtttgatttagttttcgcgtttttagttttttgtcgcggttgcgagatttttttagcgttgttcgaggtttcgcgcggttatagtatgatgggcggttagcgggaggcggcgattcgggacgacgacgacgatttgttgtaattcgttatttagtagagtttgtttgaggcgggtagtgagtatgattaggtgcgttttcgcgggcgcgcggggttacgggatttcgcgtcgttacggttaacgtttacgttttttcgtaggttattatttgggaggcgttaattaatagtaagttaggtatttattttatgttttacgagggtcgtcgataggataggttagtgttcgttgggtcggagagaatttttcggagaggattttgttttttttaagttaggatatagtcggagaattcgcggggttttcggtagggatttttttggtatcgggatggtttttgttattatttttgttttcgaggcggtaggtaggggttagggatttaggttttatcgcggagtttagattttttttaggtattgacggggagaatttggtagggtttgggtttcgttacgattaggtgggggttaggacgtcgcgggattgatcgtttttattagagggtggtggtcgcgggtcgttttggagtttttacgtcgtgtttcggtttcggtcggtgggtgggtgcgttcgggagttcgcgatattttttttttatttttaggagcgtttcgtttacgtcgtagcgttagtttgcgttttcggcgttagtgtttagttttcggtttagtttagggttaggtttcggcggttacgtgtttcggagttacgacgagtagttgcggttggcgatggaattgtcggcgtaggagtaggaggagaggcggcggcgcgcgcgttaggaggaggaggagttggagcgtattttgaggtttttattgatcgagtagtagcgttttttgtcgggattttcgttagcgttacgcgcgttacgtttagggttaggagttagataaatttcggtttgcgcgtttgtagagcggcggttggagattggagttatcgtttcgcgggtgtagtagtatagtaggtacggttcggggagggattcggtatggtcgcggggtatttttttaggttagggttttggaggtaattggtacggtttggtttttttgttttgttgtattttgattttttaattcgtttttttgggtttagatttgttttgttttagggcggagttaggcggttttgagggggagatgaatttttagaggagcgttgtttttattttttgttttttttggtcggttcgtatttttgtttattaattttattttaggatattgtttttgaagtttttgtatttttgttttttatttttggggggtagttgagtttttcgcgtgttgtgttattgttttgttttagatataaattagtacgtttagggtttagttttttttttatttcggtattttagcgttaagtgtatttagcggggtattcggtttttttagtttttatattcgttttgggttttagggtggttttagtttttttttgggtagttagaagttggagttttattttttaaggtatatttttttttttttttttttgtgattagggagtgtgtttaacgtagttttttggtttgtgtaagttttgatttttttatggtgtttcggagagtggggagtatattgggttggggtaagtattagatttaagtagattggatataaagggttcgtttagggttttggcgttatttttatttttttttattagttgttgttagtttttgtggttgtatattttatttgtttttatacggagattgattttaaaattttttatttaatggtgttaattttcggtttttttttgttttattttatttatttagagaagtatagatttcgttaggggtaggggtttatcgtatatttttgtttcgggtttgtttgggattggttttttcggtttagttagtgaggtttagaagggatataaagagggatggaagaaaagaataaagagaaattgttttttttatttttttttttgatgttaggggtattagattgattttgaggtataaataaaagaggttttatatcgga

SEQ ID NO: 8 - DNA, 24993 bp, Artificial Sequence
  rc C to T (bis1)
tccgatataaaacctcttttatttatacctcaaaatcaatctaatacccctaacatcaaaaaaaaaaataaaaaaaacaatttctctttattcttttcttccatccctctttatatcccttctaaacctcactaactaaaccgaaaaaaccaatcccaaacaaacccgaaacaaaaatatacgataaacccctacccctaacgaaatctatacttctctaaataaataaaataaaacaaaaaaaaaccgaaaattaacaccattaaataaaaaattttaaaatcaatctccgtataaaaacaaataaaatatacaaccacaaaaactaacaacaactaataaaaaaaaataaaaataacgccaaaaccctaaacgaaccctttatatccaatctacttaaatctaatacttaccccaacccaatatactccccactctccgaaacaccataaaaaaatcaaaacttacacaaaccaaaaaactacgttaaacacactccctaatcacaaaaaaaaaaaaaaaaaaatataccttaaaaaataaaactccaacttctaactacccaaaaaaaaactaaaaccaccctaaaacccaaaacgaatataaaaactaaaaaaaccgaataccccgctaaatacacttaacgctaaaataccgaaataaaaaaaaaactaaaccctaaacgtactaatttatatctaaaacaaaacaataacacaacacgcgaaaaactcaactaccccccaaaaataaaaaacaaaaatacaaaaacttcaaaaacaatatcctaaaataaaattaataaacaaaaatacgaaccgaccaaaaaaaacaaaaaataaaaacaacgctcctctaaaaattcatctccccctcaaaaccgcctaactccgccctaaaacaaaacaaatctaaacccaaaaaaacgaattaaaaaatcaaaatacaacaaaacaaaaaaaccaaaccgtaccaattacctccaaaaccctaacctaaaaaaataccccgcgaccataccgaatccctccccgaaccgtacctactatactactacacccgcgaaacgataactccaatctccaaccgccgctctacaaacgcgcaaaccgaaatttatctaactcctaaccctaaacgtaacgcgcgtaacgctaacgaaaatcccgacaaaaaacgctactactcgatcaataaaaacctcaaaatacgctccaactcctcctcctcctaacgcgcgcgccgccgcctctcctcctactcctacgccgacaattccatcgccaaccgcaactactcgtcgtaactccgaaacacgtaaccgccgaaacctaaccctaaactaaaccgaaaactaaacactaacgccgaaaacgcaaactaacgctacgacgtaaacgaaacgctcctaaaaataaaaaaaaaatatcgcgaactcccgaacgcacccacccaccgaccgaaaccgaaacacgacgtaaaaactccaaaacgacccgcgaccaccaccctctaataaaaacgatcaatcccgcgacgtcctaacccccacctaatcgtaacgaaacccaaaccctaccaaattctccccgtcaatacctaaaaaaaatctaaactccgcgataaaacctaaatccctaacccctacctaccgcctcgaaaacaaaaataataacaaaaaccatcccgataccaaaaaaatccctaccgaaaaccccgcgaattctccgactatatcctaacttaaaaaaaacaaaatcctctccgaaaaattctctccgacccaacgaacactaacctatcctatcgacgaccctcgtaaaacataaaataaatacctaacttactattaattaacgcctcccaaataataacctacgaaaaaacgtaaacgttaaccgtaacgacgcgaaatcccgtaaccccgcgcgcccgcgaaaacgcacctaatcatactcactacccgcctcaaacaaactctactaaataacgaattacaacaaatcgtcgtcgtcgtcccgaatcgccgcctcccgctaaccgcccatcatactataaccgcgcgaaacctcgaacaacgctaaaaaaatctcgcaaccgcgacaaaaaactaaaaacgcgaaaactaaatcaaacacgaccgaacgcgcccctcccacccaccccgaaaaaaaccgaaaaacaaacgttctcgcgaaaaacctcactcgtaaaactaaaactactaacgctaaaaaaatcgctacctaaaaaaaacgtctcgctactaaaactacctcgcaccgataacaccgattcgtcgcaaccgttaaaattcccgaaaataatacgaacgttaaaaatataaaaaatcgaaatttctaaaaataaaaaaacctttaaacgccaccactcaacccctcacacctcaacctcaaccccaccccgacctcatctaaaccccgatcgacccgccacgaactcaaaaaaaataaccgtacgatctcaccaatcttaactaaaaaaccaaaaaacaaacgcaaaataataaaatcccgaaacttaacaaaaaacgcattactaacgaccataaaatcaataataaaaaccacctactcacacaaaaacaaaaaatactcctcacacaaccacaacttaaccttaaacctacccccaccaaatcccaaaaaataaaaaacactacaaaaaaccataacctcccaacatctcctaaaaccccgaccccccaccttcccaacaccgacaaaaacctcacttctatatcttaataatcaattccataaaacgacccatatcacgattacccaactcaaaattaaaattaaaatattcttctacaataataacaataaaattaacttaactcaaaatctaaataatcaaaatctataccacataaaaaaaaacccaaaaactcccctcaattcctaataccaaaccaactcatttattatcacaaaacccccaaactatcccctctaccaatataacgctaacataaccttaaacattataaaaaaaaaatccacataaaccatactaaacaaaacgcttcccaaacctcctcctaaaccacatccacatccctccacttacgaatacccctacacacactcaccccattttaaaaacccccgtactactcaacgattcccaaaaaaaactacaaaaatatcttacaacctacaaaaaatataacatctcaaaaaacaccgcaactccacacacacctaaacacctcatcaaaaataacaacacccaaaacctaaaaaaaaaaccgattcctaaaataaaacctactcacccaaccacatactcaaacaccttcacctaaaaaaaactaaatacttcaaaaaccaaaaaccaaaacctctataaacacaacttaaaacactaaaaaaaaaacctaaaaatcaaaaacaacttccaaaaatactcctctccaactcgataaccctaaacaataaaacgcctaccccgacaaacactataaaatatacatatacgtatatatatttacttcaaacacttccataaacataatttcatattattcccctataaaataaaaattatactttttcacctcgaacacgatatctaatacccaaaaaatcaaatataacatcaataaacatacaaaatctataacaaaatcccctaactttctacctaaaatatatcccactaaactaaaataaccaataaataacatacataacatttctctcctctcccaaattcaacaacaacattaataatcacttacaacataactctccactaaacccaaataaatccttaaaaacttcttaatactctaaacaaccactacccatccttaaaacttaacacctaaattaaaatctatcgacctaaataaaacatccaacctcttactaaaataccaataaaaatactaataaaaacactaaaataaaaactaattcccgcaatcctacaacacctctccccatccaactctacctcattacctttaaccttacccttatactattctaaaaaatattctatccgtatacgaataataaactccacgttaaataccccatacacctaaaaacaaataaaaaaaaaactcataaacaattctaatcttaccctatatcttacccctaaaaacactaaaaacactccctataacaaaaaatcctaaaaaaactctacttcaaacttttaaataaataaatatataaaatcattcattcattcattcattcacttattcattcaacaaacattttttaaaaaacctttatataccaaacattaaaataaacatcaaaaatacaataaacaaaccaaacataatccctaccctcctaaaacttacaatctctataaaaaaacaataaaataaaattataacaacataatccatacactaataaaaataacacaaaaaccttcccaaactacaaaaacaaaaaaaactttcaaaaaaaataccacacacaaaacccataacatttattaattcctactttcatatcgtaaacaacataaaaatcccaaaataacaaacaaaacctttttttttttttttttttaaataaaatctcgctctattacccaaactaaaatactataacgaaatcgctacacactacaaactccgcctcccaaattcaaacaattctcctacctcaacctcccgaataactaaaattacaaacgcctactaccacacccgactaattttttatattattaataaaaacgaaatttcaccatattaaccaaactaatctcgaactaacctcaaataatccgctcacctcgacctcccaaaacgctaaaattacaaacataaaccaccatacccaaccaaacaatcatttttaaaaataaaaacctaactctaaaatcaaaccaaccaaaatctaaaccccaactctaccacttaacaactatataaccttatacaaatcacaaaaccactctaaacctctatttcctcatcataaaataaaccgatcatccctacttcctaaaattattataaaaaataaataaaataccaaaaaaaaaactcaataaacatacgtaaaataaaaatactaacaaaacaacacctaccaaaaaaaattactataaaaaataaatatatatatatatatacgtatacacgtaccctatatatacatccatacatccatataaaacaccaaaaaaataccttaaacccaaatataaatacttaaccacgctacattacttctatacctccaaaactaaaaaaaaaaaatcaaaatcccctatacaacttactataaacaaaaatacaactaaactaacaactaaaaactacaacctcaccttaacttcatacccattcaccatctccgtcttttcactacgccaacccaaaataccaatcttattcctaaaaaaacaaaataatccaaataaaacaaacaccccaccgaactaactcaaaaataaccaaaaccatatccacccacctctcaaaaaaaatattcttaatatcaaactaaataataacgacgaacgcgataaaccgactcaacacctattcctcaataaactaaacaacaaccaacaacaactcccgatcctacccaaccaataccaaaatctctatatacaccacccgacgatcgtaatcaatctccataaccacgacgcttatatctaccaaacacgaaacaacacaaaaaaatcaaaaataacctaaaactacctcccatcgtccccaccctaccccacttcctacctacctaaccttaacccctaaaaacaaaactacgattccctcgctaccaaatcatataatcaaaacccaaaaatataatatctaccctcaaattctaaccgctcttccacactttataaatatcactaaaacaaatcttaaacaccaaaaacactaataaaaacgaaaattaaaaataactttaactaatctaacctacacgacctaaaccaactcaaaacataaaatttaaaatccgtataaccaaaaacaaaaaaaaaaactaaaaaaaaaacaacctctcctccaaaaccccctccctaaccaatataaaccatactcacacaaaaaaacaacctaaaatcgaaacgaacatatttctatcaccactaaatccctaatatccatcatttattaattcactcactcactctttcatccattctttcaacaaatatttataaaacacctactaaatattccaaccactaaaaatacaacaataaaaaaaacaaaactcctaccctctcaaaacttaccttctaacaaaaaacgacaaatcataaatacaataaacaaatcataacaaaataaaaaaaataataataaaatcaaaacaatatctaaaacaatctaaaaaaacctaactaaaacgataaccctaaactaaactaaaacataaaaaaaaccgccgaaaaaactataaaaacacattccaaacaaaaaaacaaacgcaaaacctaaaataaaaaaacccaaaaacgacctactacaacccgcttaccccaactaataaactcccatttcatctccacgtaaaaatcctaaacctaaaaaacgaaaaaaaaaaaaactaaatctacactaaaaaaaaactcaaaaactcccgtaaaaactaaaaaactaaacctcaccttacgcaacttctccaaaaacacgaaaatacccgccaaccgcttcaccacccgctaataatcccgataccgaaacaccaactacaccaactccaaatcccgaatactcacaacctcctaaaacactaaaaaaaaacgaaacaaaatcacaaaacaaaacccttcaaccaaccataaatctataatactaaaaaaaccccgactataaaactaaaataaacaaaactacccacctatccaaccgctacgattctccctacccacgtctacgccgtacgccaaaaacacacgaacacactcaaaataccccaacgtaataaccaaatacaaaaaaatccgaccgcgaaaatccaactactcgatatccacctaaaaaaaaaaaaaaaataaaaaataaaaccccaatcacgtcgaaaacaaccctccgaaaccaaacaaccctaaaacaaacaacaacccccaccccctactaaaactactctacctcaccaacctcacaaaacaacgaaaaaacaaacactataaacaacgaaaaaacaaacactataaacaacgaaaaaacaaacacgtaaataaaaaaaaacttaaaaaacaaaacaaaaaataactctaaaaaaaaaaaaacttcctcccttcctatccaccaaaaacccctaactaaatcctctcctccaaaacccaataacctacctaccaaaaataaacctaaaactaaaataaaataacaaaaaaactattaaccaaaaaactcacctaaaaccaaacctaccctaaaaatcccaaaccaccttcaaaaaaaactaccaatttaaatcactaacattatcactaaataaaatttaacaaacgattacaataatacacaaacaaaaataaaataacaaattcataatattaatacaatttcacaaccatatcctatacttataaaacactatacattaaaatttatacaaatcctataattttataaataacataattacattacataaaatttctattatataataaaaataataaaaactttttttaaaatttttttttatattttttttaaaaaaacgaaatctcactctattaactaaactaaaatacaataacgtaatatcaactcgctataacctccgtctcccaaattcaaacgattctcctacctcaacctcccaaataactaaaattacaaacattcgccaacacgtctaactaattttttatatttttaataaaaataaattttcaccatattaaccaaactaatcttaaactcctaacctcaaataatccacctaactcgaactcccaaaatactaaaattacaaatataaaccgcaatacccaaacaaaaaattttttttttttttttttttttttttttttttacttaaaacaaaatctcactatatcacccaaactaatctcaaactcctaaacttaaacaatcctcctatttcaacctcccaaacaactaaaattacaaacccctacacctaacttaaaaaacatatttattaaacgtaaattttatttatttatttatttatttattttttaaaacaaaatctcactatatcacccaaactaaaatacaataataccatcttaactcattacaacttccgcctcccaaattcaaacgattcttatacctcaaccttctaaataactaaaattacaaacgaacaccactataccaaactaatttttatattttaataaaaacgaaattttaatatattacccaaactaatctctaactcctaacctcaaataattcgcctaccttaacctcccaaaatattaaaattacaaacgtaaaccaccacgcccgatcttaaacataaatatttaaatatatttcgaaaatctaaaacttctaattaaaaacaataaactaacaaaccaaacgcgataactcacgcctataatcccaacactttaaaaaaccgaaacgaataaatcacctaaaattaaaaattcgaaaccaacctaacaacataaaaaaaccccatctctactaaaaatacaaaattaaccaaacgtaataacccatacctataatcccaactaatcaaaaaactaaaacaaaaaaaccgcttaaacccgaaaaacgaaaattacaataaaccgaaatcataccactacactccaacctaaacgacaaaaacaaaactccgtctcaaaaaaaaaaaaaacaataaactaaccacatacatataactccctcctcttctctaaacttaattaaaacgccaataaaaaaacttctactcctaccataataaataaaattactctaccaccataaacaataaaaaaattattactacaaaatatataaaaactaaacacaaaaactcacccctataatcccaacaatttaaaaaacaaaaattaacgaattacttaaacccaaaaattaaaaatcaacctaaacaatataacaaaaccccatctctacaaaaaatacaaaaaaattaaccgaatataataacctatacctataatcccaactactcaaaaactaaaataaaaaaatcgcttaaacctaaaaaattaaaactacaataaaatatcatcacacctctacactccaaactaaacaacaaaataaaacgctatctcaaatatatatatacatatacgtatatatatatatatatatatatatatatatatatatatatatatatatttatatatatatatatatatatttctctatataaaaaatatatataaaaaaaaataactatttttaaaaatccaaaactataatccctaaaataaaaaaaataaacaaaataaactctataacatccctaaatttctacctaaaaaaacattccaaactataattcaaaaaaaaaaaacccgaacaaaacataatactcttcctaaattaaaaaaataaaaacaaaattcaaaaaaaccaaaatattaaaaattacaacaaaacacaattctaaaaaaaaataaactactcaaaaaactccaaaaatctacataaaaatctcttcaaatcttcctaaatactaaacttcacatatatataataaaactcaataaaaccacacaaaaaaaaacaataaaataataaattctcaaaactcaccaaaaacaaaaaaataatcaaactccaacctcctaaaataaaaatacatatttaatcaaacctcaaaaaaattataccttaacaataaaactaaactatccctaaaaaaaaaactcacctaaacccaccctaacaaattaaaaattaacctcaaaccgaatacaataactcatacctataatcccaacactttaaaaaacgaaaacgaacaaatcacctaaaatcaaaaattcaaaaccaacctaaccaaaataacgaaaccacatctctactaaaaatacaaaaaattaaccgaacttaataataaatacctataatcccaactactcaaaaaactaaaacacaaaaatcacttaaacccaaaaaacgaaaattacaataaaccaaaactacaccactacactctaacctaaataacaaaacaaaactccatctcaaaaaaaaaaaaaaaaaaaaaaaaaaaaaaaaaaaaaaaattaacatcaaaaaccaaacacgataactcacacctctaatcccaacactttaaaaaactaaaacaaacaaatcacttaaacctaaaaattcaaaaccaacctaaacaacataccaaaaccccatatctacaaaaaatacaaaaaattaaccaaatataataacatatacctataacctcaactactcaataactaaaacaaaaaaatcccttaaacccaaaaaattaaaactacaataaactaaaattaccccactacactcaaacctaaataacaaaacaaaactctatctcaaaaaaaaaaacctcaaaaaaatcaaactaatttacaaataatttacctaatctacctaaacaaaacccaacactctttaaaaaacaataacaaatccaaatacttaacatcatatttacaatatccaaaattcaattaaaaattactaaatataccaaaaaataaaaaaataaaacttataaacaaaatacgataactcacgtaaacctataatcccaacattttaaaaaactaaaacgaataaatcacgaaatcaaaaaatcgaacttacaataaaccgaaataacgcccctacactccaacctaaacaacaaaaaaaaaaactccatctcaaaaaaaaaaaaaaaaaaaaaaaaatataacctataatcaaaaaaaaaataatttcataaaaacaaaactcaaaaataataaaaataataaataactcaatatactcaaaaatttaaaaaaaaacataaaaaaaatattcataaaaaaaaaaataaaaaatataaaaaaaaacccaataaaccatctaaaaataataaatacaataactaaaataaaaaattcactaaataaaaataacaacaaattaaacactacacaatttaaaaatcaataaatttaaaaacaacaataaaactttccaaactaaaacacaaaaaaaaaaaacaatactaaaaaataaaattaactaaacttctataatcccaacacttttaaaaaccaaaacgaaaaattaacttaaattcaaaaatttaaaaccaacccaaacaatacaacaaaactctatctctacaaacaaaacaaaacaaaacaaaacaacttttacattaactaaacataataacaaacaactataatcccaactcctctaaaactaaaacaaaaaaatcccttaaacccaaaaattcgaaactacaataaactataatcacgccactacactccaacctaaacaacaaaacaaaaccctatctctataaaacctcataatctataaaacattatcaaacattataacatatatctattaaaatcccaaaaaacaaaataaaaaaataaaacaaataaaacaaatttaaaaaaataaaccgaatacgataactcacgcctataatcccaatactttaaaaaaccaaaacgaataaatcacaacatcaaaaatttaaaaccaacctaaccaatataataaaaccccatttttactaaaaatacaaaaattaaccaaacgtaataataaacacctataatcccaactacttaaaaactaaaacaaaaaaatcgcttaaacccgaaaaaaaaaaattacaataaaccgaaatcgtatcactacactccaacttaaacgacaaaaaaaaactccatttcaaaataaataaataaataataaaaaaaaaaaaaaacgtccaaaatttttccaaacttaataaaaactactataataaattaaaaaataatacccctcctaaaacatatccacatcacattctaaccctcacaacctataaataaaaccttatttcaaaaaaaaatctttacaaacataattaaattaaaaatctcaaaataaaataatcctaaatcacccaaaaaaccctaaatccaataacaaatatctttctaaaacactcaaaaaaataaaaaaaccatataaaaacgaaaacaaaaactaaaattctacaaccacaaaccaaaaaaattataacccaatcaccaaaatctaaaaaaaacaaaacaaaactcttccctaaaacctttaaaaaaactaccaccctaccaacatctcaaatttatatttatatctcccgaactataacaaaataaattttttttttttttttttaaaataaaatctcactctatcgcccaaactaaaatacaataacgtaatctcaactcactataaactccgcttccccgattcacgccattctcctacctcaacctcccaaataactaaaattacaaacacccaccaccacgcccgactaattttttatatttttaataaaaacgaaatttcaccgtattaaccaacataatctcgatctcctaacctcgtaatccgcccgcctcgacctcccaaaatactaaaattacaaacgtaaaccaccacacccgaccaaatatttattattttaacccacctaatttataataatttattataaaaactaataccaaaataaaaccaaaaaccaaaaaattcaataaaccccaaataaaacaaacacgaaataaactacaccaaaatccatcataatcaaatactaaaaactaataataaaaaaaaaatcctaaaaacattcaaaaaaataaaatccattatatataaaaaaacaaatacaaaaaatactatattcttctcatcaaaaactatataaaccaaaaaacaatataataaaatctttaaaatactaaaaaaaaaaaacaaaaacaaaaactttcaacctaaaattctttttttttttttctctaatccaatataactaatattaacctaaaattccatacccgataaaaatattcttcaaaactaaaaaaaaaataaatatattaacaaacaaacaaattctaaaaaaatttattaccaaatatacaaaaaatattaaaaaaaattcttcaaataaaaaaaaaataatcccaaataaaaacttaaatctatacaaaaaattaaaaaataccaaaaaatattaaatatataaaaatatcaaaaaaccaaacacaataactcatacctataatcccaacactttaaaaaaccgaaacgaacaaatcaccaaaaatcaaaaatttaaaaccaacctaaccaacataataaaaccccatctctactaaaaatacaaaaattaactaaacgtaataaaaaattcctataatcccaactactaaaaaaactaaaacacaaaaatcgcttaaacctaaaaaataaaaattacaataaacaaaaatcgcaccactacactccaacctaaataacaaaaaaaaactctatctcaaaaaaaaaaaaaaaaaatatcaaactaaacgcaataactcatacctataaactttaaaaaaccgaaataaacaaatcacttaaacccaaaaatttaaaaccaacgtaaacaatataataaaactctatactacaaaaaaatactaaaattaaccaaacgtaataatacatacctatcgtcccaactactaaaaaactaaaataaaaaaatcccttaaaccaaaaaaccaaaaattacaataaacaaaaatcatcccactacactccaacctaaacaacaaaaccaaaccctatctcaaaaaaaaaaaaaaaaaaaaatcaataaaatatttaaaacccacaaaaataaaaaaaaaaaatatcaacaaataaaaaacttcaacacaactttaaaacataaaaaataactaaaacctcacaactaacttaaaaaaacaaaaaaaactaaaactaaaacaaccacaaaaaaaaacgtccacataaaaaacaaaccaaataacccccaacccccctaaaaaatataaataaaacctacaaacaataaaaataacaaaaataaaaataaaactaaaactaaatacaaaaaaactaattacaattcaaaatcccctaatccccttcccaacctcattaaactaaaaaataccccccttcctcaccacaaaacaccaaaaatttattctttataaaaattaaacataaaatactctaaactcaaaaacattaaccacaacaaaaaataaaatataatactaaaaaccaataatccgtaaaaccccaaccccttccctacctaaatcctaaaccactaacaaccaaatcacaccaccaccaccctatctacccgaataaaaaattatcccaaaaacctcaaaatacaaacatctaataaccctacaataaacaaaccaacctaccacctaatcaccttacaataacacccacacatccctaaactccccaaccccattcttaaatataacccaacaaccaaaaaaaactaaacacttaataaaaacttcccatataaaataaaccaaaacatacaaattaaatactaaaacgactaaatacaataactcacgcctataatcccaactctttaaaaaaccgaaataaacgaatcacgaaatcaaaaaatcgaaaccatcctaactaacacgataaaaccccgtctctactaaaaatacaaaaaattaactaaacgtaataacgaacgcctataatcacaactactcgaaaaactaaaacaaaaaaataatataaacccgaaaaacgaaacttacaataaaccgaaattacgccactacactctaacgcgaaaaacaaaacgaaactccgtatcaaaaaaaaaaaaaaaaaaaaaaaaaaaaacaaattaaatactaaaaacccaaaaaaaattctcttaatacaaaaaataaaaaaaaactctttaaaaaaaaacaataatttacatcctcaaaaaaaatataaaaaaatcattaaattcataaaacaaaataaaacaacctaactttccataacgtctcctaccctttctcttaccttcttcattctaaaaataactttcttaacttttccttattttctacattcctaaacaactacacctacccccataaacaataaacatcacctaaatttactacattttcaaataaaaaaaaaaaccaactttaaaactatctacatctcttctttttcccgcaccctccacatctaacccatcaaaaaaacttataaactctacctccaaaacaaacctaaaaaccgcccaatttccactaccttacaactattacccccccatctctcactaacaaccccctactacctctttactactccccgattaccaaactctattatccacctcacctataacaactaaaatcaccctataaaatattactcaaatcctaacactctttaattcaaaatcttccaataactttccatcgtaaataacaaaaaatccaataaccccaaacttctctttaaactcatttactccacccttcgccaataaccttccccgaaacgttctccaaaatcctccaaaaaaccccaaaactttctccctcccttcactcaaactactactcaaatatcacctccttaaaaaaacccaccctaacaacccatctaaaataacaactactataactctatccactacccgtccaaatacctattaaacacctcctacacctcgaacaaaaaccccatcaaccaaatccctacctactttattcactactaattccccactccccaaacaacacctaacacataaatatttactaaacaaatacataaaatactaaactaaaaaaacacaaaaaaaaaaaaataattaaccaaaaaatcattacaaaaatatattatttataccgaaaaactcacgtctataatcccaacactttaaaaaaccaaaataaataaatcacttaaactcaaaaattcgaaaccaacctaaacaacataacaaaaccccatctctacaaaaaaaaatacaaaaattaaccaaacataataacaccacctataatcctaactccttaaaaaactaaaataaaaaaatcacctaaacctaaaaaacaaaaactacactaaactataatcacactactacactccaacctaaataacaaaataaaacgctatctcataaaaaaaaaaaaaaaaaaaaaaaaaaaaaaaaaaaaaaaaaaaaaacaaaaaaaaaaaaaaaaaaaaaaaaaaaaaaaaaaaaaaaacaatataaacaatatattatttataattaaaaaaataaataacaaaaaaaatccaaaatactaaaaaaataaaaaaaacgaaacaaaaaacactacttttcattacgcatcttctaacaacaattaaatattttaaaacataaccataaactccattatcaaaaataaaacattttaaataatttaaaattatttatataatttttataaccttatcctaaaatttcttcatttttcaatatactaaaaacctcaaaaaaaccaacgaacctaacccctattaacctctaaactataacccctcacaaaaaaaaaaaatattatttactcttatccaatcctaattaaactaaactccgaaacttacaacctaaataaaatcctaaacccgacaacgaaaataaaaaaaaaccacaaaacccgaactaactaaaaaaatactaaacaatccaaacctcccaaccctaccccaaatactacaaccgcaaccgctacaactaataaaaccctaaaaaactaacaaaccgctacctaacctcaaaactccaaatactacctccacctccccatcaaatacctcaactccaaactccaaaaaacgactaacacttccttacaaacaaaatactcctccccatccccacacctcaaaaacactccccaaaaaaacctaaataactcaacaccccatacaccccatacaaaaccccatacactcaaccaaactccaaaacaactctccccacaaacccaaaataccgcctacaatataaataacaccttaccctaaacccaaataaaaaaattcattaatctcctcaacaaaaacctccaacttctcctcaacaaaaacctctaactatttaattactaaaataaaaaaatttcccataaaacccaacacccaaccctccccaccaaaaaaacgaaaattccttatcccaacaaacctcaactaaaatcaaaaaataaaatctttaaaattttataactaaaaatccctaaacaaaaaacctccctacctccactcaaacacacacaccacactctaatacacactaataccatacaaatacacactcgtacgctcataaatactcacgtatacccttaaatatacaaacacatacatacccaactaccttctaaccctacaaaaatccactcctatataacgtatatatacgtatttacacaaaaacacccctcacacccatatacactaacaaaatactttccaaactcctttaacataaacaaaatccttttattaaaaaaaatataaaaaacatacatctcatatataaactaaacacaatacttacgaaaaaaataaaaaacgcaaaacctatactcaaaataatacctactcaaccccttccccaacccacgaaaaaaaaaacaaaaatctaatataatcgttacttaacctctcctacccaacgtaaaatacaaaaacaaatctacctaaactcattcaaaaaaaaaaaaacaaaatacatcctcaaactacgtaaaaaaccacgaactataaaaaccgcaccctaaacttctccctccatatcacccctcccatcctacccttacaacccctccccctcatcccaaaacacattaatttttaatttctaaaatttataactccctctcccgaacttcctaacttaccaactataataataccccacatccaaaactacccaatataaacaaaaaaaaaaatctaaaatactcctcgcacatcctaaaccccacaacccatctcccctacctctaaatcaaaaaaataaacaaaaaaaacaaaaaacaaacccacgataaaaaacgccccaaaaaaaaaaaaaataattctctaaaaccacaatctacccacttcaaaattctaattaccaaaaacaaaatcctactccccaaacccaacccacacatatccctcccacgaaaactacacaaactaacccttccccctattcccaccccaaaaaacaccaaaaactcacgactccaaaaccaaaaccatacccaactaaccataccaaacaaaaaaaaactaacatattccctaacttacaaccctatcccccccgacctaacaaaaaacatacataacgacaaacaaaacaccgaactaacatcacaacactactaaataccccttcccttcaccaaacacctcctatctacccatcactccctacttccaacctccaacaaaacaatttaaaactaaacaaaacccattaacctactctaaaaataaccatactaaccccctcctcaaccaactacactaccaaacctacccacgaaaaacctctacgaaactttcttaaaataaaaaaaaaacaactataccaaaccaaaaccaaaaaaacctaactcctaaatacttaaaaaaaaccgaactatttctataacgactaataccaaaaaaactaaaaaccaaaaacccctaactaaaataccaaaattccacaatacttttctcataatattaaataactatccccaaatcccccttacaaaaaacaaaacctaataccctaaaaaataaacaatatacatctaaatacaaacctcactctaaaccaatcctcgaaaaaaaaaacaactaaaaaactctcccacctacacgaaataacattcctctttttaacacgcctaaaaaaaaaaaaaaactaacctaactcctctataattaaacaaaaattaacctccaccaataccctatattccccctaacctaaatccaaaacaaacaatatccatttcaaaaaaacattaactcactaaaacaaaaataaaaataaatctaaaaccttatttctaaaacaaccaaaaaaataaaaaaaaaaaacacataaacaacccccaacacctctacctacaacgactccgataccccccaccccaaccttaccccaacaaaataaccacccacttcaaaattatcaacaaaaaaacctactaaaaaaatcttttctcccaaaacattctacctctctccaatctctacaataaaaaaaccacccaccctcaaacaaaaaaataaaactaaaacattctaaaaattcaaccttctacctaataatccttaaacccctaaaaaattcttcccacataaaacttatcttcttttactttcaaaaaaaaaaaacaaaaaaaaaccaacaaaaactaactaaccatatcttaacgctttacacatcaccctaaaatttcctattcacacttacttcaccaaaacaaaaactccttaaaaacaaaaattaataccctatttattcatctatttcctaaaaacactataacccactctctttaacaaacttctcgtaactacaaaacactacctttataataaataaacaaaaacaaaatctaaaaaattcaatctaaaaaaaaactcgaaaaatactaacataaacacaaataacaaaaaataaccacccaaaccgacccaaaaacctacgaacacaaatcactcgcatatttacaaaaactaccatacaaaactaaataccatacaaacctaaaaactaactcaacgtaaaacttcaaaaacacatcctaacccccaacctactcaatccgataacctaccctccacctccatacttcccttaacgattacacaactcctcaaactaaacttctcataactcaataaacaaccctcaaaaaataaattcccacaacgaacaactacgctaaccacccccaacccataaccccaaaatctcaaacccaatccaaaactaaaattctcaacctacaacaaaccataaaacccgaacccaactctaactcttacaacccaccctaaaaacgaaaaatcatctctaccataaatacctacctataacctaaataccaaaaacaaaaataacaatctataacctatacctacctttattctaaaacataaccaaaaaacatcctaaaacataaccaaaaaacatccccccttcccctattttctaaaaaccactacccaacccaaaactaataacccacgtaaccttactaaccaacaaaaaccaaaaaacccacctaatacgcaaaacctcaaatccttccaacaaccaaaacccctcaacttcctctacgcctaaaaaccaaaccccaacaccaaaaaacaaaaaaacgcttttcaacacctaaacaaaacccttaaaacctcccaaaaaaatctttctccactccctattcctaaactaaaactaaactctaaaaaatccaaaaatctacccaatttaaaaactaaaaaaaaaaacgctcaccgttaaaaaaaaaacgctaaataaaactaaaatacctaaaaatataacacaacctcttccccattcttaacctataaccccctccccacgcaaacctttcccacctccgcaccctcactcgaaaaatatcgccgctcaactaactaaaacgaactctcccaccacataaaacaccgacacaacccgcaacccctccctacaaccctcactaccccgacgaaaaaaaaacacaaaaacctctactctcatctaaataaatccgaaacacgtataatcccgcccgtcccgaccgaaaaaaatcaccctttcccgatcaacaaacacaaaaaccgcgaccgcaaacaaaaacgcgccgcaaactcgccaaaaaaacgaaacaacccgcgccgcaccccctccccaaaccgaacgaacgtacccgaccgcgaaatccccgcgacgccccgaaaacgctcctacctaacccgcgcgaacctccttctccaactcgcgataacgattataccacacgaaataatacaacgaatacttaccctcgaaccccttcctaacgaaaacgttaacgaaaatcatcgcccgctcctcataccgaaaccgcgacgcccgaccgaaaaaaaaaaacgacgccgaaaccgaaacccgaaaccgcgaaacgaaaaaccgacgctacctactcgcgaaactacgactcgaacatatacgaacgacgacgaacgaaaacgacgcgcccgacgcgatacgaacgacgcgaacgacgaacgtcctcgcgaaacgacgacgacgaacgacgcgaaaaaacccccacccgccctaaaaaaaaacgaacactcgacgacgctacgcgaactcgcgctcgcctcccacacccccgcacacaaaaacgccgctcgacgaaaaaaacaaacgcccgcaacgaacgcgaaaacgcacgaaacgcgaaccccgaaaacgccgccgcaaaaacgcgcgcccgcaacccccgaatccccacaactacataacccgaccctcaacccgaacgaccgacgcgaaatacgaaaatataaaaataataaaaaaaaaaaaaaaaaaccaaacgccccgaataaaacttatcaactcaaccccgcgacatcataaaatttataatccgcctcgtaaaactaaaaataacaaataaccgaaaaaaatctacactatccccgaatctcgtaaaaaaataaacgaaaaatcaaacctaacccaaacgcgaacgaaaccctaacgccaaataaactaaaacgcacctcccccgctaacattttaccttttactaaaaaaataaaaaaacacgaacctaaatcgaacgtttaaaaaacgaaataaaaatataatcttcaaaattaaacttaaatcccaaaaaccataaaaaaaaatccgaattcccaaaaaaaaacgtctaattaaaaactcctaaaaaaaatataaaacatcaataccaaaaatcattaaaacaaccaaaaatctaacccctaaaacatttctaaaaaatcttccctaccctattaaaaaattaaactccatcttccacacatatcattaaaaacaaaatatccaataacgcgaaaaaaataatccctttccccccgcacactatccccaacaaaaaccaaaataaaattaaacaaaaaaaacaacaaataacaactccgttcctccacccaactaacccttcaaaaaaaaaaataactaattccaaaaactatctccttcctaaataaccccaaaataaaaaaatacttccaaaataatccctacaaaaaatataataaaaattaaattaacctctcaaacgccaattacaaaacctaaaaaaaccaaaaaacttaaaccaatccctaaaaaaaaaaaactataatatcaaaaaaaccaaaattcgaataactccaactacctaaccttaaaaaaacaaactacttaatttttccgactttctcgatccactccccttcaaaataaaaatctaaatactacctcctaaaataaactaaaaataataactaccctaaaaacaacgcctccctcccccaaccaaacgaaccgaaacaaataacgaaaccaaacacgataccttcttaaacccacctcaaaacaaaacaaaaataaaaaattccacaccgaccctacttaaaacaacaatccaaaaaatatttatataaaaaataccaacaaaaacttacaaactctctcaaatttctttatataatcttccctccttcctcctccacaccctataataccaaaccccaacgaaaaaaaataaaaaaaaaacgaactacctcgcccctttctcccgcctaaaaaaaaccaactaacgtctccgaaaacccgaaaccgctacccgcctacaccaccaaaaatcaacaaaatatcgtaactacaaccaatacaaaaaaaaaaactaacgcgattaaaaaacatctaaaaataaccgaaaacatacctatacatttccttattaaattatttttcgaaccttatatataattccactataacaatcctacttcctaaaataataacatctccacgaaaaaatccaaaaacccttttatctccaatcccaaacccaaaaatttaactataacgaaactaaaaaaaacaaaatttaaacgatatatccgcgccaaaaccactcccaaataatctctaaaccaaccaaaaaataaaaaataaaataaaaaaataaacaaaataaatcatccttcttccccaacaaaacccaaaaatccgaaaacaaaaaaaattcaaaataaattataaaaaattatcgattataaaaaactatcccctaaacgaccgtattctttttttaccaaacgacgataaacactaaacccaaatcgcttacgcttcgacccgcgctctcaactaccacgtactcgaaacgcgcccacacaacgaaaaaacaaaaacaaccaaacgacaaaactaccaacaacctcctcgacatttaataaataaaattccataactaaaaatcgatcgaaaataaacgaacgaccaccgctcgtaaactaaacgcctaacacgaactacctaaccactcctcccgtctcactccccccgccccttacccccttcccgctaaaaccaccaaacccataaactctaataaaaaaacaactcgaaacgacaaataatactcccccctacacaccaactaaatatcgttacttacaaaaaccccaccaactaaacgactaactatcgaaaaaaaaaaaacctacaaaatttttttaaaatacaattataaataaaacccataaatcgcgatttcaaacaaacttatcaatctaaaccgcaacaaaaaacgataaaaacaactttacatatatttcgaataatataactcataaacattacttatctcccctaaaaaaaaaacctacccacccacaaatcactaccgctctaacaccgttaaaataatcgaccaacttaaacacccctaccaaaaaactacccccatcttaacaaacaaaaatctctaactcttaaaaaacccctcctcaattatcaccactaacctaacccccaaatctaaccctaaaaacctctaccctctccccacaaacaaaatacccgaaccttttactactacaaaaattaaaaattaaatacacgcgcgacacacgcgtataaaaacgcatactcaatacgaaaactacgctcatatacgacctctacctaaactccctaccccccaacccacccacgtccctcacctaccttacctttacctacctcgtcgtataaaatccaaaaaaaaaaaccgtcacctaaaacgacccctctatattatatacaccctttctaaacacacacacctctaataacccaaaaacaccgtaaatatatataaaacgaataacaaataaatataaatacacacaaacacaataatcactcctcgaaaaatctttaaaaaccgcccaaattctctcctctctaaataaaaaaatacataaaaaaataaatatatttttaatccgaaaacaaaaaaatacactacctaacctttctaacacctaaacgtccatattattaacaataaacgtattcaacaaaaatataacacatacacacacacccctaaacacacaaatataaacacctacgaaacaaaaacgcacacctcaccccaaccaaaaataaacgaataccccaaaacacaacccctttaacctaaaacgaaacttaaacctccaaatccttcttccctaatccccaccctcgccgtccgtaaacccaacgtcccccgatccaccccacgcgaaaaataaaaaaaaaaaaactataaaaataactcacattacctccgaaccaaacgaacgctacaacgaaaaccaaaaccgcaaaccacgctacccgccgaaaccgaacatctaccgcgacccctttaaac

SEQ ID NO: 9 - DNA, 24993 bp, Artificial Sequence
  G to A (bis2 rc)
acttaaaaaaaccgcgacaaatacccgaccccgacgaacaacgtaacctacgaccctaacctccgctacaacgctcgcctaacccgaaaacaatataaatcaccctcacaaccccctccccttcactttccgcgtaaaataaaccgaaaaacgctaaacccacgaacgacgaaaataaaaattaaaaaaaaaaaacttaaaaacccaaatcccgctccaaatcaaaaaaactataccttaaaatacccgtctatctctaattaaaataaaatatacgtccctatcccgtaaatatccacatctatatatccaaaaatatatatatatatatcacactcttactaaatacgcccactactaacaatataaacgcccaaataccaaaaaaatcaaacaatatattcccctacctccgaactaaaaatatatctatctctccatacatccttccatccaaaaaaaaaaaaatctaaacgatttttaaaaacctcccgaaaaataaccactatacctatatacactcacatccacttatcatccgccttacacacacccacgatatttctaaaccaccaaaaatatatatatccaaaaaaaatacatataacataaaaaaaccgtttcaaataacgacctttcttcctaaacttcacacgacgaaacaaacaaaaacaaaacaaataaaaaacgtaaataaactaaaaaacaaaaaacctaaataaaaaccgcacataaacgcaacccccgcactaaacatacgcccccatacgcgtataccgcgcgtatacccaacccccaatccctacaacaacaaaaaacccgaacactctacttataaaaaaaaaataaaaatccccaaaaccaaacctaaaaaccaaatcaataataacaattaaaaaaaaattctccaaaaatcaaaaactcctacttattaaaataaaaacaatcctttaacaaaaatactcaaattaatcgattatcccaacgataccaaaacgacaataatttataaataaacaaactccttccctaaaaaaaacaaataatactcataaatcacaccacccgaaatacatacaaaactacctccatcgccttttactacgacccaaattaacaaatttatttaaaatcgcgatccataaactttatttataattacaccttaaaaaaatcttacaaacctcccctccctcgacaaccaaccgctcaactaataaaacttttacaaacaacgatacctaactaatatataaaaaaaaacaccacctaccgccccgaactactctctcaccaaaatccataaacttaataacctcaacgaaaaaaaaataaaaaacgaaaaaaataaaacgaaaaaaataaccaaacaacccgtaccaaacgctcaatccacgaacgataaccgcccgttcacccccgatcgacccccaactataaaatttcatttattaaatatcgaaaaaactactaacaaccctaccgcttaactatctttatttctccgctatataaacgcgtctcgaacacgtaacaactaaaaacgcgaaccgaaacgcaaacgacctaaattcaatatctaccgccgcctaacaaaaaaaaaacacgaccgcccaaaaaacaattccccacaatcgacaactccccacaatccatcctaaactccccctatcctcgaactcctaaactttactaaaaaaaaaaaataattcactctacttacccctccaccccactccccatctcctaattaactcaaaaactacctaaaaataaccctaacgcgaacacatcgtccaaactttatttcccccaaccccgtcacaaccaaacttctaaacctaaaactaaaaataaaaaaatttctaaattcccccgtaaaaatatcaccaccccaaaaaacaaaactactacaataaaatcacacacaaaattcgaaaaacaatttaataaaaaaatacacaaacatactcccgaccactcctaaatacccctcaaccgcgccaaccccctcccctacactaactacaaccacgacactctactaacccctaataatacaaacgaacaacgatcccgaacccccgaaaacgccaactaactcctcccaaacgaaaaaaaaaaacgaaacaacccgctcctccctcatctcttcccgctaaaacctaacaccacaaaatataaaaaaaaaaaaaaaaaaaaccacacaaaaaaacctaaaaaaatttacaaacttttactaacacctcccacacaaacacttcttaaattattattttaaataaaaccgatataaaatcccttattcctaccttattctaaaataaactcaaaaaaacaccgtacctaatcccgccacctatctcgacccgcctaattaaaaaaaaaaaacgctatttccaaaacaatcattatccttaactcaccccaaaaaataatatctaaattctcattttaaaaaaaaataaaccgaaaaaatcgaaaaaattaaacaatttactcttttaaaatcaaacaattaaaactattcgaactctaatctctctaacatcacaatcccctccctccaaaaactaatccaaacctcttaatccttccaaaccttacaattaacgcttaaaaaaccaattcaacttttaccacaccctctacaaaaaccattctaaaaatacctcttcaccctaaaatcattcaaaaaaaaaacaatctctaaaatcaatcacttcccttcctaaaaaaccaactaaataaaaaaacgaaactaccacctactactttttctatccaacctcactctaattcttactaaaaacaatatacgaaaaaaaaaaaaccatctttcccgcgttactaaacattctatttccaataacatatataaaaaataaaatttaattttctaacaaaacaaaaaaaactcctcaaaaatattccaaaaaccaaacccctaactactccaataacccttaatactaataccccacacctttctcaaaaattcccaatcaaacgctctcttctaaaaatccgaatccttcttcataacccctaaaacccaaactcaattctaaaaaccacacctccaccccgtctcccaaacgctcgacctaaacccgtacccccccacttccccaacaaaaaacaaaataccaacgaaaaaaatacgtcccaacccacctaacgtcaaaaccccgcccgcgtctaaaccaaacctaactccccgcccactctcccacgaaatccgaaaacaatacaaaccctcttcgaccacctaccacccccaatttcacgaaacgaactacaaaccccataataccgcgaaactaaactaacaaactctacccgaaacgcctaatccccttcctctctccccatcatccccacatccccgtatcccgcgccgaccgctcgaactaaaaaccgaactatacaactataaaaacccgaaaactacgaacgcgcgtccctacgacgacgtccccgaaacccgcgtcccgtacgcccccgcgcccgctacgaacgcctactccctccgccgaacgacgtctttatatacgaaaatataaaaaacgaacgcgaatccgcgcaacgccgccgaatacccgctccctcccaaaacgaataaaaacctctccgcgccgcccgccgccgccgcctcgcgaaaacgcccgtcgcccgcgccgcccgcaccgcgccgaacgcgccgcccccgcccgccgccgctcgcacatacccgaaccgcaaccccgcgaacaaacaacgccgaccccccgccccgcgaccccgaaccccgactccgacgccgtccctcctccccgaccgaacgccgcgaccccgacataaaaaacgaacgataatccccgccaacgcctccgccaaaaaaaaacccgaaaacaaatatccgctacactacctcgtataacacaaccgccaccgcgaactaaaaaaaaaaatccgcgcgaaccaaataaaaacgccttcgaaacgccgcgaaaaccccgcgaccgaacacgcccgtccgacctaaaaaaaaaatacgacgcgaactatcccgcctccctaacgaatttacgacgcgtctttatttacgaccgcgacttttatacttattaaccgaaaaaaaataatcccctccgaccgaaacgaacgaaaccacacgtatttcgaactcacctaaataaaaataaaaacctctatacccctcctccgccgaaacaataaaaactacaaaaaaaaactacgaactatatcgatattccatataataaaaaaatccgccccaaccaattaaacgacgacacctcccgaataaaaatacgaaaataaaaaaaacttacgtaaaaaaaaaaccataaatcaaaaataaaaaaaaaactatatcacactcccaaacaccccaaccccacccaacgccctctccccaacgataaacgctttctcttttaactctcaaactaaacaaatccttaaatctctcaaaacccaaccccaactcaaaaacaaaaaataaaaaaaaaccctcttaaaaaaccccaaaaaccttatccaaatactaaaaaacgctctcctaccctctaatactaaaacctaatttctaaacgcaaaaaaaactaaaaaaccctaactactaaaaaaacttaaaattctacgcaccaaataaactccctaatttctactaatcaataaaaccacgtaaatcaccaactttaaactaaacaataatctccaaaaaacaaaaaaaaaaaaaatatcttctaaccatacttcaaaatatcttctaaccatacttcaaaacaaaaacaaacacaaatcacaaattaccacttctacccttaacacccaaaccacaaataaacactcataacaaaaataaccccccgcctccaaaataaactacaaaaaccaaaactaaacccgaatcccataacttactacaaactaaaaaccccaattttaaactaaatctaaaaccttaaaaccataaactaaaaataattaacgcaattacccgctataaaaatttaccttctaaaaactacttattaaatcataaaaaattcaatctaaaaaactatacaatcgccaaaaaaaacataaaaataaaaaacaaaccatcgaactaaacaaactaaaaatcaaaatatatctctaaaatcccacgctaaaccaacccccaaacctacataacatccaactctacataacaatccctataaatatacgaataacctatacccgcaaacctctaaaccgatctaaataaccacttcctattacctatacctataccaacactctccgaatttctcctcaaactaaactcctcaaaccctatctttatttatctatcataaaaacaatactctacaaccacgaaaaacctattaaaaaaaataaatcacaatacccccaaaaaacaaataaacaaacaaaacatcaacccctaccctcaaaaaatctctattctaataaaacaaatataaacaaaaaattccaaaataatatacaaaacgctaaaacataaccaaccaacctctactaactcttctctactttccttccctaaaaacaaaaaaaaacaaacctcatataaaaaaaacttcccaaaaatccaaaaatcactaaacaaaaaactaaatctccaaaatacctcaatcccactcccttacctaaaaataaataatccttttactacaaaaactaaaaaaaaacaaaataccctaaaaaaaaaaacttctccaacaaacctctctactaataatcctaaaataaataaccatcttactaaaataaaattaaaataaaaaacaccgaaaccgctacaaataaaaatattaaaaactactcatatatttctctctcccacccctctaactacctcaaaaacaaaatcccaaattcacccctacccctaccccaataaattaatatctccttaaaataaacactacctatcctaaatccaaaccaaaaaaaatataaaacactaataaaaattaacccttattcaaccacaaaaaaaccaaaccaatcctctccttccctcaaacgtaccaaaaaaaaaaataccactccgtataaataaaaaaattccctaactatctcccctctcgaaaactaacccaaaataaaacttatatccaaatatacactacctactccccaaaacaccaaactctattttctacaaaaaaaacctaaaaacaaccacctaacatcataaaaaaaacactataaaaccctaacatcccaaccaaaaatccctaacctctaatccccctaataccaaccgccacaaaaacaactcgactttcctcaaacactcaaaaaccaaatttccctaatcttaacttaacataactacctcttcttcactccaaaaaaaccccgcaaaaaccctccgtaaacaaacttaacaatacaactaactaaaaaaaaaaccaacataaccaccttcaaaacaaattaataaactttactcaaccccaaattactctactaaaaactaaaaacaaaaaataataaacaaataaaaaatacctaataaaaaaaaaaaacacccaacaatactataataccaacccgataccctacttaccgctatacatattctctaccaaatcgaaaaaaacaaaattataaaccaaaaaatataccaattcccccttacctaacataaccaactaaacataatcctaattctaaaatcgtaaattcctaatattccctaaaataaaaacaaaaaaaaaaattaacctatacaactcccgtaaaaaaaacatatataaactaaacctaaaaaacaaaactctacccctaacaaccaaaaccctaaaataaacaaattataatcccaaaaaatcattttccttctccctaaaacgttctccaccgtaaacttacttcctactttccctattcacccttctaacctaaaaacaaaaaaaataaattataaaacccaaaatatacgaaaaacacctcaaacccctccctttacctacactaaacaatcctaaatataaaacatcaccacaactaataaactaaaaaactcgaaaaaaaaaaccacaaaccccaaaaaccaaaaatcaatatattctaaaataaaaaaaaaaaactacaaaaacaaaataaaaaaaataacataaaaaaaaaaatccaaaatacgatccccacaacccgtaacctcctacgcaacttaaaaatacatcctacctccctccccttaaataaactcaaacaaacctacccctacaccccacgctaaacaaaaaaaatcaaacaacgactacaccaaactcctaccttcctcctcgtaaactaaaaaaaaaactaaacaaacaccaccttaaacacaaactctacgtccctcaccttcctcgcaaacactatatttaatccatacataaaatatatacttttcatacttcccttaacaaaaaaattctactcatactaaaaaaatttaaaaaataccctactaatacacataaatataaaaaatattcctatacaaatacgcacacacacgttacacaaaaataaactcctacaaaaccaaaaaacaactaaacatacatatacttatacacttaaaaacacacgtaaatacctataaacgtacgaatatatatctatataataccaatatatactaaaatataatatatatacctaaataaaaataaaaaaactctctacccaaaaacccccaactacaaaactccaaaaactccaccttttaactccaactaaaacctactaaaataaaaaatctccgttctcttaataaaaaaaactaaatattaaatttcataaaaaaccttttcattccaacaattaaataactaaaaacctctactaaaaaaaaactaaaaacctctactaaaaaaattaataaattctcctacctaaacccaaaacaaaataccacttacactacaaacgacactctaaacttataaaaaaaactactctaaaacttaactaaatatataaaattctacataaaatatataaaatactaaaccatccaaacctccctaaaaaatactcctaaaatataaaaataaaaaaaaacaccctacttacaaaaaaataccaaccgctctctaaaacctaaaactaaaacacctaataaaaaaataaaaacaacatctaaaaccctaaaaccaaacaacgacctaccaactccctaaaatcttattaactacaacgactacgactacaacatctaaaacaaaactaaaaaacctaaattactcaacacttccccaatcaactcgaaccctataaccctctcccactcccgctaccgaactcaaaaccccacccaaattacaaaccccgaaatccaacccaaccaaaattaaacaaaaataaacaacactccccttctctataaaaaaccacaactcaaaaaccaacaaaaaccaaacccgctaatttttttaaaactcccaatatattaaaaaataaaaaaattccaaaacaaaactataaaaattatataaataatcttaaattatttaaaatatttcatttttaacaataaaattcataatcatactttaaaatatttaactattactaaaaaatacgtaataaaaaacaatactccttactccgcctctcccacctccccaacactctaaactccttttatcatttacctccctaattataaacaatatattatttatactaccctctcccctccccttctccctccctccctcccttccctacctccctccctttctctttctttcttcttcttttttttcttttttcataaaacaacgtctcactctatcacccaaactaaaatacaataatataatcacaactcaatacaacctctacctcccaaactcaaataatcctcccatctcaacctcccaaaaaactaaaactacaaataataccaccatacctaactaatttttatatttttttttataaaaataaaatcttaccatattactcaaactaatctcgaactcctaaactcaaataatccacctactttaacctcccaaaatactaaaattacaaacgtaaaccccccgacataaacaatatacttctacaataatttcttaattaattaccttcccctccttataccccctcaacctaatactctatacatttatctaacaaatatttatataccaaatactacctaaaaaataaaaaaccaacaataaacaaaacaaacaaaaacctaactaataaaacttctattcgaaatacaaaaaatactcaacaaacacttaaacgaacaataaataaaaccataacaactattacctcaaataaactatcaaaataaacttttctaaaaaaataacatttaaacaacaacctaaataaaaaaaaaaaaaaaactttaaaactctctaaaaaatcctaaaaaacgttccgaaaaaaaccattaacgaaaaataaaacaaataaattcaaaaaaaaatctaaaaccattaaattccctactacctacgataaaaaaccactaaaaaattttaaactaaaaaatatcaaaacctaaataacacttcacaaaataactttaactaccataaataaaataaacaataaaacctaacaaccgaaaaacaacaaaaaaacaataaaaaactaccaataaaaaataaaaaaacaacaactacaaaataataaaaactaaacgacttctaaatctattttaaaaacaaaacctacaaatttttctaataaattaaatataaaaaatacgaaaaaaaaaaaaaatataaacaattttaaaattaatttttttttccacctaaaaatacaataaatccaaataatatttactatttataaaaacaaatacaactatccaaaaatacaaaaaacaaaaaaaaattaaaaaaatcacttccaaaataaaaaaaacaaaaaaaaaaacaaaaaacgtcataaaaaaccaaactatcccattttatttcataaattcaataatctttttatatttttcctaaaaatataaattactattttcccccaaaaaattttcttttattccctacatcaaaaaaatttcctctaaattcttaacatctaatttatttttttttttttttttttttttttttttaatacgaaatctcgctctatcccccgcgctaaaatacaataacgcaatctcgactcactacaaactccgcctcccgaattcacaccattctcctacctcaacctcccgaataactataactacaaacgcccgccaccacgcccaactaattttttatatttttaataaaaacgaaatttcaccgtattaaccaaaataatctcgatctcctaacctcgtaatccgcccacctcgacctcccaaaaaactaaaattacaaacgtaaaccactacacccaaccgtcttaacatctaatttatatattttaatttatttcacataaaaaactttcatcaaatatccaatttctcctaactattaaatcatatttaaaaataaaactaaaaaactcaaaaatatataaatactactataaaataatcaaataacaaactaacctattcattataaaatcaccaaatatctatattctaaaatctttaaaacaacttcctactcgaataaataaaataataataatataacctaactaccaataattcaaaacccaaataaaaaaaaaactaaaatttcacgaatcactaactttcaacaccatacctcatcctctactataaccaatactcctaaatccaaaacatctcatacccaatttctacaaaaaataaacccctaatatcctataataaaaaaaaaaaacatctcccaacttaataaaactaaaaaaaaaaccaaaaaatcctaaattataaccaacctccctacactcaactctaacttcacctccacctctaccatccccattacctacaaatcctacctacacctttcaaaaaaactaaaaatcacctaacttactccttatataaacgtttccctctataactactttaatttcaacttcctctactcccctaaatcaattataaaaccccaaccactttccatattctaaaattatattaaaatttctcatctactaacatctcttctctttattcttataaattttaaatattttactaacttttttttttttttttttttaaaacaaaatctaactttattacctaaactaaaatacaataaaataatctctactcactacaacctctaactccctaactcaaaaaatcctcccacctcaacctcccaataactaaaacgataaacatacaccaccacgcctaactaattttaatatttttttataacacaaaatttcaccacattacccacgctaatttcaaactcctaaactcaaataatctacccacctcgacctcccaaaacttacaaacataaaccactacgcccaacctaacattctttttttttttttttaaaacaaaatctctctctatcacccaaactaaaatacaataatacgatctctattcactacaacctccacctcccaaattcaaacgattcttatacctcaacctccctaataactaaaattacaaaaatcccccaccacgcccaactaatttttatatttttaataaaaataaaatttcaccatattaaccaaactaatctcaaactcctaacctctaataacctacccgcctcgacctcccaaaatactaaaattacaaacataaaccactatacctaacctcctaacattcttatacatttaacattttttaacactcttcaatcctttatacaaattcaaatttctatctaaaatcattttctttccacctaaaaaactccctttaacatttcctacacatctaacaataaattcccttaaaatttatttatctaccaacatatttatttcttcttcaattttaaaaaatattttcaccgaatataaaattctaaatcaataccaatcatactaaattaaaaaaaaaaaaaaaaaaaattctaaattaaaaatttttatttttatttttttcccccaacactttaaaaatttcattatattatttcctaacttacataatttctaataaaaaaaatataatatttcctatatctattcttccatacataataaacctcatttctttaaatacttttaaaattttctttttaccactaattttcaacatttaattataataaaccttaatataatttacttcgtatttatcttacttaaaattcattaaatttcttaattcttaactttatcttaatattaatttccacaacaaattactacaaactaaataaattaaaacaacaaatatttaaccgaatataataactcacgcctataatcccaacattttaaaaaaccgaaacgaacgaatcacgaaatcaaaaaatcgaaaccatactaactaacacgataaaaccccgtctctactaaaaatacaaaaaattaaccgaacgtaataataaatacctataatcccaactacttaaaaaactaaaacaaaaaaataacgtaaaccgaaaaaacgaaacttacaataaactaaaatcacgccactacactccaacctaaacgacaaaataaaattccatctcaaaaaaaaaaaaaaaaaatttattctatcacaattcgaaaaacataaatacaaatttaaaatattaacaaaataacaatccttccaaaaactctaaaaaaaaatcctaccttatctctttcaaattctaataactaaaccacaaccctcttaacttataactacaaaactctaatctctacctccgtcttcacataaccttcccacctctctaaatatcttaaaaaaacacctatcattaaatttaaaaccccctaaataatccaaaattatttcatcttaaaatccttaacttaattatatctacaaaaacccttttttaaaataaaatctcattcataaactataaaaatcaaaatataatataaacatatcttaaaaaaaacaccattcttcaacccaccataataatttttatcaaatttaaaaaaattttaaacgttctttctttcttttattatttatttacttattttaaaataaaatctccctctatcgcccaaactaaaatacaataacacgatctcgactcattacaacctccccttcccgaattcaaacgattctcctacctcaacccccaaataactaaaactacaaatacccaccaccacgcctaactaatttttatatttttaataaaaataaaatttcaccatattaaccaaactaatctcaaactcctaatattataatccacccgccttaacctcccaaaatactaaaattacaaacgtaaaccaccgcacccgacctatttctctaaatttatcttatttatcctacttctttattctatcctttaaaattccaataaatatatattacaatacttaataatatcttacaaattataaaactccataaaaacaaaatcttactctattacccaaactaaaatacaataacgtaatcataactcactacaacctcgaactcctaaactcaaaaaatcctcctacctcaacttcaaaaaaactaaaactacaactacttaccaccatacccaactaatataaaaattattttattttattttattttatttataaaaacaaaatcttactatattacctaaactaatcttaaactcctaaactcaaaccaacctcccgccttaacctccaaaaatactaaaactataaaaacccaaccaactttatttttcaatactatttttctcctctatacttcaatttaaaaaattctattactatcttcaaattcactaatttttaaattatacaatatctaatctactattatttccattcaataaatttttcatttcaattactatacttactatctttaaataatccactaaattcttttttatacctctcattcctctcctcataaacatctttttcatatttttctttaaactcttaaatatattaaaccatctatcatctttatcatttctaaattttatttctataaaattatttttctcctaattataaattatattttctttcttttttttttttttttaaaataaaatctctctctctattacccaaactaaaatacaaaaacgccatctcgactcactacaaactcgatctcctaacctcgtaatccacccgcctcaacctcccaaaatactaaaattacaaactcacgtaaaccaccgcaccctacctataaattttattttcctactttttaacatatctaataatttttaactaaattttaaacattataaatataatattaaacatctaaatttattattattctttaaaaaatattaaactttattcaaacaaactaaataaattacttacaaatcaatttaacctttttaaaacttttttttttaaaacaaaatcttactctatcacccaaacttaaatacaataaaacaatctcaactcattacaacctcaacctcctaaacttaaaaaatcctcctacctcaatcactaaataactaaaactacaaacacatactaccatacctaactaattttttatattttttataaacataaaattttaatatattacccaaactaatcttaaactcctaaactcaaataatctacctacctcaacctcccaaaatactaaaattaaaaatataaaccaccgtacctaacctttaatactaatttttctttttctttttcttttcttttcttttttttttttaaaataaaatcttactctatcacccaaaccaaaatataataatacaatcttaactcactacaacctccgcctcctaaattcaaataattcttatacctcaacctcctaaataactaaaattacaaacacccatcaccaaacccgactaattttttatatttttaataaaaatataatttcgccattttaaccaaactaatcttaaactcctaacctcaaataatctacccgcctccgcctcccaaaatactaaaattacaaacataaaccactacacccgacctaaaactaatttttaatctattaaaataaatctaaataaaccttttctctaaaaataatttaactctactactaaaacataacccttctaaaatctaattaaatatacatctccactctaaaaaactaaaacttaattatctccttacttttaataaactctaaaaatttaccattttattactcctttttatataatcttactaaatttcactatacacatataaaatttaatattcaaaaaaacttaaaaaaacccctatacaaatttctaaaattttttaaataatttactcttttccaaaactatactctactacaacctttaataccttaacttccctaaatcctatctccatcttctcaactcaaaaaaaacaccatactctactcgaacttcccctccttaaattacaatctaaaatattcctccaaacaaaaatccaaaaatattacaaaactcaccttattcattttccttacttcaaaaatcacaattctaaacttctaaaaacaactatttctctttacatatattttctatataaaaaaatatatatatatacacacacaaacacacacacacacacacatacacacacacatatatatatacacacacacgcatatatatatatatatttaaaacaacgtctcactctattacccaacctaaaatacaaaaatataataatacctcactacaacctcaacctcccaaacttaaacgatcctcccacctcaacctctaaataactaaaactacaaacacaaaccatcatacccgactaattcttttatattttttataaaaataaaattttaccatattacccaaactaatctctaactcctaaactcaaacaatccgccaacctttacctcccaaattactaaaattacaaaaataaacctctatacccaaccttcatatattttacaacaataattttctcattatttataataacaaaataatttcatttattataataaaaataaaaacctttttactaacgttttaatcaaattcaaaaaaaaaaaaaaaattacatacatataatcaattcactattccttttttttttaaaacgaaattttactcttatcgcccaaactaaaatacaataacataatctcgactcactacaacctccgcctcccgaattcaaacgattctcttacctcaacctcctaattaactaaaattacaaacataaaccaccacgcctaactaattttatatttttaataaaaataaaatttctccatattatcaaactaatctcgaactcccaacctcaaataatctacccgcctcgacctcccaaaatactaaaattacaaacgtaaactaccgcgcctaacctatcaattcactattcttaaccaaaaatcctaaactctcgaaatatatttaaatacttatacttaaaaccgaacgtaataactcacgcctataatcccaacactttaaaaaaccaaaacaaacgaatcacttaaaatcaaaaattaaaaaccaacctaaacaacatatcaaaaccccgtctctactaaaatacaaaaattaacctaacataataatactcgcctataatcccaactactcaaaaaactaaaacacaaaaatcgcttaaacctaaaaaacgaaaattacaataaaccaaaataacaccactacactctaacctaaataacacaataaaactctatctcaaaaaacaaacaaacaaacaaacaaacaaaacttacgtttaacaaacatactttctaaaccaaatacaaaaacttataatcccaactacttaaaaaactaaaacaaaaaaattactcaaacctaaaaatttaaaaccaacctaaataacataataaaaccctatctcaaataaaaaaaaaaaaaaaaaaaaaaaaaaaaaaaatcttttatctaaacactacgactcacacctataatcccaacactttaaaaacccgaaccaaataaatcacctaaaatcaaaaattcaaaactaacctaaccaacataataaaaacccatctctactaaaaatacaaaaaattaaccaaacgtattaacgaatatctataatcccaactacttaaaaaactaaaacaaaaaaatcgcttaaacctaaaaaacgaaaattacaacgaactaatatcacgtcattatactccaacctaaccaacaaaataaaactccgtccccccaaaaaaaacacaaaaaaaaaccccaaaaaaaacttttatcacttttatcacacaacaaaaatctcatacaatataatcatattattcacaaaattataaaatttatacaaattttaatacataatatcccacaaacacaaaacataattataaaattatattaataccataaacttattatttcattcctatctatatattactataaccgtttattaaacctcactcaataataatatcaataatctaaattaataactcttcctaaaaataacctaaaacccttaaaataaatctaatcccaaataaactccttaaccaacaacctctttaccaccccacttcaatcccaaacttattcttaacaaacaaaccactaaaccctaaaaaaaaaaacccaaccaaaaacccttaataaacaaaaaaaaaaaaaaccctccctcttccaaaattactttctatcctatcttctaaacccctttccatccacgtatctatctttccgttactcataatatctatctttccgttacccataatatctatctttccgttaccttataaaattaataaaacaaaacaaccccaacaaaaaataaaaattactacctactccaaaactatctaactccgaaaaactacctccgacgtaactaaaactttatcttccactcctcctcctcctccaaataaacatcgaacaactaaatccccgcgaccgaactcccctacacctaaccaccacgctaaaacaccttaaatatacccgtatactcctaacgcacgacgcaaacgtaaacaaaaaaaatcgcaacgactaaacaaataaacaaccctactcaccccaaccccacaaccgaaacctccccaacatcataaacctataattaactaaaaaatcctaccctataaccttacctcgccctcccccaatactccaaaaaactataaatacccgaaacctaaaactaatacaactaatacttcgataccgaaactaccaacgaataataaaacgactaacgaacatccccgtactcctaaaaaaactacgcaaaataaaacccaacctctcaacctccacgaaaacccttaaacccttctccaatacaaacttaacctctctccccttcgtcctccaaacccaaaacttctacgtaaaaataaaataaaaattcactaactaaaataaacgaactacaacaaatcgcttctaaactctcccactttaaatcctacgcttactcccctacctaaaatatattctcataattcttccgacgattccctctataccttaactcaactcaaaaccaccgcctcaactaaacctttccaaattaccccaaatactatcttaactccattattattctcttcactctatcataatttacttactatattcataacctaccgctccttattaaaaaataaactctaaaaaaacaaaaatcctatctttttcactattatattcccaataactaaaacactcaataaatatttcataaatatttattaaaaaaataaataaaaaaataaataaataaattaacaaataataaacactaaaaacttaataataacaaaaacatacccgtcccgacctcaaattactcttctatataaatataatctacactaaccaaaaaaaaaattttaaaaaaaaaactactctctcttcaattccctcccctattcctaaccacacgaatcccaaaccccataccctaaactaatccaaaccgtataaaccaaaccaatcaaaaccacctccaacctccgcttccaccaatacccctaatatccaaaatctaccctaataacacctacaaaatataaaaaaacgaccaaaacctaaaaataaacaccacactcctaaactttaaccacataacctaacaacgaaaaaaccgcaactttatcttcaaaaaccaaaatcaaacaaacaaaaaataaaacaaaataaaaacgataaaaaacaaccccaaaccacccctaatccccctatactattccgtatctaacaaacacaaacgccgtaatcataaaaattaaccacgaccgccgaataatatacacaaaaactctaacactaactaaacaaaaccgaaaactactactaactactactcaacccactaaaaaacaaatactaaaccgacttaccgcgcccgtcgtcaccactcaacttaacaccaaaaatatctcctttaaaaaataaataaacataaccttaatcacccttaaaccaacccgataaaatacctacctcacctaaaccactctacttccccaaaaacaaaactaacatcctaaactaacgcaataaaaaaacgaaaataataaataaatataaaactaaaataaaactacaactcccaactaccaacccaactacactcttacctacaacaaactatacaaaaaattctaacctcccttccccaaccctaaaaatacaaaaacaatacaacgtaatcaaacacttatatttaaattcaaaacacttctctaatattttatataaatatataaatatatacacaaaacacgtacacacgcacacacacacacacatttattcctcacaacaaccctttctaataaatactattctattaatattcccattttacgcatatttattaaatcctttccttaacatcccatttactcttcacaacaaccccaaaaaataaaaataatcgatccattttataataaaaaaataaaaacttaaaataattctataacctatacaaaatcacacaactattaaataacaaaattaaaattcaaatcctaactaacctaaccctaaaaccaaacctttatccctaaaaataactacctaactaaacataataactcatacctataatcccaacgctttaaaaaaccgaaataaacgaatcacctaaaatcaattcgaaaccaacctaactaacataataaaaccccgtctctactaacaatacaaaaaattaaccgaatataataacaaacgcctataatcccaactactcgaaaaactaaaacaaaaaaattacttaaacctaaaaaacgaaacttacaatatacaacgatcccgccacaacactccaacctaaacaacaaaacgaaactccatctaaaaaaaaaaaaaaaaaaaaactctacctattactctaaaacccctatattacccacgacataaaaacaaaaactaacaaataccataaattttatatataacatctcctctaaaaacctcccctacttctataatctaaaaaaacctctatactacccccaccaatacataaaccatactattataactccattttattatctccttataaaaattataaatctcaaaaaaacaaaaatcatatttaacttatttactatatccctaatacctacctcaatacctaacacataaaaactcctcaaaaaatatttattaaataaataaataaataaataaataaataaataacctcatatattcacttacccaaaaacctaaaacaaaatctctccaaaaccctttactacaaaaaatattcccaatacccttaaaaataaaacacaaaataaaaccaaaactacttataaaccctttcttcatctatccccaaatatataaaacatctaacgtaaaactcatcacccgcacacgaacaaaacatctttcaaaacaacacaaaaacaaaatcaaaaataataaaacaaaactaaataaaaaaaaatattacaaaactacgaaaaccaactcccacttcaatacttccatcaatattcccactaacatcctaacaaaaaactaaatactttattcaaaccgataaatttcaattcaaataccaaaccctaaaaataaataataactacctaaaatactaaaaaatttctaaaaactcatctaaattcaataaaaaaccatactacaaataattactaatattactattaaatttaaaaaaaaaaaaaaataccatatataccatttattaaccattctaatctaataaaacatatcctaaataaaaaatcaaaaaaccttaccacaaattctatatacccattaataccacacctaattctctaaataccaaataccgtatccgaaataaaaaaacataatttctacctcacaaaaaaacaacataaaatcatacctataaaaatacctaaaacaaacacacacacgcacatacacaccccacaatacctaccgaaacaaacgttttactatccaaaatcaccgaactaaaaaaaaacacttttaaaaattacttctaacctctaaaccttccttttaatattttaaactatactcacaaaaaccctaacccctaatccttaaaacactcaatccccttcaaataaaaatacctaaatatataattaaataaacaaaccccaccccaaaaaccgacctcctccctaaatcttaaatactatcacctctaataaaatacccaaatatatataaaattacgatatcctctaaaataccacatttcttataaactataaaacacctttacaatccttcctaaaaatcgctaaacaacacgaaaacccccaaaataaaataaatatatacaaaaatacccgtaaataaaaaaatataaatataactcaaaaaaaaacttaaaaaacgtcctacttaacataacctatataaacctcctttccacaatacccaaaaccatatcaacgccacactaacaaaaaaaacaacttaaaaaccttataacaacaaataaattaacctaacattaaaaactaaaaaaaactcctaaacccctccccatataatacaaaccctaatcactcaaactctaaaccaaaccaaccccactaccatcactacaaaaaaatacttcaaccccaactttaaactaaacaaccgtaatataaaccgccccataaaactaaccaccaaaacacaaaaataaaacccctaccgatactaaaaaaataaaaaaccgaaactccaaaaaatactaaaaaaccataacttcctacaatatcccttaccccttaaaatctaataaaaacaaattcaaaaccaaactataactatataaaaaacatcccctatccctatataaacaaataacccccatcattaacctcataaccgtcaacaatacgctttttaccaaactccgaaacttcatcaccctacgtctacctcctaacttcccaattaaaattaataaaaccgcacgaccatttctcctaaacccgtaacgaaccgaccgaaatttaaataaaatcgaaataaaactaaaactaaaatataaaaaactaaataataacgcctaaaaatttcctcatcctcaaaaatcccgatcttccacatcctcaacgcccgcatcaccttcgaaaacctcaacgactacgacgaaccgataccatcgatacgaaacaaccccaacaacgaaacgccttccccaaacaacgactcctccaacgtcaacaactccaactccacgaataaaaccccccgcgaaaacgcctacccctcgactctccccgaaataaataaaaaaaacgcgcccgaccgtacctaacccaacccccgcgcccccaacctcctaccgcgactacgaaatctccccaacgttattcgaaaccccgcgcgactacaacataataaacgaccaacgaaaaacgacgacccgaaacgacgacgacgacctactacaattcgccatccaacaaaacctacttaaaacgaacaataaatataaccaaatacgtctccgcgaacgcgcgaaaccacgaaactccgcgccgccacgactaacgcccacgcctccccgcaaatcaccatctaaaaaacgctaaccaacaacaaaccaaacacccaccccatatcctacgaaaatcgccgacaaaacaaatcaatacccgctaaaccgaaaaaaatcctccgaaaaaaatcctatctcccctaaaccaaaacacaaccgaaaaacccgcgaaaccctcgacaaaaaccctcctaatatcgaaataacttctaccaccactcctacctccgaaacgacaaacaaaaatcaaaaatccaaacttcaccgcgaaattcaaactctccccaaacattaacgaaaaaaacttaataaaatctaaactccgccacgaccaaataaaaaccaaaacgccgcgaaactaaccgcctccactaaaaaataataaccgcgaaccgccctaaaacctccacgccgtatcccgaccccgaccgataaataaatacgcccgaaaacccgcgacattccttccccacccccaaaaacgccccgcccacgccgcaacgccaacctacgcccccgacgtcaatacccaaccctcgacccaactcaaaaccaaattccgacgaccacgtattccgaaactacgacgaacaactacgactaacgataaaactatcgacgcaaaaacaaaaaaaaaaacgacgacgcgcgcgccaaaaaaaaaaaaaactaaaacgcatcctaaaactctcactaaccgaacaataacgccccctaccgaaaccctcgccaacgccacgcgcgccacgcccaaaaccaaaaaccaaacaaaccccgacctacgcgcctacaaaacgacgactaaaaactaaaaccaccgcctcgcgaatacaacaacacaacaaacacgattcgaaaaaaaattcgacataaccgcgaaataccttcccaaaccaaaaccctaaaaacaactaacacgacctaatccccctactttactatattctaattccccaacccgctcccctaaactcaaatctatcctatcctaaaacgaaaccaaacgatcctaaaaaaaaaataaatccttaaaaaaacgctatccctatcccttactccttctaaccgatccgcatttctattcactaaccccactccaaaacactacccctaaaacctttacatctctactcttcactcctaaaaaacaactaaactccccgcgtactatatcactactttattccaaacacaaaccaacacgtctaaaacccaacccctcccccaccccgacatttcaacgtcaaatacacttaacgaaatacccgactcccccaacccccacacccgtcctaaatctcaaaataattccaacttctccttaaacaaccaaaaattaaaatcccatcccccaaaacacatttttttttttttttttttataatcaaaaaatatatccaacgtaaccccctaacctatacaaaccctaactccctcataatacctcgaaaaataaaaaacatattaaactaaaataaacactaaacccaaataaactaaacacaaaaaactcgcccaaaaccctaacgccacccccaccccttcccaccaactactactaacctctataattatacatcccacttacccccacacgaaaactaactctaaaacccttcatccaataatactaacccccgactctcccctaccccacctcacccacccaaaaaaacacaaaccccgccaaaaacaaaaacccaccgcacacccttatcccgaacctatctaaaactaaccttcccgactcaaccaataaaactcaaaaaaaacacaaaaaaaaataaaaaaaaaaaacaaaaaaaaactattcctcccacccccttccctaataccaaaaacaccaaactaattctaaaacacaaataaaaaaaacttcataccgaa

SEQ ID NO: 10 - DNA, 24993 bp, Artificial Sequence
  G to A (bis2 rc) rc
ttcggtatgaagttttttttatttgtgttttagaattagtttggtgtttttggtattagggaagggggtgggaggaatagtttttttttgttttttttttttatttttttttgtgttttttttgagttttattggttgagtcgggaaggttagttttagataggttcgggataagggtgtgcggtgggtttttgtttttggcggggtttgtgtttttttgggtgggtgaggtggggtaggggagagtcgggggttagtattattggatgaagggttttagagttagttttcgtgtgggggtaagtgggatgtataattatagaggttagtagtagttggtgggaaggggtgggggtggcgttagggttttgggcgagttttttgtgtttagtttatttgggtttagtgtttattttagtttaatatgttttttatttttcgaggtattatgagggagttagggtttgtataggttagggggttacgttggatatattttttgattataaaaaaaaaaaaaaaaaaatgtgttttgggggatgggattttaatttttggttgtttaaggagaagttggaattattttgagatttaggacgggtgtgggggttgggggagtcgggtatttcgttaagtgtatttgacgttgaaatgtcggggtgggggaggggttgggttttagacgtgttggtttgtgtttggaataaagtagtgatatagtacgcggggagtttagttgttttttaggagtgaagagtagagatgtaaaggttttaggggtagtgttttggagtggggttagtgaatagaaatgcggatcggttagaaggagtaagggatagggatagcgtttttttaaggatttattttttttttaggatcgtttggtttcgttttaggataggatagatttgagtttaggggagcgggttggggaattagaatatagtaaagtagggggattaggtcgtgttagttgtttttagggttttggtttgggaaggtatttcgcggttatgtcgaattttttttcgaatcgtgtttgttgtgttgttgtattcgcgaggcggtggttttagtttttagtcgtcgttttgtaggcgcgtaggtcggggtttgtttggtttttggttttgggcgtggcgcgcgtggcgttggcgagggtttcggtagggggcgttattgttcggttagtgagagttttaggatgcgttttagttttttttttttttggcgcgcgcgtcgtcgtttttttttttgtttttgcgtcgatagttttatcgttagtcgtagttgttcgtcgtagtttcggaatacgtggtcgtcggaatttggttttgagttgggtcgagggttgggtattgacgtcgggggcgtaggttggcgttgcggcgtgggcggggcgtttttgggggtggggaaggaatgtcgcgggttttcgggcgtatttatttatcggtcggggtcgggatacggcgtggaggttttagggcggttcgcggttattattttttagtggaggcggttagtttcgcggcgttttggtttttatttggtcgtggcggagtttagattttattaagtttttttcgttaatgtttggggagagtttgaatttcgcggtgaagtttggatttttgatttttgtttgtcgtttcggaggtaggagtggtggtagaagttatttcgatattaggagggtttttgtcgagggtttcgcgggtttttcggttgtgttttggtttaggggagataggatttttttcggaggatttttttcggtttagcgggtattgatttgttttgtcggcgattttcgtaggatatggggtgggtgtttggtttgttgttggttagcgttttttagatggtgatttgcggggaggcgtgggcgttagtcgtggcggcgcggagtttcgtggtttcgcgcgttcgcggagacgtatttggttatatttattgttcgttttaagtaggttttgttggatggcgaattgtagtaggtcgtcgtcgtcgtttcgggtcgtcgtttttcgttggtcgtttattatgttgtagtcgcgcggggtttcgaataacgttggggagatttcgtagtcgcggtaggaggttgggggcgcgggggttgggttaggtacggtcgggcgcgttttttttatttatttcggggagagtcgaggggtaggcgttttcgcggggggttttattcgtggagttggagttgttgacgttggaggagtcgttgtttggggaaggcgtttcgttgttggggttgtttcgtatcgatggtatcggttcgtcgtagtcgttgaggttttcgaaggtgatgcgggcgttgaggatgtggaagatcgggatttttgaggatgaggaaatttttaggcgttattatttagttttttatattttagttttagttttatttcgattttatttaaatttcggtcggttcgttacgggtttaggagaaatggtcgtgcggttttattaattttaattgggaagttaggaggtagacgtagggtgatgaagtttcggagtttggtaaaaagcgtattgttgacggttatgaggttaatgatgggggttatttgtttatatagggataggggatgttttttatatagttatagtttggttttgaatttgtttttattagattttaaggggtaagggatattgtaggaagttatggttttttagtattttttggagtttcggttttttatttttttagtatcggtaggggttttatttttgtgttttggtggttagttttatggggcggtttatattacggttgtttagtttaaagttggggttgaagtatttttttgtagtgatggtagtggggttggtttggtttagagtttgagtgattagggtttgtattatatggggaggggtttaggagttttttttagtttttaatgttaggttaatttatttgttgttataaggtttttaagttgttttttttgttagtgtggcgttgatatggttttgggtattgtggaaaggaggtttatataggttatgttaagtaggacgttttttaagtttttttttgagttatatttatatttttttatttacgggtatttttgtatatatttattttattttgggggttttcgtgttgtttagcgatttttaggaaggattgtaaaggtgttttatagtttataagaaatgtggtattttagaggatatcgtaattttatatatatttgggtattttattagaggtgatagtatttaagatttagggaggaggtcggtttttggggtggggtttgtttatttaattatatatttaggtatttttatttgaaggggattgagtgttttaaggattaggggttagggtttttgtgagtatagtttaaaatattaaaaggaaggtttagaggttagaagtaatttttaaaagtgtttttttttagttcggtgattttggatagtaaaacgtttgtttcggtaggtattgtggggtgtgtatgtgcgtgtgtgtgtttgttttaggtatttttataggtatgattttatgttgtttttttgtgaggtagaaattatgtttttttatttcggatacggtatttggtatttagagaattaggtgtggtattaatgggtatatagaatttgtggtaaggttttttgattttttatttaggatatgttttattagattagaatggttaataaatggtatatatggtatttttttttttttttaaatttaatagtaatattagtaattatttgtagtatggttttttattgaatttagatgagtttttagaaattttttagtattttaggtagttattatttatttttagggtttggtatttgaattgaaatttatcggtttgaataaagtatttagttttttgttaggatgttagtgggaatattgatggaagtattgaagtgggagttggttttcgtagttttgtaatatttttttttatttagttttgttttattatttttgattttgtttttgtgttgttttgaaagatgttttgttcgtgtgcgggtgatgagttttacgttagatgttttatatatttggggatagatgaagaaagggtttataagtagttttggttttattttgtgttttatttttaagggtattgggaatattttttgtagtaaagggttttggagagattttgttttaggtttttgggtaagtgaatatatgaggttatttatttatttatttatttatttatttatttaataaatattttttgaggagtttttatgtgttaggtattgaggtaggtattagggatatagtaaataagttaaatatgatttttgtttttttgagatttataatttttataaggagataataaaatggagttataatagtatggtttatgtattggtgggggtagtatagaggtttttttagattatagaagtaggggaggtttttagaggagatgttatatataaaatttatggtatttgttagtttttgtttttatgtcgtgggtaatataggggttttagagtaataggtagagtttttttttttttttttttttagatggagtttcgttttgttgtttaggttggagtgttgtggcgggatcgttgtatattgtaagtttcgttttttaggtttaagtaatttttttgttttagtttttcgagtagttgggattataggcgtttgttattatattcggttaattttttgtattgttagtagagacggggttttattatgttagttaggttggtttcgaattgattttaggtgattcgtttatttcggttttttaaagcgttgggattataggtatgagttattatgtttagttaggtagttatttttagggataaaggtttggttttagggttaggttagttaggatttgaattttaattttgttatttaatagttgtgtgattttgtataggttatagaattattttaagtttttatttttttattataaaatggatcgattatttttattttttggggttgttgtgaagagtaaatgggatgttaaggaaaggatttaataaatatgcgtaaaatgggaatattaatagaatagtatttattagaaagggttgttgtgaggaataaatgtgtgtgtgtgtgtgcgtgtgtacgtgttttgtgtatatatttatatatttatataaaatattagagaagtgttttgaatttaaatataagtgtttgattacgttgtattgtttttgtatttttagggttggggaagggaggttagaattttttgtatagtttgttgtaggtaagagtgtagttgggttggtagttgggagttgtagttttattttagttttatatttatttattattttcgtttttttattgcgttagtttaggatgttagttttgtttttggggaagtagagtggtttaggtgaggtaggtattttatcgggttggtttaagggtgattaaggttatgtttatttattttttaaaggagatatttttggtgttaagttgagtggtgacgacgggcgcggtaagtcggtttagtatttgttttttagtgggttgagtagtagttagtagtagttttcggttttgtttagttagtgttagagtttttgtgtatattattcggcggtcgtggttaatttttatgattacggcgtttgtgtttgttagatacggaatagtatagggggattaggggtggtttggggttgttttttatcgtttttattttgttttattttttgtttgtttgattttggtttttgaagataaagttgcggttttttcgttgttaggttatgtggttaaagtttaggagtgtggtgtttatttttaggttttggtcgtttttttatattttgtaggtgttattagggtagattttggatattaggggtattggtggaagcggaggttggaggtggttttgattggtttggtttatacggtttggattagtttagggtatggggtttgggattcgtgtggttaggaataggggagggaattgaagagagagtagttttttttttaaaattttttttttggttagtgtagattatatttatatagaagagtaatttgaggtcgggacgggtatgtttttgttattattaagtttttagtgtttattatttgttaatttatttatttatttttttatttatttttttaataaatatttatgaaatatttattgagtgttttagttattgggaatataatagtgaaaaagataggatttttgtttttttagagtttattttttaataaggagcggtaggttatgaatatagtaagtaaattatgatagagtgaagagaataataatggagttaagatagtatttggggtaatttggaaaggtttagttgaggcggtggttttgagttgagttaaggtatagagggaatcgtcggaagaattatgagaatatattttaggtaggggagtaagcgtaggatttaaagtgggagagtttagaagcgatttgttgtagttcgtttattttagttagtgaatttttattttatttttacgtagaagttttgggtttggaggacgaaggggagagaggttaagtttgtattggagaagggtttaagggttttcgtggaggttgagaggttgggttttattttgcgtagtttttttaggagtacggggatgttcgttagtcgttttattattcgttggtagtttcggtatcgaagtattagttgtattagttttaggtttcgggtatttatagttttttggagtattgggggagggcgaggtaaggttatagggtaggattttttagttaattataggtttatgatgttggggaggtttcggttgtggggttggggtgagtagggttgtttatttgtttagtcgttgcgattttttttgtttacgtttgcgtcgtgcgttaggagtatacgggtatatttaaggtgttttagcgtggtggttaggtgtaggggagttcggtcgcggggatttagttgttcgatgtttatttggaggaggaggaggagtggaagataaagttttagttacgtcggaggtagtttttcggagttagatagttttggagtaggtagtaatttttattttttgttggggttgttttgttttattaattttataaggtaacggaaagatagatattatgggtaacggaaagatagatattatgagtaacggaaagatagatacgtggatggaaaggggtttagaagataggatagaaagtaattttggaagagggagggttttttttttttttgtttattaagggtttttggttgggtttttttttttagggtttagtggtttgtttgttaagaataagtttgggattgaagtggggtggtaaagaggttgttggttaaggagtttatttgggattagatttattttaagggttttaggttatttttaggaagagttattaatttagattattgatattattattgagtgaggtttaataaacggttatagtaatatatagataggaatgaaataataagtttatggtattaatataattttataattatgttttgtgtttgtgggatattatgtattaaaatttgtataaattttataattttgtgaataatatgattatattgtatgagatttttgttgtgtgataaaagtgataaaagttttttttggggtttttttttgtgttttttttggggggacggagttttattttgttggttaggttggagtataatgacgtgatattagttcgttgtaattttcgttttttaggtttaagcgatttttttgttttagttttttaagtagttgggattatagatattcgttaatacgtttggttaattttttgtatttttagtagagatgggtttttattatgttggttaggttagttttgaatttttgattttaggtgatttatttggttcgggtttttaaagtgttgggattataggtgtgagtcgtagtgtttagataaaagattttttttttttttttttttttttttttttttatttgagatagggttttattatgttatttaggttggttttaaatttttaggtttgagtaatttttttgttttagttttttaagtagttgggattataagtttttgtatttggtttagaaagtatgtttgttaaacgtaagttttgtttgtttgtttgtttgtttgttttttgagatagagttttattgtgttatttaggttagagtgtagtggtgttattttggtttattgtaattttcgttttttaggtttaagcgatttttgtgttttagttttttgagtagttgggattataggcgagtattattatgttaggttaatttttgtattttagtagagacggggttttgatatgttgtttaggttggtttttaatttttgattttaagtgattcgtttgttttggttttttaaagtgttgggattataggcgtgagttattacgttcggttttaagtataagtatttaaatatatttcgagagtttaggatttttggttaagaatagtgaattgataggttaggcgcggtagtttacgtttgtaattttagtattttgggaggtcgaggcgggtagattatttgaggttgggagttcgagattagtttgataatatggagaaattttatttttattaaaaatataaaattagttaggcgtggtggtttatgtttgtaattttagttaattaggaggttgaggtaagagaatcgtttgaattcgggaggcggaggttgtagtgagtcgagattatgttattgtattttagtttgggcgataagagtaaaatttcgttttaaaaaaaaaaggaatagtgaattgattatatgtatgtaattttttttttttttttgaatttgattaaaacgttagtaaaaaggtttttatttttattataataaatgaaattattttgttattataaataatgagaaaattattgttgtaaaatatatgaaggttgggtatagaggtttatttttgtaattttagtaatttgggaggtaaaggttggcggattgtttgagtttaggagttagagattagtttgggtaatatggtaaaattttatttttataaaaaatataaaagaattagtcgggtatgatggtttgtgtttgtagttttagttatttagaggttgaggtgggaggatcgtttaagtttgggaggttgaggttgtagtgaggtattattatatttttgtattttaggttgggtaatagagtgagacgttgttttaaatatatatatatatatgcgtgtgtgtgtatatatatatgtgtgtgtgtatgtgtgtgtgtgtgtgtgtttgtgtgtgtatatatatatatttttttatatagaaaatatatgtaaagagaaatagttgtttttagaagtttagaattgtgatttttgaagtaaggaaaatgaataaggtgagttttgtaatatttttggatttttgtttggaggaatattttagattgtaatttaaggaggggaagttcgagtagagtatggtgttttttttgagttgagaagatggagataggatttagggaagttaaggtattaaaggttgtagtagagtatagttttggaaaagagtaaattatttaaaaaattttagaaatttgtataggggtttttttaagtttttttgaatattaaattttatatgtgtatagtgaaatttagtaagattatataaaaaggagtaataaaatggtaaatttttagagtttattaaaagtaaggagataattaagttttagttttttagagtggagatgtatatttaattagattttagaagggttatgttttagtagtagagttaaattatttttagagaaaaggtttatttagatttattttaatagattaaaaattagttttaggtcgggtgtagtggtttatgtttgtaattttagtattttgggaggcggaggcgggtagattatttgaggttaggagtttaagattagtttggttaaaatggcgaaattatatttttattaaaaatataaaaaattagtcgggtttggtgatgggtgtttgtaattttagttatttaggaggttgaggtataagaattatttgaatttaggaggcggaggttgtagtgagttaagattgtattattatattttggtttgggtgatagagtaagattttattttaaaaaaaaaaaagaaaagaaaagaaaaagaaaaagaaaaattagtattaaaggttaggtacggtggtttatatttttaattttagtattttgggaggttgaggtaggtagattatttgagtttaggagtttaagattagtttgggtaatatattaaaattttatgtttataaaaaatataaaaaattagttaggtatggtagtatgtgtttgtagttttagttatttagtgattgaggtaggaggattttttaagtttaggaggttgaggttgtaatgagttgagattgttttattgtatttaagtttgggtgatagagtaagattttgttttaaaaaaaaaagttttaaaaaggttaaattgatttgtaagtaatttatttagtttgtttgaataaagtttaatattttttaaagaataataataaatttagatgtttaatattatatttataatgtttaaaatttagttaaaaattattagatatgttaaaaagtaggaaaataaaatttataggtagggtgcggtggtttacgtgagtttgtaattttagtattttgggaggttgaggcgggtggattacgaggttaggagatcgagtttgtagtgagtcgagatggcgtttttgtattttagtttgggtaatagagagagagattttattttaaaaaaaaaaaaaaaagaaagaaaatataatttataattaggagaaaaataattttatagaaataaaatttagaaatgataaagatgatagatggtttaatatatttaagagtttaaagaaaaatatgaaaaagatgtttatgaggagaggaatgagaggtataaaaaagaatttagtggattatttaaagatagtaagtatagtaattgaaatgaaaaatttattgaatggaaataatagtagattagatattgtataatttaaaaattagtgaatttgaagatagtaatagaattttttaaattgaagtatagaggagaaaaatagtattgaaaaataaagttggttgggtttttatagttttagtatttttggaggttaaggcgggaggttggtttgagtttaggagtttaagattagtttaggtaatatagtaagattttgtttttataaataaaataaaataaaataaaataatttttatattagttgggtatggtggtaagtagttgtagttttagtttttttgaagttgaggtaggaggattttttgagtttaggagttcgaggttgtagtgagttatgattacgttattgtattttagtttgggtaatagagtaagattttgtttttatggagttttataatttgtaagatattattaagtattgtaatatatatttattggaattttaaaggatagaataaagaagtaggataaataagataaatttagagaaataggtcgggtgcggtggtttacgtttgtaattttagtattttgggaggttaaggcgggtggattataatattaggagtttgagattagtttggttaatatggtgaaattttatttttattaaaaatataaaaattagttaggcgtggtggtgggtatttgtagttttagttatttgggggttgaggtaggagaatcgtttgaattcgggaaggggaggttgtaatgagtcgagatcgtgttattgtattttagtttgggcgatagagggagattttattttaaaataagtaaataaataataaaagaaagaaagaacgtttaaaatttttttaaatttgataaaaattattatggtgggttgaagaatggtgttttttttaagatatgtttatattatattttgatttttatagtttatgaatgagattttattttaaaaaagggtttttgtagatataattaagttaaggattttaagatgaaataattttggattatttagggggttttaaatttaatgataggtgtttttttaagatatttagagaggtgggaaggttatgtgaagacggaggtagagattagagttttgtagttataagttaagagggttgtggtttagttattagaatttgaaagagataaggtaggatttttttttagagtttttggaaggattgttattttgttaatattttaaatttgtatttatgtttttcgaattgtgatagaataaattttttttttttttttttgagatggaattttattttgtcgtttaggttggagtgtagtggcgtgattttagtttattgtaagtttcgttttttcggtttacgttatttttttgttttagttttttaagtagttgggattataggtatttattattacgttcggttaattttttgtatttttagtagagacggggttttatcgtgttagttagtatggtttcgattttttgatttcgtgattcgttcgtttcggttttttaaaatgttgggattataggcgtgagttattatattcggttaaatatttgttgttttaatttatttagtttgtagtaatttgttgtggaaattaatattaagataaagttaagaattaagaaatttaatgaattttaagtaagataaatacgaagtaaattatattaaggtttattataattaaatgttgaaaattagtggtaaaaagaaaattttaaaagtatttaaagaaatgaggtttattatgtatggaagaatagatataggaaatattatattttttttattagaaattatgtaagttaggaaataatataatgaaatttttaaagtgttgggggaaaaaaataaaaataaaaatttttaatttagaattttttttttttttttttttaatttagtatgattggtattgatttagaattttatattcggtgaaaatattttttaaaattgaagaagaaataaatatgttggtagataaataaattttaagggaatttattgttagatgtgtaggaaatgttaaagggagttttttaggtggaaagaaaatgattttagatagaaatttgaatttgtataaaggattgaagagtgttaaaaaatgttaaatgtataagaatgttaggaggttaggtatagtggtttatgtttgtaattttagtattttgggaggtcgaggcgggtaggttattagaggttaggagtttgagattagtttggttaatatggtgaaattttatttttattaaaaatataaaaattagttgggcgtggtgggggatttttgtaattttagttattagggaggttgaggtataagaatcgtttgaatttgggaggtggaggttgtagtgaatagagatcgtattattgtattttagtttgggtgatagagagagattttgttttaaaaaaaaaaaaaaagaatgttaggttgggcgtagtggtttatgtttgtaagttttgggaggtcgaggtgggtagattatttgagtttaggagtttgaaattagcgtgggtaatgtggtgaaattttgtgttataaaaaaatattaaaattagttaggcgtggtggtgtatgtttatcgttttagttattgggaggttgaggtgggaggattttttgagttagggagttagaggttgtagtgagtagagattattttattgtattttagtttaggtaataaagttagattttgttttaaaaaaaaaaaaaaaaaaaagttagtaaaatatttaaaatttataagaataaagagaagagatgttagtagatgagaaattttaatataattttagaatatggaaagtggttggggttttataattgatttaggggagtagaggaagttgaaattaaagtagttatagagggaaacgtttatataaggagtaagttaggtgatttttagtttttttgaaaggtgtaggtaggatttgtaggtaatggggatggtagaggtggaggtgaagttagagttgagtgtagggaggttggttataatttaggattttttggttttttttttagttttattaagttgggagatgttttttttttttattataggatattaggggtttattttttgtagaaattgggtatgagatgttttggatttaggagtattggttatagtagaggatgaggtatggtgttgaaagttagtgattcgtgaaattttagttttttttttatttgggttttgaattattggtagttaggttatattattattattttatttattcgagtaggaagttgttttaaagattttagaatatagatatttggtgattttataatgaataggttagtttgttatttgattattttatagtagtatttatatatttttgagttttttagttttatttttaaatatgatttaatagttaggagaaattggatatttgatgaaagttttttatgtgaaataaattaaaatatataaattagatgttaagacggttgggtgtagtggtttacgtttgtaattttagttttttgggaggtcgaggtgggcggattacgaggttaggagatcgagattattttggttaatacggtgaaatttcgtttttattaaaaatataaaaaattagttgggcgtggtggcgggcgtttgtagttatagttattcgggaggttgaggtaggagaatggtgtgaattcgggaggcggagtttgtagtgagtcgagattgcgttattgtattttagcgcgggggatagagcgagatttcgtattaaaaaaaaaaaaaaaaaaaaaaaaaaaaataaattagatgttaagaatttagaggaaatttttttgatgtagggaataaaagaaaattttttgggggaaaatagtaatttatatttttaggaaaaatataaaaagattattgaatttatgaaataaaatgggatagtttggttttttatgacgttttttgtttttttttttgttttttttattttggaagtgatttttttaatttttttttgttttttgtatttttggatagttgtatttgtttttataaatagtaaatattatttggatttattgtatttttaggtggaaaaaaaaattaattttaaaattgtttatattttttttttttttcgtattttttatatttaatttattagaaaaatttgtaggttttgtttttaaaatagatttagaagtcgtttagtttttattattttgtagttgttgtttttttattttttattggtagttttttattgtttttttgttgtttttcggttgttaggttttattgtttattttatttatggtagttaaagttattttgtgaagtgttatttaggttttgatattttttagtttaaaattttttagtggttttttatcgtaggtagtagggaatttaatggttttagatttttttttgaatttatttgttttatttttcgttaatggtttttttcggaacgttttttaggattttttagagagttttaaagttttttttttttttttatttaggttgttgtttaaatgttatttttttagaaaagtttattttgatagtttatttgaggtaatagttgttatggttttatttattgttcgtttaagtgtttgttgagtattttttgtatttcgaatagaagttttattagttaggtttttgtttgttttgtttattgttggttttttattttttaggtagtatttggtatataaatatttgttagataaatgtatagagtattaggttgagggggtataaggaggggaaggtaattaattaagaaattattgtagaagtatattgtttatgtcggggggtttacgtttgtaattttagtattttgggaggttaaagtaggtggattatttgagtttaggagttcgagattagtttgagtaatatggtaagattttatttttataaaaaaaaatataaaaattagttaggtatggtggtattatttgtagttttagttttttgggaggttgagatgggaggattatttgagtttgggaggtagaggttgtattgagttgtgattatattattgtattttagtttgggtgatagagtgagacgttgttttatgaaaaaagaaaaaaaagaagaagaaagaaagagaaagggagggaggtagggaagggagggagggagggagaaggggaggggagagggtagtataaataatatattgtttataattagggaggtaaatgataaaaggagtttagagtgttggggaggtgggagaggcggagtaaggagtattgttttttattacgtattttttagtaatagttaaatattttaaagtatgattatgaattttattgttaaaaatgaaatattttaaataatttaagattatttatataatttttatagttttgttttggaatttttttattttttaatatattgggagttttaaaaaaattagcgggtttggtttttgttggtttttgagttgtggttttttatagagaaggggagtgttgtttatttttgtttaattttggttgggttggatttcggggtttgtaatttgggtggggttttgagttcggtagcgggagtgggagagggttatagggttcgagttgattggggaagtgttgagtaatttaggttttttagttttgttttagatgttgtagtcgtagtcgttgtagttaataagattttagggagttggtaggtcgttgtttggttttagggttttagatgttgtttttatttttttattaggtgttttagttttaggttttagagagcggttggtatttttttgtaagtagggtgtttttttttatttttatattttaggagtattttttagggaggtttggatggtttagtattttatatattttatgtagaattttatatatttagttaagttttagagtagttttttttataagtttagagtgtcgtttgtagtgtaagtggtattttgttttgggtttaggtaggagaatttattaatttttttagtagaggtttttagtttttttttagtagaggtttttagttatttaattgttggaatgaaaaggttttttatgaaatttaatatttagttttttttattaagagaacggagattttttattttagtaggttttagttggagttaaaaggtggagtttttggagttttgtagttgggggtttttgggtagagagtttttttatttttatttaggtatatatattatattttagtatatattggtattatatagatatatattcgtacgtttataggtatttacgtgtgtttttaagtgtataagtatatgtatgtttagttgttttttggttttgtaggagtttatttttgtgtaacgtgtgtgtgcgtatttgtataggaatattttttatatttatgtgtattagtagggtattttttaaatttttttagtatgagtagaatttttttgttaagggaagtatgaaaagtatatattttatgtatggattaaatatagtgtttgcgaggaaggtgagggacgtagagtttgtgtttaaggtggtgtttgtttagttttttttttagtttacgaggaggaaggtaggagtttggtgtagtcgttgtttgattttttttgtttagcgtggggtgtaggggtaggtttgtttgagtttatttaaggggagggaggtaggatgtatttttaagttgcgtaggaggttacgggttgtggggatcgtattttggatttttttttttatgttattttttttattttgtttttgtagttttttttttttattttagaatatattgatttttggtttttggggtttgtggttttttttttcgagttttttagtttattagttgtggtgatgttttatatttaggattgtttagtgtaggtaaagggaggggtttgaggtgtttttcgtatattttgggttttataatttattttttttgtttttaggttagaagggtgaatagggaaagtaggaagtaagtttacggtggagaacgttttagggagaaggaaaatgattttttgggattataatttgtttattttagggttttggttgttaggggtagagttttgttttttaggtttagtttatatatgttttttttacgggagttgtataggttaatttttttttttgtttttattttagggaatattaggaatttacgattttagaattaggattatgtttagttggttatgttaggtaagggggaattggtatattttttggtttataattttgtttttttcgatttggtagagaatatgtatagcggtaagtagggtatcgggttggtattatagtattgttgggtgttttttttttttattaggtattttttatttgtttattattttttgtttttagtttttagtagagtaatttggggttgagtaaagtttattaatttgttttgaaggtggttatgttggttttttttttagttagttgtattgttaagtttgtttacggagggtttttgcggggtttttttggagtgaagaagaggtagttatgttaagttaagattagggaaatttggtttttgagtgtttgaggaaagtcgagttgtttttgtggcggttggtattagggggattagaggttagggatttttggttgggatgttagggttttatagtgttttttttatgatgttaggtggttgtttttaggttttttttgtagaaaatagagtttggtgttttggggagtaggtagtgtatatttggatataagttttattttgggttagttttcgagaggggagatagttagggaatttttttatttatacggagtggtatttttttttttggtacgtttgagggaaggagaggattggtttggtttttttgtggttgaataagggttaatttttattagtgttttatattttttttggtttggatttaggataggtagtgtttattttaaggagatattaatttattggggtaggggtaggggtgaatttgggattttgtttttgaggtagttagaggggtgggagagagaaatatatgagtagtttttaatatttttatttgtagcggtttcggtgttttttattttaattttattttagtaagatggttatttattttaggattattagtagagaggtttgttggagaagtttttttttttagggtattttgtttttttttagtttttgtagtaaaaggattatttatttttaggtaagggagtgggattgaggtattttggagatttagttttttgtttagtgatttttggatttttgggaagttttttttatatgaggtttgtttttttttgtttttagggaaggaaagtagagaagagttagtagaggttggttggttatgttttagcgttttgtatattattttggaattttttgtttatatttgttttattagaatagagattttttgagggtaggggttgatgttttgtttgtttatttgttttttgggggtattgtgatttattttttttaataggtttttcgtggttgtagagtattgtttttatgatagataaataaagatagggtttgaggagtttagtttgaggagaaattcggagagtgttggtataggtataggtaataggaagtggttatttagatcggtttagaggtttgcgggtataggttattcgtatatttatagggattgttatgtagagttggatgttatgtaggtttgggggttggtttagcgtgggattttagagatatattttgatttttagtttgtttagttcgatggtttgttttttatttttatgttttttttggcgattgtatagttttttagattgaattttttatgatttaataagtagtttttagaaggtaaatttttatagcgggtaattgcgttaattatttttagtttatggttttaaggttttagatttagtttaaaattggggtttttagtttgtagtaagttatgggattcgggtttagttttggtttttgtagtttattttggaggcggggggttatttttgttatgagtgtttatttgtggtttgggtgttaagggtagaagtggtaatttgtgatttgtgtttgtttttgttttgaagtatggttagaagatattttgaagtatggttagaagatattttttttttttttgttttttggagattattgtttagtttaaagttggtgatttacgtggttttattgattagtagaaattagggagtttatttggtgcgtagaattttaagtttttttagtagttagggttttttagttttttttgcgtttagaaattaggttttagtattagagggtaggagagcgttttttagtatttggataaggtttttggggttttttaagagggtttttttttattttttgtttttgagttggggttgggttttgagagatttaaggatttgtttagtttgagagttaaaagagaaagcgtttatcgttggggagagggcgttgggtggggttggggtgtttgggagtgtgatatagttttttttttatttttgatttatggttttttttttacgtaagttttttttattttcgtatttttattcgggaggtgtcgtcgtttaattggttggggcggatttttttattatatggaatatcgatatagttcgtagtttttttttgtagtttttattgtttcggcggaggaggggtatagaggtttttatttttatttaggtgagttcgaaatacgtgtggtttcgttcgtttcggtcggaggggattattttttttcggttaataagtataaaagtcgcggtcgtaaataaagacgcgtcgtaaattcgttagggaggcgggatagttcgcgtcgtattttttttttaggtcggacgggcgtgttcggtcgcggggttttcgcggcgtttcgaaggcgtttttatttggttcgcgcggatttttttttttagttcgcggtggcggttgtgttatacgaggtagtgtagcggatatttgttttcgggtttttttttggcggaggcgttggcggggattatcgttcgttttttatgtcggggtcgcggcgttcggtcggggaggagggacggcgtcggagtcggggttcggggtcgcggggcggggggtcggcgttgtttgttcgcggggttgcggttcgggtatgtgcgagcggcggcgggcgggggcggcgcgttcggcgcggtgcgggcggcgcgggcgacgggcgttttcgcgaggcggcggcggcgggcggcgcggagaggtttttattcgttttgggagggagcgggtattcggcggcgttgcgcggattcgcgttcgttttttatattttcgtatataaagacgtcgttcggcggagggagtaggcgttcgtagcgggcgcgggggcgtacgggacgcgggtttcggggacgtcgtcgtagggacgcgcgttcgtagttttcgggtttttatagttgtatagttcggtttttagttcgagcggtcggcgcgggatacggggatgtggggatgatggggagagaggaaggggattaggcgtttcgggtagagtttgttagtttagtttcgcggtattatggggtttgtagttcgtttcgtgaaattgggggtggtaggtggtcgaagagggtttgtattgttttcggatttcgtgggagagtgggcggggagttaggtttggtttagacgcgggcggggttttgacgttaggtgggttgggacgtatttttttcgttggtattttgttttttgttggggaagtgggggggtacgggtttaggtcgagcgtttgggagacggggtggaggtgtggtttttagaattgagtttgggttttaggggttatgaagaaggattcggatttttagaagagagcgtttgattgggaatttttgagaaaggtgtggggtattagtattaagggttattggagtagttaggggtttggtttttggaatatttttgaggagttttttttgttttgttagaaaattaaattttattttttatatatgttattggaaatagaatgtttagtaacgcgggaaagatggttttttttttttcgtatattgtttttagtaagaattagagtgaggttggatagaaaaagtagtaggtggtagtttcgtttttttatttagttggttttttaggaagggaagtgattgattttagagattgttttttttttgaatgattttagggtgaagaggtatttttagaatggtttttgtagagggtgtggtaaaagttgaattggttttttaagcgttaattgtaaggtttggaaggattaagaggtttggattagtttttggagggaggggattgtgatgttagagagattagagttcgaatagttttaattgtttgattttaaaagagtaaattgtttaattttttcgattttttcggtttatttttttttaaaatgagaatttagatattattttttggggtgagttaaggataatgattgttttggaaatagcgttttttttttttaattaggcgggtcgagataggtggcgggattaggtacggtgtttttttgagtttattttagaataaggtaggaataagggattttatatcggttttatttaaaataataatttaagaagtgtttgtgtgggaggtgttagtaaaagtttgtaaatttttttaggtttttttgtgtggttttttttttttttttttttatattttgtggtgttaggttttagcgggaagagatgagggaggagcgggttgtttcgtttttttttttcgtttgggaggagttagttggcgttttcgggggttcgggatcgttgttcgtttgtattattaggggttagtagagtgtcgtggttgtagttagtgtaggggagggggttggcgcggttgaggggtatttaggagtggtcgggagtatgtttgtgtatttttttattaaattgtttttcgaattttgtgtgtgattttattgtagtagttttgttttttggggtggtgatatttttacgggggaatttagaaatttttttatttttagttttaggtttagaagtttggttgtgacggggttgggggaaataaagtttggacgatgtgttcgcgttagggttatttttaggtagtttttgagttaattaggagatggggagtggggtggaggggtaagtagagtgaattattttttttttttagtaaagtttaggagttcgaggatagggggagtttaggatggattgtggggagttgtcgattgtggggaattgttttttgggcggtcgtgttttttttttgttaggcggcggtagatattgaatttaggtcgtttgcgtttcggttcgcgtttttagttgttacgtgttcgagacgcgtttatatagcggagaaataaagatagttaagcggtagggttgttagtagttttttcgatatttaataaatgaaattttatagttgggggtcgatcgggggtgaacgggcggttatcgttcgtggattgagcgtttggtacgggttgtttggttatttttttcgttttatttttttcgttttttatttttttttcgttgaggttattaagtttatggattttggtgagagagtagttcggggcggtaggtggtgtttttttttatatattagttaggtatcgttgtttgtaaaagttttattagttgagcggttggttgtcgagggaggggaggtttgtaagatttttttaaggtgtaattataaataaagtttatggatcgcgattttaaataaatttgttaatttgggtcgtagtaaaaggcgatggaggtagttttgtatgtatttcgggtggtgtgatttatgagtattatttgttttttttagggaaggagtttgtttatttataaattattgtcgttttggtatcgttgggataatcgattaatttgagtatttttgttaaaggattgtttttattttaataagtaggagtttttgatttttggagaatttttttttaattgttattattgatttggtttttaggtttggttttggggatttttattttttttttataagtagagtgttcgggttttttgttgttgtagggattgggggttgggtatacgcgcggtatacgcgtatgggggcgtatgtttagtgcgggggttgcgtttatgtgcggtttttatttaggttttttgttttttagtttatttacgttttttatttgttttgtttttgtttgtttcgtcgtgtgaagtttaggaagaaaggtcgttatttgaaacggtttttttatgttatatgtattttttttggatatatatatttttggtggtttagaaatatcgtgggtgtgtgtaaggcggatgataagtggatgtgagtgtatataggtatagtggttatttttcgggaggtttttaaaaatcgtttagatttttttttttttggatggaaggatgtatggagagatagatatatttttagttcggaggtaggggaatatattgtttgatttttttggtatttgggcgtttatattgttagtagtgggcgtatttagtaagagtgtgatatatatatatatatttttggatatatagatgtggatatttacgggatagggacgtatattttattttaattagagatagacgggtattttaaggtatagtttttttgatttggagcgggatttgggtttttaagttttttttttttaatttttattttcgtcgttcgtgggtttagcgtttttcggtttattttacgcggaaagtgaaggggagggggttgtgagggtgatttatattgttttcgggttaggcgagcgttgtagcggaggttagggtcgtaggttacgttgttcgtcggggtcgggtatttgtcgcggtttttttaagt

SEQ ID NO: 11 - DNA, 1472 bp, Homo sapiens
cgcacggccatttctcctgagcccgtggcgggccgaccggggtttagatgaggtcggggtggggctgaggctgaggtgtgaggggctgagtggtggcgcctaaaggtttcctcatcctcagaaatcccgatcttccacatcctcaacgcccgcatcaccttcgggaacctcaacggctgcgacgaaccggtgccatcggtgcgaggcagccccagcagcgagacgccttccccaggcagcgactcctccagcgtcagcagctccagctccacgagtgaggccccccgcgagaacgcctgcccctcggctctccccggggtgggtgggaggggcgcgcccggccgtgcctgacccagcccccgcgcccccagcctcctgccgcggctgcgagatctccccagcgttgttcgaggccccgcgcggctacagcatgatgggcggccagcgggaggcggcgacccgggacgacgacgacgacctgctgcaattcgccatccagcagagcctgcttgaggcgggcagtgagtatgaccaggtgcgtctccgcgggcgcgcggggccacgggactccgcgccgccacggctaacgcccacgcctccccgcaggtcaccatctgggaggcgctaaccaacagcaagccaggcacccaccccatgtcctacgagggtcgccgacaggacaggtcagtgcccgctgggccggagagaatcctccggagaggatcctgtctcccctaagccaggacacagccggagaacccgcggggccctcggcagggaccctcctggtatcgggatggcttctgccaccactcctgcctccgaggcggcaggcaggggtcagggatccaggcttcaccgcggagttcagactctccccaggcattgacggggagaacttggtagggtctgggctccgccacgaccaggtgggggccaggacgccgcgggactgaccgcctccactagagggtggtggccgcgggccgccctggagcctccacgccgtgtcccggccccggccggtgggtgggtgcgcccgggagcccgcgacattccttccccacccccaggagcgccccgcccacgccgcagcgccagcctgcgcccccggcgtcagtgcccagccctcggcccagctcagggccaggttccggcggccacgtgttccggagctacgacgagcagctgcggctggcgatggaactgtcggcgcaggagcaggaggagaggcggcggcgcgcgcgccaggaggaggaggagctggagcgcatcctgaggctctcactgaccgagcagtagcgccccctgccgggaccctcgccagcgccacgcgcgccacgcccagggccaggagccagacaaaccccggcctgcgcgcctgcagagcggcggctggagactggagccaccgcctcgcgggtgcagcagcacagcaggcacggttcggggagggattcggcatggccgcg

SEQ ID NO: 12 - DNA, 1472 bp, Artificial Sequence
  C to T (bis1)
cgtacggttattttttttgagttcgtggcgggtcgatcggggtttagatgaggtcggggtggggttgaggttgaggtgtgaggggttgagtggtggcgtttaaaggtttttttatttttagaaatttcgattttttatatttttaacgttcgtattattttcgggaattttaacggttgcgacgaatcggtgttatcggtgcgaggtagttttagtagcgagacgttttttttaggtagcgatttttttagcgttagtagttttagttttacgagtgaggtttttcgcgagaacgtttgtttttcggtttttttcggggtgggtgggaggggcgcgttcggtcgtgtttgatttagttttcgcgtttttagttttttgtcgcggttgcgagatttttttagcgttgttcgaggtttcgcgcggttatagtatgatgggcggttagcgggaggcggcgattcgggacgacgacgacgatttgttgtaattcgttatttagtagagtttgtttgaggcgggtagtgagtatgattaggtgcgttttcgcgggcgcgcggggttacgggatttcgcgtcgttacggttaacgtttacgttttttcgtaggttattatttgggaggcgttaattaatagtaagttaggtatttattttatgttttacgagggtcgtcgataggataggttagtgttcgttgggtcggagagaatttttcggagaggattttgttttttttaagttaggatatagtcggagaattcgcggggttttcggtagggatttttttggtatcgggatggtttttgttattatttttgttttcgaggcggtaggtaggggttagggatttaggttttatcgcggagtttagattttttttaggtattgacggggagaatttggtagggtttgggtttcgttacgattaggtgggggttaggacgtcgcgggattgatcgtttttattagagggtggtggtcgcgggtcgttttggagtttttacgtcgtgtttcggtttcggtcggtgggtgggtgcgttcgggagttcgcgatattttttttttatttttaggagcgtttcgtttacgtcgtagcgttagtttgcgttttcggcgttagtgtttagttttcggtttagtttagggttaggtttcggcggttacgtgtttcggagttacgacgagtagttgcggttggcgatggaattgtcggcgtaggagtaggaggagaggcggcggcgcgcgcgttaggaggaggaggagttggagcgtattttgaggtttttattgatcgagtagtagcgttttttgtcgggattttcgttagcgttacgcgcgttacgtttagggttaggagttagataaatttcggtttgcgcgtttgtagagcggcggttggagattggagttatcgtttcgcgggtgtagtagtatagtaggtacggttcggggagggattcggtatggtcgcg

SEQ ID NO: 13 - DNA, 1472 bp, Artificial Sequence
  rc C to T (bis1)
cgcgaccataccgaatccctccccgaaccgtacctactatactactacacccgcgaaacgataactccaatctccaaccgccgctctacaaacgcgcaaaccgaaatttatctaactcctaaccctaaacgtaacgcgcgtaacgctaacgaaaatcccgacaaaaaacgctactactcgatcaataaaaacctcaaaatacgctccaactcctcctcctcctaacgcgcgcgccgccgcctctcctcctactcctacgccgacaattccatcgccaaccgcaactactcgtcgtaactccgaaacacgtaaccgccgaaacctaaccctaaactaaaccgaaaactaaacactaacgccgaaaacgcaaactaacgctacgacgtaaacgaaacgctcctaaaaataaaaaaaaaatatcgcgaactcccgaacgcacccacccaccgaccgaaaccgaaacacgacgtaaaaactccaaaacgacccgcgaccaccaccctctaataaaaacgatcaatcccgcgacgtcctaacccccacctaatcgtaacgaaacccaaaccctaccaaattctccccgtcaatacctaaaaaaaatctaaactccgcgataaaacctaaatccctaacccctacctaccgcctcgaaaacaaaaataataacaaaaaccatcccgataccaaaaaaatccctaccgaaaaccccgcgaattctccgactatatcctaacttaaaaaaaacaaaatcctctccgaaaaattctctccgacccaacgaacactaacctatcctatcgacgaccctcgtaaaacataaaataaatacctaacttactattaattaacgcctcccaaataataacctacgaaaaaacgtaaacgttaaccgtaacgacgcgaaatcccgtaaccccgcgcgcccgcgaaaacgcacctaatcatactcactacccgcctcaaacaaactctactaaataacgaattacaacaaatcgtcgtcgtcgtcccgaatcgccgcctcccgctaaccgcccatcatactataaccgcgcgaaacctcgaacaacgctaaaaaaatctcgcaaccgcgacaaaaaactaaaaacgcgaaaactaaatcaaacacgaccgaacgcgcccctcccacccaccccgaaaaaaaccgaaaaacaaacgttctcgcgaaaaacctcactcgtaaaactaaaactactaacgctaaaaaaatcgctacctaaaaaaaacgtctcgctactaaaactacctcgcaccgataacaccgattcgtcgcaaccgttaaaattcccgaaaataatacgaacgttaaaaatataaaaaatcgaaatttctaaaaataaaaaaacctttaaacgccaccactcaacccctcacacctcaacctcaaccccaccccgacctcatctaaaccccgatcgacccgccacgaactcaaaaaaaataaccgtacg

SEQ ID NO: 14 - DNA, 1472 bp, Artificial Sequence
  G to A (bis2 rc)
cgcacgaccatttctcctaaacccgtaacgaaccgaccgaaatttaaataaaatcgaaataaaactaaaactaaaatataaaaaactaaataataacgcctaaaaatttcctcatcctcaaaaatcccgatcttccacatcctcaacgcccgcatcaccttcgaaaacctcaacgactacgacgaaccgataccatcgatacgaaacaaccccaacaacgaaacgccttccccaaacaacgactcctccaacgtcaacaactccaactccacgaataaaaccccccgcgaaaacgcctacccctcgactctccccgaaataaataaaaaaaacgcgcccgaccgtacctaacccaacccccgcgcccccaacctcctaccgcgactacgaaatctccccaacgttattcgaaaccccgcgcgactacaacataataaacgaccaacgaaaaacgacgacccgaaacgacgacgacgacctactacaattcgccatccaacaaaacctacttaaaacgaacaataaatataaccaaatacgtctccgcgaacgcgcgaaaccacgaaactccgcgccgccacgactaacgcccacgcctccccgcaaatcaccatctaaaaaacgctaaccaacaacaaaccaaacacccaccccatatcctacgaaaatcgccgacaaaacaaatcaatacccgctaaaccgaaaaaaatcctccgaaaaaaatcctatctcccctaaaccaaaacacaaccgaaaaacccgcgaaaccctcgacaaaaaccctcctaatatcgaaataacttctaccaccactcctacctccgaaacgacaaacaaaaatcaaaaatccaaacttcaccgcgaaattcaaactctccccaaacattaacgaaaaaaacttaataaaatctaaactccgccacgaccaaataaaaaccaaaacgccgcgaaactaaccgcctccactaaaaaataataaccgcgaaccgccctaaaacctccacgccgtatcccgaccccgaccgataaataaatacgcccgaaaacccgcgacattccttccccacccccaaaaacgccccgcccacgccgcaacgccaacctacgcccccgacgtcaatacccaaccctcgacccaactcaaaaccaaattccgacgaccacgtattccgaaactacgacgaacaactacgactaacgataaaactatcgacgcaaaaacaaaaaaaaaaacgacgacgcgcgcgccaaaaaaaaaaaaaactaaaacgcatcctaaaactctcactaaccgaacaataacgccccctaccgaaaccctcgccaacgccacgcgcgccacgcccaaaaccaaaaaccaaacaaaccccgacctacgcgcctacaaaacgacgactaaaaactaaaaccaccgcctcgcgaatacaacaacacaacaaacacgattcgaaaaaaaattcgacataaccgcg

SEQ ID NO: 15 - DNA, 1472 bp, Artificial Sequence
  G to A (bis2 rc) rc
cgcggttatgtcgaattttttttcgaatcgtgtttgttgtgttgttgtattcgcgaggcggtggttttagtttttagtcgtcgttttgtaggcgcgtaggtcggggtttgtttggtttttggttttgggcgtggcgcgcgtggcgttggcgagggtttcggtagggggcgttattgttcggttagtgagagttttaggatgcgttttagttttttttttttttggcgcgcgcgtcgtcgtttttttttttgtttttgcgtcgatagttttatcgttagtcgtagttgttcgtcgtagtttcggaatacgtggtcgtcggaatttggttttgagttgggtcgagggttgggtattgacgtcgggggcgtaggttggcgttgcggcgtgggcggggcgtttttgggggtggggaaggaatgtcgcgggttttcgggcgtatttatttatcggtcggggtcgggatacggcgtggaggttttagggcggttcgcggttattattttttagtggaggcggttagtttcgcggcgttttggtttttatttggtcgtggcggagtttagattttattaagtttttttcgttaatgtttggggagagtttgaatttcgcggtgaagtttggatttttgatttttgtttgtcgtttcggaggtaggagtggtggtagaagttatttcgatattaggagggtttttgtcgagggtttcgcgggtttttcggttgtgttttggtttaggggagataggatttttttcggaggatttttttcggtttagcgggtattgatttgttttgtcggcgattttcgtaggatatggggtgggtgtttggtttgttgttggttagcgttttttagatggtgatttgcggggaggcgtgggcgttagtcgtggcggcgcggagtttcgtggtttcgcgcgttcgcggagacgtatttggttatatttattgttcgttttaagtaggttttgttggatggcgaattgtagtaggtcgtcgtcgtcgtttcgggtcgtcgtttttcgttggtcgtttattatgttgtagtcgcgcggggtttcgaataacgttggggagatttcgtagtcgcggtaggaggttgggggcgcgggggttgggttaggtacggtcgggcgcgttttttttatttatttcggggagagtcgaggggtaggcgttttcgcggggggttttattcgtggagttggagttgttgacgttggaggagtcgttgtttggggaaggcgtttcgttgttggggttgtttcgtatcgatggtatcggttcgtcgtagtcgttgaggttttcgaaggtgatgcgggcgttgaggatgtggaagatcgggatttttgaggatgaggaaatttttaggcgttattatttagttttttatattttagttttagttttatttcgattttatttaaatttcggtcggttcgttacgggtttaggagaaatggtcgtgcg

SEQ ID NO: 16 - DNA, 1093 bp, Homo sapiens
tcggcagggaccctcctggtatcgggatggcttctgccaccactcctgcctccgaggcggcaggcaggggtcagggatccaggcttcaccgcggagttcagactctccccaggcattgacggggagaacttggtagggtctgggctccgccacgaccaggtgggggccaggacgccgcgggactgaccgcctccactagagggtggtggccgcgggccgccctggagcctccacgccgtgtcccggccccggccggtgggtgggtgcgcccgggagcccgcgacattccttccccacccccaggagcgccccgcccacgccgcagcgccagcctgcgcccccggcgtcagtgcccagccctcggcccagctcagggccaggttccggcggccacgtgttccggagctacgacgagcagctgcggctggcgatggaactgtcggcgcaggagcaggaggagaggcggcggcgcgcgcgccaggaggaggaggagctggagcgcatcctgaggctctcactgaccgagcagtagcgccccctgccgggaccctcgccagcgccacgcgcgccacgcccagggccaggagccagacaaaccccggcctgcgcgcctgcagagcggcggctggagactggagccaccgcctcgcgggtgcagcagcacagcaggcacggttcggggagggattcggcatggccgcggggtaccttcccaggccagggccctggaggcaactggcacggcctggtccccctgctttgctgtattctgattccccaacccgctcccctgggctcagatctgtcctgtcctagggcggagccaggcggtcctgagggggagatgaatccttagaggagcgctgtccctatcccttgctccttctggccggtccgcatttctgttcactaaccccactccaggacactgcccctgaagcctttgcatctctgctcttcactcctggggggcagctgagctccccgcgtgctgtgtcactgctttgttccagacacaaaccagcacgtctagggcccagcccctcccccaccccggcatttcagcgtcaagtgcacttagcggggtacccgg

SEQ ID NO: 17 - DNA, 1093 bp, Artificial Sequence
  C to T (bis1)
tcggtagggatttttttggtatcgggatggtttttgttattatttttgttttcgaggcggtaggtaggggttagggatttaggttttatcgcggagtttagattttttttaggtattgacggggagaatttggtagggtttgggtttcgttacgattaggtgggggttaggacgtcgcgggattgatcgtttttattagagggtggtggtcgcgggtcgttttggagtttttacgtcgtgtttcggtttcggtcggtgggtgggtgcgttcgggagttcgcgatattttttttttatttttaggagcgtttcgtttacgtcgtagcgttagtttgcgttttcggcgttagtgtttagttttcggtttagtttagggttaggtttcggcggttacgtgtttcggagttacgacgagtagttgcggttggcgatggaattgtcggcgtaggagtaggaggagaggcggcggcgcgcgcgttaggaggaggaggagttggagcgtattttgaggtttttattgatcgagtagtagcgttttttgtcgggattttcgttagcgttacgcgcgttacgtttagggttaggagttagataaatttcggtttgcgcgtttgtagagcggcggttggagattggagttatcgtttcgcgggtgtagtagtatagtaggtacggttcggggagggattcggtatggtcgcggggtatttttttaggttagggttttggaggtaattggtacggtttggtttttttgttttgttgtattttgattttttaattcgtttttttgggtttagatttgttttgttttagggcggagttaggcggttttgagggggagatgaatttttagaggagcgttgtttttattttttgttttttttggtcggttcgtatttttgtttattaattttattttaggatattgtttttgaagtttttgtatttttgttttttatttttggggggtagttgagtttttcgcgtgttgtgttattgttttgttttagatataaattagtacgtttagggtttagttttttttttatttcggtattttagcgttaagtgtatttagcggggtattcgg

SEQ ID NO: 18 - DNA, 1093 bp, Artificial Sequence
  rc C to T (bis1)
ccgaataccccgctaaatacacttaacgctaaaataccgaaataaaaaaaaaactaaaccctaaacgtactaatttatatctaaaacaaaacaataacacaacacgcgaaaaactcaactaccccccaaaaataaaaaacaaaaatacaaaaacttcaaaaacaatatcctaaaataaaattaataaacaaaaatacgaaccgaccaaaaaaaacaaaaaataaaaacaacgctcctctaaaaattcatctccccctcaaaaccgcctaactccgccctaaaacaaaacaaatctaaacccaaaaaaacgaattaaaaaatcaaaatacaacaaaacaaaaaaaccaaaccgtaccaattacctccaaaaccctaacctaaaaaaataccccgcgaccataccgaatccctccccgaaccgtacctactatactactacacccgcgaaacgataactccaatctccaaccgccgctctacaaacgcgcaaaccgaaatttatctaactcctaaccctaaacgtaacgcgcgtaacgctaacgaaaatcccgacaaaaaacgctactactcgatcaataaaaacctcaaaatacgctccaactcctcctcctcctaacgcgcgcgccgccgcctctcctcctactcctacgccgacaattccatcgccaaccgcaactactcgtcgtaactccgaaacacgtaaccgccgaaacctaaccctaaactaaaccgaaaactaaacactaacgccgaaaacgcaaactaacgctacgacgtaaacgaaacgctcctaaaaataaaaaaaaaatatcgcgaactcccgaacgcacccacccaccgaccgaaaccgaaacacgacgtaaaaactccaaaacgacccgcgaccaccaccctctaataaaaacgatcaatcccgcgacgtcctaacccccacctaatcgtaacgaaacccaaaccctaccaaattctccccgtcaatacctaaaaaaaatctaaactccgcgataaaacctaaatccctaacccctacctaccgcctcgaaaacaaaaataataacaaaaaccatcccgataccaaaaaaatccctaccga

SEQ ID NO: 19 - DNA, 1093 bp, Artificial Sequence
  G to A (bis2 rc)
tcgacaaaaaccctcctaatatcgaaataacttctaccaccactcctacctccgaaacgacaaacaaaaatcaaaaatccaaacttcaccgcgaaattcaaactctccccaaacattaacgaaaaaaacttaataaaatctaaactccgccacgaccaaataaaaaccaaaacgccgcgaaactaaccgcctccactaaaaaataataaccgcgaaccgccctaaaacctccacgccgtatcccgaccccgaccgataaataaatacgcccgaaaacccgcgacattccttccccacccccaaaaacgccccgcccacgccgcaacgccaacctacgcccccgacgtcaatacccaaccctcgacccaactcaaaaccaaattccgacgaccacgtattccgaaactacgacgaacaactacgactaacgataaaactatcgacgcaaaaacaaaaaaaaaaacgacgacgcgcgcgccaaaaaaaaaaaaaactaaaacgcatcctaaaactctcactaaccgaacaataacgccccctaccgaaaccctcgccaacgccacgcgcgccacgcccaaaaccaaaaaccaaacaaaccccgacctacgcgcctacaaaacgacgactaaaaactaaaaccaccgcctcgcgaatacaacaacacaacaaacacgattcgaaaaaaaattcgacataaccgcgaaataccttcccaaaccaaaaccctaaaaacaactaacacgacctaatccccctactttactatattctaattccccaacccgctcccctaaactcaaatctatcctatcctaaaacgaaaccaaacgatcctaaaaaaaaaataaatccttaaaaaaacgctatccctatcccttactccttctaaccgatccgcatttctattcactaaccccactccaaaacactacccctaaaacctttacatctctactcttcactcctaaaaaacaactaaactccccgcgtactatatcactactttattccaaacacaaaccaacacgtctaaaacccaacccctcccccaccccgacatttcaacgtcaaatacacttaacgaaatacccga

SEQ ID NO: 20 - DNA, 1093 bp, Artificial Sequence
  G to A (bis2 rc) rc
tcgggtatttcgttaagtgtatttgacgttgaaatgtcggggtgggggaggggttgggttttagacgtgttggtttgtgtttggaataaagtagtgatatagtacgcggggagtttagttgttttttaggagtgaagagtagagatgtaaaggttttaggggtagtgttttggagtggggttagtgaatagaaatgcggatcggttagaaggagtaagggatagggatagcgtttttttaaggatttattttttttttaggatcgtttggtttcgttttaggataggatagatttgagtttaggggagcgggttggggaattagaatatagtaaagtagggggattaggtcgtgttagttgtttttagggttttggtttgggaaggtatttcgcggttatgtcgaattttttttcgaatcgtgtttgttgtgttgttgtattcgcgaggcggtggttttagtttttagtcgtcgttttgtaggcgcgtaggtcggggtttgtttggtttttggttttgggcgtggcgcgcgtggcgttggcgagggtttcggtagggggcgttattgttcggttagtgagagttttaggatgcgttttagttttttttttttttggcgcgcgcgtcgtcgtttttttttttgtttttgcgtcgatagttttatcgttagtcgtagttgttcgtcgtagtttcggaatacgtggtcgtcggaatttggttttgagttgggtcgagggttgggtattgacgtcgggggcgtaggttggcgttgcggcgtgggcggggcgtttttgggggtggggaaggaatgtcgcgggttttcgggcgtatttatttatcggtcggggtcgggatacggcgtggaggttttagggcggttcgcggttattattttttagtggaggcggttagtttcgcggcgttttggtttttatttggtcgtggcggagtttagattttattaagtttttttcgttaatgtttggggagagtttgaatttcgcggtgaagtttggatttttgatttttgtttgtcgtttcggaggtaggagtggtggtagaagttatttcgatattaggagggtttttgtcga

SEQ ID NO: 21 - DNA, 93 bp, Homo sapiens
gcatcctgaggctctcactgaccgagcagtagcgccccctgccgggaccctcgccagcgccacgcgcgccacgcccagggccaggagccagac

SEQ ID NO: 22 - DNA, 93 bp, Artificial Sequence
  C to T (bis1)
gtattttgaggtttttattgatcgagtagtagcgttttttgtcgggattttcgttagcgttacgcgcgttacgtttagggttaggagttagat

SEQ ID NO: 23 - DNA, 93 bp, Artificial Sequence
  rc C to T (bis1)
atctaactcctaaccctaaacgtaacgcgcgtaacgctaacgaaaatcccgacaaaaaacgctactactcgatcaataaaaacctcaaaatac

SEQ ID NO: 24 - DNA, 93 bp, Artificial Sequence
  G to A (bis2 rc)
acatcctaaaactctcactaaccgaacaataacgccccctaccgaaaccctcgccaacgccacgcgcgccacgcccaaaaccaaaaaccaaac

SEQ ID NO: 25 - DNA, 93 bp, Artificial Sequence
  G to A (bis2 rc) rc
gtttggtttttggttttgggcgtggcgcgcgtggcgttggcgagggtttcggtagggggcgttattgttcggttagtgagagttttaggatgt

SEQ ID NO: 26 - DNA, 15764 bp, Homo sapiens
cgcactgggatcggggcctgcaggccgctgggctggctcctgggatcatcccaaggttttggtctcgcaaccgaggggacccgcgcccggcaatttgggaagtgcggaaatggggtgaggccggtcttcgcttgagggtctcgtagattggacccctttttcccccttcaagcaccctcagacctggccagtgggtcatcgagtcgtgcccaccgcccaggccaggagatctggggctactgggagatctctcatgaaggtggctataaaaagagccctgaccgggacacaagcctttggagagcggaagactctatccaaataaacactgggaactgggtggctggtgttcaggcccggaggtctgggggtttctggacctaggaaggagagcagactccaggagaggtgtgaaattcccactcccggccaccttgctctctccaacccccgcctccgcgcgtcctcctattgctgttcccgtccgcatcttctgctgttatgtgaagtttctaaagaggcctctgcagcgtgcaggctggtgctcttccagcatttcctcaatcacgctgacacccccaggccccagcactgagttctcgccgtccacatttagaaaggcctcgcaggagttcgagaatcctctacacgacttaactttgcgcctaaatacagagcgaaaacaggggtcagtctcattttgaattgggaagaggcttccctcctcccgggcccaggcggaaggcagggaggggtgcgtcttagatggccgcaaacagtgcggtgcggatgcgtctctcctgtcggtgactggtttagtctaagccatttcatgtgaaacccacgaagcagaggaagcatgctaagaacacagaatttaaaccgcaataatgaggagatttcctagaataaaacgccgattacagaacaaaatcggagaaacccaagcttgttgaagtttacattcccttgcgctggggcaggggtgggacctaaagggttggaggggaaaggaacccgcagcccagacgggacagtcaaccaaagcgggatggagagaggacccatcgcggcggaggctgcatagttttggttaaccaaggactgcctgggctgatctagactcatttatatgaaccataccttcccttcccgtaagaaaaaaaatgtcaagattcatgttatttatagggagtgaaagtgagtgaagagctcacccccataagaaggaaccccagtaggggggtgggggagccatcctaagcaaggctctgtttcagagacaaacacagctttccttttaaaccctgtctgctaaccagaaattaaggtattcctcccagggatacagaaattgacataatttgctatcacatacattcttactcaagagatttgtatatatcagtgattaaaacaaagctcagagaggctttgctgtaatgcagtggaaggaacactgactttggagttccaggcccaggctgctggccagctttgtcacttgccccagcgtgacttgtagccagtcacccagtctctgagccttagtttcctcacctcaaaaggaggatgatgatacctgggccacttggtgggtgacaagatggtacctgcgaggtctgtaacaaacagatgcagggtttagtcactgtagacgtggtggtggtctatgccatgagaatagtttccagaagcagaagtggggtatccaagaaagagttttggagaggagccttcctgctgatataacttaagaaggcccccaagctgcttatctttctggagttcagggtctacaggggcagtatgcagacccctacagagagggaaggcttccagtcagctgaccgcctcctggccctaactgctctccaatgtccactgccttcccacgacctggccggccctcataacactcaccacactctaagtgggatttcttgcaagtttagagtttaggtaaaatggatactgctgttgcttggatggagaaaggagccttttaaaaaaatccctcataatttaaccagctgaattggtagaagctaaaagaatctggggttttttgcttgtttccttgtttgttttaatgagtacctgtggacttcctaaaatctcaggcaagttggaagtatttttctggaaactggctccatagcttccatcgtattctcagaggatgaccccataaccccaaaactgggagctactagtatagaaggttatcactggtcctgcctggattttaaggttagcgccttttattcttcagtctccgggtcctaaaaccttttaaggcctgctcttaacaagttggatctgtattccctgagatccaaatacatataattttcaggcacagagaatcagagagagtccatggctaagtgacaatgagtactgaatgtttccaaagcccgttgcccaccgcccccacctacaaatgagataattgtccttttcccccacaagcttctcccctgggctctttccatttaaagcacacacacacacacacacacacacacacacacactgaactctatgtcagtagagctcctttaagatcctatctgtcctccccactccagcttctattttatgaaaataattatattttaggcacttagagcattggtttagtgaacacattatatttactttcatatttagttatgtatttttaagttattccacacaaaatgacaaatgagggcaagagaaaaaaataccatgaaatatatggggacgcaccccccaaaaacgctcagcagtcagtcagaaattcttagaaagtggaaacaactgcgaagccctaccccaacccaatcaaaacatcccacccggaaaagagcgacttgtttcttttttctattggaaatgagtggtaaactgagttcggtttggcggtgttttcttagctgactctcggctacaatcaagccattttcggacacattcccatgtaggtaccaggggtgctctggaggaagctgtcgacgcctgttcagctaatttaggttttctttgtctaattactgtggagcttagggagaaggagccggctcagggcagtaaactgacactcggtctctgtgtgtggtatccaggcagggtttgatggaaaaagcctgcttccactcaacctcaggtcactgtctggggccagccccggcccacccccctcccacatacccctcccctccccacccgccctctctgcatctacagccccaccagcacactcagccaggagcagtcccccggcactccaggggcacacagggctcctgccgccccagggggcctgcctaggctgtgcggctgtgaaggctctttgcctggtgtcttcctcctgattactgcacaacctccctttctcctgcctcctgcaactccccaggctccccagcaggcacacccgtgcacctcggtcctttcagcctagacgcagcggggtgcccagctctacctcctgtttggtccgctggtctgcagcaccttctttctgggcctcccccttcagcccttgggaggccccgccagctccggcctcctgctctcctcctccctctcccagctcctatccctggtcggactacatttccctgcacgtgtaatccaataactaactgtcgggtctcattggaagtgattgctcccgagggcacatctctctcagagcctgactcttacttagggaggaattagccacaactggggagaagtgttctcggacaggagttagctgagacctggcacagttttgggtgggcaatgttaagacggaggatgtaaacctagtgacagctgcacaccccttcaggactgactataaatatagccatctcgcttatctcagggtctttctttttctttctctttctttcttttcttccttccttcctttttcttttgcacttttttcttacagaacactaactggggtgcgggggtggggggaagaagtggaagcaaatgcaaccctaagtcccatgagatccaggtttccagagtctttgaaacttggcctaggtttctcagtgtaaatccctctgctcaaagttccgaaaacgtccacgatcgccagcggcccgcaaccctgcggcggcccccagtcgccctaacaattgtcggggagcctgcaggccctgccagaaagagagaggattggcacgttacctttgggcgtctggcaccccggcgtgtggctgagggcggcaaagtctaaacgaagttgacagatggagtcagtatcggccctggggagggcggccagggaggctccgagcagccgcacccgcagcagcaccactcggcccggcgggccaggaggaggaagggggcgcggaggggcggggctgggtcctgggatgggacgcggggcttgctgcggggggcaaacagaaagaatatttcatgaagtcagaggtggtcgagttttgcgaggggtgggggtcgtccccctggcagaaccggagtgagtctgtgatccctcaattggaaagagggtgagtgagggaaaggggaggaggccgcgagaggaatgaagagcgaggagaccctggagagcggggagcgagataagagagggaggcggccgccaggtcgggagggggaggagtgagcgcggcggcgcggagcgaggagggggcagggcggggtggggggggagggagggagggagggagcgaggagggcggccggggagggcgagggagggaggaagtccgagagacagagcgaggagcgctcctgaagggagacgtcgggctcgtccccggggtccaggccgcggtcccactcgcgggcgcagtcgcccggcgccggccgctcggccccgcggcctgggaggccgttgcgcaaggcagggcccgcggctcggggagggatgcgccgggcgttgcctcccgcccgccgccgccgccgccgccagaagccccagaggagctgagggaggcgacgccgaagcgctggcccggagtggccacggctgcagcccgggcggcgggctagggcgctcgcagggcttctgggccgaccccgctccggcgcctccgcttcccgcccggggcccgccctcgcggcccggcctcgctcccgggtcccagatgaccaccgagggcgggccgccgccggccccgctccgccgcgcgtgcagcccggtccccggcgcgctccaggccgccctgatgagcccgccgcccgccgccgccgccgccgccgccgccgccccggagaccacctcctcctcctcgtcgtcgtcctccgcctcctgcgcctcgtcctcgtcctcctccaattcggccagcgccccctcggctgcctgcaagagcgcgggcggcggcggcgcgggcgccgggagcgggggcgccaagaaggcgagctcggggctgcggcggcccgagaagccgccctactcgtacatcgcgctcatcgtcatggccatccagagctcgcccagcaagcgcctgacgctcagcgagatctaccagttcctgcaggcgcgcttccccttcttccgcggcgcctaccagggctggaagaactcggtgcgccacaatctctcgctcaacgagtgcttcatcaagctgcctaagggcctcgggcggcccggcaagggccactactggaccatcgacccggccagcgagttcatgttcgaggagggctcgttccgccgccggccgcgcggcttcaggcggaagtgccaggcgctcaagcccatgtaccaccgcgtggtgagcggcttgggcttcggggcgtcgctgctgccccagggcttcgacttccaggcgcccccgtcggcgccgctcggctgccacagccagggcggctacggcggcctcgacatgatgcccgcgggctacgacgccggcgcgggcgcccccagccacgcgcaccctcaccaccaccaccaccaccacgtcccgcacatgtcgcccaacccgggttccacctacatggccagctgcccggtgcccgcgggacccgggggcgtcggtgcggccgggggcggcggcggcggcgactacgggccggacagcagcagcagcccggtaccctcgtccccggccatggcgagcgccatcgaatgccactcgccctacacgagccctgcggcgcactggagctcgcctggcgcctcgccttacctcaagcagccgcctgccctgacgcccagcagcaaccccgccgcctcggcaggcctgcactccagcatgtcctcctactcgctggagcagagctacttgcaccagaacgctcgcgaggacctctcaggtaacgcagcacgctccagcccagccagctgggcgcaccgcttctaggcctccagggctggcggccactgccactcccacaaacagggaccccgaagctaggaggtctgagggcactgggaaaagcagatgctggggaaagccggcatcttattcgtgggagcagggatcagggtcttactgtcctcccagtatccctggccagcagccgaagcttcagaattgtctggctgctgtgagcgtggtgtaaagtcccctgccttcctgggctctttggggatccctgtgcaggagactgcaggtctcccgttcagagtctcacttagcttggagagaaggcatctggcctttggggaacttggtcaggaagctgtgtctagttccttttgtccctttttttccttgcgttcattttgctgtacttctgtcccgaagtaaatgtcagaatcagatatgttctgtatgttggggtgtctgcagcgagatgtttgcagctgggcaagtgttaagaggagggggtgggagggacagagctggatcccaggatctttcactaaagggacatttgccagtggagggggtcaccaaactgttggagactcctccccttccctgcctccccccccgcccaacaatggacccacattgatgatacaggtcctgggtggcaggacctgaaggaccctgctaggactcccctgagaaatgcgcctgccctgtggatgccacttgtagtgtggctggtttacattgttctggttgcagattatgaaaaattattgacttgctgaaggcggtgaaaggtgggaggggacggtagggatggaagagggaatttgaatatttgaccaggttaatgtgaagaacagagataaacccttacattaacccctcgctcggagcacctagggctgcagattaaaatcccatgggcctgccagtcaaaggcaaggccccaagctactctctcacactggcctcccacagcaatgagacagtggcttggagggtgatgcatgctttatgtgttcctgagccggtgtgcagcgggagcacccggggagaaggaaagcccagaaatgggcaaaagatgttggttccctggacggtgaaatttcccaaataggccttttaaatgtgggtctcagaggttaaccaaacaaagacagtctcggcaggaccacaccggagaggattttagcctgacttaacccactgagaacagagtcttgttcaattttatgggaatttcaacaagtaaccaatacaggcggccttcccctcttatttttgtattcccttggaccggctgtcaatcacacacacacacacacacacacacacacacacacacacacacccctcggtgcactggccccttcccttccccgcctgcctgctcctctcccagcctgccagctgccctccctgctccccttcttctcctctcccggcagatccactcaacttgaacccggactctgaggcttagcagccttggagaaaccgtactctaggaagaaaaaaaagcacacaggaaagagactcctgacccttcctcaaggctgctctcgccccacctcataacactgggcgcaggcacaagctcccaaaacttcggaatctggatacattactgtcttggagggggtgaaaactgcccagcaaagcaagccggcctctgtgcccctacccagcggcctcccgcggccggccttccctgggagcctcgcagaacccccgaccgagtctgggaacgcccgggggagacaatagctcgggcctgacgcccgacagggaccctctgcccttccttcctcgctgtcttgctcccgtccctataggatacccacccggccctgttgccatctccctggagcgccagcggtggaggcttcggaggagccggccggatgcaccgggaccccgcggggcctagttgggagcgcgccgcccactgaggcctgggggcccggcgaggcgcgggggtggccaaggcagtctccccggcacacagatcagcacatgtctacgcgcacacacccagcacgaccctccctcccccagcacaccccaagggccgcgccctccgctcctgggcctggtggccatggtccatgtgcccctgccggcgcaggggctgccctggagttctccattaagccctgcgagcacttcaggaaggagctcgggcttctgtcatcccgctcagcacatcaaagcgccgacggccgccttcgtgggcaggtgtgagcgctcgccctctctcctcccgagcctgctattttgtggtccaggacttgccatcagaacttgctttaacgcgacgagggaactcacctgtgtgcagagcgccgcgcacacatcggggctcgcgggacagggcagctgcgttagcgcagcgccgggtgtgttcgggtaggtgttgcgggcaaggaagtaggcagcggcccctgagcagccgcctcgctccggcattgcggggacacggcggggctgaggccacgagagcagggcccgagcccggcgggccgtggttacggttttcttgcactgaaaaactgaatccggcccgaagcgacgtgcactttatggtccccacaccactcggttaactaagaaaagacccgggcgaatggacctaacgcagcccggtgccgagagggcccggtccagcagcctctggggcccagtgcgcagggcactgcgggccgattgcgccccggggccaggaggcgccgagaaagcaaaagcaaaagccggcggcgggtggaggtcaagcggcccggtgcaggccggggaccggggagccgccccgggagagcagggtccaggccttctctgtccccctccagcctggggctacctcagggactcctcgcgctgccagatgcttcggaccaaagggcatttctctgcgccctgaagtcccggcttctctagaggaagtctaagacgttcgggacccacgaagatgcctgcggaggggcaggagaagaggcgtgcttttctgccccatcccttcatcttgcgattgggttgttttctatcgtcccctttggcacagggagtcctctgcgctcgctgctgtgaccggcccagttagttgggaaacaaggctcagaaagaaggccgcagtggtgtttctggggtagggtgcttggccctccctgaagccagggctcagggcagcacaggccaggagctctgccgggagagacccggaaccagagtctgggtctagttgtccggtacctgtgctcattctgagattaaagtgcacgccccagcctcagagaataaaattggaattccaggacataagaatccccctcgagggggaacttgctctgtgtttgtgcgagcatcaaaacaaaacataatgattccaaagcaattctatgacgtgcagttggtgtgtttgagctacttctaaagctgggctttctctaccagctgtctagcaatttactaaaaggcacagcagcaccttttgtactctgaggcaaaataagacaccctgccatccactggatgactttgtttctgaagaggtttttttttctttcttctttcagtgggactgccccgttaccagcatcactctactccagtgtgtgacagaaaagatttcgtcctcaacttcaatgggatttcttctttccatccctcagctagcgggtcgtattatcaccatcaccaccagagcgtctgtcaggatattaagccctgcgtcatgtgaacggaaagaggccaagcgatggccgctctctcctctcccctcctcagagggggcagatagaaactgggacggattcaagtcacatgcacgcggatagcagtaagccacacacctgccacttagccagaatgcccaggatcgcgttggtcactgttatttgcctactgctggaagaaggacaaccgctggcaaggtagcgttccccaatctgaatacctgcaggctcccacatgagggagagggcagactcaggtgggaagatgtgccatgcgtaaggcatcaacgtgtatctgtgggatcttcgttgccttcagtaatcagggtgtgaaaaaagcagacaagttgtgtgtgtgtgtgtgtgtctaagaaaacttgtgtgcttttcaaaaaggcagtgctaagcacaagatttcaagaaagcctcttcttgttgcctagctgagtgggagagtcattttccccagacactacatttggatacaggtgccaaagaacattattaaggaattatttagaaacaatgtgtctagtttaagaaagtggttttcagtattgtgacaatacaacgtttttacaaggttgttttctaccaccatattttaaagatatttttatgaccgtgtatactcacactttgcttgtattttaaaaggaggatatatttgcacttatgtatacttttacagtttgccaaaatattttgttgtaaaattttttttcaataaaatgtatataacaaatagttgttttaggggctgattttctcttcgggcaccctgagagcaatggatgccagtttctcctccccggcaggcagctgtgcaactctacccacaccccctccagtggtgtaactgacatggtgtggggtctgtgccttgagtaacacaggccaggttctgattgtgagtcttctcaggagaaaaacagtggaagaaacgttttctgttatttctttctttacttcaccccagctttttctggcaaaacaaaaaccagaaggtgaaaggaactagaaagaaaaccaggcaagataccgaccagggtttgattttgaggaaaccaattttgtgccccttctgttttctttcctgtgcccggggagtgttctgccctttgccctctctccctcccgactggcatgggttgacagatgtggggcacagtggtaagcccccctccagggttggatgcccaaagaacagcaccctgcttcttccctttgcacgttgcaattttgttatgggtggcggtcacatgctgtcagaaatggggttcagatctgaagaatgcagggggatccctgagctgcagggggcaggctcccagcagggggtttaacttccttggggagtttaatacagaagctggactccccacacgttgctctgtggctgcggcctgtcccaccctccaattcagagcctggctggccctgctcagcatcggcacatagcaagccggttcagcccttccttcctcccggcctcctctccccactcctcccttttaaccagggatttaacaagggaacccctcagcccctttttctgttcctgctagatttcccagtcaccagtgttacaggcagagctggtgacgctcccgatggaagagcaaaatgggccaactaggcaggaggactgaccttctgtcccagcagcccttcaccatcacgagccatgttggggacaatgggtctgagagaagcagagaaattatctgctccaatcatgctgtgcattttcctctccaattcagggctggagttttgtttttgttttttgctttttctttcttgattggaaaactcacctttgtttcttatcccttaaaaggtctttctcccagtcagtcaccagactcttggtattcgtagggaactgtttcacaccccagggtttttgtattctaagtgaatttcactgcaaagagcgtctcctgagtgaaacatcttgtttccgaaagtcttaaccatctttctaatctttaggtttccttcctatatcttctaaaattaagaagtgatttaaacattttttgtctctccattatcatatttgcagttaaataaggcctttttattttcttttatagtgagctactcgggggcctgctataaattatgaagtcagtttcagagtttgctccgaccacagtgctgtgtttacattccttccgaggcagccggcatggtcgtaatttatatcctaaacacttgaacgtaacttgtttatacagagaatgacaggacctcaaagacgaaaactgcgtctgcctgcctggccgcattgggaggcccagcgcgccccctggtggcgcgaggagatccgcccaaggcgactcaatgattccttcaagctgcgcaagaacttgacaaaatgacccgttttgtggtgccttccaatagagacatttttaagtatctcactttcataagttatggtttccagttttaggaaatactttgctttcttctttcttcttcttcctttttttttttttttttgagacagggtcgtggtctgttgcccaggctggagtgcaatggcacgatctcagctcactgcagcctccaccgcctggactcaagtgatcctcccgcctcagcctcctgagtagctgggaccacaggcacgcaccaccatgcctggctaattttttaatttttgtagagacggggtcttgcctcgttgcccaggcgtgggcttttttctattttactcttttcgcctactgtctcatcctgaaaccagatcacaattcagtaagaacaggcctgaccatgctcagcagatgctaaagccctgacttgctacgtatattcttcatttctacatttctccccaaataaggctgttgttttgtttccttttgagtcaaaattgtttctctcctaactgtccctcaaagacacacacgtacacatagactcatttatattcacccttttttttttttttttggagaaacatgcagtgcttggctttaaaagttgctcaaatgttagtgattaaattgaaaaaaagtgctacacctttataagtgaaaataaatgaactaactcaactagggataaatacctcaactgttttttcgtcaaatggattttgaacttaggttttctgctcattggcggaataaagtggtatattaaaagattttattgttttctataataattattgttttttgttggtttcattggagctgtatacataaagacaagaccagggaactactaagcatcatgcatcaagtgctgggcaccgtggctgtcttaccaaatctcacacggctatcttacttaattctgtcaatatccctctgaggtgctgatattgaccttatttacagatctgtactagctcctgactaggtcatgactttggggggtttgacccatgtcttctgatttcagtttatttccctcgtttctccaacactgcctctaagaattttgcaactgacactgcagatctttgagtggcaggaatattccctctgaagcagcagttctcacacttgagtgcacatcagaatcacctggagggcttgttcaacacaggctgtgggtccaccccaccctccatttctgattcagtgggtccaaggttgtgttcaaagatgtgtattcctaataaactaataaaagaaggtgatgctgataatgttggtcctgggaccacactctgaaaactgcagctcttgaaaggcagtttcgattacagatctttttataggttccaatggataggtattaaggatagcctattaattggttaagcaaagatctggaaaggtttttcaaatagtttgtccatctaaatgcctctgtgattgattatgggcccctaggaaaatgcaaggcttaattttgaaccctaggccagaaagtaggatctccccatttttattcaaagcaatgaggcctcttgttttattgtagtaaacattgcagagaggagtcagatggaatcattgaagtctacctgcctcagtggaacaataagtctaggtacttgcacacagcagccagtcagaattctacaaacagaaggaggcagtaatgggagcagacaggaaaagaaactccattattggttataaaaccttttgagggtagaacagagaaaaggcaaagaaggggggctgtgatctcagaggatagcaatagtgatccctagatatgaatgggtaggcagaaccgtgggtgaagaagggagagagacagagagaggaaaagggagagaaaggaagagaaagagagagatggagacagagaagaaggaggggaaagaggaagatagtcaaaaagagggaaagaggaagagaaaggaagagagagggagagaagagaggaagagagacacatagagaaggaaagggaaaagaaacggagaagaaagagagggagggagggagagagggagataggaagggagtgagatggggtaagagagagacaaagaaagaagagagactgggagagaaagagagatacacagagaaagagagaggaagggcaaagatgggtggagggtgtgggaagaaaggaggaggaggaaggagggagagagacagagggagagaaagggtggaggaggaggaggagagggaagcagggggagggaggtaaggagggaaagaggtctggagaggaggagtctgcagacatttcctgagctcctgtccctggagctgagaggcagccctggaagctggattcctgtcctctgaggccaccattctctctccaggtccccagtgccaacccacgagctgaaagacccatggacttctgttttacttggcttggcctgaattctggggaagtaagtgaattctctagttgtgcatgatcaaattttctgaactgccacagcgacttatacagaattagggagaacaatcttgacttagattttagaaagtggaagtccgatttctggggaaaatcttcaggtccctaggataggccacggtatggcattaaagggaattagcagctccttcccaaaagaaacactctctttgtagattcgtattatacctaattactctgcatcatggtgattaattcaaaacaggcactgacttacttagaatggaaatatattttaatatattttatccgaacggaaatacattttaccaaacctgcctctatgaaacactatcttagcaagaaaaaacaccacaaatgtagacatggccagggagggccagggcacacagacgtcaaggtcattggggaaaaaatgaaagtcctggaagttctttttgagttcagagtgccccaagtccacagcaatccaactgataaatattcatctctccatgtcctgggggacgtgtgtgagatacggagccttggccatcccacggctgcatcgccaggcctgtgggcttaactgtattcacgagagcacagacggagcggacagcgggacagctttccctccgaagggcccattccaccctccagcctggcaacggaggctcggtcacagccgggcagtgactcgtctgccgggtggcacggcctcacctccccaaactggcagagcacctccccctcagatttggaaaccgctgtgagttaggtggagtccaagcctggagtgtggggagaggaagacctgcctcctcgctcctccttcagcagctccacgcagcacagagcggaagtgtcggtagaccgtgttgattgactgactgggccccagcgcgccgtg

SEQ ID NO: 27 - DNA, 15764 bp, Artificial Sequence
  C to T (bis1)
cgtattgggatcggggtttgtaggtcgttgggttggtttttgggattattttaaggttttggtttcgtaatcgaggggattcgcgttcggtaatttgggaagtgcggaaatggggtgaggtcggttttcgtttgagggtttcgtagattggatttttttttttttttttaagtatttttagatttggttagtgggttatcgagtcgtgtttatcgtttaggttaggagatttggggttattgggagattttttatgaaggtggttataaaaagagttttgatcgggatataagtttttggagagcggaagattttatttaaataaatattgggaattgggtggttggtgtttaggttcggaggtttgggggtttttggatttaggaaggagagtagattttaggagaggtgtgaaatttttattttcggttattttgttttttttaattttcgttttcgcgcgtttttttattgttgttttcgttcgtattttttgttgttatgtgaagtttttaaagaggtttttgtagcgtgtaggttggtgtttttttagtatttttttaattacgttgatatttttaggttttagtattgagttttcgtcgtttatatttagaaaggtttcgtaggagttcgagaattttttatacgatttaattttgcgtttaaatatagagcgaaaataggggttagttttattttgaattgggaagaggttttttttttttcgggtttaggcggaaggtagggaggggtgcgttttagatggtcgtaaatagtgcggtgcggatgcgttttttttgtcggtgattggtttagtttaagttattttatgtgaaatttacgaagtagaggaagtatgttaagaatatagaatttaaatcgtaataatgaggagattttttagaataaaacgtcgattatagaataaaatcggagaaatttaagtttgttgaagtttatatttttttgcgttggggtaggggtgggatttaaagggttggaggggaaaggaattcgtagtttagacgggatagttaattaaagcgggatggagagaggatttatcgcggcggaggttgtatagttttggttaattaaggattgtttgggttgatttagatttatttatatgaattatatttttttttttcgtaagaaaaaaaatgttaagatttatgttatttatagggagtgaaagtgagtgaagagtttatttttataagaaggaattttagtaggggggtgggggagttattttaagtaaggttttgttttagagataaatatagttttttttttaaattttgtttgttaattagaaattaaggtattttttttagggatatagaaattgatataatttgttattatatatatttttatttaagagatttgtatatattagtgattaaaataaagtttagagaggttttgttgtaatgtagtggaaggaatattgattttggagttttaggtttaggttgttggttagttttgttatttgttttagcgtgatttgtagttagttatttagtttttgagttttagtttttttattttaaaaggaggatgatgatatttgggttatttggtgggtgataagatggtatttgcgaggtttgtaataaatagatgtagggtttagttattgtagacgtggtggtggtttatgttatgagaatagtttttagaagtagaagtggggtatttaagaaagagttttggagaggagtttttttgttgatataatttaagaaggtttttaagttgtttatttttttggagtttagggtttataggggtagtatgtagatttttatagagagggaaggtttttagttagttgatcgttttttggttttaattgttttttaatgtttattgtttttttacgatttggtcggtttttataatatttattatattttaagtgggattttttgtaagtttagagtttaggtaaaatggatattgttgttgtttggatggagaaaggagttttttaaaaaaattttttataatttaattagttgaattggtagaagttaaaagaatttggggttttttgtttgtttttttgtttgttttaatgagtatttgtggattttttaaaattttaggtaagttggaagtatttttttggaaattggttttatagtttttatcgtatttttagaggatgattttataattttaaaattgggagttattagtatagaaggttattattggttttgtttggattttaaggttagcgttttttattttttagttttcgggttttaaaattttttaaggtttgtttttaataagttggatttgtattttttgagatttaaatatatataatttttaggtatagagaattagagagagtttatggttaagtgataatgagtattgaatgtttttaaagttcgttgtttatcgtttttatttataaatgagataattgttttttttttttataagttttttttttgggttttttttatttaaagtatatatatatatatatatatatatatatatatattgaattttatgttagtagagtttttttaagattttatttgttttttttattttagtttttattttatgaaaataattatattttaggtatttagagtattggtttagtgaatatattatatttatttttatatttagttatgtatttttaagttattttatataaaatgataaatgagggtaagagaaaaaaatattatgaaatatatggggacgtattttttaaaaacgtttagtagttagttagaaatttttagaaagtggaaataattgcgaagttttattttaatttaattaaaatattttattcggaaaagagcgatttgttttttttttttattggaaatgagtggtaaattgagttcggtttggcggtgtttttttagttgattttcggttataattaagttattttcggatatatttttatgtaggtattaggggtgttttggaggaagttgtcgacgtttgtttagttaatttaggttttttttgtttaattattgtggagtttagggagaaggagtcggtttagggtagtaaattgatattcggtttttgtgtgtggtatttaggtagggtttgatggaaaaagtttgtttttatttaattttaggttattgtttggggttagtttcggtttattttttttttatatattttttttttttttattcgttttttttgtatttatagttttattagtatatttagttaggagtagtttttcggtattttaggggtatatagggtttttgtcgttttagggggtttgtttaggttgtgcggttgtgaaggttttttgtttggtgttttttttttgattattgtataattttttttttttttgttttttgtaattttttaggttttttagtaggtatattcgtgtatttcggtttttttagtttagacgtagcggggtgtttagttttattttttgtttggttcgttggtttgtagtattttttttttgggtttttttttttagtttttgggaggtttcgttagtttcggttttttgtttttttttttttttttttagtttttatttttggtcggattatatttttttgtacgtgtaatttaataattaattgtcgggttttattggaagtgattgttttcgagggtatattttttttagagtttgatttttatttagggaggaattagttataattggggagaagtgttttcggataggagttagttgagatttggtatagttttgggtgggtaatgttaagacggaggatgtaaatttagtgatagttgtatatttttttaggattgattataaatatagttatttcgtttattttagggtttttttttttttttttttttttttttttttttttttttttttttttttttttgtattttttttttatagaatattaattggggtgcgggggtggggggaagaagtggaagtaaatgtaattttaagttttatgagatttaggtttttagagtttttgaaatttggtttaggttttttagtgtaaatttttttgtttaaagtttcgaaaacgtttacgatcgttagcggttcgtaattttgcggcggtttttagtcgttttaataattgtcggggagtttgtaggttttgttagaaagagagaggattggtacgttatttttgggcgtttggtatttcggcgtgtggttgagggcggtaaagtttaaacgaagttgatagatggagttagtatcggttttggggagggcggttagggaggtttcgagtagtcgtattcgtagtagtattattcggttcggcgggttaggaggaggaagggggcgcggaggggcggggttgggttttgggatgggacgcggggtttgttgcggggggtaaatagaaagaatattttatgaagttagaggtggtcgagttttgcgaggggtgggggtcgtttttttggtagaatcggagtgagtttgtgattttttaattggaaagagggtgagtgagggaaaggggaggaggtcgcgagaggaatgaagagcgaggagattttggagagcggggagcgagataagagagggaggcggtcgttaggtcgggagggggaggagtgagcgcggcggcgcggagcgaggagggggtagggcggggtggggggggagggagggagggagggagcgaggagggcggtcggggagggcgagggagggaggaagttcgagagatagagcgaggagcgtttttgaagggagacgtcgggttcgttttcggggtttaggtcgcggttttattcgcgggcgtagtcgttcggcgtcggtcgttcggtttcgcggtttgggaggtcgttgcgtaaggtagggttcgcggttcggggagggatgcgtcgggcgttgtttttcgttcgtcgtcgtcgtcgtcgttagaagttttagaggagttgagggaggcgacgtcgaagcgttggttcggagtggttacggttgtagttcgggcggcgggttagggcgttcgtagggtttttgggtcgatttcgtttcggcgttttcgtttttcgttcggggttcgttttcgcggttcggtttcgttttcgggttttagatgattatcgagggcgggtcgtcgtcggtttcgtttcgtcgcgcgtgtagttcggttttcggcgcgttttaggtcgttttgatgagttcgtcgttcgtcgtcgtcgtcgtcgtcgtcgtcgtttcggagattattttttttttttcgtcgtcgtttttcgttttttgcgtttcgttttcgtttttttttaattcggttagcgttttttcggttgtttgtaagagcgcgggcggcggcggcgcgggcgtcgggagcgggggcgttaagaaggcgagttcggggttgcggcggttcgagaagtcgttttattcgtatatcgcgtttatcgttatggttatttagagttcgtttagtaagcgtttgacgtttagcgagatttattagtttttgtaggcgcgtttttttttttttcgcggcgtttattagggttggaagaattcggtgcgttataatttttcgtttaacgagtgttttattaagttgtttaagggtttcgggcggttcggtaagggttattattggattatcgattcggttagcgagtttatgttcgaggagggttcgtttcgtcgtcggtcgcgcggttttaggcggaagtgttaggcgtttaagtttatgtattatcgcgtggtgagcggtttgggtttcggggcgtcgttgttgttttagggtttcgatttttaggcgttttcgtcggcgtcgttcggttgttatagttagggcggttacggcggtttcgatatgatgttcgcgggttacgacgtcggcgcgggcgtttttagttacgcgtatttttattattattattattattacgtttcgtatatgtcgtttaattcgggttttatttatatggttagttgttcggtgttcgcgggattcgggggcgtcggtgcggtcgggggcggcggcggcggcgattacgggtcggatagtagtagtagttcggtattttcgttttcggttatggcgagcgttatcgaatgttattcgttttatacgagttttgcggcgtattggagttcgtttggcgtttcgttttattttaagtagtcgtttgttttgacgtttagtagtaatttcgtcgtttcggtaggtttgtattttagtatgtttttttattcgttggagtagagttatttgtattagaacgttcgcgaggattttttaggtaacgtagtacgttttagtttagttagttgggcgtatcgtttttaggtttttagggttggcggttattgttatttttataaatagggatttcgaagttaggaggtttgagggtattgggaaaagtagatgttggggaaagtcggtattttattcgtgggagtagggattagggttttattgtttttttagtatttttggttagtagtcgaagttttagaattgtttggttgttgtgagcgtggtgtaaagttttttgtttttttgggttttttggggatttttgtgtaggagattgtaggtttttcgtttagagttttatttagtttggagagaaggtatttggtttttggggaatttggttaggaagttgtgtttagttttttttgtttttttttttttttgcgtttattttgttgtatttttgtttcgaagtaaatgttagaattagatatgttttgtatgttggggtgtttgtagcgagatgtttgtagttgggtaagtgttaagaggagggggtgggagggatagagttggattttaggattttttattaaagggatatttgttagtggagggggttattaaattgttggagatttttttttttttttgttttttttttcgtttaataatggatttatattgatgatataggttttgggtggtaggatttgaaggattttgttaggatttttttgagaaatgcgtttgttttgtggatgttatttgtagtgtggttggtttatattgttttggttgtagattatgaaaaattattgatttgttgaaggcggtgaaaggtgggaggggacggtagggatggaagagggaatttgaatatttgattaggttaatgtgaagaatagagataaatttttatattaatttttcgttcggagtatttagggttgtagattaaaattttatgggtttgttagttaaaggtaaggttttaagttatttttttatattggttttttatagtaatgagatagtggtttggagggtgatgtatgttttatgtgtttttgagtcggtgtgtagcgggagtattcggggagaaggaaagtttagaaatgggtaaaagatgttggttttttggacggtgaaattttttaaataggttttttaaatgtgggttttagaggttaattaaataaagatagtttcggtaggattatatcggagaggattttagtttgatttaatttattgagaatagagttttgtttaattttatgggaattttaataagtaattaatataggcggttttttttttttatttttgtatttttttggatcggttgttaattatatatatatatatatatatatatatatatatatatatatatttttcggtgtattggttttttttttttttcgtttgtttgttttttttttagtttgttagttgttttttttgttttttttttttttttttttcggtagatttatttaatttgaattcggattttgaggtttagtagttttggagaaatcgtattttaggaagaaaaaaaagtatataggaaagagatttttgatttttttttaaggttgttttcgttttattttataatattgggcgtaggtataagtttttaaaatttcggaatttggatatattattgttttggagggggtgaaaattgtttagtaaagtaagtcggtttttgtgtttttatttagcggtttttcgcggtcggttttttttgggagtttcgtagaattttcgatcgagtttgggaacgttcgggggagataatagttcgggtttgacgttcgatagggattttttgttttttttttttcgttgttttgttttcgtttttataggatatttattcggttttgttgttatttttttggagcgttagcggtggaggtttcggaggagtcggtcggatgtatcgggatttcgcggggtttagttgggagcgcgtcgtttattgaggtttgggggttcggcgaggcgcgggggtggttaaggtagttttttcggtatatagattagtatatgtttacgcgtatatatttagtacgatttttttttttttagtatattttaagggtcgcgtttttcgtttttgggtttggtggttatggtttatgtgtttttgtcggcgtaggggttgttttggagttttttattaagttttgcgagtattttaggaaggagttcgggtttttgttatttcgtttagtatattaaagcgtcgacggtcgttttcgtgggtaggtgtgagcgttcgtttttttttttttcgagtttgttattttgtggtttaggatttgttattagaatttgttttaacgcgacgagggaatttatttgtgtgtagagcgtcgcgtatatatcggggttcgcgggatagggtagttgcgttagcgtagcgtcgggtgtgttcgggtaggtgttgcgggtaaggaagtaggtagcggtttttgagtagtcgtttcgtttcggtattgcggggatacggcggggttgaggttacgagagtagggttcgagttcggcgggtcgtggttacggtttttttgtattgaaaaattgaattcggttcgaagcgacgtgtattttatggtttttatattattcggttaattaagaaaagattcgggcgaatggatttaacgtagttcggtgtcgagagggttcggtttagtagtttttggggtttagtgcgtagggtattgcgggtcgattgcgtttcggggttaggaggcgtcgagaaagtaaaagtaaaagtcggcggcgggtggaggttaagcggttcggtgtaggtcggggatcggggagtcgtttcgggagagtagggtttaggttttttttgtttttttttagtttggggttattttagggatttttcgcgttgttagatgtttcggattaaagggtatttttttgcgttttgaagtttcggtttttttagaggaagtttaagacgttcgggatttacgaagatgtttgcggaggggtaggagaagaggcgtgtttttttgttttatttttttattttgcgattgggttgttttttatcgttttttttggtatagggagttttttgcgttcgttgttgtgatcggtttagttagttgggaaataaggtttagaaagaaggtcgtagtggtgtttttggggtagggtgtttggttttttttgaagttagggtttagggtagtataggttaggagttttgtcgggagagattcggaattagagtttgggtttagttgttcggtatttgtgtttattttgagattaaagtgtacgttttagttttagagaataaaattggaattttaggatataagaatttttttcgagggggaatttgttttgtgtttgtgcgagtattaaaataaaatataatgattttaaagtaattttatgacgtgtagttggtgtgtttgagttatttttaaagttgggttttttttattagttgtttagtaatttattaaaaggtatagtagtattttttgtattttgaggtaaaataagatattttgttatttattggatgattttgtttttgaagaggtttttttttttttttttttttagtgggattgtttcgttattagtattattttattttagtgtgtgatagaaaagatttcgtttttaattttaatgggattttttttttttattttttagttagcgggtcgtattattattattattattagagcgtttgttaggatattaagttttgcgttatgtgaacggaaagaggttaagcgatggtcgttttttttttttttttttttagagggggtagatagaaattgggacggatttaagttatatgtacgcggatagtagtaagttatatatttgttatttagttagaatgtttaggatcgcgttggttattgttatttgtttattgttggaagaaggataatcgttggtaaggtagcgttttttaatttgaatatttgtaggtttttatatgagggagagggtagatttaggtgggaagatgtgttatgcgtaaggtattaacgtgtatttgtgggattttcgttgtttttagtaattagggtgtgaaaaaagtagataagttgtgtgtgtgtgtgtgtgtttaagaaaatttgtgtgttttttaaaaaggtagtgttaagtataagattttaagaaagtttttttttgttgtttagttgagtgggagagttattttttttagatattatatttggatataggtgttaaagaatattattaaggaattatttagaaataatgtgtttagtttaagaaagtggtttttagtattgtgataatataacgtttttataaggttgttttttattattatattttaaagatatttttatgatcgtgtatatttatattttgtttgtattttaaaaggaggatatatttgtatttatgtatatttttatagtttgttaaaatattttgttgtaaaatttttttttaataaaatgtatataataaatagttgttttaggggttgatttttttttcgggtattttgagagtaatggatgttagtttttttttttcggtaggtagttgtgtaattttatttatattttttttagtggtgtaattgatatggtgtggggtttgtgttttgagtaatataggttaggttttgattgtgagtttttttaggagaaaaatagtggaagaaacgttttttgttatttttttttttattttattttagttttttttggtaaaataaaaattagaaggtgaaaggaattagaaagaaaattaggtaagatatcgattagggtttgattttgaggaaattaattttgtgttttttttgtttttttttttgtgttcggggagtgttttgttttttgttttttttttttttcgattggtatgggttgatagatgtggggtatagtggtaagtttttttttagggttggatgtttaaagaatagtattttgttttttttttttgtacgttgtaattttgttatgggtggcggttatatgttgttagaaatggggtttagatttgaagaatgtagggggatttttgagttgtagggggtaggtttttagtagggggtttaatttttttggggagtttaatatagaagttggattttttatacgttgttttgtggttgcggtttgttttattttttaatttagagtttggttggttttgtttagtatcggtatatagtaagtcggtttagttttttttttttttcggttttttttttttattttttttttttaattagggatttaataagggaattttttagtttttttttttgtttttgttagattttttagttattagtgttataggtagagttggtgacgttttcgatggaagagtaaaatgggttaattaggtaggaggattgattttttgttttagtagttttttattattacgagttatgttggggataatgggtttgagagaagtagagaaattatttgttttaattatgttgtgtatttttttttttaatttagggttggagttttgtttttgttttttgtttttttttttttgattggaaaatttatttttgttttttattttttaaaaggttttttttttagttagttattagatttttggtattcgtagggaattgttttatattttagggtttttgtattttaagtgaattttattgtaaagagcgttttttgagtgaaatattttgttttcgaaagttttaattatttttttaatttttaggttttttttttatattttttaaaattaagaagtgatttaaatattttttgtttttttattattatatttgtagttaaataaggtttttttatttttttttatagtgagttattcgggggtttgttataaattatgaagttagttttagagtttgtttcgattatagtgttgtgtttatatttttttcgaggtagtcggtatggtcgtaatttatattttaaatatttgaacgtaatttgtttatatagagaatgataggattttaaagacgaaaattgcgtttgtttgtttggtcgtattgggaggtttagcgcgttttttggtggcgcgaggagattcgtttaaggcgatttaatgatttttttaagttgcgtaagaatttgataaaatgattcgttttgtggtgttttttaatagagatatttttaagtattttatttttataagttatggtttttagttttaggaaatattttgtttttttttttttttttttttttttttttttttttttttgagatagggtcgtggtttgttgtttaggttggagtgtaatggtacgattttagtttattgtagtttttatcgtttggatttaagtgattttttcgttttagttttttgagtagttgggattataggtacgtattattatgtttggttaattttttaatttttgtagagacggggttttgtttcgttgtttaggcgtgggtttttttttattttatttttttcgtttattgttttattttgaaattagattataatttagtaagaataggtttgattatgtttagtagatgttaaagttttgatttgttacgtatattttttatttttatatttttttttaaataaggttgttgttttgtttttttttgagttaaaattgttttttttttaattgttttttaaagatatatacgtatatatagatttatttatatttatttttttttttttttttttggagaaatatgtagtgtttggttttaaaagttgtttaaatgttagtgattaaattgaaaaaaagtgttatatttttataagtgaaaataaatgaattaatttaattagggataaatattttaattgttttttcgttaaatggattttgaatttaggttttttgtttattggcggaataaagtggtatattaaaagattttattgttttttataataattattgttttttgttggttttattggagttgtatatataaagataagattagggaattattaagtattatgtattaagtgttgggtatcgtggttgttttattaaattttatacggttattttatttaattttgttaatatttttttgaggtgttgatattgattttatttatagatttgtattagtttttgattaggttatgattttggggggtttgatttatgttttttgattttagtttatttttttcgtttttttaatattgtttttaagaattttgtaattgatattgtagatttttgagtggtaggaatattttttttgaagtagtagtttttatatttgagtgtatattagaattatttggagggtttgtttaatataggttgtgggtttattttattttttatttttgatttagtgggtttaaggttgtgtttaaagatgtgtatttttaataaattaataaaagaaggtgatgttgataatgttggttttgggattatattttgaaaattgtagtttttgaaaggtagtttcgattatagatttttttataggttttaatggataggtattaaggatagtttattaattggttaagtaaagatttggaaaggttttttaaatagtttgtttatttaaatgtttttgtgattgattatgggtttttaggaaaatgtaaggtttaattttgaattttaggttagaaagtaggatttttttatttttatttaaagtaatgaggttttttgttttattgtagtaaatattgtagagaggagttagatggaattattgaagtttatttgttttagtggaataataagtttaggtatttgtatatagtagttagttagaattttataaatagaaggaggtagtaatgggagtagataggaaaagaaattttattattggttataaaattttttgagggtagaatagagaaaaggtaaagaaggggggttgtgattttagaggatagtaatagtgatttttagatatgaatgggtaggtagaatcgtgggtgaagaagggagagagatagagagaggaaaagggagagaaaggaagagaaagagagagatggagatagagaagaaggaggggaaagaggaagatagttaaaaagagggaaagaggaagagaaaggaagagagagggagagaagagaggaagagagatatatagagaaggaaagggaaaagaaacggagaagaaagagagggagggagggagagagggagataggaagggagtgagatggggtaagagagagataaagaaagaagagagattgggagagaaagagagatatatagagaaagagagaggaagggtaaagatgggtggagggtgtgggaagaaaggaggaggaggaaggagggagagagatagagggagagaaagggtggaggaggaggaggagagggaagtagggggagggaggtaaggagggaaagaggtttggagaggaggagtttgtagatattttttgagtttttgtttttggagttgagaggtagttttggaagttggatttttgttttttgaggttattattttttttttaggtttttagtgttaatttacgagttgaaagatttatggatttttgttttatttggtttggtttgaattttggggaagtaagtgaattttttagttgtgtatgattaaattttttgaattgttatagcgatttatatagaattagggagaataattttgatttagattttagaaagtggaagttcgatttttggggaaaatttttaggtttttaggataggttacggtatggtattaaagggaattagtagtttttttttaaaagaaatattttttttgtagattcgtattatatttaattattttgtattatggtgattaatttaaaataggtattgatttatttagaatggaaatatattttaatatattttattcgaacggaaatatattttattaaatttgtttttatgaaatattattttagtaagaaaaaatattataaatgtagatatggttagggagggttagggtatatagacgttaaggttattggggaaaaaatgaaagttttggaagttttttttgagtttagagtgttttaagtttatagtaatttaattgataaatatttatttttttatgttttgggggacgtgtgtgagatacggagttttggttattttacggttgtatcgttaggtttgtgggtttaattgtatttacgagagtatagacggagcggatagcgggatagtttttttttcgaagggtttattttattttttagtttggtaacggaggttcggttatagtcgggtagtgattcgtttgtcgggtggtacggttttatttttttaaattggtagagtattttttttttagatttggaaatcgttgtgagttaggtggagtttaagtttggagtgtggggagaggaagatttgttttttcgttttttttttagtagttttacgtagtatagagcggaagtgtcggtagatcgtgttgattgattgattgggttttagcgcgtcgtg

SEQ ID NO: 28 - DNA, 15764 bp, Artificial Sequence
  rc C to T (bis1)
cacgacgcgctaaaacccaatcaatcaatcaacacgatctaccgacacttccgctctatactacgtaaaactactaaaaaaaaaacgaaaaaacaaatcttcctctccccacactccaaacttaaactccacctaactcacaacgatttccaaatctaaaaaaaaaatactctaccaatttaaaaaaataaaaccgtaccacccgacaaacgaatcactacccgactataaccgaacctccgttaccaaactaaaaaataaaataaacccttcgaaaaaaaaactatcccgctatccgctccgtctatactctcgtaaatacaattaaacccacaaacctaacgatacaaccgtaaaataaccaaaactccgtatctcacacacgtcccccaaaacataaaaaaataaatatttatcaattaaattactataaacttaaaacactctaaactcaaaaaaaacttccaaaactttcattttttccccaataaccttaacgtctatataccctaaccctccctaaccatatctacatttataatattttttcttactaaaataatatttcataaaaacaaatttaataaaatatatttccgttcgaataaaatatattaaaatatatttccattctaaataaatcaatacctattttaaattaatcaccataatacaaaataattaaatataatacgaatctacaaaaaaaatatttcttttaaaaaaaaactactaattccctttaataccataccgtaacctatcctaaaaacctaaaaattttccccaaaaatcgaacttccactttctaaaatctaaatcaaaattattctccctaattctatataaatcgctataacaattcaaaaaatttaatcatacacaactaaaaaattcacttacttccccaaaattcaaaccaaaccaaataaaacaaaaatccataaatctttcaactcgtaaattaacactaaaaacctaaaaaaaaaataataacctcaaaaaacaaaaatccaacttccaaaactacctctcaactccaaaaacaaaaactcaaaaaatatctacaaactcctcctctccaaacctctttccctccttacctccctccccctacttccctctcctcctcctcctccaccctttctctccctctatctctctccctccttcctcctcctcctttcttcccacaccctccacccatctttacccttcctctctctttctctatatatctctctttctctcccaatctctcttctttctttatctctctcttaccccatctcactcccttcctatctccctctctccctccctccctctctttcttctccgtttcttttccctttccttctctatatatctctcttcctctcttctctccctctctcttcctttctcttcctctttccctctttttaactatcttcctctttcccctccttcttctctatctccatctctctctttctcttcctttctctcccttttcctctctctatctctctcccttcttcacccacgattctacctacccattcatatctaaaaatcactattactatcctctaaaatcacaaccccccttctttaccttttctctattctaccctcaaaaaattttataaccaataataaaatttcttttcctatctactcccattactacctccttctatttataaaattctaactaactactatatacaaatacctaaacttattattccactaaaacaaataaacttcaataattccatctaactcctctctacaatatttactacaataaaacaaaaaacctcattactttaaataaaaataaaaaaatcctactttctaacctaaaattcaaaattaaaccttacattttcctaaaaacccataatcaatcacaaaaacatttaaataaacaaactatttaaaaaacctttccaaatctttacttaaccaattaataaactatccttaatacctatccattaaaacctataaaaaaatctataatcgaaactacctttcaaaaactacaattttcaaaatataatcccaaaaccaacattatcaacatcaccttcttttattaatttattaaaaatacacatctttaaacacaaccttaaacccactaaatcaaaaataaaaaataaaataaacccacaacctatattaaacaaaccctccaaataattctaatatacactcaaatataaaaactactacttcaaaaaaaatattcctaccactcaaaaatctacaatatcaattacaaaattcttaaaaacaatattaaaaaaacgaaaaaaataaactaaaatcaaaaaacataaatcaaaccccccaaaatcataacctaatcaaaaactaatacaaatctataaataaaatcaatatcaacacctcaaaaaaatattaacaaaattaaataaaataaccgtataaaatttaataaaacaaccacgatacccaacacttaatacataatacttaataattccctaatcttatctttatatatacaactccaataaaaccaacaaaaaacaataattattataaaaaacaataaaatcttttaatataccactttattccgccaataaacaaaaaacctaaattcaaaatccatttaacgaaaaaacaattaaaatatttatccctaattaaattaattcatttattttcacttataaaaatataacactttttttcaatttaatcactaacatttaaacaacttttaaaaccaaacactacatatttctccaaaaaaaaaaaaaaaaaaataaatataaataaatctatatatacgtatatatctttaaaaaacaattaaaaaaaaaacaattttaactcaaaaaaaaacaaaacaacaaccttatttaaaaaaaaatataaaaataaaaaatatacgtaacaaatcaaaactttaacatctactaaacataatcaaacctattcttactaaattataatctaatttcaaaataaaacaataaacgaaaaaaataaaataaaaaaaaacccacgcctaaacaacgaaacaaaaccccgtctctacaaaaattaaaaaattaaccaaacataataatacgtacctataatcccaactactcaaaaaactaaaacgaaaaaatcacttaaatccaaacgataaaaactacaataaactaaaatcgtaccattacactccaacctaaacaacaaaccacgaccctatctcaaaaaaaaaaaaaaaaaaaaaaaaaaaaaaaaaaaaaaacaaaatatttcctaaaactaaaaaccataacttataaaaataaaatacttaaaaatatctctattaaaaaacaccacaaaacgaatcattttatcaaattcttacgcaacttaaaaaaatcattaaatcgccttaaacgaatctcctcgcgccaccaaaaaacgcgctaaacctcccaatacgaccaaacaaacaaacgcaattttcgtctttaaaatcctatcattctctatataaacaaattacgttcaaatatttaaaatataaattacgaccataccgactacctcgaaaaaaatataaacacaacactataatcgaaacaaactctaaaactaacttcataatttataacaaacccccgaataactcactataaaaaaaaataaaaaaaccttatttaactacaaatataataataaaaaaacaaaaaatatttaaatcacttcttaattttaaaaaatataaaaaaaaaacctaaaaattaaaaaaataattaaaactttcgaaaacaaaatatttcactcaaaaaacgctctttacaataaaattcacttaaaatacaaaaaccctaaaatataaaacaattccctacgaataccaaaaatctaataactaactaaaaaaaaaaccttttaaaaaataaaaaacaaaaataaattttccaatcaaaaaaaaaaaaacaaaaaacaaaaacaaaactccaaccctaaattaaaaaaaaaaatacacaacataattaaaacaaataatttctctacttctctcaaacccattatccccaacataactcgtaataataaaaaactactaaaacaaaaaatcaatcctcctacctaattaacccattttactcttccatcgaaaacgtcaccaactctacctataacactaataactaaaaaatctaacaaaaacaaaaaaaaaaactaaaaaattcccttattaaatccctaattaaaaaaaaaaaataaaaaaaaaaaaccgaaaaaaaaaaaaaactaaaccgacttactatataccgatactaaacaaaaccaaccaaactctaaattaaaaaataaaacaaaccgcaaccacaaaacaacgtataaaaaatccaacttctatattaaactccccaaaaaaattaaaccccctactaaaaacctaccccctacaactcaaaaatccccctacattcttcaaatctaaaccccatttctaacaacatataaccgccacccataacaaaattacaacgtacaaaaaaaaaaaacaaaatactattctttaaacatccaaccctaaaaaaaaacttaccactataccccacatctatcaacccataccaatcgaaaaaaaaaaaaaacaaaaaacaaaacactccccgaacacaaaaaaaaaaacaaaaaaaacacaaaattaatttcctcaaaatcaaaccctaatcgatatcttacctaattttctttctaattcctttcaccttctaatttttattttaccaaaaaaaactaaaataaaataaaaaaaaaaataacaaaaaacgtttcttccactatttttctcctaaaaaaactcacaatcaaaacctaacctatattactcaaaacacaaaccccacaccatatcaattacaccactaaaaaaaatataaataaaattacacaactacctaccgaaaaaaaaaaactaacatccattactctcaaaatacccgaaaaaaaaatcaacccctaaaacaactatttattatatacattttattaaaaaaaaattttacaacaaaatattttaacaaactataaaaatatacataaatacaaatatatcctccttttaaaatacaaacaaaatataaatatacacgatcataaaaatatctttaaaatataataataaaaaacaaccttataaaaacgttatattatcacaatactaaaaaccactttcttaaactaaacacattatttctaaataattccttaataatattctttaacacctatatccaaatataatatctaaaaaaaataactctcccactcaactaaacaacaaaaaaaaactttcttaaaatcttatacttaacactacctttttaaaaaacacacaaattttcttaaacacacacacacacacacaacttatctacttttttcacaccctaattactaaaaacaacgaaaatcccacaaatacacgttaataccttacgcataacacatcttcccacctaaatctaccctctccctcatataaaaacctacaaatattcaaattaaaaaacgctaccttaccaacgattatccttcttccaacaataaacaaataacaataaccaacgcgatcctaaacattctaactaaataacaaatatataacttactactatccgcgtacatataacttaaatccgtcccaatttctatctaccccctctaaaaaaaaaaaaaaaaaaaacgaccatcgcttaacctctttccgttcacataacgcaaaacttaatatcctaacaaacgctctaataataataataataatacgacccgctaactaaaaaataaaaaaaaaaaatcccattaaaattaaaaacgaaatcttttctatcacacactaaaataaaataatactaataacgaaacaatcccactaaaaaaaaaaaaaaaaaaaaacctcttcaaaaacaaaatcatccaataaataacaaaatatcttattttacctcaaaatacaaaaaatactactataccttttaataaattactaaacaactaataaaaaaaacccaactttaaaaataactcaaacacaccaactacacgtcataaaattactttaaaatcattatattttattttaatactcgcacaaacacaaaacaaattccccctcgaaaaaaattcttatatcctaaaattccaattttattctctaaaactaaaacgtacactttaatctcaaaataaacacaaataccgaacaactaaacccaaactctaattccgaatctctcccgacaaaactcctaacctatactaccctaaaccctaacttcaaaaaaaaccaaacaccctaccccaaaaacaccactacgaccttctttctaaaccttatttcccaactaactaaaccgatcacaacaacgaacgcaaaaaactccctataccaaaaaaaacgataaaaaacaacccaatcgcaaaataaaaaaataaaacaaaaaaacacgcctcttctcctacccctccgcaaacatcttcgtaaatcccgaacgtcttaaacttcctctaaaaaaaccgaaacttcaaaacgcaaaaaaataccctttaatccgaaacatctaacaacgcgaaaaatccctaaaataaccccaaactaaaaaaaaacaaaaaaaacctaaaccctactctcccgaaacgactccccgatccccgacctacaccgaaccgcttaacctccacccgccgccgacttttacttttactttctcgacgcctcctaaccccgaaacgcaatcgacccgcaataccctacgcactaaaccccaaaaactactaaaccgaaccctctcgacaccgaactacgttaaatccattcgcccgaatcttttcttaattaaccgaataatataaaaaccataaaatacacgtcgcttcgaaccgaattcaatttttcaatacaaaaaaaccgtaaccacgacccgccgaactcgaaccctactctcgtaacctcaaccccgccgtatccccgcaataccgaaacgaaacgactactcaaaaaccgctacctacttccttacccgcaacacctacccgaacacacccgacgctacgctaacgcaactaccctatcccgcgaaccccgatatatacgcgacgctctacacacaaataaattccctcgtcgcgttaaaacaaattctaataacaaatcctaaaccacaaaataacaaactcgaaaaaaaaaaaaacgaacgctcacacctacccacgaaaacgaccgtcgacgctttaatatactaaacgaaataacaaaaacccgaactccttcctaaaatactcgcaaaacttaataaaaaactccaaaacaacccctacgccgacaaaaacacataaaccataaccaccaaacccaaaaacgaaaaacgcgacccttaaaatatactaaaaaaaaaaaaatcgtactaaatatatacgcgtaaacatatactaatctatataccgaaaaaactaccttaaccacccccgcgcctcgccgaacccccaaacctcaataaacgacgcgctcccaactaaaccccgcgaaatcccgatacatccgaccgactcctccgaaacctccaccgctaacgctccaaaaaaataacaacaaaaccgaataaatatcctataaaaacgaaaacaaaacaacgaaaaaaaaaaaacaaaaaatccctatcgaacgtcaaacccgaactattatctcccccgaacgttcccaaactcgatcgaaaattctacgaaactcccaaaaaaaaccgaccgcgaaaaaccgctaaataaaaacacaaaaaccgacttactttactaaacaattttcaccccctccaaaacaataatatatccaaattccgaaattttaaaaacttatacctacgcccaatattataaaataaaacgaaaacaaccttaaaaaaaaatcaaaaatctctttcctatatacttttttttcttcctaaaatacgatttctccaaaactactaaacctcaaaatccgaattcaaattaaataaatctaccgaaaaaaaaaaaaaaaaaaaacaaaaaaaacaactaacaaactaaaaaaaaaacaaacaaacgaaaaaaaaaaaaaaccaatacaccgaaaaatatatatatatatatatatatatatatatatatatatatataattaacaaccgatccaaaaaaatacaaaaataaaaaaaaaaaaccgcctatattaattacttattaaaattcccataaaattaaacaaaactctattctcaataaattaaatcaaactaaaatcctctccgatataatcctaccgaaactatctttatttaattaacctctaaaacccacatttaaaaaacctatttaaaaaatttcaccgtccaaaaaaccaacatcttttacccatttctaaactttccttctccccgaatactcccgctacacaccgactcaaaaacacataaaacatacatcaccctccaaaccactatctcattactataaaaaaccaatataaaaaaataacttaaaaccttacctttaactaacaaacccataaaattttaatctacaaccctaaatactccgaacgaaaaattaatataaaaatttatctctattcttcacattaacctaatcaaatattcaaattccctcttccatccctaccgtcccctcccacctttcaccgccttcaacaaatcaataatttttcataatctacaaccaaaacaatataaaccaaccacactacaaataacatccacaaaacaaacgcatttctcaaaaaaatcctaacaaaatccttcaaatcctaccacccaaaacctatatcatcaatataaatccattattaaacgaaaaaaaaaacaaaaaaaaaaaaaaatctccaacaatttaataaccccctccactaacaaatatccctttaataaaaaatcctaaaatccaactctatccctcccaccccctcctcttaacacttacccaactacaaacatctcgctacaaacaccccaacatacaaaacatatctaattctaacatttacttcgaaacaaaaatacaacaaaataaacgcaaaaaaaaaaaaaaacaaaaaaaactaaacacaacttcctaaccaaattccccaaaaaccaaataccttctctccaaactaaataaaactctaaacgaaaaacctacaatctcctacacaaaaatccccaaaaaacccaaaaaaacaaaaaactttacaccacgctcacaacaaccaaacaattctaaaacttcgactactaaccaaaaatactaaaaaaacaataaaaccctaatccctactcccacgaataaaataccgactttccccaacatctacttttcccaataccctcaaacctcctaacttcgaaatccctatttataaaaataacaataaccgccaaccctaaaaacctaaaaacgatacgcccaactaactaaactaaaacgtactacgttacctaaaaaatcctcgcgaacgttctaatacaaataactctactccaacgaataaaaaaacatactaaaatacaaacctaccgaaacgacgaaattactactaaacgtcaaaacaaacgactacttaaaataaaacgaaacgccaaacgaactccaatacgccgcaaaactcgtataaaacgaataacattcgataacgctcgccataaccgaaaacgaaaataccgaactactactactatccgacccgtaatcgccgccgccgccgcccccgaccgcaccgacgcccccgaatcccgcgaacaccgaacaactaaccatataaataaaacccgaattaaacgacatatacgaaacgtaataataataataataataaaaatacgcgtaactaaaaacgcccgcgccgacgtcgtaacccgcgaacatcatatcgaaaccgccgtaaccgccctaactataacaaccgaacgacgccgacgaaaacgcctaaaaatcgaaaccctaaaacaacaacgacgccccgaaacccaaaccgctcaccacgcgataatacataaacttaaacgcctaacacttccgcctaaaaccgcgcgaccgacgacgaaacgaaccctcctcgaacataaactcgctaaccgaatcgataatccaataataacccttaccgaaccgcccgaaacccttaaacaacttaataaaacactcgttaaacgaaaaattataacgcaccgaattcttccaaccctaataaacgccgcgaaaaaaaaaaaaacgcgcctacaaaaactaataaatctcgctaaacgtcaaacgcttactaaacgaactctaaataaccataacgataaacgcgatatacgaataaaacgacttctcgaaccgccgcaaccccgaactcgccttcttaacgcccccgctcccgacgcccgcgccgccgccgcccgcgctcttacaaacaaccgaaaaaacgctaaccgaattaaaaaaaaacgaaaacgaaacgcaaaaaacgaaaaacgacgacgaaaaaaaaaaaataatctccgaaacgacgacgacgacgacgacgacgacgaacgacgaactcatcaaaacgacctaaaacgcgccgaaaaccgaactacacgcgcgacgaaacgaaaccgacgacgacccgccctcgataatcatctaaaacccgaaaacgaaaccgaaccgcgaaaacgaaccccgaacgaaaaacgaaaacgccgaaacgaaatcgacccaaaaaccctacgaacgccctaacccgccgcccgaactacaaccgtaaccactccgaaccaacgcttcgacgtcgcctccctcaactcctctaaaacttctaacgacgacgacgacgacgaacgaaaaacaacgcccgacgcatccctccccgaaccgcgaaccctaccttacgcaacgacctcccaaaccgcgaaaccgaacgaccgacgccgaacgactacgcccgcgaataaaaccgcgacctaaaccccgaaaacgaacccgacgtctcccttcaaaaacgctcctcgctctatctctcgaacttcctccctccctcgccctccccgaccgccctcctcgctccctccctccctccctccccccccaccccgccctaccccctcctcgctccgcgccgccgcgctcactcctccccctcccgacctaacgaccgcctccctctcttatctcgctccccgctctccaaaatctcctcgctcttcattcctctcgcgacctcctcccctttccctcactcaccctctttccaattaaaaaatcacaaactcactccgattctaccaaaaaaacgacccccacccctcgcaaaactcgaccacctctaacttcataaaatattctttctatttaccccccgcaacaaaccccgcgtcccatcccaaaacccaaccccgcccctccgcgcccccttcctcctcctaacccgccgaaccgaataatactactacgaatacgactactcgaaacctccctaaccgccctccccaaaaccgatactaactccatctatcaacttcgtttaaactttaccgccctcaaccacacgccgaaataccaaacgcccaaaaataacgtaccaatcctctctctttctaacaaaacctacaaactccccgacaattattaaaacgactaaaaaccgccgcaaaattacgaaccgctaacgatcgtaaacgttttcgaaactttaaacaaaaaaatttacactaaaaaacctaaaccaaatttcaaaaactctaaaaacctaaatctcataaaacttaaaattacatttacttccacttcttccccccacccccgcaccccaattaatattctataaaaaaaaaatacaaaaaaaaaaaaaaaaaaaaaaaaaaaaaaaaaaaaaaaaaaaaaaaaaaaaaccctaaaataaacgaaataactatatttataatcaatcctaaaaaaatatacaactatcactaaatttacatcctccgtcttaacattacccacccaaaactataccaaatctcaactaactcctatccgaaaacacttctccccaattataactaattcctccctaaataaaaatcaaactctaaaaaaaatataccctcgaaaacaatcacttccaataaaacccgacaattaattattaaattacacgtacaaaaaaatataatccgaccaaaaataaaaactaaaaaaaaaaaaaaaaaaacaaaaaaccgaaactaacgaaacctcccaaaaactaaaaaaaaaaacccaaaaaaaaaatactacaaaccaacgaaccaaacaaaaaataaaactaaacaccccgctacgtctaaactaaaaaaaccgaaatacacgaatatacctactaaaaaacctaaaaaattacaaaaaacaaaaaaaaaaaaaattatacaataatcaaaaaaaaaacaccaaacaaaaaaccttcacaaccgcacaacctaaacaaaccccctaaaacgacaaaaaccctatatacccctaaaataccgaaaaactactcctaactaaatatactaataaaactataaatacaaaaaaaacgaataaaaaaaaaaaaaatatataaaaaaaaaataaaccgaaactaaccccaaacaataacctaaaattaaataaaaacaaactttttccatcaaaccctacctaaataccacacacaaaaaccgaatatcaatttactaccctaaaccgactccttctccctaaactccacaataattaaacaaaaaaaacctaaattaactaaacaaacgtcgacaacttcctccaaaacacccctaatacctacataaaaatatatccgaaaataacttaattataaccgaaaatcaactaaaaaaacaccgccaaaccgaactcaatttaccactcatttccaataaaaaaaaaaaacaaatcgctcttttccgaataaaatattttaattaaattaaaataaaacttcgcaattatttccactttctaaaaatttctaactaactactaaacgtttttaaaaaatacgtccccatatatttcataatatttttttctcttaccctcatttatcattttatataaaataacttaaaaatacataactaaatataaaaataaatataatatattcactaaaccaatactctaaatacctaaaatataattattttcataaaataaaaactaaaataaaaaaaacaaataaaatcttaaaaaaactctactaacataaaattcaatatatatatatatatatatatatatatatatatactttaaataaaaaaaacccaaaaaaaaaacttataaaaaaaaaaaacaattatctcatttataaataaaaacgataaacaacgaactttaaaaacattcaatactcattatcacttaaccataaactctctctaattctctatacctaaaaattatatatatttaaatctcaaaaaatacaaatccaacttattaaaaacaaaccttaaaaaattttaaaacccgaaaactaaaaaataaaaaacgctaaccttaaaatccaaacaaaaccaataataaccttctatactaataactcccaattttaaaattataaaatcatcctctaaaaatacgataaaaactataaaaccaatttccaaaaaaatacttccaacttacctaaaattttaaaaaatccacaaatactcattaaaacaaacaaaaaaacaaacaaaaaaccccaaattcttttaacttctaccaattcaactaattaaattataaaaaatttttttaaaaaactcctttctccatccaaacaacaacaatatccattttacctaaactctaaacttacaaaaaatcccacttaaaatataataaatattataaaaaccgaccaaatcgtaaaaaaacaataaacattaaaaaacaattaaaaccaaaaaacgatcaactaactaaaaaccttccctctctataaaaatctacatactacccctataaaccctaaactccaaaaaaataaacaacttaaaaaccttcttaaattatatcaacaaaaaaactcctctccaaaactctttcttaaataccccacttctacttctaaaaactattctcataacataaaccaccaccacgtctacaataactaaaccctacatctatttattacaaacctcgcaaataccatcttatcacccaccaaataacccaaatatcatcatcctccttttaaaataaaaaaactaaaactcaaaaactaaataactaactacaaatcacgctaaaacaaataacaaaactaaccaacaacctaaacctaaaactccaaaatcaatattccttccactacattacaacaaaacctctctaaactttattttaatcactaatatatacaaatctcttaaataaaaatatatataataacaaattatatcaatttctatatccctaaaaaaaataccttaatttctaattaacaaacaaaatttaaaaaaaaaactatatttatctctaaaacaaaaccttacttaaaataactcccccacccccctactaaaattccttcttataaaaataaactcttcactcactttcactccctataaataacataaatcttaacattttttttcttacgaaaaaaaaaaatataattcatataaataaatctaaatcaacccaaacaatccttaattaaccaaaactatacaacctccgccgcgataaatcctctctccatcccgctttaattaactatcccgtctaaactacgaattcctttcccctccaaccctttaaatcccacccctaccccaacgcaaaaaaatataaacttcaacaaacttaaatttctccgattttattctataatcgacgttttattctaaaaaatctcctcattattacgatttaaattctatattcttaacatacttcctctacttcgtaaatttcacataaaataacttaaactaaaccaatcaccgacaaaaaaaacgcatccgcaccgcactatttacgaccatctaaaacgcacccctccctaccttccgcctaaacccgaaaaaaaaaaaacctcttcccaattcaaaataaaactaacccctattttcgctctatatttaaacgcaaaattaaatcgtataaaaaattctcgaactcctacgaaacctttctaaatataaacgacgaaaactcaatactaaaacctaaaaatatcaacgtaattaaaaaaatactaaaaaaacaccaacctacacgctacaaaaacctctttaaaaacttcacataacaacaaaaaatacgaacgaaaacaacaataaaaaaacgcgcgaaaacgaaaattaaaaaaaacaaaataaccgaaaataaaaatttcacacctctcctaaaatctactctccttcctaaatccaaaaacccccaaacctccgaacctaaacaccaaccacccaattcccaatatttatttaaataaaatcttccgctctccaaaaacttatatcccgatcaaaactctttttataaccaccttcataaaaaatctcccaataaccccaaatctcctaacctaaacgataaacacgactcgataacccactaaccaaatctaaaaatacttaaaaaaaaaaaaaaaaatccaatctacgaaaccctcaaacgaaaaccgacctcaccccatttccgcacttcccaaattaccgaacgcgaatcccctcgattacgaaaccaaaaccttaaaataatcccaaaaaccaacccaacgacctacaaaccccgatcccaatacg

SEQ ID NO: 29 - DNA, 15764 bp, Artificial Sequence
  G to A (bis2 rc)
cgcactaaaatcgaaacctacaaaccgctaaactaactcctaaaatcatcccaaaattttaatctcgcaaccgaaaaaacccgcgcccgacaatttaaaaaatacgaaaataaaataaaaccgatcttcgcttaaaaatctcgtaaattaaacccctttttcccccttcaaacaccctcaaacctaaccaataaatcatcgaatcgtacccaccgcccaaaccaaaaaatctaaaactactaaaaaatctctcataaaaataactataaaaaaaaccctaaccgaaacacaaacctttaaaaaacgaaaaactctatccaaataaacactaaaaactaaataactaatattcaaacccgaaaatctaaaaatttctaaacctaaaaaaaaaaacaaactccaaaaaaaatataaaattcccactcccgaccaccttactctctccaacccccgcctccgcgcgtcctcctattactattcccgtccgcatcttctactattatataaaatttctaaaaaaacctctacaacgtacaaactaatactcttccaacatttcctcaatcacgctaacacccccaaaccccaacactaaattctcgccgtccacatttaaaaaaacctcgcaaaaattcgaaaatcctctacacgacttaactttacgcctaaatacaaaacgaaaacaaaaatcaatctcattttaaattaaaaaaaaacttccctcctcccgaacccaaacgaaaaacaaaaaaaaatacgtcttaaataaccgcaaacaatacgatacgaatacgtctctcctatcgataactaatttaatctaaaccatttcatataaaacccacgaaacaaaaaaaacatactaaaaacacaaaatttaaaccgcaataataaaaaaatttcctaaaataaaacgccgattacaaaacaaaatcgaaaaaacccaaacttattaaaatttacattcccttacgctaaaacaaaaataaaacctaaaaaattaaaaaaaaaaaaaacccgcaacccaaacgaaacaatcaaccaaaacgaaataaaaaaaaaacccatcgcgacgaaaactacataattttaattaaccaaaaactacctaaactaatctaaactcatttatataaaccataccttcccttcccgtaaaaaaaaaaatatcaaaattcatattatttataaaaaataaaaataaataaaaaactcacccccataaaaaaaaaccccaataaaaaaataaaaaaaccatcctaaacaaaactctatttcaaaaacaaacacaactttccttttaaaccctatctactaaccaaaaattaaaatattcctcccaaaaatacaaaaattaacataatttactatcacatacattcttactcaaaaaatttatatatatcaataattaaaacaaaactcaaaaaaactttactataatacaataaaaaaaacactaactttaaaattccaaacccaaactactaaccaactttatcacttaccccaacgtaacttataaccaatcacccaatctctaaaccttaatttcctcacctcaaaaaaaaaataataatacctaaaccacttaataaataacaaaataatacctacgaaatctataacaaacaaatacaaaatttaatcactataaacgtaataataatctataccataaaaataatttccaaaaacaaaaataaaatatccaaaaaaaaattttaaaaaaaaaccttcctactaatataacttaaaaaaacccccaaactacttatctttctaaaattcaaaatctacaaaaacaatatacaaacccctacaaaaaaaaaaaacttccaatcaactaaccgcctcctaaccctaactactctccaatatccactaccttcccacgacctaaccgaccctcataacactcaccacactctaaataaaatttcttacaaatttaaaatttaaataaaataaatactactattacttaaataaaaaaaaaaaccttttaaaaaaatccctcataatttaaccaactaaattaataaaaactaaaaaaatctaaaattttttacttatttccttatttattttaataaatacctataaacttcctaaaatctcaaacaaattaaaaatatttttctaaaaactaactccataacttccatcgtattctcaaaaaataaccccataaccccaaaactaaaaactactaatataaaaaattatcactaatcctacctaaattttaaaattaacgccttttattcttcaatctccgaatcctaaaaccttttaaaacctactcttaacaaattaaatctatattccctaaaatccaaatacatataattttcaaacacaaaaaatcaaaaaaaatccataactaaataacaataaatactaaatatttccaaaacccgttacccaccgcccccacctacaaataaaataattatccttttcccccacaaacttctcccctaaactctttccatttaaaacacacacacacacacacacacacacacacacacactaaactctatatcaataaaactcctttaaaatcctatctatcctccccactccaacttctattttataaaaataattatattttaaacacttaaaacattaatttaataaacacattatatttactttcatatttaattatatatttttaaattattccacacaaaataacaaataaaaacaaaaaaaaaaaataccataaaatatataaaaacgcaccccccaaaaacgctcaacaatcaatcaaaaattcttaaaaaataaaaacaactacgaaaccctaccccaacccaatcaaaacatcccacccgaaaaaaaacgacttatttcttttttctattaaaaataaataataaactaaattcgatttaacgatattttcttaactaactctcgactacaatcaaaccattttcgaacacattcccatataaataccaaaaatactctaaaaaaaactatcgacgcctattcaactaatttaaattttctttatctaattactataaaacttaaaaaaaaaaaaccgactcaaaacaataaactaacactcgatctctatatataatatccaaacaaaatttaataaaaaaaacctacttccactcaacctcaaatcactatctaaaaccaaccccgacccacccccctcccacatacccctcccctccccacccgccctctctacatctacaaccccaccaacacactcaaccaaaaacaatcccccgacactccaaaaacacacaaaactcctaccgccccaaaaaacctacctaaactatacgactataaaaactctttacctaatatcttcctcctaattactacacaacctccctttctcctacctcctacaactccccaaactccccaacaaacacacccgtacacctcgatcctttcaacctaaacgcaacgaaatacccaactctacctcctatttaatccgctaatctacaacaccttctttctaaacctcccccttcaacccttaaaaaaccccgccaactccgacctcctactctcctcctccctctcccaactcctatccctaatcgaactacatttccctacacgtataatccaataactaactatcgaatctcattaaaaataattactcccgaaaacacatctctctcaaaacctaactcttacttaaaaaaaaattaaccacaactaaaaaaaaatattctcgaacaaaaattaactaaaacctaacacaattttaaataaacaatattaaaacgaaaaatataaacctaataacaactacacaccccttcaaaactaactataaatataaccatctcgcttatctcaaaatctttctttttctttctctttctttcttttcttccttccttcctttttcttttacacttttttcttacaaaacactaactaaaatacgaaaataaaaaaaaaaaataaaaacaaatacaaccctaaatcccataaaatccaaatttccaaaatctttaaaacttaacctaaatttctcaatataaatccctctactcaaaattccgaaaacgtccacgatcgccaacgacccgcaaccctacgacgacccccaatcgccctaacaattatcgaaaaacctacaaaccctaccaaaaaaaaaaaaaattaacacgttacctttaaacgtctaacaccccgacgtataactaaaaacgacaaaatctaaacgaaattaacaaataaaatcaatatcgaccctaaaaaaaacgaccaaaaaaactccgaacaaccgcacccgcaacaacaccactcgacccgacgaaccaaaaaaaaaaaaaaaacgcgaaaaaacgaaactaaatcctaaaataaaacgcgaaacttactacgaaaaacaaacaaaaaaaatatttcataaaatcaaaaataatcgaattttacgaaaaataaaaatcgtccccctaacaaaaccgaaataaatctataatccctcaattaaaaaaaaaataaataaaaaaaaaaaaaaaaaaccgcgaaaaaaataaaaaacgaaaaaaccctaaaaaacgaaaaacgaaataaaaaaaaaaaacgaccgccaaatcgaaaaaaaaaaaaataaacgcgacgacgcgaaacgaaaaaaaaacaaaacgaaataaaaaaaaaaaaaaaaaaaaaaaaaacgaaaaaaacgaccgaaaaaaacgaaaaaaaaaaaaaatccgaaaaacaaaacgaaaaacgctcctaaaaaaaaacgtcgaactcgtccccgaaatccaaaccgcgatcccactcgcgaacgcaatcgcccgacgccgaccgctcgaccccgcgacctaaaaaaccgttacgcaaaacaaaacccgcgactcgaaaaaaaatacgccgaacgttacctcccgcccgccgccgccgccgccgccaaaaaccccaaaaaaactaaaaaaaacgacgccgaaacgctaacccgaaataaccacgactacaacccgaacgacgaactaaaacgctcgcaaaacttctaaaccgaccccgctccgacgcctccgcttcccgcccgaaacccgccctcgcgacccgacctcgctcccgaatcccaaataaccaccgaaaacgaaccgccgccgaccccgctccgccgcgcgtacaacccgatccccgacgcgctccaaaccgccctaataaacccgccgcccgccgccgccgccgccgccgccgccgccccgaaaaccacctcctcctcctcgtcgtcgtcctccgcctcctacgcctcgtcctcgtcctcctccaattcgaccaacgccccctcgactacctacaaaaacgcgaacgacgacgacgcgaacgccgaaaacgaaaacgccaaaaaaacgaactcgaaactacgacgacccgaaaaaccgccctactcgtacatcgcgctcatcgtcataaccatccaaaactcgcccaacaaacgcctaacgctcaacgaaatctaccaattcctacaaacgcgcttccccttcttccgcgacgcctaccaaaactaaaaaaactcgatacgccacaatctctcgctcaacgaatacttcatcaaactacctaaaaacctcgaacgacccgacaaaaaccactactaaaccatcgacccgaccaacgaattcatattcgaaaaaaactcgttccgccgccgaccgcgcgacttcaaacgaaaataccaaacgctcaaacccatataccaccgcgtaataaacgacttaaacttcgaaacgtcgctactaccccaaaacttcgacttccaaacgcccccgtcgacgccgctcgactaccacaaccaaaacgactacgacgacctcgacataatacccgcgaactacgacgccgacgcgaacgcccccaaccacgcgcaccctcaccaccaccaccaccaccacgtcccgcacatatcgcccaacccgaattccacctacataaccaactacccgatacccgcgaaacccgaaaacgtcgatacgaccgaaaacgacgacgacgacgactacgaaccgaacaacaacaacaacccgataccctcgtccccgaccataacgaacgccatcgaataccactcgccctacacgaaccctacgacgcactaaaactcgcctaacgcctcgccttacctcaaacaaccgcctaccctaacgcccaacaacaaccccgccgcctcgacaaacctacactccaacatatcctcctactcgctaaaacaaaactacttacaccaaaacgctcgcgaaaacctctcaaataacgcaacacgctccaacccaaccaactaaacgcaccgcttctaaacctccaaaactaacgaccactaccactcccacaaacaaaaaccccgaaactaaaaaatctaaaaacactaaaaaaaacaaatactaaaaaaaaccgacatcttattcgtaaaaacaaaaatcaaaatcttactatcctcccaatatccctaaccaacaaccgaaacttcaaaattatctaactactataaacgtaatataaaatcccctaccttcctaaactctttaaaaatccctatacaaaaaactacaaatctcccgttcaaaatctcacttaacttaaaaaaaaaacatctaacctttaaaaaacttaatcaaaaaactatatctaattccttttatccctttttttccttacgttcattttactatacttctatcccgaaataaatatcaaaatcaaatatattctatatattaaaatatctacaacgaaatatttacaactaaacaaatattaaaaaaaaaaaataaaaaaaacaaaactaaatcccaaaatctttcactaaaaaaacatttaccaataaaaaaaatcaccaaactattaaaaactcctccccttccctacctccccccccgcccaacaataaacccacattaataatacaaatcctaaataacaaaacctaaaaaaccctactaaaactcccctaaaaaatacgcctaccctataaataccacttataatataactaatttacattattctaattacaaattataaaaaattattaacttactaaaaacgataaaaaataaaaaaaaacgataaaaataaaaaaaaaaatttaaatatttaaccaaattaatataaaaaacaaaaataaacccttacattaacccctcgctcgaaacacctaaaactacaaattaaaatcccataaacctaccaatcaaaaacaaaaccccaaactactctctcacactaacctcccacaacaataaaacaataacttaaaaaataatacatactttatatattcctaaaccgatatacaacgaaaacacccgaaaaaaaaaaaaacccaaaaataaacaaaaaatattaattccctaaacgataaaatttcccaaataaaccttttaaatataaatctcaaaaattaaccaaacaaaaacaatctcgacaaaaccacaccgaaaaaaattttaacctaacttaacccactaaaaacaaaatcttattcaattttataaaaatttcaacaaataaccaatacaaacgaccttcccctcttatttttatattcccttaaaccgactatcaatcacacacacacacacacacacacacacacacacacacacacacccctcgatacactaaccccttcccttccccgcctacctactcctctcccaacctaccaactaccctccctactccccttcttctcctctcccgacaaatccactcaacttaaacccgaactctaaaacttaacaaccttaaaaaaaccgtactctaaaaaaaaaaaaaaacacacaaaaaaaaaactcctaacccttcctcaaaactactctcgccccacctcataacactaaacgcaaacacaaactcccaaaacttcgaaatctaaatacattactatcttaaaaaaaataaaaactacccaacaaaacaaaccgacctctatacccctacccaacgacctcccgcgaccgaccttccctaaaaacctcgcaaaacccccgaccgaatctaaaaacgcccgaaaaaaacaataactcgaacctaacgcccgacaaaaaccctctacccttccttcctcgctatcttactcccgtccctataaaatacccacccgaccctattaccatctccctaaaacgccaacgataaaaacttcgaaaaaaccgaccgaatacaccgaaaccccgcgaaacctaattaaaaacgcgccgcccactaaaacctaaaaacccgacgaaacgcgaaaataaccaaaacaatctccccgacacacaaatcaacacatatctacgcgcacacacccaacacgaccctccctcccccaacacaccccaaaaaccgcgccctccgctcctaaacctaataaccataatccatatacccctaccgacgcaaaaactaccctaaaattctccattaaaccctacgaacacttcaaaaaaaaactcgaacttctatcatcccgctcaacacatcaaaacgccgacgaccgccttcgtaaacaaatataaacgctcgccctctctcctcccgaacctactattttataatccaaaacttaccatcaaaacttactttaacgcgacgaaaaaactcacctatatacaaaacgccgcgcacacatcgaaactcgcgaaacaaaacaactacgttaacgcaacgccgaatatattcgaataaatattacgaacaaaaaaataaacaacgacccctaaacaaccgcctcgctccgacattacgaaaacacgacgaaactaaaaccacgaaaacaaaacccgaacccgacgaaccgtaattacgattttcttacactaaaaaactaaatccgacccgaaacgacgtacactttataatccccacaccactcgattaactaaaaaaaaacccgaacgaataaacctaacgcaacccgataccgaaaaaacccgatccaacaacctctaaaacccaatacgcaaaacactacgaaccgattacgccccgaaaccaaaaaacgccgaaaaaacaaaaacaaaaaccgacgacgaataaaaatcaaacgacccgatacaaaccgaaaaccgaaaaaccgccccgaaaaaacaaaatccaaaccttctctatccccctccaacctaaaactacctcaaaaactcctcgcgctaccaaatacttcgaaccaaaaaacatttctctacgccctaaaatcccgacttctctaaaaaaaatctaaaacgttcgaaacccacgaaaatacctacgaaaaaacaaaaaaaaaaacgtacttttctaccccatcccttcatcttacgattaaattattttctatcgtcccctttaacacaaaaaatcctctacgctcgctactataaccgacccaattaattaaaaaacaaaactcaaaaaaaaaaccgcaataatatttctaaaataaaatacttaaccctccctaaaaccaaaactcaaaacaacacaaaccaaaaactctaccgaaaaaaacccgaaaccaaaatctaaatctaattatccgatacctatactcattctaaaattaaaatacacgccccaacctcaaaaaataaaattaaaattccaaaacataaaaatccccctcgaaaaaaaacttactctatatttatacgaacatcaaaacaaaacataataattccaaaacaattctataacgtacaattaatatatttaaactacttctaaaactaaactttctctaccaactatctaacaatttactaaaaaacacaacaacaccttttatactctaaaacaaaataaaacaccctaccatccactaaataactttatttctaaaaaaatttttttttctttcttctttcaataaaactaccccgttaccaacatcactctactccaatatataacaaaaaaaatttcgtcctcaacttcaataaaatttcttctttccatccctcaactaacgaatcgtattatcaccatcaccaccaaaacgtctatcaaaatattaaaccctacgtcatataaacgaaaaaaaaccaaacgataaccgctctctcctctcccctcctcaaaaaaaacaaataaaaactaaaacgaattcaaatcacatacacgcgaataacaataaaccacacacctaccacttaaccaaaatacccaaaatcgcgttaatcactattatttacctactactaaaaaaaaaacaaccgctaacaaaataacgttccccaatctaaatacctacaaactcccacataaaaaaaaaaacaaactcaaataaaaaaatataccatacgtaaaacatcaacgtatatctataaaatcttcgttaccttcaataatcaaaatataaaaaaaacaaacaaattatatatatatatatatatctaaaaaaacttatatacttttcaaaaaaacaatactaaacacaaaatttcaaaaaaacctcttcttattacctaactaaataaaaaaatcattttccccaaacactacatttaaatacaaataccaaaaaacattattaaaaaattatttaaaaacaatatatctaatttaaaaaaataattttcaatattataacaatacaacgtttttacaaaattattttctaccaccatattttaaaaatatttttataaccgtatatactcacactttacttatattttaaaaaaaaaatatatttacacttatatatacttttacaatttaccaaaatattttattataaaattttttttcaataaaatatatataacaaataattattttaaaaactaattttctcttcgaacaccctaaaaacaataaataccaatttctcctccccgacaaacaactatacaactctacccacaccccctccaataatataactaacataatataaaatctataccttaaataacacaaaccaaattctaattataaatcttctcaaaaaaaaaacaataaaaaaaacgttttctattatttctttctttacttcaccccaactttttctaacaaaacaaaaaccaaaaaataaaaaaaactaaaaaaaaaaccaaacaaaataccgaccaaaatttaattttaaaaaaaccaattttataccccttctattttctttcctatacccgaaaaatattctaccctttaccctctctccctcccgactaacataaattaacaaatataaaacacaataataaacccccctccaaaattaaatacccaaaaaacaacaccctacttcttccctttacacgttacaattttattataaataacgatcacatactatcaaaaataaaattcaaatctaaaaaatacaaaaaaatccctaaactacaaaaaacaaactcccaacaaaaaatttaacttccttaaaaaatttaatacaaaaactaaactccccacacgttactctataactacgacctatcccaccctccaattcaaaacctaactaaccctactcaacatcgacacataacaaaccgattcaacccttccttcctcccgacctcctctccccactcctcccttttaaccaaaaatttaacaaaaaaacccctcaacccctttttctattcctactaaatttcccaatcaccaatattacaaacaaaactaataacgctcccgataaaaaaacaaaataaaccaactaaacaaaaaaactaaccttctatcccaacaacccttcaccatcacgaaccatattaaaaacaataaatctaaaaaaaacaaaaaaattatctactccaatcatactatacattttcctctccaattcaaaactaaaattttatttttattttttactttttctttcttaattaaaaaactcacctttatttcttatcccttaaaaaatctttctcccaatcaatcaccaaactcttaatattcgtaaaaaactatttcacaccccaaaatttttatattctaaataaatttcactacaaaaaacgtctcctaaataaaacatcttatttccgaaaatcttaaccatctttctaatctttaaatttccttcctatatcttctaaaattaaaaaataatttaaacattttttatctctccattatcatatttacaattaaataaaacctttttattttcttttataataaactactcgaaaacctactataaattataaaatcaatttcaaaatttactccgaccacaatactatatttacattccttccgaaacaaccgacataatcgtaatttatatcctaaacacttaaacgtaacttatttatacaaaaaataacaaaacctcaaaaacgaaaactacgtctacctacctaaccgcattaaaaaacccaacgcgccccctaataacgcgaaaaaatccgcccaaaacgactcaataattccttcaaactacgcaaaaacttaacaaaataacccgttttataataccttccaataaaaacatttttaaatatctcactttcataaattataatttccaattttaaaaaatactttactttcttctttcttcttcttcctttttttttttttttttaaaacaaaatcgtaatctattacccaaactaaaatacaataacacgatctcaactcactacaacctccaccgcctaaactcaaataatcctcccgcctcaacctcctaaataactaaaaccacaaacacgcaccaccatacctaactaattttttaatttttataaaaacgaaatcttacctcgttacccaaacgtaaacttttttctattttactcttttcgcctactatctcatcctaaaaccaaatcacaattcaataaaaacaaacctaaccatactcaacaaatactaaaaccctaacttactacgtatattcttcatttctacatttctccccaaataaaactattattttatttccttttaaatcaaaattatttctctcctaactatccctcaaaaacacacacgtacacataaactcatttatattcacccttttttttttttttttaaaaaaacatacaatacttaactttaaaaattactcaaatattaataattaaattaaaaaaaaatactacacctttataaataaaaataaataaactaactcaactaaaaataaatacctcaactattttttcgtcaaataaattttaaacttaaattttctactcattaacgaaataaaataatatattaaaaaattttattattttctataataattattattttttattaatttcattaaaactatatacataaaaacaaaaccaaaaaactactaaacatcatacatcaaatactaaacaccgtaactatcttaccaaatctcacacgactatcttacttaattctatcaatatccctctaaaatactaatattaaccttatttacaaatctatactaactcctaactaaatcataactttaaaaaatttaacccatatcttctaatttcaatttatttccctcgtttctccaacactacctctaaaaattttacaactaacactacaaatctttaaataacaaaaatattccctctaaaacaacaattctcacacttaaatacacatcaaaatcacctaaaaaacttattcaacacaaactataaatccaccccaccctccatttctaattcaataaatccaaaattatattcaaaaatatatattcctaataaactaataaaaaaaaataatactaataatattaatcctaaaaccacactctaaaaactacaactcttaaaaaacaatttcgattacaaatctttttataaattccaataaataaatattaaaaataacctattaattaattaaacaaaaatctaaaaaaatttttcaaataatttatccatctaaatacctctataattaattataaacccctaaaaaaatacaaaacttaattttaaaccctaaaccaaaaaataaaatctccccatttttattcaaaacaataaaacctcttattttattataataaacattacaaaaaaaaatcaaataaaatcattaaaatctacctacctcaataaaacaataaatctaaatacttacacacaacaaccaatcaaaattctacaaacaaaaaaaaacaataataaaaacaaacaaaaaaaaaaactccattattaattataaaaccttttaaaaataaaacaaaaaaaaaacaaaaaaaaaaaactataatctcaaaaaataacaataataatccctaaatataaataaataaacaaaaccgtaaataaaaaaaaaaaaaaaacaaaaaaaaaaaaaaaaaaaaaaaaaaaaaaaaaaaaaaaaataaaaacaaaaaaaaaaaaaaaaaaaaaaaaaaataatcaaaaaaaaaaaaaaaaaaaaaaaaaaaaaaaaaaaaaaaaaaaaaaaaaaaaaaaaaacacataaaaaaaaaaaaaaaaaaaaaacgaaaaaaaaaaaaaaaaaaaaaaaaaaaaaaaaaaataaaaaaaaaataaaataaaataaaaaaaaaacaaaaaaaaaaaaaaaactaaaaaaaaaaaaaaaatacacaaaaaaaaaaaaaaaaaaaacaaaaataaataaaaaatataaaaaaaaaaaaaaaaaaaaaaaaaaaaaaaaaaacaaaaaaaaaaaaaaaataaaaaaaaaaaaaaaaaaaaaaacaaaaaaaaaaaaataaaaaaaaaaaaaaatctaaaaaaaaaaaatctacaaacatttcctaaactcctatccctaaaactaaaaaacaaccctaaaaactaaattcctatcctctaaaaccaccattctctctccaaatccccaataccaacccacgaactaaaaaacccataaacttctattttacttaacttaacctaaattctaaaaaaataaataaattctctaattatacataatcaaattttctaaactaccacaacgacttatacaaaattaaaaaaaacaatcttaacttaaattttaaaaaataaaaatccgatttctaaaaaaaatcttcaaatccctaaaataaaccacgatataacattaaaaaaaattaacaactccttcccaaaaaaaacactctctttataaattcgtattatacctaattactctacatcataataattaattcaaaacaaacactaacttacttaaaataaaaatatattttaatatattttatccgaacgaaaatacattttaccaaacctacctctataaaacactatcttaacaaaaaaaaacaccacaaatataaacataaccaaaaaaaaccaaaacacacaaacgtcaaaatcattaaaaaaaaaataaaaatcctaaaaattctttttaaattcaaaataccccaaatccacaacaatccaactaataaatattcatctctccatatcctaaaaaacgtatataaaatacgaaaccttaaccatcccacgactacatcgccaaacctataaacttaactatattcacgaaaacacaaacgaaacgaacaacgaaacaactttccctccgaaaaacccattccaccctccaacctaacaacgaaaactcgatcacaaccgaacaataactcgtctaccgaataacacgacctcacctccccaaactaacaaaacacctccccctcaaatttaaaaaccgctataaattaaataaaatccaaacctaaaatataaaaaaaaaaaaacctacctcctcgctcctccttcaacaactccacgcaacacaaaacgaaaatatcgataaaccgtattaattaactaactaaaccccaacgcgccgta

SEQ ID NO: 30 - DNA, 15764 bp, Artificial Sequence
  G to A (bis2 rc) rc
tacggcgcgttggggtttagttagttaattaatacggtttatcgatattttcgttttgtgttgcgtggagttgttgaaggaggagcgaggaggtaggtttttttttttttatattttaggtttggattttatttaatttatagcggtttttaaatttgagggggaggtgttttgttagtttggggaggtgaggtcgtgttattcggtagacgagttattgttcggttgtgatcgagttttcgttgttaggttggagggtggaatgggtttttcggagggaaagttgtttcgttgttcgtttcgtttgtgttttcgtgaatatagttaagtttataggtttggcgatgtagtcgtgggatggttaaggtttcgtattttatatacgttttttaggatatggagagatgaatatttattagttggattgttgtggatttggggtattttgaatttaaaaagaatttttaggatttttattttttttttaatgattttgacgtttgtgtgttttggttttttttggttatgtttatatttgtggtgtttttttttgttaagatagtgttttatagaggtaggtttggtaaaatgtattttcgttcggataaaatatattaaaatatatttttattttaagtaagttagtgtttgttttgaattaattattatgatgtagagtaattaggtataatacgaatttataaagagagtgttttttttgggaaggagttgttaattttttttaatgttatatcgtggtttattttagggatttgaagattttttttagaaatcggatttttattttttaaaatttaagttaagattgttttttttaattttgtataagtcgttgtggtagtttagaaaatttgattatgtataattagagaatttatttatttttttagaatttaggttaagttaagtaaaatagaagtttatgggttttttagttcgtgggttggtattggggatttggagagagaatggtggttttagaggataggaatttagtttttagggttgttttttagttttagggataggagtttaggaaatgtttgtagattttttttttttagatttttttttttttttatttttttttttttgtttttttttttttttttttttttattttttttttttttttgtttttttttttttttttttttttttttttttttttatattttttatttatttttgttttttttttttttttttttgtgtattttttttttttttttagttttttttttttttttgttttttttttattttattttattttttttttatttttttttttttttttttttttttttttttttttcgttttttttttttttttttttttatgtgttttttttttttttttttttttttttttttttttttttttttttttttttttttttttgattatttttttttttttttttttttttttttgtttttatttttttttttttttttttttttttttttttttttttttttgttttttttttttttttatttacggttttgtttatttatttatatttagggattattattgttattttttgagattatagttttttttttttgttttttttttgttttatttttaaaaggttttataattaataatggagtttttttttttgtttgtttttattattgtttttttttgtttgtagaattttgattggttgttgtgtgtaagtatttagatttattgttttattgaggtaggtagattttaatgattttatttgatttttttttgtaatgtttattataataaaataagaggttttattgttttgaataaaaatggggagattttattttttggtttagggtttaaaattaagttttgtatttttttaggggtttataattaattatagaggtatttagatggataaattatttgaaaaatttttttagatttttgtttaattaattaataggttatttttaatatttatttattggaatttataaaaagatttgtaatcgaaattgttttttaagagttgtagtttttagagtgtggttttaggattaatattattagtattatttttttttattagtttattaggaatatatatttttgaatataattttggatttattgaattagaaatggagggtggggtggatttatagtttgtgttgaataagttttttaggtgattttgatgtgtatttaagtgtgagaattgttgttttagagggaatatttttgttatttaaagatttgtagtgttagttgtaaaatttttagaggtagtgttggagaaacgagggaaataaattgaaattagaagatatgggttaaattttttaaagttatgatttagttaggagttagtatagatttgtaaataaggttaatattagtattttagagggatattgatagaattaagtaagatagtcgtgtgagatttggtaagatagttacggtgtttagtatttgatgtatgatgtttagtagttttttggttttgtttttatgtatatagttttaatgaaattaataaaaaataataattattatagaaaataataaaattttttaatatattattttatttcgttaatgagtagaaaatttaagtttaaaatttatttgacgaaaaaatagttgaggtatttatttttagttgagttagtttatttatttttatttataaaggtgtagtatttttttttaatttaattattaatatttgagtaatttttaaagttaagtattgtatgtttttttaaaaaaaaaaaaaaaagggtgaatataaatgagtttatgtgtacgtgtgtgtttttgagggatagttaggagagaaataattttgatttaaaaggaaataaaataatagttttatttggggagaaatgtagaaatgaagaatatacgtagtaagttagggttttagtatttgttgagtatggttaggtttgtttttattgaattgtgatttggttttaggatgagatagtaggcgaaaagagtaaaatagaaaaaagtttacgtttgggtaacgaggtaagatttcgtttttataaaaattaaaaaattagttaggtatggtggtgcgtgtttgtggttttagttatttaggaggttgaggcgggaggattatttgagtttaggcggtggaggttgtagtgagttgagatcgtgttattgtattttagtttgggtaatagattacgattttgttttaaaaaaaaaaaaaaaaaggaagaagaagaaagaagaaagtaaagtattttttaaaattggaaattataatttatgaaagtgagatatttaaaaatgtttttattggaaggtattataaaacgggttattttgttaagtttttgcgtagtttgaaggaattattgagtcgttttgggcggattttttcgcgttattagggggcgcgttgggttttttaatgcggttaggtaggtagacgtagttttcgtttttgaggttttgttattttttgtataaataagttacgtttaagtgtttaggatataaattacgattatgtcggttgtttcggaaggaatgtaaatatagtattgtggtcggagtaaattttgaaattgattttataatttatagtaggttttcgagtagtttattataaaagaaaataaaaaggttttatttaattgtaaatatgataatggagagataaaaaatgtttaaattattttttaattttagaagatataggaaggaaatttaaagattagaaagatggttaagattttcggaaataagatgttttatttaggagacgttttttgtagtgaaatttatttagaatataaaaattttggggtgtgaaatagttttttacgaatattaagagtttggtgattgattgggagaaagattttttaagggataagaaataaaggtgagttttttaattaagaaagaaaaagtaaaaaataaaaataaaattttagttttgaattggagaggaaaatgtatagtatgattggagtagataatttttttgttttttttagatttattgtttttaatatggttcgtgatggtgaagggttgttgggatagaaggttagtttttttgtttagttggtttattttgtttttttatcgggagcgttattagttttgtttgtaatattggtgattgggaaatttagtaggaatagaaaaaggggttgaggggtttttttgttaaatttttggttaaaagggaggagtggggagaggaggtcgggaggaaggaagggttgaatcggtttgttatgtgtcgatgttgagtagggttagttaggttttgaattggagggtgggataggtcgtagttatagagtaacgtgtggggagtttagtttttgtattaaattttttaaggaagttaaattttttgttgggagtttgttttttgtagtttagggatttttttgtattttttagatttgaattttatttttgatagtatgtgatcgttatttataataaaattgtaacgtgtaaagggaagaagtagggtgttgttttttgggtatttaattttggaggggggtttattattgtgttttatatttgttaatttatgttagtcgggagggagagagggtaaagggtagaatatttttcgggtataggaaagaaaatagaaggggtataaaattggtttttttaaaattaaattttggtcggtattttgtttggttttttttttagttttttttattttttggtttttgttttgttagaaaaagttggggtgaagtaaagaaagaaataatagaaaacgttttttttattgttttttttttgagaagatttataattagaatttggtttgtgttatttaaggtatagattttatattatgttagttatattattggagggggtgtgggtagagttgtatagttgtttgtcggggaggagaaattggtatttattgtttttagggtgttcgaagagaaaattagtttttaaaataattatttgttatatatattttattgaaaaaaaattttataataaaatattttggtaaattgtaaaagtatatataagtgtaaatatattttttttttaaaatataagtaaagtgtgagtatatacggttataaaaatatttttaaaatatggtggtagaaaataattttgtaaaaacgttgtattgttataatattgaaaattatttttttaaattagatatattgtttttaaataattttttaataatgttttttggtatttgtatttaaatgtagtgtttggggaaaatgatttttttatttagttaggtaataagaagaggtttttttgaaattttgtgtttagtattgtttttttgaaaagtatataagtttttttagatatatatatatatatataatttgtttgttttttttatattttgattattgaaggtaacgaagattttatagatatacgttgatgttttacgtatggtatatttttttatttgagtttgtttttttttttatgtgggagtttgtaggtatttagattggggaacgttattttgttagcggttgttttttttttagtagtaggtaaataatagtgattaacgcgattttgggtattttggttaagtggtaggtgtgtggtttattgttattcgcgtgtatgtgatttgaattcgttttagtttttatttgttttttttgaggaggggagaggagagagcggttatcgtttggttttttttcgtttatatgacgtagggtttaatattttgatagacgttttggtggtgatggtgataatacgattcgttagttgagggatggaaagaagaaattttattgaagttgaggacgaaattttttttgttatatattggagtagagtgatgttggtaacggggtagttttattgaaagaagaaagaaaaaaaaatttttttagaaataaagttatttagtggatggtagggtgttttattttgttttagagtataaaaggtgttgttgtgttttttagtaaattgttagatagttggtagagaaagtttagttttagaagtagtttaaatatattaattgtacgttatagaattgttttggaattattatgttttgttttgatgttcgtataaatatagagtaagttttttttcgagggggatttttatgttttggaattttaattttattttttgaggttggggcgtgtattttaattttagaatgagtataggtatcggataattagatttagattttggtttcgggtttttttcggtagagtttttggtttgtgttgttttgagttttggttttagggagggttaagtattttattttagaaatattattgcggttttttttttgagttttgttttttaattaattgggtcggttatagtagcgagcgtagaggattttttgtgttaaaggggacgatagaaaataatttaatcgtaagatgaagggatggggtagaaaagtacgtttttttttttgttttttcgtaggtattttcgtgggtttcgaacgttttagattttttttagagaagtcgggattttagggcgtagagaaatgttttttggttcgaagtatttggtagcgcgaggagtttttgaggtagttttaggttggagggggatagagaaggtttggattttgttttttcggggcggtttttcggttttcggtttgtatcgggtcgtttgatttttattcgtcgtcggtttttgtttttgttttttcggcgttttttggtttcggggcgtaatcggttcgtagtgttttgcgtattgggttttagaggttgttggatcgggttttttcggtatcgggttgcgttaggtttattcgttcgggtttttttttagttaatcgagtggtgtggggattataaagtgtacgtcgtttcgggtcggatttagttttttagtgtaagaaaatcgtaattacggttcgtcgggttcgggttttgttttcgtggttttagtttcgtcgtgttttcgtaatgtcggagcgaggcggttgtttaggggtcgttgtttatttttttgttcgtaatatttattcgaatatattcggcgttgcgttaacgtagttgttttgtttcgcgagtttcgatgtgtgcgcggcgttttgtatataggtgagttttttcgtcgcgttaaagtaagttttgatggtaagttttggattataaaatagtaggttcgggaggagagagggcgagcgtttatatttgtttacgaaggcggtcgtcggcgttttgatgtgttgagcgggatgatagaagttcgagtttttttttgaagtgttcgtagggtttaatggagaattttagggtagtttttgcgtcggtaggggtatatggattatggttattaggtttaggagcggagggcgcggtttttggggtgtgttgggggagggagggtcgtgttgggtgtgtgcgcgtagatatgtgttgatttgtgtgtcggggagattgttttggttattttcgcgtttcgtcgggtttttaggttttagtgggcggcgcgtttttaattaggtttcgcggggtttcggtgtattcggtcggttttttcgaagtttttatcgttggcgttttagggagatggtaatagggtcgggtgggtattttatagggacgggagtaagatagcgaggaaggaagggtagagggtttttgtcgggcgttaggttcgagttattgtttttttcgggcgtttttagattcggtcgggggttttgcgaggtttttagggaaggtcggtcgcgggaggtcgttgggtaggggtatagaggtcggtttgttttgttgggtagtttttattttttttaagatagtaatgtatttagatttcgaagttttgggagtttgtgtttgcgtttagtgttatgaggtggggcgagagtagttttgaggaagggttaggagttttttttttgtgtgtttttttttttttttagagtacggtttttttaaggttgttaagttttagagttcgggtttaagttgagtggatttgtcgggagaggagaagaaggggagtagggagggtagttggtaggttgggagaggagtaggtaggcggggaagggaaggggttagtgtatcgaggggtgtgtgtgtgtgtgtgtgtgtgtgtgtgtgtgtgtgtgtgtgattgatagtcggtttaagggaatataaaaataagaggggaaggtcgtttgtattggttatttgttgaaatttttataaaattgaataagattttgtttttagtgggttaagttaggttaaaatttttttcggtgtggttttgtcgagattgtttttgtttggttaatttttgagatttatatttaaaaggtttatttgggaaattttatcgtttagggaattaatattttttgtttatttttgggtttttttttttttcgggtgttttcgttgtatatcggtttaggaatatataaagtatgtattattttttaagttattgttttattgttgtgggaggttagtgtgagagagtagtttggggttttgtttttgattggtaggtttatgggattttaatttgtagttttaggtgtttcgagcgaggggttaatgtaagggtttatttttgttttttatattaatttggttaaatatttaaatttttttttttatttttatcgtttttttttattttttatcgtttttagtaagttaataattttttataatttgtaattagaataatgtaaattagttatattataagtggtatttatagggtaggcgtattttttaggggagttttagtagggttttttaggttttgttatttaggatttgtattattaatgtgggtttattgttgggcggggggggaggtagggaaggggaggagtttttaatagtttggtgattttttttattggtaaatgtttttttagtgaaagattttgggatttagttttgttttttttattttttttttttaatatttgtttagttgtaaatatttcgttgtagatattttaatatatagaatatatttgattttgatatttatttcgggatagaagtatagtaaaatgaacgtaaggaaaaaaagggataaaaggaattagatatagttttttgattaagttttttaaaggttagatgttttttttttaagttaagtgagattttgaacgggagatttgtagttttttgtatagggatttttaaagagtttaggaaggtaggggattttatattacgtttatagtagttagataattttgaagtttcggttgttggttagggatattgggaggatagtaagattttgatttttgtttttacgaataagatgtcggttttttttagtatttgttttttttagtgtttttagattttttagtttcggggtttttgtttgtgggagtggtagtggtcgttagttttggaggtttagaagcggtgcgtttagttggttgggttggagcgtgttgcgttatttgagaggttttcgcgagcgttttggtgtaagtagttttgttttagcgagtaggaggatatgttggagtgtaggtttgtcgaggcggcggggttgttgttgggcgttagggtaggcggttgtttgaggtaaggcgaggcgttaggcgagttttagtgcgtcgtagggttcgtgtagggcgagtggtattcgatggcgttcgttatggtcggggacgagggtatcgggttgttgttgttgttcggttcgtagtcgtcgtcgtcgtcgttttcggtcgtatcgacgttttcgggtttcgcgggtatcgggtagttggttatgtaggtggaattcgggttgggcgatatgtgcgggacgtggtggtggtggtggtggtgagggtgcgcgtggttgggggcgttcgcgtcggcgtcgtagttcgcgggtattatgtcgaggtcgtcgtagtcgttttggttgtggtagtcgagcggcgtcgacgggggcgtttggaagtcgaagttttggggtagtagcgacgtttcgaagtttaagtcgtttattacgcggtggtatatgggtttgagcgtttggtattttcgtttgaagtcgcgcggtcggcggcggaacgagtttttttcgaatatgaattcgttggtcgggtcgatggtttagtagtggtttttgtcgggtcgttcgaggtttttaggtagtttgatgaagtattcgttgagcgagagattgtggcgtatcgagtttttttagttttggtaggcgtcgcggaagaaggggaagcgcgtttgtaggaattggtagatttcgttgagcgttaggcgtttgttgggcgagttttggatggttatgacgatgagcgcgatgtacgagtagggcggtttttcgggtcgtcgtagtttcgagttcgtttttttggcgttttcgttttcggcgttcgcgtcgtcgtcgttcgcgtttttgtaggtagtcgagggggcgttggtcgaattggaggaggacgaggacgaggcgtaggaggcggaggacgacgacgaggaggaggaggtggttttcggggcggcggcggcggcggcggcggcggcgggcggcgggtttattagggcggtttggagcgcgtcggggatcgggttgtacgcgcggcggagcggggtcggcggcggttcgttttcggtggttatttgggattcgggagcgaggtcgggtcgcgagggcgggtttcgggcgggaagcggaggcgtcggagcggggtcggtttagaagttttgcgagcgttttagttcgtcgttcgggttgtagtcgtggttatttcgggttagcgtttcggcgtcgttttttttagtttttttggggtttttggcggcggcggcggcggcgggcgggaggtaacgttcggcgtattttttttcgagtcgcgggttttgttttgcgtaacggttttttaggtcgcggggtcgagcggtcggcgtcgggcgattgcgttcgcgagtgggatcgcggtttggatttcggggacgagttcgacgtttttttttaggagcgtttttcgttttgtttttcggattttttttttttttcgtttttttcggtcgtttttttcgttttttttttttttttttttttttttatttcgttttgtttttttttcgtttcgcgtcgtcgcgtttatttttttttttttcgatttggcggtcgttttttttttttatttcgtttttcgttttttagggttttttcgttttttatttttttcgcggttttttttttttttttttatttattttttttttaattgagggattatagatttatttcggttttgttagggggacgatttttatttttcgtaaaattcgattatttttgattttatgaaatattttttttgtttgtttttcgtagtaagtttcgcgttttattttaggatttagtttcgttttttcgcgttttttttttttttttggttcgtcgggtcgagtggtgttgttgcgggtgcggttgttcggagtttttttggtcgttttttttagggtcgatattgattttatttgttaatttcgtttagattttgtcgtttttagttatacgtcggggtgttagacgtttaaaggtaacgtgttaattttttttttttttggtagggtttgtaggtttttcgataattgttagggcgattgggggtcgtcgtagggttgcgggtcgttggcgatcgtggacgttttcggaattttgagtagagggatttatattgagaaatttaggttaagttttaaagattttggaaatttggattttatgggatttagggttgtatttgtttttattttttttttttattttcgtattttagttagtgttttgtaagaaaaaagtgtaaaagaaaaaggaaggaaggaagaaaagaaagaaagagaaagaaaaagaaagattttgagataagcgagatggttatatttatagttagttttgaaggggtgtgtagttgttattaggtttatatttttcgttttaatattgtttatttaaaattgtgttaggttttagttaatttttgttcgagaatatttttttttagttgtggttaatttttttttaagtaagagttaggttttgagagagatgtgttttcgggagtaattatttttaatgagattcgatagttagttattggattatacgtgtagggaaatgtagttcgattagggataggagttgggagagggaggaggagagtaggaggtcggagttggcggggttttttaagggttgaagggggaggtttagaaagaaggtgttgtagattagcggattaaataggaggtagagttgggtatttcgttgcgtttaggttgaaaggatcgaggtgtacgggtgtgtttgttggggagtttggggagttgtaggaggtaggagaaagggaggttgtgtagtaattaggaggaagatattaggtaaagagtttttatagtcgtatagtttaggtaggttttttggggcggtaggagttttgtgtgtttttggagtgtcgggggattgtttttggttgagtgtgttggtggggttgtagatgtagagagggcgggtggggaggggaggggtatgtgggaggggggtgggtcggggttggttttagatagtgatttgaggttgagtggaagtaggttttttttattaaattttgtttggatattatatatagagatcgagtgttagtttattgttttgagtcggttttttttttttaagttttatagtaattagataaagaaaatttaaattagttgaataggcgtcgatagttttttttagagtatttttggtatttatatgggaatgtgttcgaaaatggtttgattgtagtcgagagttagttaagaaaatatcgttaaatcgaatttagtttattatttatttttaatagaaaaaagaaataagtcgttttttttcgggtgggatgttttgattgggttggggtagggtttcgtagttgtttttattttttaagaatttttgattgattgttgagcgtttttggggggtgcgtttttatatattttatggtattttttttttttgtttttatttgttattttgtgtggaataatttaaaaatatataattaaatatgaaagtaaatataatgtgtttattaaattaatgttttaagtgtttaaaatataattatttttataaaatagaagttggagtggggaggatagataggattttaaaggagttttattgatatagagtttagtgtgtgtgtgtgtgtgtgtgtgtgtgtgtgtgtgttttaaatggaaagagtttaggggagaagtttgtgggggaaaaggataattattttatttgtaggtgggggcggtgggtaacgggttttggaaatatttagtatttattgttatttagttatggattttttttgattttttgtgtttgaaaattatatgtatttggattttagggaatatagatttaatttgttaagagtaggttttaaaaggttttaggattcggagattgaagaataaaaggcgttaattttaaaatttaggtaggattagtgataattttttatattagtagtttttagttttggggttatggggttattttttgagaatacgatggaagttatggagttagtttttagaaaaatatttttaatttgtttgagattttaggaagtttataggtatttattaaaataaataaggaaataagtaaaaaattttagatttttttagtttttattaatttagttggttaaattatgagggatttttttaaaaggtttttttttttatttaagtaatagtagtatttattttatttaaattttaaatttgtaagaaattttatttagagtgtggtgagtgttatgagggtcggttaggtcgtgggaaggtagtggatattggagagtagttagggttaggaggcggttagttgattggaagttttttttttttgtaggggtttgtatattgtttttgtagattttgaattttagaaagataagtagtttgggggtttttttaagttatattagtaggaaggtttttttttaaaatttttttttggatattttatttttgtttttggaaattatttttatggtatagattattattacgtttatagtgattaaattttgtatttgtttgttatagatttcgtaggtattattttgttatttattaagtggtttaggtattattattttttttttgaggtgaggaaattaaggtttagagattgggtgattggttataagttacgttggggtaagtgataaagttggttagtagtttgggtttggaattttaaagttagtgttttttttattgtattatagtaaagtttttttgagttttgttttaattattgatatatataaattttttgagtaagaatgtatgtgatagtaaattatgttaatttttgtatttttgggaggaatattttaatttttggttagtagatagggtttaaaaggaaagttgtgtttgtttttgaaatagagttttgtttaggatggtttttttatttttttattggggtttttttttatgggggtgagttttttatttatttttattttttataaataatatgaattttgatatttttttttttacgggaagggaaggtatggtttatataaatgagtttagattagtttaggtagtttttggttaattaaaattatgtagttttcgtcgcgatgggttttttttttatttcgttttggttgattgtttcgtttgggttgcgggttttttttttttttaattttttaggttttatttttgttttagcgtaagggaatgtaaattttaataagtttgggttttttcgattttgttttgtaatcggcgttttattttaggaaatttttttattattgcggtttaaattttgtgtttttagtatgttttttttgtttcgtgggttttatatgaaatggtttagattaaattagttatcgataggagagacgtattcgtatcgtattgtttgcggttatttaagacgtatttttttttgtttttcgtttgggttcgggaggagggaagtttttttttaatttaaaatgagattgatttttgttttcgttttgtatttaggcgtaaagttaagtcgtgtagaggattttcgaatttttgcgaggtttttttaaatgtggacggcgagaatttagtgttggggtttgggggtgttagcgtgattgaggaaatgttggaagagtattagtttgtacgttgtagaggtttttttagaaattttatataatagtagaagatgcggacgggaatagtaataggaggacgcgcggaggcgggggttggagagagtaaggtggtcgggagtgggaattttatattttttttggagtttgtttttttttttaggtttagaaatttttagattttcgggtttgaatattagttatttagtttttagtgtttatttggatagagtttttcgttttttaaaggtttgtgtttcggttagggttttttttatagttatttttatgagagattttttagtagttttagattttttggtttgggcggtgggtacgattcgatgatttattggttaggtttgagggtgtttgaagggggaaaaaggggtttaatttacgagatttttaagcgaagatcggttttattttattttcgtattttttaaattgtcgggcgcgggttttttcggttgcgagattaaaattttgggatgattttaggagttagtttagcggtttgtaggtttcgattttagtgcg

SEQ ID NO: 31 - DNA, 5764 bp, Homo sapiens
agcccgggcggcgggctagggcgctcgcagggcttctgggccgaccccgctccggcgcctccgcttcccgcccggggcccgccctcgcggcccggcctcgctcccgggtcccagatgaccaccgagggcgggccgccgccggccccgctccgccgcgcgtgcagcccggtccccggcgcgctccaggccgccctgatgagcccgccgcccgccgccgccgccgccgccgccgccgccccggagaccacctcctcctcctcgtcgtcgtcctccgcctcctgcgcctcgtcctcgtcctcctccaattcggccagcgccccctcggctgcctgcaagagcgcgggcggcggcggcgcgggcgccgggagcgggggcgccaagaaggcgagctcggggctgcggcggcccgagaagccgccctactcgtacatcgcgctcatcgtcatggccatccagagctcgcccagcaagcgcctgacgctcagcgagatctaccagttcctgcaggcgcgcttccccttcttccgcggcgcctaccagggctggaagaactcggtgcgccacaatctctcgctcaacgagtgcttcatcaagctgcctaagggcctcgggcggcccggcaagggccactactggaccatcgacccggccagcgagttcatgttcgaggagggctcgttccgccgccggccgcgcggcttcaggcggaagtgccaggcgctcaagcccatgtaccaccgcgtggtgagcggcttgggcttcggggcgtcgctgctgccccagggcttcgacttccaggcgcccccgtcggcgccgctcggctgccacagccagggcggctacggcggcctcgacatgatgcccgcgggctacgacgccggcgcgggcgcccccagccacgcgcaccctcaccaccaccaccaccaccacgtcccgcacatgtcgcccaacccgggttccacctacatggccagctgcccggtgcccgcgggacccgggggcgtcggtgcggccgggggcggcggcggcggcgactacgggccggacagcagcagcagcccggtaccctcgtccccggccatggcgagcgccatcgaatgccactcgccctacacgagccctgcggcgcactggagctcgcctggcgcctcgccttacctcaagcagccgcctgccctgacgcccagcagcaaccccgccgcctcggcaggcctgcactccagcatgtcctcctactcgctggagcagagctacttgcaccagaacgctcgcgaggacctctcaggtaacgcagcacgctccagcccagccagctgggcgcaccgcttctaggcctccagggctggcggccactgccactcccacaaacagggaccccgaagctaggaggtctgagggcactgggaaaagcagatgctggggaaagccggcatcttattcgtgggagcagggatcagggtcttactgtcctcccagtatccctggccagcagccgaagcttcagaattgtctggctgctgtgagcgtggtgtaaagtcccctgccttcctgggctctttggggatccctgtgcaggagactgcaggtctcccgttcagagtctcacttagcttggagagaaggcatctggcctttggggaacttggtcaggaagctgtgtctagttccttttgtccctttttttccttgcgttcattttgctgtacttctgtcccgaagtaaatgtcagaatcagatatgttctgtatgttggggtgtctgcagcgagatgtttgcagctgggcaagtgttaagaggagggggtgggagggacagagctggatcccaggatctttcactaaagggacatttgccagtggagggggtcaccaaactgttggagactcctccccttccctgcctccccccccgcccaacaatggacccacattgatgatacaggtcctgggtggcaggacctgaaggaccctgctaggactcccctgagaaatgcgcctgccctgtggatgccacttgtagtgtggctggtttacattgttctggttgcagattatgaaaaattattgacttgctgaaggcggtgaaaggtgggaggggacggtagggatggaagagggaatttgaatatttgaccaggttaatgtgaagaacagagataaacccttacattaacccctcgctcggagcacctagggctgcagattaaaatcccatgggcctgccagtcaaaggcaaggccccaagctactctctcacactggcctcccacagcaatgagacagtggcttggagggtgatgcatgctttatgtgttcctgagccggtgtgcagcgggagcacccggggagaaggaaagcccagaaatgggcaaaagatgttggttccctggacggtgaaatttcccaaataggccttttaaatgtgggtctcagaggttaaccaaacaaagacagtctcggcaggaccacaccggagaggattttagcctgacttaacccactgagaacagagtcttgttcaattttatgggaatttcaacaagtaaccaatacaggcggccttcccctcttatttttgtattcccttggaccggctgtcaatcacacacacacacacacacacacacacacacacacacacacacccctcggtgcactggccccttcccttccccgcctgcctgctcctctcccagcctgccagctgccctccctgctccccttcttctcctctcccggcagatccactcaacttgaacccggactctgaggcttagcagccttggagaaaccgtactctaggaagaaaaaaaagcacacaggaaagagactcctgacccttcctcaaggctgctctcgccccacctcataacactgggcgcaggcacaagctcccaaaacttcggaatctggatacattactgtcttggagggggtgaaaactgcccagcaaagcaagccggcctctgtgcccctacccagcggcctcccgcggccggccttccctgggagcctcgcagaacccccgaccgagtctgggaacgcccgggggagacaatagctcgggcctgacgcccgacagggaccctctgcccttccttcctcgctgtcttgctcccgtccctataggatacccacccggccctgttgccatctccctggagcgccagcggtggaggcttcggaggagccggccggatgcaccgggaccccgcggggcctagttgggagcgcgccgcccactgaggcctgggggcccggcgaggcgcgggggtggccaaggcagtctccccggcacacagatcagcacatgtctacgcgcacacacccagcacgaccctccctcccccagcacaccccaagggccgcgccctccgctcctgggcctggtggccatggtccatgtgcccctgccggcgcaggggctgccctggagttctccattaagccctgcgagcacttcaggaaggagctcgggcttctgtcatcccgctcagcacatcaaagcgccgacggccgccttcgtgggcaggtgtgagcgctcgccctctctcctcccgagcctgctattttgtggtccaggacttgccatcagaacttgctttaacgcgacgagggaactcacctgtgtgcagagcgccgcgcacacatcggggctcgcgggacagggcagctgcgttagcgcagcgccgggtgtgttcgggtaggtgttgcgggcaaggaagtaggcagcggcccctgagcagccgcctcgctccggcattgcggggacacggcggggctgaggccacgagagcagggcccgagcccggcgggccgtggttacggttttcttgcactgaaaaactgaatccggcccgaagcgacgtgcactttatggtccccacaccactcggttaactaagaaaagacccgggcgaatggacctaacgcagcccggtgccgagagggcccggtccagcagcctctggggcccagtgcgcagggcactgcgggccgattgcgccccggggccaggaggcgccgagaaagcaaaagcaaaagccggcggcgggtggaggtcaagcggcccggtgcaggccggggaccggggagccgccccgggagagcagggtccaggccttctctgtccccctccagcctggggctacctcagggactcctcgcgctgccagatgcttcggaccaaagggcatttctctgcgccctgaagtcccggcttctctagaggaagtctaagacgttcgggacccacgaagatgcctgcggaggggcaggagaagaggcgtgcttttctgccccatcccttcatcttgcgattgggttgttttctatcgtcccctttggcacagggagtcctctgcgctcgctgctgtgaccggcccagttagttgggaaacaaggctcagaaagaaggccgcagtggtgtttctggggtagggtgcttggccctccctgaagccagggctcagggcagcacaggccaggagctctgccgggagagacccggaaccagagtctgggtctagttgtccggtacctgtgctcattctgagattaaagtgcacgccccagcctcagagaataaaattggaattccaggacataagaatccccctcgagggggaacttgctctgtgtttgtgcgagcatcaaaacaaaacataatgattccaaagcaattctatgacgtgcagttggtgtgtttgagctacttctaaagctgggctttctctaccagctgtctagcaatttactaaaaggcacagcagcaccttttgtactctgaggcaaaataagacaccctgccatccactggatgactttgtttctgaagaggtttttttttctttcttctttcagtgggactgccccgttaccagcatcactctactccagtgtgtgacagaaaagatttcgtcctcaacttcaatgggatttcttctttccatccctcagctagcgggtcgtattatcaccatcaccaccagagcgtctgtcaggatattaagccctgcgtcatgtgaacggaaagaggccaagcgatggccgctctctcctctcccctcctcagagggggcagatagaaactgggacggattcaagtcacatgcacgcggatagcagtaagccacacacctgccacttagccagaatgcccaggatcgcgttggtcactgttatttgcctactgctggaagaaggacaaccgctggcaaggtagcgttccccaatctgaatacctgcaggctcccacatgagggagagggcagactcaggtgggaagatgtgccatgcgtaaggcatcaacgtgtatctgtgggatcttcgttgccttcagtaatcagggtgtgaaaaaagcagacaagttgtgtgtgtgtgtgtgtgtctaagaaaacttgtgtgcttttcaaaaaggcagtgctaagcacaagatttcaagaaagcctcttcttgttgcctagctgagtgggagagtcattttccccagacactacatttggatacaggtgccaaagaacattattaaggaattatttagaaacaatgtgtctagtttaagaaagtggttttcagtattgtgacaatacaacgtttttacaaggttgttttctaccaccatattttaaagatatttttatgaccgtgtatactcacactttgcttgtattttaaaaggaggatatatttgcacttatgtatacttttacagtttgccaaaatattttgttgtaaaattttttttcaataaaatgtatataaca

SEQ ID NO: 32 - DNA, 5764 bp, Artificial Sequence
  C to T (bis1)
agttcgggcggcgggttagggcgttcgtagggtttttgggtcgatttcgtttcggcgttttcgtttttcgttcggggttcgttttcgcggttcggtttcgttttcgggttttagatgattatcgagggcgggtcgtcgtcggtttcgtttcgtcgcgcgtgtagttcggttttcggcgcgttttaggtcgttttgatgagttcgtcgttcgtcgtcgtcgtcgtcgtcgtcgtcgtttcggagattattttttttttttcgtcgtcgtttttcgttttttgcgtttcgttttcgtttttttttaattcggttagcgttttttcggttgtttgtaagagcgcgggcggcggcggcgcgggcgtcgggagcgggggcgttaagaaggcgagttcggggttgcggcggttcgagaagtcgttttattcgtatatcgcgtttatcgttatggttatttagagttcgtttagtaagcgtttgacgtttagcgagatttattagtttttgtaggcgcgtttttttttttttcgcggcgtttattagggttggaagaattcggtgcgttataatttttcgtttaacgagtgttttattaagttgtttaagggtttcgggcggttcggtaagggttattattggattatcgattcggttagcgagtttatgttcgaggagggttcgtttcgtcgtcggtcgcgcggttttaggcggaagtgttaggcgtttaagtttatgtattatcgcgtggtgagcggtttgggtttcggggcgtcgttgttgttttagggtttcgatttttaggcgttttcgtcggcgtcgttcggttgttatagttagggcggttacggcggtttcgatatgatgttcgcgggttacgacgtcggcgcgggcgtttttagttacgcgtatttttattattattattattattacgtttcgtatatgtcgtttaattcgggttttatttatatggttagttgttcggtgttcgcgggattcgggggcgtcggtgcggtcgggggcggcggcggcggcgattacgggtcggatagtagtagtagttcggtattttcgttttcggttatggcgagcgttatcgaatgttattcgttttatacgagttttgcggcgtattggagttcgtttggcgtttcgttttattttaagtagtcgtttgttttgacgtttagtagtaatttcgtcgtttcggtaggtttgtattttagtatgtttttttattcgttggagtagagttatttgtattagaacgttcgcgaggattttttaggtaacgtagtacgttttagtttagttagttgggcgtatcgtttttaggtttttagggttggcggttattgttatttttataaatagggatttcgaagttaggaggtttgagggtattgggaaaagtagatgttggggaaagtcggtattttattcgtgggagtagggattagggttttattgtttttttagtatttttggttagtagtcgaagttttagaattgtttggttgttgtgagcgtggtgtaaagttttttgtttttttgggttttttggggatttttgtgtaggagattgtaggtttttcgtttagagttttatttagtttggagagaaggtatttggtttttggggaatttggttaggaagttgtgtttagttttttttgtttttttttttttttgcgtttattttgttgtatttttgtttcgaagtaaatgttagaattagatatgttttgtatgttggggtgtttgtagcgagatgtttgtagttgggtaagtgttaagaggagggggtgggagggatagagttggattttaggattttttattaaagggatatttgttagtggagggggttattaaattgttggagatttttttttttttttgttttttttttcgtttaataatggatttatattgatgatataggttttgggtggtaggatttgaaggattttgttaggatttttttgagaaatgcgtttgttttgtggatgttatttgtagtgtggttggtttatattgttttggttgtagattatgaaaaattattgatttgttgaaggcggtgaaaggtgggaggggacggtagggatggaagagggaatttgaatatttgattaggttaatgtgaagaatagagataaatttttatattaatttttcgttcggagtatttagggttgtagattaaaattttatgggtttgttagttaaaggtaaggttttaagttatttttttatattggttttttatagtaatgagatagtggtttggagggtgatgtatgttttatgtgtttttgagtcggtgtgtagcgggagtattcggggagaaggaaagtttagaaatgggtaaaagatgttggttttttggacggtgaaattttttaaataggttttttaaatgtgggttttagaggttaattaaataaagatagtttcggtaggattatatcggagaggattttagtttgatttaatttattgagaatagagttttgtttaattttatgggaattttaataagtaattaatataggcggttttttttttttatttttgtatttttttggatcggttgttaattatatatatatatatatatatatatatatatatatatatatatttttcggtgtattggttttttttttttttcgtttgtttgttttttttttagtttgttagttgttttttttgttttttttttttttttttttcggtagatttatttaatttgaattcggattttgaggtttagtagttttggagaaatcgtattttaggaagaaaaaaaagtatataggaaagagatttttgatttttttttaaggttgttttcgttttattttataatattgggcgtaggtataagtttttaaaatttcggaatttggatatattattgttttggagggggtgaaaattgtttagtaaagtaagtcggtttttgtgtttttatttagcggtttttcgcggtcggttttttttgggagtttcgtagaattttcgatcgagtttgggaacgttcgggggagataatagttcgggtttgacgttcgatagggattttttgttttttttttttcgttgttttgttttcgtttttataggatatttattcggttttgttgttatttttttggagcgttagcggtggaggtttcggaggagtcggtcggatgtatcgggatttcgcggggtttagttgggagcgcgtcgtttattgaggtttgggggttcggcgaggcgcgggggtggttaaggtagttttttcggtatatagattagtatatgtttacgcgtatatatttagtacgatttttttttttttagtatattttaagggtcgcgtttttcgtttttgggtttggtggttatggtttatgtgtttttgtcggcgtaggggttgttttggagttttttattaagttttgcgagtattttaggaaggagttcgggtttttgttatttcgtttagtatattaaagcgtcgacggtcgttttcgtgggtaggtgtgagcgttcgtttttttttttttcgagtttgttattttgtggtttaggatttgttattagaatttgttttaacgcgacgagggaatttatttgtgtgtagagcgtcgcgtatatatcggggttcgcgggatagggtagttgcgttagcgtagcgtcgggtgtgttcgggtaggtgttgcgggtaaggaagtaggtagcggtttttgagtagtcgtttcgtttcggtattgcggggatacggcggggttgaggttacgagagtagggttcgagttcggcgggtcgtggttacggtttttttgtattgaaaaattgaattcggttcgaagcgacgtgtattttatggtttttatattattcggttaattaagaaaagattcgggcgaatggatttaacgtagttcggtgtcgagagggttcggtttagtagtttttggggtttagtgcgtagggtattgcgggtcgattgcgtttcggggttaggaggcgtcgagaaagtaaaagtaaaagtcggcggcgggtggaggttaagcggttcggtgtaggtcggggatcggggagtcgtttcgggagagtagggtttaggttttttttgtttttttttagtttggggttattttagggatttttcgcgttgttagatgtttcggattaaagggtatttttttgcgttttgaagtttcggtttttttagaggaagtttaagacgttcgggatttacgaagatgtttgcggaggggtaggagaagaggcgtgtttttttgttttatttttttattttgcgattgggttgttttttatcgttttttttggtatagggagttttttgcgttcgttgttgtgatcggtttagttagttgggaaataaggtttagaaagaaggtcgtagtggtgtttttggggtagggtgtttggttttttttgaagttagggtttagggtagtataggttaggagttttgtcgggagagattcggaattagagtttgggtttagttgttcggtatttgtgtttattttgagattaaagtgtacgttttagttttagagaataaaattggaattttaggatataagaatttttttcgagggggaatttgttttgtgtttgtgcgagtattaaaataaaatataatgattttaaagtaattttatgacgtgtagttggtgtgtttgagttatttttaaagttgggttttttttattagttgtttagtaatttattaaaaggtatagtagtattttttgtattttgaggtaaaataagatattttgttatttattggatgattttgtttttgaagaggtttttttttttttttttttttagtgggattgtttcgttattagtattattttattttagtgtgtgatagaaaagatttcgtttttaattttaatgggattttttttttttattttttagttagcgggtcgtattattattattattattagagcgtttgttaggatattaagttttgcgttatgtgaacggaaagaggttaagcgatggtcgttttttttttttttttttttagagggggtagatagaaattgggacggatttaagttatatgtacgcggatagtagtaagttatatatttgttatttagttagaatgtttaggatcgcgttggttattgttatttgtttattgttggaagaaggataatcgttggtaaggtagcgttttttaatttgaatatttgtaggtttttatatgagggagagggtagatttaggtgggaagatgtgttatgcgtaaggtattaacgtgtatttgtgggattttcgttgtttttagtaattagggtgtgaaaaaagtagataagttgtgtgtgtgtgtgtgtgtttaagaaaatttgtgtgttttttaaaaaggtagtgttaagtataagattttaagaaagtttttttttgttgtttagttgagtgggagagttattttttttagatattatatttggatataggtgttaaagaatattattaaggaattatttagaaataatgtgtttagtttaagaaagtggtttttagtattgtgataatataacgtttttataaggttgttttttattattatattttaaagatatttttatgatcgtgtatatttatattttgtttgtattttaaaaggaggatatatttgtatttatgtatatttttatagtttgttaaaatattttgttgtaaaatttttttttaataaaatgtatataata

SEQ ID NO: 33 - DNA, 5764 bp, Artificial Sequence
  rc C to T (bis1)
tattatatacattttattaaaaaaaaattttacaacaaaatattttaacaaactataaaaatatacataaatacaaatatatcctccttttaaaatacaaacaaaatataaatatacacgatcataaaaatatctttaaaatataataataaaaaacaaccttataaaaacgttatattatcacaatactaaaaaccactttcttaaactaaacacattatttctaaataattccttaataatattctttaacacctatatccaaatataatatctaaaaaaaataactctcccactcaactaaacaacaaaaaaaaactttcttaaaatcttatacttaacactacctttttaaaaaacacacaaattttcttaaacacacacacacacacacaacttatctacttttttcacaccctaattactaaaaacaacgaaaatcccacaaatacacgttaataccttacgcataacacatcttcccacctaaatctaccctctccctcatataaaaacctacaaatattcaaattaaaaaacgctaccttaccaacgattatccttcttccaacaataaacaaataacaataaccaacgcgatcctaaacattctaactaaataacaaatatataacttactactatccgcgtacatataacttaaatccgtcccaatttctatctaccccctctaaaaaaaaaaaaaaaaaaaacgaccatcgcttaacctctttccgttcacataacgcaaaacttaatatcctaacaaacgctctaataataataataataatacgacccgctaactaaaaaataaaaaaaaaaaatcccattaaaattaaaaacgaaatcttttctatcacacactaaaataaaataatactaataacgaaacaatcccactaaaaaaaaaaaaaaaaaaaaacctcttcaaaaacaaaatcatccaataaataacaaaatatcttattttacctcaaaatacaaaaaatactactataccttttaataaattactaaacaactaataaaaaaaacccaactttaaaaataactcaaacacaccaactacacgtcataaaattactttaaaatcattatattttattttaatactcgcacaaacacaaaacaaattccccctcgaaaaaaattcttatatcctaaaattccaattttattctctaaaactaaaacgtacactttaatctcaaaataaacacaaataccgaacaactaaacccaaactctaattccgaatctctcccgacaaaactcctaacctatactaccctaaaccctaacttcaaaaaaaaccaaacaccctaccccaaaaacaccactacgaccttctttctaaaccttatttcccaactaactaaaccgatcacaacaacgaacgcaaaaaactccctataccaaaaaaaacgataaaaaacaacccaatcgcaaaataaaaaaataaaacaaaaaaacacgcctcttctcctacccctccgcaaacatcttcgtaaatcccgaacgtcttaaacttcctctaaaaaaaccgaaacttcaaaacgcaaaaaaataccctttaatccgaaacatctaacaacgcgaaaaatccctaaaataaccccaaactaaaaaaaaacaaaaaaaacctaaaccctactctcccgaaacgactccccgatccccgacctacaccgaaccgcttaacctccacccgccgccgacttttacttttactttctcgacgcctcctaaccccgaaacgcaatcgacccgcaataccctacgcactaaaccccaaaaactactaaaccgaaccctctcgacaccgaactacgttaaatccattcgcccgaatcttttcttaattaaccgaataatataaaaaccataaaatacacgtcgcttcgaaccgaattcaatttttcaatacaaaaaaaccgtaaccacgacccgccgaactcgaaccctactctcgtaacctcaaccccgccgtatccccgcaataccgaaacgaaacgactactcaaaaaccgctacctacttccttacccgcaacacctacccgaacacacccgacgctacgctaacgcaactaccctatcccgcgaaccccgatatatacgcgacgctctacacacaaataaattccctcgtcgcgttaaaacaaattctaataacaaatcctaaaccacaaaataacaaactcgaaaaaaaaaaaaacgaacgctcacacctacccacgaaaacgaccgtcgacgctttaatatactaaacgaaataacaaaaacccgaactccttcctaaaatactcgcaaaacttaataaaaaactccaaaacaacccctacgccgacaaaaacacataaaccataaccaccaaacccaaaaacgaaaaacgcgacccttaaaatatactaaaaaaaaaaaaatcgtactaaatatatacgcgtaaacatatactaatctatataccgaaaaaactaccttaaccacccccgcgcctcgccgaacccccaaacctcaataaacgacgcgctcccaactaaaccccgcgaaatcccgatacatccgaccgactcctccgaaacctccaccgctaacgctccaaaaaaataacaacaaaaccgaataaatatcctataaaaacgaaaacaaaacaacgaaaaaaaaaaaacaaaaaatccctatcgaacgtcaaacccgaactattatctcccccgaacgttcccaaactcgatcgaaaattctacgaaactcccaaaaaaaaccgaccgcgaaaaaccgctaaataaaaacacaaaaaccgacttactttactaaacaattttcaccccctccaaaacaataatatatccaaattccgaaattttaaaaacttatacctacgcccaatattataaaataaaacgaaaacaaccttaaaaaaaaatcaaaaatctctttcctatatacttttttttcttcctaaaatacgatttctccaaaactactaaacctcaaaatccgaattcaaattaaataaatctaccgaaaaaaaaaaaaaaaaaaaacaaaaaaaacaactaacaaactaaaaaaaaaacaaacaaacgaaaaaaaaaaaaaaccaatacaccgaaaaatatatatatatatatatatatatatatatatatatatatataattaacaaccgatccaaaaaaatacaaaaataaaaaaaaaaaaccgcctatattaattacttattaaaattcccataaaattaaacaaaactctattctcaataaattaaatcaaactaaaatcctctccgatataatcctaccgaaactatctttatttaattaacctctaaaacccacatttaaaaaacctatttaaaaaatttcaccgtccaaaaaaccaacatcttttacccatttctaaactttccttctccccgaatactcccgctacacaccgactcaaaaacacataaaacatacatcaccctccaaaccactatctcattactataaaaaaccaatataaaaaaataacttaaaaccttacctttaactaacaaacccataaaattttaatctacaaccctaaatactccgaacgaaaaattaatataaaaatttatctctattcttcacattaacctaatcaaatattcaaattccctcttccatccctaccgtcccctcccacctttcaccgccttcaacaaatcaataatttttcataatctacaaccaaaacaatataaaccaaccacactacaaataacatccacaaaacaaacgcatttctcaaaaaaatcctaacaaaatccttcaaatcctaccacccaaaacctatatcatcaatataaatccattattaaacgaaaaaaaaaacaaaaaaaaaaaaaaatctccaacaatttaataaccccctccactaacaaatatccctttaataaaaaatcctaaaatccaactctatccctcccaccccctcctcttaacacttacccaactacaaacatctcgctacaaacaccccaacatacaaaacatatctaattctaacatttacttcgaaacaaaaatacaacaaaataaacgcaaaaaaaaaaaaaaacaaaaaaaactaaacacaacttcctaaccaaattccccaaaaaccaaataccttctctccaaactaaataaaactctaaacgaaaaacctacaatctcctacacaaaaatccccaaaaaacccaaaaaaacaaaaaactttacaccacgctcacaacaaccaaacaattctaaaacttcgactactaaccaaaaatactaaaaaaacaataaaaccctaatccctactcccacgaataaaataccgactttccccaacatctacttttcccaataccctcaaacctcctaacttcgaaatccctatttataaaaataacaataaccgccaaccctaaaaacctaaaaacgatacgcccaactaactaaactaaaacgtactacgttacctaaaaaatcctcgcgaacgttctaatacaaataactctactccaacgaataaaaaaacatactaaaatacaaacctaccgaaacgacgaaattactactaaacgtcaaaacaaacgactacttaaaataaaacgaaacgccaaacgaactccaatacgccgcaaaactcgtataaaacgaataacattcgataacgctcgccataaccgaaaacgaaaataccgaactactactactatccgacccgtaatcgccgccgccgccgcccccgaccgcaccgacgcccccgaatcccgcgaacaccgaacaactaaccatataaataaaacccgaattaaacgacatatacgaaacgtaataataataataataataaaaatacgcgtaactaaaaacgcccgcgccgacgtcgtaacccgcgaacatcatatcgaaaccgccgtaaccgccctaactataacaaccgaacgacgccgacgaaaacgcctaaaaatcgaaaccctaaaacaacaacgacgccccgaaacccaaaccgctcaccacgcgataatacataaacttaaacgcctaacacttccgcctaaaaccgcgcgaccgacgacgaaacgaaccctcctcgaacataaactcgctaaccgaatcgataatccaataataacccttaccgaaccgcccgaaacccttaaacaacttaataaaacactcgttaaacgaaaaattataacgcaccgaattcttccaaccctaataaacgccgcgaaaaaaaaaaaaacgcgcctacaaaaactaataaatctcgctaaacgtcaaacgcttactaaacgaactctaaataaccataacgataaacgcgatatacgaataaaacgacttctcgaaccgccgcaaccccgaactcgccttcttaacgcccccgctcccgacgcccgcgccgccgccgcccgcgctcttacaaacaaccgaaaaaacgctaaccgaattaaaaaaaaacgaaaacgaaacgcaaaaaacgaaaaacgacgacgaaaaaaaaaaaataatctccgaaacgacgacgacgacgacgacgacgacgaacgacgaactcatcaaaacgacctaaaacgcgccgaaaaccgaactacacgcgcgacgaaacgaaaccgacgacgacccgccctcgataatcatctaaaacccgaaaacgaaaccgaaccgcgaaaacgaaccccgaacgaaaaacgaaaacgccgaaacgaaatcgacccaaaaaccctacgaacgccctaacccgccgcccgaact

SEQ ID NO: 34 - DNA, 5764 bp, Artificial Sequence
  G to A (bis2 rc)
aacccgaacgacgaactaaaacgctcgcaaaacttctaaaccgaccccgctccgacgcctccgcttcccgcccgaaacccgccctcgcgacccgacctcgctcccgaatcccaaataaccaccgaaaacgaaccgccgccgaccccgctccgccgcgcgtacaacccgatccccgacgcgctccaaaccgccctaataaacccgccgcccgccgccgccgccgccgccgccgccgccccgaaaaccacctcctcctcctcgtcgtcgtcctccgcctcctacgcctcgtcctcgtcctcctccaattcgaccaacgccccctcgactacctacaaaaacgcgaacgacgacgacgcgaacgccgaaaacgaaaacgccaaaaaaacgaactcgaaactacgacgacccgaaaaaccgccctactcgtacatcgcgctcatcgtcataaccatccaaaactcgcccaacaaacgcctaacgctcaacgaaatctaccaattcctacaaacgcgcttccccttcttccgcgacgcctaccaaaactaaaaaaactcgatacgccacaatctctcgctcaacgaatacttcatcaaactacctaaaaacctcgaacgacccgacaaaaaccactactaaaccatcgacccgaccaacgaattcatattcgaaaaaaactcgttccgccgccgaccgcgcgacttcaaacgaaaataccaaacgctcaaacccatataccaccgcgtaataaacgacttaaacttcgaaacgtcgctactaccccaaaacttcgacttccaaacgcccccgtcgacgccgctcgactaccacaaccaaaacgactacgacgacctcgacataatacccgcgaactacgacgccgacgcgaacgcccccaaccacgcgcaccctcaccaccaccaccaccaccacgtcccgcacatatcgcccaacccgaattccacctacataaccaactacccgatacccgcgaaacccgaaaacgtcgatacgaccgaaaacgacgacgacgacgactacgaaccgaacaacaacaacaacccgataccctcgtccccgaccataacgaacgccatcgaataccactcgccctacacgaaccctacgacgcactaaaactcgcctaacgcctcgccttacctcaaacaaccgcctaccctaacgcccaacaacaaccccgccgcctcgacaaacctacactccaacatatcctcctactcgctaaaacaaaactacttacaccaaaacgctcgcgaaaacctctcaaataacgcaacacgctccaacccaaccaactaaacgcaccgcttctaaacctccaaaactaacgaccactaccactcccacaaacaaaaaccccgaaactaaaaaatctaaaaacactaaaaaaaacaaatactaaaaaaaaccgacatcttattcgtaaaaacaaaaatcaaaatcttactatcctcccaatatccctaaccaacaaccgaaacttcaaaattatctaactactataaacgtaatataaaatcccctaccttcctaaactctttaaaaatccctatacaaaaaactacaaatctcccgttcaaaatctcacttaacttaaaaaaaaaacatctaacctttaaaaaacttaatcaaaaaactatatctaattccttttatccctttttttccttacgttcattttactatacttctatcccgaaataaatatcaaaatcaaatatattctatatattaaaatatctacaacgaaatatttacaactaaacaaatattaaaaaaaaaaaataaaaaaaacaaaactaaatcccaaaatctttcactaaaaaaacatttaccaataaaaaaaatcaccaaactattaaaaactcctccccttccctacctccccccccgcccaacaataaacccacattaataatacaaatcctaaataacaaaacctaaaaaaccctactaaaactcccctaaaaaatacgcctaccctataaataccacttataatataactaatttacattattctaattacaaattataaaaaattattaacttactaaaaacgataaaaaataaaaaaaaacgataaaaataaaaaaaaaaatttaaatatttaaccaaattaatataaaaaacaaaaataaacccttacattaacccctcgctcgaaacacctaaaactacaaattaaaatcccataaacctaccaatcaaaaacaaaaccccaaactactctctcacactaacctcccacaacaataaaacaataacttaaaaaataatacatactttatatattcctaaaccgatatacaacgaaaacacccgaaaaaaaaaaaaacccaaaaataaacaaaaaatattaattccctaaacgataaaatttcccaaataaaccttttaaatataaatctcaaaaattaaccaaacaaaaacaatctcgacaaaaccacaccgaaaaaaattttaacctaacttaacccactaaaaacaaaatcttattcaattttataaaaatttcaacaaataaccaatacaaacgaccttcccctcttatttttatattcccttaaaccgactatcaatcacacacacacacacacacacacacacacacacacacacacacccctcgatacactaaccccttcccttccccgcctacctactcctctcccaacctaccaactaccctccctactccccttcttctcctctcccgacaaatccactcaacttaaacccgaactctaaaacttaacaaccttaaaaaaaccgtactctaaaaaaaaaaaaaaacacacaaaaaaaaaactcctaacccttcctcaaaactactctcgccccacctcataacactaaacgcaaacacaaactcccaaaacttcgaaatctaaatacattactatcttaaaaaaaataaaaactacccaacaaaacaaaccgacctctatacccctacccaacgacctcccgcgaccgaccttccctaaaaacctcgcaaaacccccgaccgaatctaaaaacgcccgaaaaaaacaataactcgaacctaacgcccgacaaaaaccctctacccttccttcctcgctatcttactcccgtccctataaaatacccacccgaccctattaccatctccctaaaacgccaacgataaaaacttcgaaaaaaccgaccgaatacaccgaaaccccgcgaaacctaattaaaaacgcgccgcccactaaaacctaaaaacccgacgaaacgcgaaaataaccaaaacaatctccccgacacacaaatcaacacatatctacgcgcacacacccaacacgaccctccctcccccaacacaccccaaaaaccgcgccctccgctcctaaacctaataaccataatccatatacccctaccgacgcaaaaactaccctaaaattctccattaaaccctacgaacacttcaaaaaaaaactcgaacttctatcatcccgctcaacacatcaaaacgccgacgaccgccttcgtaaacaaatataaacgctcgccctctctcctcccgaacctactattttataatccaaaacttaccatcaaaacttactttaacgcgacgaaaaaactcacctatatacaaaacgccgcgcacacatcgaaactcgcgaaacaaaacaactacgttaacgcaacgccgaatatattcgaataaatattacgaacaaaaaaataaacaacgacccctaaacaaccgcctcgctccgacattacgaaaacacgacgaaactaaaaccacgaaaacaaaacccgaacccgacgaaccgtaattacgattttcttacactaaaaaactaaatccgacccgaaacgacgtacactttataatccccacaccactcgattaactaaaaaaaaacccgaacgaataaacctaacgcaacccgataccgaaaaaacccgatccaacaacctctaaaacccaatacgcaaaacactacgaaccgattacgccccgaaaccaaaaaacgccgaaaaaacaaaaacaaaaaccgacgacgaataaaaatcaaacgacccgatacaaaccgaaaaccgaaaaaccgccccgaaaaaacaaaatccaaaccttctctatccccctccaacctaaaactacctcaaaaactcctcgcgctaccaaatacttcgaaccaaaaaacatttctctacgccctaaaatcccgacttctctaaaaaaaatctaaaacgttcgaaacccacgaaaatacctacgaaaaaacaaaaaaaaaaacgtacttttctaccccatcccttcatcttacgattaaattattttctatcgtcccctttaacacaaaaaatcctctacgctcgctactataaccgacccaattaattaaaaaacaaaactcaaaaaaaaaaccgcaataatatttctaaaataaaatacttaaccctccctaaaaccaaaactcaaaacaacacaaaccaaaaactctaccgaaaaaaacccgaaaccaaaatctaaatctaattatccgatacctatactcattctaaaattaaaatacacgccccaacctcaaaaaataaaattaaaattccaaaacataaaaatccccctcgaaaaaaaacttactctatatttatacgaacatcaaaacaaaacataataattccaaaacaattctataacgtacaattaatatatttaaactacttctaaaactaaactttctctaccaactatctaacaatttactaaaaaacacaacaacaccttttatactctaaaacaaaataaaacaccctaccatccactaaataactttatttctaaaaaaatttttttttctttcttctttcaataaaactaccccgttaccaacatcactctactccaatatataacaaaaaaaatttcgtcctcaacttcaataaaatttcttctttccatccctcaactaacgaatcgtattatcaccatcaccaccaaaacgtctatcaaaatattaaaccctacgtcatataaacgaaaaaaaaccaaacgataaccgctctctcctctcccctcctcaaaaaaaacaaataaaaactaaaacgaattcaaatcacatacacgcgaataacaataaaccacacacctaccacttaaccaaaatacccaaaatcgcgttaatcactattatttacctactactaaaaaaaaaacaaccgctaacaaaataacgttccccaatctaaatacctacaaactcccacataaaaaaaaaaacaaactcaaataaaaaaatataccatacgtaaaacatcaacgtatatctataaaatcttcgttaccttcaataatcaaaatataaaaaaaacaaacaaattatatatatatatatatatctaaaaaaacttatatacttttcaaaaaaacaatactaaacacaaaatttcaaaaaaacctcttcttattacctaactaaataaaaaaatcattttccccaaacactacatttaaatacaaataccaaaaaacattattaaaaaattatttaaaaacaatatatctaatttaaaaaaataattttcaatattataacaatacaacgtttttacaaaattattttctaccaccatattttaaaaatatttttataaccgtatatactcacactttacttatattttaaaaaaaaaatatatttacacttatatatacttttacaatttaccaaaatattttattataaaattttttttcaataaaatatatataaca

SEQ ID NO: 35 - DNA, 5764 bp, Artificial Sequence
  G to A (bis2 rc) rc
tgttatatatattttattgaaaaaaaattttataataaaatattttggtaaattgtaaaagtatatataagtgtaaatatattttttttttaaaatataagtaaagtgtgagtatatacggttataaaaatatttttaaaatatggtggtagaaaataattttgtaaaaacgttgtattgttataatattgaaaattatttttttaaattagatatattgtttttaaataattttttaataatgttttttggtatttgtatttaaatgtagtgtttggggaaaatgatttttttatttagttaggtaataagaagaggtttttttgaaattttgtgtttagtattgtttttttgaaaagtatataagtttttttagatatatatatatatatataatttgtttgttttttttatattttgattattgaaggtaacgaagattttatagatatacgttgatgttttacgtatggtatatttttttatttgagtttgtttttttttttatgtgggagtttgtaggtatttagattggggaacgttattttgttagcggttgttttttttttagtagtaggtaaataatagtgattaacgcgattttgggtattttggttaagtggtaggtgtgtggtttattgttattcgcgtgtatgtgatttgaattcgttttagtttttatttgttttttttgaggaggggagaggagagagcggttatcgtttggttttttttcgtttatatgacgtagggtttaatattttgatagacgttttggtggtgatggtgataatacgattcgttagttgagggatggaaagaagaaattttattgaagttgaggacgaaattttttttgttatatattggagtagagtgatgttggtaacggggtagttttattgaaagaagaaagaaaaaaaaatttttttagaaataaagttatttagtggatggtagggtgttttattttgttttagagtataaaaggtgttgttgtgttttttagtaaattgttagatagttggtagagaaagtttagttttagaagtagtttaaatatattaattgtacgttatagaattgttttggaattattatgttttgttttgatgttcgtataaatatagagtaagttttttttcgagggggatttttatgttttggaattttaattttattttttgaggttggggcgtgtattttaattttagaatgagtataggtatcggataattagatttagattttggtttcgggtttttttcggtagagtttttggtttgtgttgttttgagttttggttttagggagggttaagtattttattttagaaatattattgcggttttttttttgagttttgttttttaattaattgggtcggttatagtagcgagcgtagaggattttttgtgttaaaggggacgatagaaaataatttaatcgtaagatgaagggatggggtagaaaagtacgtttttttttttgttttttcgtaggtattttcgtgggtttcgaacgttttagattttttttagagaagtcgggattttagggcgtagagaaatgttttttggttcgaagtatttggtagcgcgaggagtttttgaggtagttttaggttggagggggatagagaaggtttggattttgttttttcggggcggtttttcggttttcggtttgtatcgggtcgtttgatttttattcgtcgtcggtttttgtttttgttttttcggcgttttttggtttcggggcgtaatcggttcgtagtgttttgcgtattgggttttagaggttgttggatcgggttttttcggtatcgggttgcgttaggtttattcgttcgggtttttttttagttaatcgagtggtgtggggattataaagtgtacgtcgtttcgggtcggatttagttttttagtgtaagaaaatcgtaattacggttcgtcgggttcgggttttgttttcgtggttttagtttcgtcgtgttttcgtaatgtcggagcgaggcggttgtttaggggtcgttgtttatttttttgttcgtaatatttattcgaatatattcggcgttgcgttaacgtagttgttttgtttcgcgagtttcgatgtgtgcgcggcgttttgtatataggtgagttttttcgtcgcgttaaagtaagttttgatggtaagttttggattataaaatagtaggttcgggaggagagagggcgagcgtttatatttgtttacgaaggcggtcgtcggcgttttgatgtgttgagcgggatgatagaagttcgagtttttttttgaagtgttcgtagggtttaatggagaattttagggtagtttttgcgtcggtaggggtatatggattatggttattaggtttaggagcggagggcgcggtttttggggtgtgttgggggagggagggtcgtgttgggtgtgtgcgcgtagatatgtgttgatttgtgtgtcggggagattgttttggttattttcgcgtttcgtcgggtttttaggttttagtgggcggcgcgtttttaattaggtttcgcggggtttcggtgtattcggtcggttttttcgaagtttttatcgttggcgttttagggagatggtaatagggtcgggtgggtattttatagggacgggagtaagatagcgaggaaggaagggtagagggtttttgtcgggcgttaggttcgagttattgtttttttcgggcgtttttagattcggtcgggggttttgcgaggtttttagggaaggtcggtcgcgggaggtcgttgggtaggggtatagaggtcggtttgttttgttgggtagtttttattttttttaagatagtaatgtatttagatttcgaagttttgggagtttgtgtttgcgtttagtgttatgaggtggggcgagagtagttttgaggaagggttaggagttttttttttgtgtgtttttttttttttttagagtacggtttttttaaggttgttaagttttagagttcgggtttaagttgagtggatttgtcgggagaggagaagaaggggagtagggagggtagttggtaggttgggagaggagtaggtaggcggggaagggaaggggttagtgtatcgaggggtgtgtgtgtgtgtgtgtgtgtgtgtgtgtgtgtgtgtgtgtgattgatagtcggtttaagggaatataaaaataagaggggaaggtcgtttgtattggttatttgttgaaatttttataaaattgaataagattttgtttttagtgggttaagttaggttaaaatttttttcggtgtggttttgtcgagattgtttttgtttggttaatttttgagatttatatttaaaaggtttatttgggaaattttatcgtttagggaattaatattttttgtttatttttgggtttttttttttttcgggtgttttcgttgtatatcggtttaggaatatataaagtatgtattattttttaagttattgttttattgttgtgggaggttagtgtgagagagtagtttggggttttgtttttgattggtaggtttatgggattttaatttgtagttttaggtgtttcgagcgaggggttaatgtaagggtttatttttgttttttatattaatttggttaaatatttaaatttttttttttatttttatcgtttttttttattttttatcgtttttagtaagttaataattttttataatttgtaattagaataatgtaaattagttatattataagtggtatttatagggtaggcgtattttttaggggagttttagtagggttttttaggttttgttatttaggatttgtattattaatgtgggtttattgttgggcggggggggaggtagggaaggggaggagtttttaatagtttggtgattttttttattggtaaatgtttttttagtgaaagattttgggatttagttttgttttttttattttttttttttaatatttgtttagttgtaaatatttcgttgtagatattttaatatatagaatatatttgattttgatatttatttcgggatagaagtatagtaaaatgaacgtaaggaaaaaaagggataaaaggaattagatatagttttttgattaagttttttaaaggttagatgttttttttttaagttaagtgagattttgaacgggagatttgtagttttttgtatagggatttttaaagagtttaggaaggtaggggattttatattacgtttatagtagttagataattttgaagtttcggttgttggttagggatattgggaggatagtaagattttgatttttgtttttacgaataagatgtcggttttttttagtatttgttttttttagtgtttttagattttttagtttcggggtttttgtttgtgggagtggtagtggtcgttagttttggaggtttagaagcggtgcgtttagttggttgggttggagcgtgttgcgttatttgagaggttttcgcgagcgttttggtgtaagtagttttgttttagcgagtaggaggatatgttggagtgtaggtttgtcgaggcggcggggttgttgttgggcgttagggtaggcggttgtttgaggtaaggcgaggcgttaggcgagttttagtgcgtcgtagggttcgtgtagggcgagtggtattcgatggcgttcgttatggtcggggacgagggtatcgggttgttgttgttgttcggttcgtagtcgtcgtcgtcgtcgttttcggtcgtatcgacgttttcgggtttcgcgggtatcgggtagttggttatgtaggtggaattcgggttgggcgatatgtgcgggacgtggtggtggtggtggtggtgagggtgcgcgtggttgggggcgttcgcgtcggcgtcgtagttcgcgggtattatgtcgaggtcgtcgtagtcgttttggttgtggtagtcgagcggcgtcgacgggggcgtttggaagtcgaagttttggggtagtagcgacgtttcgaagtttaagtcgtttattacgcggtggtatatgggtttgagcgtttggtattttcgtttgaagtcgcgcggtcggcggcggaacgagtttttttcgaatatgaattcgttggtcgggtcgatggtttagtagtggtttttgtcgggtcgttcgaggtttttaggtagtttgatgaagtattcgttgagcgagagattgtggcgtatcgagtttttttagttttggtaggcgtcgcggaagaaggggaagcgcgtttgtaggaattggtagatttcgttgagcgttaggcgtttgttgggcgagttttggatggttatgacgatgagcgcgatgtacgagtagggcggtttttcgggtcgtcgtagtttcgagttcgtttttttggcgttttcgttttcggcgttcgcgtcgtcgtcgttcgcgtttttgtaggtagtcgagggggcgttggtcgaattggaggaggacgaggacgaggcgtaggaggcggaggacgacgacgaggaggaggaggtggttttcggggcggcggcggcggcggcggcggcggcgggcggcgggtttattagggcggtttggagcgcgtcggggatcgggttgtacgcgcggcggagcggggtcggcggcggttcgttttcggtggttatttgggattcgggagcgaggtcgggtcgcgagggcgggtttcgggcgggaagcggaggcgtcggagcggggtcggtttagaagttttgcgagcgttttagttcgtcgttcgggtt

SEQ ID NO: 36 - DNA, 2254 bp, Homo sapiens
cgaaaacgtccacgatcgccagcggcccgcaaccctgcggcggcccccagtcgccctaacaattgtcggggagcctgcaggccctgccagaaagagagaggattggcacgttacctttgggcgtctggcaccccggcgtgtggctgagggcggcaaagtctaaacgaagttgacagatggagtcagtatcggccctggggagggcggccagggaggctccgagcagccgcacccgcagcagcaccactcggcccggcgggccaggaggaggaagggggcgcggaggggcggggctgggtcctgggatgggacgcggggcttgctgcggggggcaaacagaaagaatatttcatgaagtcagaggtggtcgagttttgcgaggggtgggggtcgtccccctggcagaaccggagtgagtctgtgatccctcaattggaaagagggtgagtgagggaaaggggaggaggccgcgagaggaatgaagagcgaggagaccctggagagcggggagcgagataagagagggaggcggccgccaggtcgggagggggaggagtgagcgcggcggcgcggagcgaggagggggcagggcggggtggggggggagggagggagggagggagcgaggagggcggccggggagggcgagggagggaggaagtccgagagacagagcgaggagcgctcctgaagggagacgtcgggctcgtccccggggtccaggccgcggtcccactcgcgggcgcagtcgcccggcgccggccgctcggccccgcggcctgggaggccgttgcgcaaggcagggcccgcggctcggggagggatgcgccgggcgttgcctcccgcccgccgccgccgccgccgccagaagccccagaggagctgagggaggcgacgccgaagcgctggcccggagtggccacggctgcagcccgggcggcgggctagggcgctcgcagggcttctgggccgaccccgctccggcgcctccgcttcccgcccggggcccgccctcgcggcccggcctcgctcccgggtcccagatgaccaccgagggcgggccgccgccggccccgctccgccgcgcgtgcagcccggtccccggcgcgctccaggccgccctgatgagcccgccgcccgccgccgccgccgccgccgccgccgccccggagaccacctcctcctcctcgtcgtcgtcctccgcctcctgcgcctcgtcctcgtcctcctccaattcggccagcgccccctcggctgcctgcaagagcgcgggcggcggcggcgcgggcgccgggagcgggggcgccaagaaggcgagctcggggctgcggcggcccgagaagccgccctactcgtacatcgcgctcatcgtcatggccatccagagctcgcccagcaagcgcctgacgctcagcgagatctaccagttcctgcaggcgcgcttccccttcttccgcggcgcctaccagggctggaagaactcggtgcgccacaatctctcgctcaacgagtgcttcatcaagctgcctaagggcctcgggcggcccggcaagggccactactggaccatcgacccggccagcgagttcatgttcgaggagggctcgttccgccgccggccgcgcggcttcaggcggaagtgccaggcgctcaagcccatgtaccaccgcgtggtgagcggcttgggcttcggggcgtcgctgctgccccagggcttcgacttccaggcgcccccgtcggcgccgctcggctgccacagccagggcggctacggcggcctcgacatgatgcccgcgggctacgacgccggcgcgggcgcccccagccacgcgcaccctcaccaccaccaccaccaccacgtcccgcacatgtcgcccaacccgggttccacctacatggccagctgcccggtgcccgcgggacccgggggcgtcggtgcggccgggggcggcggcggcggcgactacgggccggacagcagcagcagcccggtaccctcgtccccggccatggcgagcgccatcgaatgccactcgccctacacgagccctgcggcgcactggagctcgcctggcgcctcgccttacctcaagcagccgcctgccctgacgcccagcagcaaccccgccgcctcggcaggcctgcactccagcatgtcctcctactcgctggagcagagctacttgcaccagaacgctcgcgaggacctctcaggtaacgcagcacgctccagcccagccagctgggcgcaccg

SEQ ID NO: 37 - DNA, 2254 bp, Artificial Sequence
  C to T (bis1)
cgaaaacgtttacgatcgttagcggttcgtaattttgcggcggtttttagtcgttttaataattgtcggggagtttgtaggttttgttagaaagagagaggattggtacgttatttttgggcgtttggtatttcggcgtgtggttgagggcggtaaagtttaaacgaagttgatagatggagttagtatcggttttggggagggcggttagggaggtttcgagtagtcgtattcgtagtagtattattcggttcggcgggttaggaggaggaagggggcgcggaggggcggggttgggttttgggatgggacgcggggtttgttgcggggggtaaatagaaagaatattttatgaagttagaggtggtcgagttttgcgaggggtgggggtcgtttttttggtagaatcggagtgagtttgtgattttttaattggaaagagggtgagtgagggaaaggggaggaggtcgcgagaggaatgaagagcgaggagattttggagagcggggagcgagataagagagggaggcggtcgttaggtcgggagggggaggagtgagcgcggcggcgcggagcgaggagggggtagggcggggtggggggggagggagggagggagggagcgaggagggcggtcggggagggcgagggagggaggaagttcgagagatagagcgaggagcgtttttgaagggagacgtcgggttcgttttcggggtttaggtcgcggttttattcgcgggcgtagtcgttcggcgtcggtcgttcggtttcgcggtttgggaggtcgttgcgtaaggtagggttcgcggttcggggagggatgcgtcgggcgttgtttttcgttcgtcgtcgtcgtcgtcgttagaagttttagaggagttgagggaggcgacgtcgaagcgttggttcggagtggttacggttgtagttcgggcggcgggttagggcgttcgtagggtttttgggtcgatttcgtttcggcgttttcgtttttcgttcggggttcgttttcgcggttcggtttcgttttcgggttttagatgattatcgagggcgggtcgtcgtcggtttcgtttcgtcgcgcgtgtagttcggttttcggcgcgttttaggtcgttttgatgagttcgtcgttcgtcgtcgtcgtcgtcgtcgtcgtcgtttcggagattattttttttttttcgtcgtcgtttttcgttttttgcgtttcgttttcgtttttttttaattcggttagcgttttttcggttgtttgtaagagcgcgggcggcggcggcgcgggcgtcgggagcgggggcgttaagaaggcgagttcggggttgcggcggttcgagaagtcgttttattcgtatatcgcgtttatcgttatggttatttagagttcgtttagtaagcgtttgacgtttagcgagatttattagtttttgtaggcgcgtttttttttttttcgcggcgtttattagggttggaagaattcggtgcgttataatttttcgtttaacgagtgttttattaagttgtttaagggtttcgggcggttcggtaagggttattattggattatcgattcggttagcgagtttatgttcgaggagggttcgtttcgtcgtcggtcgcgcggttttaggcggaagtgttaggcgtttaagtttatgtattatcgcgtggtgagcggtttgggtttcggggcgtcgttgttgttttagggtttcgatttttaggcgttttcgtcggcgtcgttcggttgttatagttagggcggttacggcggtttcgatatgatgttcgcgggttacgacgtcggcgcgggcgtttttagttacgcgtatttttattattattattattattacgtttcgtatatgtcgtttaattcgggttttatttatatggttagttgttcggtgttcgcgggattcgggggcgtcggtgcggtcgggggcggcggcggcggcgattacgggtcggatagtagtagtagttcggtattttcgttttcggttatggcgagcgttatcgaatgttattcgttttatacgagttttgcggcgtattggagttcgtttggcgtttcgttttattttaagtagtcgtttgttttgacgtttagtagtaatttcgtcgtttcggtaggtttgtattttagtatgtttttttattcgttggagtagagttatttgtattagaacgttcgcgaggattttttaggtaacgtagtacgttttagtttagttagttgggcgtatcg

SEQ ID NO: 38 - DNA, 2254 bp, Artificial Sequence
  rc C to T (bis1)
cgatacgcccaactaactaaactaaaacgtactacgttacctaaaaaatcctcgcgaacgttctaatacaaataactctactccaacgaataaaaaaacatactaaaatacaaacctaccgaaacgacgaaattactactaaacgtcaaaacaaacgactacttaaaataaaacgaaacgccaaacgaactccaatacgccgcaaaactcgtataaaacgaataacattcgataacgctcgccataaccgaaaacgaaaataccgaactactactactatccgacccgtaatcgccgccgccgccgcccccgaccgcaccgacgcccccgaatcccgcgaacaccgaacaactaaccatataaataaaacccgaattaaacgacatatacgaaacgtaataataataataataataaaaatacgcgtaactaaaaacgcccgcgccgacgtcgtaacccgcgaacatcatatcgaaaccgccgtaaccgccctaactataacaaccgaacgacgccgacgaaaacgcctaaaaatcgaaaccctaaaacaacaacgacgccccgaaacccaaaccgctcaccacgcgataatacataaacttaaacgcctaacacttccgcctaaaaccgcgcgaccgacgacgaaacgaaccctcctcgaacataaactcgctaaccgaatcgataatccaataataacccttaccgaaccgcccgaaacccttaaacaacttaataaaacactcgttaaacgaaaaattataacgcaccgaattcttccaaccctaataaacgccgcgaaaaaaaaaaaaacgcgcctacaaaaactaataaatctcgctaaacgtcaaacgcttactaaacgaactctaaataaccataacgataaacgcgatatacgaataaaacgacttctcgaaccgccgcaaccccgaactcgccttcttaacgcccccgctcccgacgcccgcgccgccgccgcccgcgctcttacaaacaaccgaaaaaacgctaaccgaattaaaaaaaaacgaaaacgaaacgcaaaaaacgaaaaacgacgacgaaaaaaaaaaaataatctccgaaacgacgacgacgacgacgacgacgacgaacgacgaactcatcaaaacgacctaaaacgcgccgaaaaccgaactacacgcgcgacgaaacgaaaccgacgacgacccgccctcgataatcatctaaaacccgaaaacgaaaccgaaccgcgaaaacgaaccccgaacgaaaaacgaaaacgccgaaacgaaatcgacccaaaaaccctacgaacgccctaacccgccgcccgaactacaaccgtaaccactccgaaccaacgcttcgacgtcgcctccctcaactcctctaaaacttctaacgacgacgacgacgacgaacgaaaaacaacgcccgacgcatccctccccgaaccgcgaaccctaccttacgcaacgacctcccaaaccgcgaaaccgaacgaccgacgccgaacgactacgcccgcgaataaaaccgcgacctaaaccccgaaaacgaacccgacgtctcccttcaaaaacgctcctcgctctatctctcgaacttcctccctccctcgccctccccgaccgccctcctcgctccctccctccctccctccccccccaccccgccctaccccctcctcgctccgcgccgccgcgctcactcctccccctcccgacctaacgaccgcctccctctcttatctcgctccccgctctccaaaatctcctcgctcttcattcctctcgcgacctcctcccctttccctcactcaccctctttccaattaaaaaatcacaaactcactccgattctaccaaaaaaacgacccccacccctcgcaaaactcgaccacctctaacttcataaaatattctttctatttaccccccgcaacaaaccccgcgtcccatcccaaaacccaaccccgcccctccgcgcccccttcctcctcctaacccgccgaaccgaataatactactacgaatacgactactcgaaacctccctaaccgccctccccaaaaccgatactaactccatctatcaacttcgtttaaactttaccgccctcaaccacacgccgaaataccaaacgcccaaaaataacgtaccaatcctctctctttctaacaaaacctacaaactccccgacaattattaaaacgactaaaaaccgccgcaaaattacgaaccgctaacgatcgtaaacgttttcg

SEQ ID NO: 39 - DNA, 2254 bp, Artificial Sequence
  G to A (bis2 rc)
cgaaaacgtccacgatcgccaacgacccgcaaccctacgacgacccccaatcgccctaacaattatcgaaaaacctacaaaccctaccaaaaaaaaaaaaaattaacacgttacctttaaacgtctaacaccccgacgtataactaaaaacgacaaaatctaaacgaaattaacaaataaaatcaatatcgaccctaaaaaaaacgaccaaaaaaactccgaacaaccgcacccgcaacaacaccactcgacccgacgaaccaaaaaaaaaaaaaaaacgcgaaaaaacgaaactaaatcctaaaataaaacgcgaaacttactacgaaaaacaaacaaaaaaaatatttcataaaatcaaaaataatcgaattttacgaaaaataaaaatcgtccccctaacaaaaccgaaataaatctataatccctcaattaaaaaaaaaataaataaaaaaaaaaaaaaaaaaccgcgaaaaaaataaaaaacgaaaaaaccctaaaaaacgaaaaacgaaataaaaaaaaaaaacgaccgccaaatcgaaaaaaaaaaaaataaacgcgacgacgcgaaacgaaaaaaaaacaaaacgaaataaaaaaaaaaaaaaaaaaaaaaaaaacgaaaaaaacgaccgaaaaaaacgaaaaaaaaaaaaaatccgaaaaacaaaacgaaaaacgctcctaaaaaaaaacgtcgaactcgtccccgaaatccaaaccgcgatcccactcgcgaacgcaatcgcccgacgccgaccgctcgaccccgcgacctaaaaaaccgttacgcaaaacaaaacccgcgactcgaaaaaaaatacgccgaacgttacctcccgcccgccgccgccgccgccgccaaaaaccccaaaaaaactaaaaaaaacgacgccgaaacgctaacccgaaataaccacgactacaacccgaacgacgaactaaaacgctcgcaaaacttctaaaccgaccccgctccgacgcctccgcttcccgcccgaaacccgccctcgcgacccgacctcgctcccgaatcccaaataaccaccgaaaacgaaccgccgccgaccccgctccgccgcgcgtacaacccgatccccgacgcgctccaaaccgccctaataaacccgccgcccgccgccgccgccgccgccgccgccgccccgaaaaccacctcctcctcctcgtcgtcgtcctccgcctcctacgcctcgtcctcgtcctcctccaattcgaccaacgccccctcgactacctacaaaaacgcgaacgacgacgacgcgaacgccgaaaacgaaaacgccaaaaaaacgaactcgaaactacgacgacccgaaaaaccgccctactcgtacatcgcgctcatcgtcataaccatccaaaactcgcccaacaaacgcctaacgctcaacgaaatctaccaattcctacaaacgcgcttccccttcttccgcgacgcctaccaaaactaaaaaaactcgatacgccacaatctctcgctcaacgaatacttcatcaaactacctaaaaacctcgaacgacccgacaaaaaccactactaaaccatcgacccgaccaacgaattcatattcgaaaaaaactcgttccgccgccgaccgcgcgacttcaaacgaaaataccaaacgctcaaacccatataccaccgcgtaataaacgacttaaacttcgaaacgtcgctactaccccaaaacttcgacttccaaacgcccccgtcgacgccgctcgactaccacaaccaaaacgactacgacgacctcgacataatacccgcgaactacgacgccgacgcgaacgcccccaaccacgcgcaccctcaccaccaccaccaccaccacgtcccgcacatatcgcccaacccgaattccacctacataaccaactacccgatacccgcgaaacccgaaaacgtcgatacgaccgaaaacgacgacgacgacgactacgaaccgaacaacaacaacaacccgataccctcgtccccgaccataacgaacgccatcgaataccactcgccctacacgaaccctacgacgcactaaaactcgcctaacgcctcgccttacctcaaacaaccgcctaccctaacgcccaacaacaaccccgccgcctcgacaaacctacactccaacatatcctcctactcgctaaaacaaaactacttacaccaaaacgctcgcgaaaacctctcaaataacgcaacacgctccaacccaaccaactaaacgcaccg

SEQ ID NO: 40 - DNA, 2254 bp, Artificial Sequence
  G to A (bis2 rc) rc
cggtgcgtttagttggttgggttggagcgtgttgcgttatttgagaggttttcgcgagcgttttggtgtaagtagttttgttttagcgagtaggaggatatgttggagtgtaggtttgtcgaggcggcggggttgttgttgggcgttagggtaggcggttgtttgaggtaaggcgaggcgttaggcgagttttagtgcgtcgtagggttcgtgtagggcgagtggtattcgatggcgttcgttatggtcggggacgagggtatcgggttgttgttgttgttcggttcgtagtcgtcgtcgtcgtcgttttcggtcgtatcgacgttttcgggtttcgcgggtatcgggtagttggttatgtaggtggaattcgggttgggcgatatgtgcgggacgtggtggtggtggtggtggtgagggtgcgcgtggttgggggcgttcgcgtcggcgtcgtagttcgcgggtattatgtcgaggtcgtcgtagtcgttttggttgtggtagtcgagcggcgtcgacgggggcgtttggaagtcgaagttttggggtagtagcgacgtttcgaagtttaagtcgtttattacgcggtggtatatgggtttgagcgtttggtattttcgtttgaagtcgcgcggtcggcggcggaacgagtttttttcgaatatgaattcgttggtcgggtcgatggtttagtagtggtttttgtcgggtcgttcgaggtttttaggtagtttgatgaagtattcgttgagcgagagattgtggcgtatcgagtttttttagttttggtaggcgtcgcggaagaaggggaagcgcgtttgtaggaattggtagatttcgttgagcgttaggcgtttgttgggcgagttttggatggttatgacgatgagcgcgatgtacgagtagggcggtttttcgggtcgtcgtagtttcgagttcgtttttttggcgttttcgttttcggcgttcgcgtcgtcgtcgttcgcgtttttgtaggtagtcgagggggcgttggtcgaattggaggaggacgaggacgaggcgtaggaggcggaggacgacgacgaggaggaggaggtggttttcggggcggcggcggcggcggcggcggcggcgggcggcgggtttattagggcggtttggagcgcgtcggggatcgggttgtacgcgcggcggagcggggtcggcggcggttcgttttcggtggttatttgggattcgggagcgaggtcgggtcgcgagggcgggtttcgggcgggaagcggaggcgtcggagcggggtcggtttagaagttttgcgagcgttttagttcgtcgttcgggttgtagtcgtggttatttcgggttagcgtttcggcgtcgttttttttagtttttttggggtttttggcggcggcggcggcggcgggcgggaggtaacgttcggcgtattttttttcgagtcgcgggttttgttttgcgtaacggttttttaggtcgcggggtcgagcggtcggcgtcgggcgattgcgttcgcgagtgggatcgcggtttggatttcggggacgagttcgacgtttttttttaggagcgtttttcgttttgtttttcggattttttttttttttcgtttttttcggtcgtttttttcgttttttttttttttttttttttttttatttcgttttgtttttttttcgtttcgcgtcgtcgcgtttatttttttttttttcgatttggcggtcgttttttttttttatttcgtttttcgttttttagggttttttcgttttttatttttttcgcggttttttttttttttttttatttattttttttttaattgagggattatagatttatttcggttttgttagggggacgatttttatttttcgtaaaattcgattatttttgattttatgaaatattttttttgtttgtttttcgtagtaagtttcgcgttttattttaggatttagtttcgttttttcgcgttttttttttttttttggttcgtcgggtcgagtggtgttgttgcgggtgcggttgttcggagtttttttggtcgttttttttagggtcgatattgattttatttgttaatttcgtttagattttgtcgtttttagttatacgtcggggtgttagacgtttaaaggtaacgtgttaattttttttttttttggtagggtttgtaggtttttcgataattgttagggcgattgggggtcgtcgtagggttgcgggtcgttggcgatcgtggacgttttcg

SEQ ID NO: 41 - DNA, 1076 bp, Homo sapiens
cttctgggccgaccccgctccggcgcctccgcttcccgcccggggcccgccctcgcggcccggcctcgctcccgggtcccagatgaccaccgagggcgggccgccgccggccccgctccgccgcgcgtgcagcccggtccccggcgcgctccaggccgccctgatgagcccgccgcccgccgccgccgccgccgccgccgccgccccggagaccacctcctcctcctcgtcgtcgtcctccgcctcctgcgcctcgtcctcgtcctcctccaattcggccagcgccccctcggctgcctgcaagagcgcgggcggcggcggcgcgggcgccgggagcgggggcgccaagaaggcgagctcggggctgcggcggcccgagaagccgccctactcgtacatcgcgctcatcgtcatggccatccagagctcgcccagcaagcgcctgacgctcagcgagatctaccagttcctgcaggcgcgcttccccttcttccgcggcgcctaccagggctggaagaactcggtgcgccacaatctctcgctcaacgagtgcttcatcaagctgcctaagggcctcgggcggcccggcaagggccactactggaccatcgacccggccagcgagttcatgttcgaggagggctcgttccgccgccggccgcgcggcttcaggcggaagtgccaggcgctcaagcccatgtaccaccgcgtggtgagcggcttgggcttcggggcgtcgctgctgccccagggcttcgacttccaggcgcccccgtcggcgccgctcggctgccacagccagggcggctacggcggcctcgacatgatgcccgcgggctacgacgccggcgcgggcgcccccagccacgcgcaccctcaccaccaccaccaccaccacgtcccgcacatgtcgcccaacccgggttccacctacatggccagctgcccggtgcccgcgggacccgggggcgtcggtgcggccgggggcggcggcggcggcgactacgggccggacagcagcagcagcccggtaccctcgtccccggccatggcgagcgccatcgaatgccactcgc

SEQ ID NO: 42 - DNA, 1076 bp, Artificial Sequence
  C to T (bis1)
tttttgggtcgatttcgtttcggcgttttcgtttttcgttcggggttcgttttcgcggttcggtttcgttttcgggttttagatgattatcgagggcgggtcgtcgtcggtttcgtttcgtcgcgcgtgtagttcggttttcggcgcgttttaggtcgttttgatgagttcgtcgttcgtcgtcgtcgtcgtcgtcgtcgtcgtttcggagattattttttttttttcgtcgtcgtttttcgttttttgcgtttcgttttcgtttttttttaattcggttagcgttttttcggttgtttgtaagagcgcgggcggcggcggcgcgggcgtcgggagcgggggcgttaagaaggcgagttcggggttgcggcggttcgagaagtcgttttattcgtatatcgcgtttatcgttatggttatttagagttcgtttagtaagcgtttgacgtttagcgagatttattagtttttgtaggcgcgtttttttttttttcgcggcgtttattagggttggaagaattcggtgcgttataatttttcgtttaacgagtgttttattaagttgtttaagggtttcgggcggttcggtaagggttattattggattatcgattcggttagcgagtttatgttcgaggagggttcgtttcgtcgtcggtcgcgcggttttaggcggaagtgttaggcgtttaagtttatgtattatcgcgtggtgagcggtttgggtttcggggcgtcgttgttgttttagggtttcgatttttaggcgttttcgtcggcgtcgttcggttgttatagttagggcggttacggcggtttcgatatgatgttcgcgggttacgacgtcggcgcgggcgtttttagttacgcgtatttttattattattattattattacgtttcgtatatgtcgtttaattcgggttttatttatatggttagttgttcggtgttcgcgggattcgggggcgtcggtgcggtcgggggcggcggcggcggcgattacgggtcggatagtagtagtagttcggtattttcgttttcggttatggcgagcgttatcgaatgttattcgt

SEQ ID NO: 43 - DNA, 1076 bp, Artificial Sequence
  rc C to T (bis1)
acgaataacattcgataacgctcgccataaccgaaaacgaaaataccgaactactactactatccgacccgtaatcgccgccgccgccgcccccgaccgcaccgacgcccccgaatcccgcgaacaccgaacaactaaccatataaataaaacccgaattaaacgacatatacgaaacgtaataataataataataataaaaatacgcgtaactaaaaacgcccgcgccgacgtcgtaacccgcgaacatcatatcgaaaccgccgtaaccgccctaactataacaaccgaacgacgccgacgaaaacgcctaaaaatcgaaaccctaaaacaacaacgacgccccgaaacccaaaccgctcaccacgcgataatacataaacttaaacgcctaacacttccgcctaaaaccgcgcgaccgacgacgaaacgaaccctcctcgaacataaactcgctaaccgaatcgataatccaataataacccttaccgaaccgcccgaaacccttaaacaacttaataaaacactcgttaaacgaaaaattataacgcaccgaattcttccaaccctaataaacgccgcgaaaaaaaaaaaaacgcgcctacaaaaactaataaatctcgctaaacgtcaaacgcttactaaacgaactctaaataaccataacgataaacgcgatatacgaataaaacgacttctcgaaccgccgcaaccccgaactcgccttcttaacgcccccgctcccgacgcccgcgccgccgccgcccgcgctcttacaaacaaccgaaaaaacgctaaccgaattaaaaaaaaacgaaaacgaaacgcaaaaaacgaaaaacgacgacgaaaaaaaaaaaataatctccgaaacgacgacgacgacgacgacgacgacgaacgacgaactcatcaaaacgacctaaaacgcgccgaaaaccgaactacacgcgcgacgaaacgaaaccgacgacgacccgccctcgataatcatctaaaacccgaaaacgaaaccgaaccgcgaaaacgaaccccgaacgaaaaacgaaaacgccgaaacgaaatcgacccaaaaa

SEQ ID NO: 44 - DNA, 1076 bp, Artificial Sequence
  G to A (bis2 rc)
cttctaaaccgaccccgctccgacgcctccgcttcccgcccgaaacccgccctcgcgacccgacctcgctcccgaatcccaaataaccaccgaaaacgaaccgccgccgaccccgctccgccgcgcgtacaacccgatccccgacgcgctccaaaccgccctaataaacccgccgcccgccgccgccgccgccgccgccgccgccccgaaaaccacctcctcctcctcgtcgtcgtcctccgcctcctacgcctcgtcctcgtcctcctccaattcgaccaacgccccctcgactacctacaaaaacgcgaacgacgacgacgcgaacgccgaaaacgaaaacgccaaaaaaacgaactcgaaactacgacgacccgaaaaaccgccctactcgtacatcgcgctcatcgtcataaccatccaaaactcgcccaacaaacgcctaacgctcaacgaaatctaccaattcctacaaacgcgcttccccttcttccgcgacgcctaccaaaactaaaaaaactcgatacgccacaatctctcgctcaacgaatacttcatcaaactacctaaaaacctcgaacgacccgacaaaaaccactactaaaccatcgacccgaccaacgaattcatattcgaaaaaaactcgttccgccgccgaccgcgcgacttcaaacgaaaataccaaacgctcaaacccatataccaccgcgtaataaacgacttaaacttcgaaacgtcgctactaccccaaaacttcgacttccaaacgcccccgtcgacgccgctcgactaccacaaccaaaacgactacgacgacctcgacataatacccgcgaactacgacgccgacgcgaacgcccccaaccacgcgcaccctcaccaccaccaccaccaccacgtcccgcacatatcgcccaacccgaattccacctacataaccaactacccgatacccgcgaaacccgaaaacgtcgatacgaccgaaaacgacgacgacgacgactacgaaccgaacaacaacaacaacccgataccctcgtccccgaccataacgaacgccatcgaataccactcgc

SEQ ID NO: 45 - DNA, 1076 bp, Artificial Sequence
  G to A (bis2 rc) rc
gcgagtggtattcgatggcgttcgttatggtcggggacgagggtatcgggttgttgttgttgttcggttcgtagtcgtcgtcgtcgtcgttttcggtcgtatcgacgttttcgggtttcgcgggtatcgggtagttggttatgtaggtggaattcgggttgggcgatatgtgcgggacgtggtggtggtggtggtggtgagggtgcgcgtggttgggggcgttcgcgtcggcgtcgtagttcgcgggtattatgtcgaggtcgtcgtagtcgttttggttgtggtagtcgagcggcgtcgacgggggcgtttggaagtcgaagttttggggtagtagcgacgtttcgaagtttaagtcgtttattacgcggtggtatatgggtttgagcgtttggtattttcgtttgaagtcgcgcggtcggcggcggaacgagtttttttcgaatatgaattcgttggtcgggtcgatggtttagtagtggtttttgtcgggtcgttcgaggtttttaggtagtttgatgaagtattcgttgagcgagagattgtggcgtatcgagtttttttagttttggtaggcgtcgcggaagaaggggaagcgcgtttgtaggaattggtagatttcgttgagcgttaggcgtttgttgggcgagttttggatggttatgacgatgagcgcgatgtacgagtagggcggtttttcgggtcgtcgtagtttcgagttcgtttttttggcgttttcgttttcggcgttcgcgtcgtcgtcgttcgcgtttttgtaggtagtcgagggggcgttggtcgaattggaggaggacgaggacgaggcgtaggaggcggaggacgacgacgaggaggaggaggtggttttcggggcggcggcggcggcggcggcggcggcgggcggcgggtttattagggcggtttggagcgcgtcggggatcgggttgtacgcgcggcggagcggggtcggcggcggttcgttttcggtggttatttgggattcgggagcgaggtcgggtcgcgagggcgggtttcgggcgggaagcggaggcgtcggagcggggtcggtttagaag

SEQ ID NO: 46 - DNA, 128 bp, Homo sapiens
ctcagcgagatctaccagttcctgcaggcgcgcttccccttcttccgcggcgcctaccagggctggaagaactcggtgcgccacaatctctcgctcaacgagtgcttcatcaagctgcctaagggcct

SEQ ID NO: 47 - DNA, 128 bp, Artificial Sequence
  C to T (bis1)
tttagcgagatttattagtttttgtaggcgcgtttttttttttttcgcggcgtttattagggttggaagaattcggtgcgttataatttttcgtttaacgagtgttttattaagttgtttaagggttt

SEQ ID NO: 48 - DNA, 128 bp, Artificial Sequence
  rc C to T (bis1)
aaacccttaaacaacttaataaaacactcgttaaacgaaaaattataacgcaccgaattcttccaaccctaataaacgccgcgaaaaaaaaaaaaacgcgcctacaaaaactaataaatctcgctaaa

SEQ ID NO: 49 - DNA, 128 bp, Artificial Sequence
  G to A (bis2 rc)
ctcaacgaaatctaccaattcctacaaacgcgcttccccttcttccgcgacgcctaccaaaactaaaaaaactcgatacgccacaatctctcgctcaacgaatacttcatcaaactacctaaaaacct

SEQ ID NO: 50 - DNA, 128 bp, Artificial Sequence
  G to A (bis2 rc) rc
aggtttttaggtagtttgatgaagtattcgttgagcgagagattgtggcgtatcgagtttttttagttttggtaggcgtcgcggaagaaggggaagcgcgtttgtaggaattggtagatttcgttgag

SEQ ID NO: 51 - DNA, 76 bp, Homo sapiens
cctaccagggctggaagaactcggtgcgccacaatctctcgctcaacgagtgcttcatcaagctgcctaagggcct

SEQ ID NO: 52 - DNA, 76 bp, Artificial Sequence
  C to T (bis1)
tttattagggttggaagaattcggtgcgttataatttttcgtttaacgagtgttttattaagttgtttaagggttt

SEQ ID NO: 53 - DNA, 76 bp, Artificial Sequence
  rc C to T (bis1)
aaacccttaaacaacttaataaaacactcgttaaacgaaaaattataacgcaccgaattcttccaaccctaataaa

SEQ ID NO: 54 - DNA, 76 bp, Artificial Sequence
  G to A (bis2 rc)
cctaccaaaactaaaaaaactcgatacgccacaatctctcgctcaacgaatacttcatcaaactacctaaaaacct

SEQ ID NO: 55 - DNA, 76 bp, Artificial Sequence
  G to A (bis2 rc) rc
aggtttttaggtagtttgatgaagtattcgttgagcgagagattgtggcgtatcgagtttttttagttttggtagg

SEQ ID NO: 56 - DNA, 22 bp, Artificial Sequence
  Primer
gtattttgaggtttttattgat

SEQ ID NO: 57 - DNA, 19 bp, Artificial Sequence
  Primer
atctaactcctaaccctaa

SEQ ID NO: 58 - DNA, 39 bp, Artificial Sequence
  Blocker
ttattgattgagtagtagtgttttttgttgggatttttg

SEQ ID NO: 59 - DNA, 17 bp, Artificial Sequence
  Probe
taacgcgcgtaacgcta

SEQ ID NO: 60 - DNA, 21 bp, Artificial Sequence
  Primer
tttattagggttggaagaatt

SEQ ID NO: 61 - DNA, 22 bp, Artificial Sequence
  Primer
aaacccttaaacaacttaataa

SEQ ID NO: 62 - DNA, 32 bp, Artificial Sequence
  Blocker
gaatttggtgtgttataattttttgtttaatg

SEQ ID NO: 63 - DNA, 24 bp, Artificial Sequence
  Probe
tcgttaaacgaaaaattataacgc